European Patent Application EP 4 512 900 A2, published February 26, 2025. Title: RNA-Guided Nucleases and Active Fragments and Variants Thereof And Methods of Use. Applicant: LifeEDIT, Inc. Application US 18/431,662, filed February 2, 2024. The sequence listing filed with the application follows.

SEQUENCE LISTING (651 sequences)

SEQ ID NO: 1 - protein, 1070 aa, Bacillus sp.
  REGION 1..1070: note = source = /note="APG05083.1"
MRELDYRIGLDIGTNSIGWGIIELSWNKDREQYEKARIVDKGVRMFDKAEIPKTGASLAEPRRIARSSRRRLNRKSQRKKDIRNLLVQHEIISQKELASLYPLTKSSMDIWDIRLDGLDRLLDRFEWTRLLIHLAQRRGFKSNRKSELKDVETGKVLSSIQANEKRLSLYRTVGEMWMKNEDFSKYDKRRNSSNEYVFSVSRADLEKEIVTLFEAQRKFQSSYASADLQKTYLQIWAHQLPFASGNAIVNKVGYCSLLKGKEKRVPKATYTFQYFSTLDQINRTRLGPNFQPFTKEQRDVILDEMFNRTDYYKKKTIPEVTYYDIRKWLALDETIQFKGLTYDPNEELKKIELKSFINLKPFYEIKKVVTNYAKKTNEAFSTLDYDTFAYALTVYKTDKDIRSYLKKSNNLSKCCYDDQLIEELLTLSYTKFGHLSFKAINHVLPIMQEGRTYQEAIHQLGYDATNLKKENRSMFLPLFPDEITNPIVKRALTQARKVVNAIIRRYGSPNSVHIELARELSKSHDERTKIMKAHDENYKKNKGAISILIENGILNPTGYDIVRYKLWKEQGERCAYSLKQIPANTFFNEMKKERSGSPVLEIDHILPYSQSFIDSYHNKVLVYGDENQKKGNRIPYTYFLEGNKDWESFESYVRLNSFFSKKKRGYLLKKAYLPRESNMIKERHLNDTRYASSYLKNFIEKNLKFKEVEGSTRKKHVQTVNGIITAHLRKRWGLEKDRQETYLHHAMDAIIVACTDHHMVTKVTEYYQIKESNKSIRKPYFPLPWVGFREEILSHLARQPIARKISEELKIGYQSFDYILVSRMPKRSVTGAAHEQTIMKKGGIDKKGKTIIIKRVYLKDIKFDENGDFKMVGKEQDLATYEAIKQRYIEYGKESKKAFETPLYKPSKKGKGNLIKKIKVEVQTKSFVREVNGGVAQNGDLVRVDLFEKDNRYYMIPIYVMDTVHSELPNKAVTSSKGYEQWLTIDNSFTFKFSLYPYDLVRLVKGNEDRFLYFSTLDINSDRLNFKDVNKPSKQAENRYSLKTIENLEKYEVGVLGDLRFVRQEIRKNF

SEQ ID NO: 2 - RNA, 19 nt, Bacillus sp.
  misc_feature 1..19: note = source = /note="crRNA"
  source 1..19: mol_type = other RNA
gtcatagttccattattgc

SEQ ID NO: 3 - RNA, 84 nt, Bacillus sp.
  misc_feature 1..84: note = source = /note="tracrRNA"
  source 1..84: mol_type = other RNA
gctttgatgtttctatgataagggcttaggcccgtggcgttggggatcgcctgcccattttaatgggcttctccccatctattt

SEQ ID NO: 4 - RNA, 137 nt, synthetic construct
  misc_feature 1..137: note = source = /note="Description of Artificial Sequence: Syntheticpolynucleotide"
  misc_feature 1..137: note = source = /note="sgRNA L1"
  source 1..137: mol_type = other RNA
gagcggacagcagcttcctatatctcgtacgtcatagttccattattgcaaaggctttgatgtttctatgataagggcttaggcccgtggcgttggggatcgcctgcccattttaatgggcttctccccatctattt

SEQ ID NO: 5 - RNA, 137 nt, synthetic construct
  misc_feature 1..137: note = source = /note="Description of Artificial Sequence: Syntheticpolynucleotide"
  misc_feature 1..137: note = source = /note="sgRNA L2"
  source 1..137: mol_type = other RNA
ccatgatatagacgttgtggctgttgtagtgtcatagttccattattgcaaaggctttgatgtttctatgataagggcttaggcccgtggcgttggggatcgcctgcccattttaatgggcttctccccatctattt

SEQ ID NO: 6-7 - skipped (2 entries)

SEQ ID NO: 8 - DNA, 38 bp, synthetic construct
  misc_difference 31..38: note = a,c,t,g, unknown, or other
  misc_feature 1..38: note = source = /note="Description of Artificial Sequence: Syntheticoligonucleotide"
  misc_feature 1..38: note = source = /note="Target seq and PAM region of plasmid library 1"
  source 1..38: mol_type = other DNA
gagcggacagcagcttcctatatctcgtacnnnnnnnn

SEQ ID NO: 9 - DNA, 38 bp, synthetic construct
  misc_difference 31..38: note = a,c,t,g, unknown, or other
  misc_feature 1..38: note = source = /note="Description of Artificial Sequence: Syntheticoligonucleotide"
  misc_feature 1..38: note = source = /note="Target seq and PAM region of plasmid library 2"
  source 1..38: mol_type = other DNA
ccatgatatagacgttgtggctgttgtagtnnnnnnnn

SEQ ID NO: 10 - RNA, 132 nt, synthetic construct
  misc_difference 1..25: note = a,c,t,g, unknown, or other
  misc_feature 1..132: note = source = /note="Description of Artificial Sequence: Syntheticpolynucleotide"
  misc_feature 1..132: note = source = /note="sgRNA with N's"
  source 1..132: mol_type = other RNA
nnnnnnnnnnnnnnnnnnnnnnnnngtcatagttccattattgcaaaggctttgatgtttctatgataagggcttaggcccgtggcgttggggatcgcctgcccattttaatgggcttctccccatctattt

SEQ ID NO: 11 - protein, 1071 aa, Bacillus sp.
  REGION 1..1071: note = source = /note="APG07433.1"
MRELDYRIGLDIGTNSIGWGVIELSWNKDRERYEKVRIVDQGVRMFDRAEMPKTGASLAEPRRIARSSRRRLNRKSQRKKNIRNLLVQHGVITQEELDSLYPLSKKSMDIWGIRLDGLDRLLNHFEWARLLIHLAQRRGFKSNRKSELKDTETGKVLSSIQLNEKRLSLYRTVGEMWMKDPDFSKYDRKRNSPNEYVFSVSRAELEKEIVTLFAAQRRFQSPYASKDLQETYLQIWTHQLPFASGNAILNKVGYCSLLKGKERRIPKATYTFQYFSALDQVNRTRLGPDFQPFTKEQREIILNNMFQRTDYYKKKTIPEVTYYDIRKWLELDETIQFKGLNYDPNEELKKIEKKPFINLKAFYEINKVVANYSERTNETFSTLDYDGIGYALTVYKTDKDIRSYLKSSHNLPKRCYDDQLIEELLSLSYTKFGHLSLKAINHVLSIMQKGNTYKEAVDQLGYDTSGLKKEKRSKFLPPISDEITNPIVKRALTQARKVVNAIIRRHGSPHSVHIELARELSKNHDERTKIVSAQDENYKKNKGAISILSEHGILNPTGYDIVRYKLWKEQGERCAYSLKEIPADTFFNELKKERNGAPILEVDHILPYSQSFIDSYHNKVLVYSDENRKKGNRIPYTYFLETNKDWEAFERYVRSNKFFSKKKREYLLKRAYLPRESELIKERHLNDTRYASTFLKNFIEQNLQFKEAEDNPRKRRVQTVNGVITAHFRKRWGLEKDRQETYLHHAMDAIIVACTDHHMVTRVTEYYQIKESNKSVKKPYFPMPWEGFRDELLSHLASQPIAKKISEELKAGYQSLDYIFVSRMPKRSITGAAHKQTIMRKGGIDKKGKTIIIERLHLKDIKFDENGDFKMVGKEQDMATYEAIKQRYLEHGKNSKKAFETPLYKPSKKGTGNLIKRVKVEGQAKSFVREVNGGVAQNGDLVRVDLFEKDDKYYMVPIYVPDTVCSELPKKVVASSKGYEQWLTLDNSFTFKFSLYPYDLVRLVKGDEDRFLYFGTLDIDSDRLNFKDVNKPSKKNEYRYSLKTIEDLEKYEVGVLGDLRLVRKETRRNFH

SEQ ID NO: 12 - RNA, 21 nt, Bacillus sp.
  misc_feature 1..21: note = source = /note="crRNA"
  source 1..21: mol_type = other RNA
gtcatagttccattaaagcca

SEQ ID NO: 13 - RNA, 85 nt, Bacillus sp.
  misc_feature 1..85: note = source = /note="tracrRNA"
  source 1..85: mol_type = other RNA
tggctttgatgtttctatgataagggtttcgacccgtggcgtcggggatcgcctgcccattgaaatgggcttctccccatttatt

SEQ ID NO: 14 - RNA, 140 nt, synthetic construct
  misc_feature 1..140: note = source = /note="Description of Artificial Sequence: Syntheticpolynucleotide"
  misc_feature 1..140: note = source = /note="sgRNA L1"
  source 1..140: mol_type = other RNA
gagcggacagcagcttcctatatctcgtacgtcatagttccattaaagccagaaatggctttgatgtttctatgataagggtttcgacccgtggcgtcggggatcgcctgcccattgaaatgggcttctccccatttatt

SEQ ID NO: 15 - RNA, 140 nt, synthetic construct
  misc_feature 1..140: note = source = /note="Description of Artificial Sequence: Syntheticpolynucleotide"
  misc_feature 1..140: note = source = /note="sgRNA L2"
  source 1..140: mol_type = other RNA
ccatgatatagacgttgtggctgttgtagtgtcatagttccattaaagccagaaatggctttgatgtttctatgataagggtttcgacccgtggcgtcggggatcgcctgcccattgaaatgggcttctccccatttatt

SEQ ID NO: 16 - DNA, 38 bp, synthetic construct; identical to SEQ ID NO: 8
  misc_difference 31..38: note = a,c,t,g, unknown, or other
  misc_feature 1..38: note = source = /note="Description of Artificial Sequence: Syntheticoligonucleotide"
  misc_feature 1..38: note = source = /note="Target seq and PAM region of plasmid library 1"
  source 1..38: mol_type = other DNA

SEQ ID NO: 17 - DNA, 38 bp, synthetic construct; identical to SEQ ID NO: 9
  misc_difference 31..38: note = a,c,t,g, unknown, or other
  misc_feature 1..38: note = source = /note="Description of Artificial Sequence: Syntheticoligonucleotide"
  misc_feature 1..38: note = source = /note="Target seq and PAM region of plasmid library 2"
  source 1..38: mol_type = other DNA

SEQ ID NO: 18 - RNA, 135 nt, synthetic construct
  misc_difference 1..25: note = a,c,t,g, unknown, or other
  misc_feature 1..135: note = source = /note="Description of Artificial Sequence: Syntheticpolynucleotide"
  misc_feature 1..135: note = source = /note="sgRNA with N's"
  source 1..135: mol_type = other RNA
nnnnnnnnnnnnnnnnnnnnnnnnngtcatagttccattaaagccaaaagtggctttgatgtttctatgataagggtttcgacccgtggcgtcggggatcgcctgcccattgaaatgggcttctccccatttatt

SEQ ID NO: 19 - protein, 1071 aa, Bacillus sp.
  REGION 1..1071: note = source = /note="APG07513.1"
MRELDYRIGLDIGTNSIGWGVIELSWNKDREQYEKTRIVDKGVRMFDKAEIPKTGASLAEPRRIARSSRRRLNRKSQRKKDIRNLLVQHEIISQKELTSLYPLSKSSMDIWDIRLDGLDRLLDRFEWARLLIHLAQRRGFKSNRKSELKDVETGKVLSSIQVNEKRLSLYRTVGEMWMKNADCSKYGKRRNSPNEYVFSVSRADLEKEIVTLFEAQRKFHSSYASVDLQKTYIQIWAHQLPFASGNAIVNKVGYCSLLKGKEKRVPKATYTFQYFNTLDQINRTRLGPNFQPFTKEQRDIILDKMFQRTDYYKKKTIPEVTYYDIRKWLALDETIQFKGLTYDPNEELKKIEMKPFINLKPFYEIKKVVTNYAKKTNEVFSALDYDTVAYALTVYKTDKDIRSYLKRSNNLSKRCYDDQLIEELLTLSYTKFGHLSFKAINHVLPIMQEGRTYQEAIHQLGYDTTNLKKENRSMFLPIIPDEITNPIVKRALTQARKVVNAIIRRYGSPNSVHIELARELSKSHDERKKIMTAHDENYKKNKGAVSILIDNGILNPTGYDIVRYKLWKEQGERCAYSLKKIPANTFFNELKKERSGPPVLEVDHILPYSQSFIDSYHNKVLVYGDENQKKGNRIPYTFFSEEDKEWESFESYVRSNSFFSKKKRGYLLKKAYLPRESNLIKERHLNDTRYASSYLKNFIEKNLKFKEAVGITRKKYVQTVNGVITAHLRKRWGLEKDRQETYLHHAMDAIIVACTDHHMVTKVTEYYQIKEGNKSIKKPYFPLPWMGFREEILSHLESQPIARKISEELKIGYQSPDYILVSRMPKRSVTGSAHDQTVMKKGDIDKKGKTIIIKRVHLKDIKFDENGDFKMVGKEQDLATYEAIKQRYLEYRKESKKAFETPLYKPSKKGKGNLIKKIKVEVQTKSFVREINGGVAQNGDLVRVDLFEKDNRYYMVPIYVVDTVRSELPNKAVTSSKGYEQWLSIDNSFTFKFSLYPYDLVRLVKGDEDRFLYFSTLDINSDRLNFKDVNKPSKQAEYRYSLKTIENLEKYEIGVLGDLRLVRQETRKIFK

SEQ ID NO: 20 - RNA, 27 nt, Bacillus sp.
  misc_feature 1..27: note = source = /note="crRNA"
  source 1..27: mol_type = other RNA
gtcatagttccattaaagccattgctg

SEQ ID NO: 21 - RNA, 93 nt, Bacillus sp.
  misc_feature 1..93: note = source = /note="tracrRNA"
  source 1..93: mol_type = other RNA
acagcaatggctttgatgtttctatgataagggcttcggcccgtggcgttggggatcgcctgcccattttaatgggcttctccccatctattt

SEQ ID NO: 22 - RNA, 154 nt, synthetic construct
  misc_feature 1..154: note = source = /note="Description of Artificial Sequence: Syntheticpolynucleotide"
  misc_feature 1..154: note = source = /note="sgRNA L1"
  source 1..154: mol_type = other RNA
gagcggacagcagcttcctatatctcgtacgtcatagttccattaaagccattgctgaaagacagcaatggctttgatgtttctatgataagggcttcggcccgtggcgttggggatcgcctgcccattttaatgggcttctccccatctattt

SEQ ID NO: 23 - RNA, 154 nt, synthetic construct
  misc_feature 1..154: note = source = /note="Description of Artificial Sequence: Syntheticpolynucleotide"
  misc_feature 1..154: note = source = /note="sgRNA L2"
  source 1..154: mol_type = other RNA
ccatgatatagacgttgtggctgttgtagtgtcatagttccattaaagccattgctgaaagacagcaatggctttgatgtttctatgataagggcttcggcccgtggcgttggggatcgcctgcccattttaatgggcttctccccatctattt

SEQ ID NO: 24 - DNA, 38 bp, synthetic construct; identical to SEQ ID NO: 8
  misc_difference 31..38: note = a,c,t,g, unknown, or other
  misc_feature 1..38: note = source = /note="Description of Artificial Sequence: Syntheticoligonucleotide"
  misc_feature 1..38: note = source = /note="Target seq and PAM region of plasmid library 1"
  source 1..38: mol_type = other DNA

SEQ ID NO: 25 - DNA, 38 bp, synthetic construct; identical to SEQ ID NO: 9
  misc_difference 31..38: note = a,c,t,g, unknown, or other
  misc_feature 1..38: note = source = /note="Description of Artificial Sequence: Syntheticoligonucleotide"
  misc_feature 1..38: note = source = /note="Target seq and PAM region of plasmid library 2"
  source 1..38: mol_type = other DNA

SEQ ID NO: 26 - RNA, 149 nt, synthetic construct
  misc_difference 1..25: note = a,c,t,g, unknown, or other
  misc_feature 1..149: note = source = /note="Description of Artificial Sequence: Syntheticpolynucleotide"
  misc_feature 1..149: note = source = /note="sgRNA with N's"
  source 1..149: mol_type = other RNA
nnnnnnnnnnnnnnnnnnnnnnnnngtcatagttccattaaagccattgctgaaagacagcaatggctttgatgtttctatgataagggcttcggcccgtggcgttggggatcgcctgcccattttaatgggcttctccccatctattt

SEQ ID NO: 27 - protein, 1072 aa, Bacillus sp.
  REGION 1..1072: note = source = /note="APG08290.1"
MSELDYRIGLDIGTNSIGWGVIELFWNKDRERYEKVRIVDKGVRMFDKAEIPNKGASLAEPRRIARSSRRRLNRKSQRKKEIRNLLVQHGMITQEELDLLYPLSKKSIDIWDIRLDGLDRLLNHLEWARLLIHLAQRRGFKSNRKSELKDAETGKVLSSIQVNEKRLFLYRTVGEMWIKDAEFSKYDRRRNSPNEYVFSVSRADLEKEIVTLFEAQRKFQSSYASKNLQETYLQIWAHQLPFASGNAILNKVGYCSLLKGKERRIPKATYTFQYFSALDQVNRTRLGPDFQPFTQEQKEIILDKMFQRTDYYKKKTIPEVSYYDIRKWLELDETIQFKGLNYDPNEELKKIEKKPFINLKAFYEIKKVVANYAERTNEAFSTLDYDAIAYALTVYKTDKDIRSYLKKSNNLSKRCYDDQLIEELFTLSYTKFGHLSFKAINHVLPIMQEGRTYQEAIHQLGYDTTNLKKENRSMFLPLIPDEITNPIVKRAITQARKVVNAIIRRYGSPNSVHIELARELSKSHDERKKIMTAHDENYKKNKGAISILIENGILNPTGYDIVRYKLWKEQGERCAYSLKEIPPDTFFNELKKERNGSPILEVDHILPYSQSFIDSYHNKVLVYSDENRNKGNRIPYTYFLETNKDWEAFERYVRSNKLFSKKKREYLLKKTYLPRESELIKERHLNDTRYASTFLKNFIEQNLQFKEVEVNLRKKRVQTVNGVITAHLRKRWGLEKNRQETYLHHAMDAIIVACTDHHMVTRITEYYQIKESNKSVKKPYFPMPWEGFRDELLSHLASQPIAKKISEELKAGYQSSDYIFVSRMPKRSVTGAAHDQTIRRKGGIDKKGKTIIIKRVRLKDIKFDENGDFKMVGKEQDLATYEAIKQRYLEHRKNSKKAFETPLYKPSKKGTGNLIKRVKIEGQTKAFVREVNGGVAQNSDLVRVDLFEKDDKYYMVPIYVPDTVCSELPKKVVKSGKGYEQWLTLDNSFTFKSSLYPYDLVRLVKGNEDRFLYFGTLDIDSDRLNFKDVNKPSKQNEYRYSLKTIENLEKYEVGVLGDLRLVKQETRRIFNR

SEQ ID NO: 28 - RNA, 21 nt, Bacillus sp.
  misc_feature 1..21: note = source = /note="crRNA"
  source 1..21: mol_type = other RNA
gtcatagttccatgaaagcca

SEQ ID NO: 29 - RNA, 85 nt, Bacillus sp.
  misc_feature 1..85: note = source = /note="tracrRNA"
  source 1..85: mol_type = other RNA
tggctttgatgtttctatgataagggtttcggcccgtggcgtcggggatcgcctgcccattccgatgggcttctccccatttatt

SEQ ID NO: 30 - RNA, 140 nt, synthetic construct
  misc_feature 1..140: note = source = /note="Description of Artificial Sequence: Syntheticpolynucleotide"
  misc_feature 1..140: note = source = /note="sgRNA L1"
  source 1..140: mol_type = other RNA
gagcggacagcagcttcctatatctcgtacgtcatagttccatgaaagccaaaagtggctttgatgtttctatgataagggtttcggcccgtggcgtcggggatcgcctgcccattccgatgggcttctccccatttatt

SEQ ID NO: 31 - RNA, 140 nt, synthetic construct
  misc_feature 1..140: note = source = /note="Description of Artificial Sequence: Syntheticpolynucleotide"
  misc_feature 1..140: note = source = /note="sgRNA L2"
  source 1..140: mol_type = other RNA
ccatgatatagacgttgtggctgttgtagtgtcatagttccatgaaagccaaaagtggctttgatgtttctatgataagggtttcggcccgtggcgtcggggatcgcctgcccattccgatgggcttctccccatttatt

SEQ ID NO: 32 - skipped

SEQ ID NO: 33 - DNA, 38 bp, synthetic construct; identical to SEQ ID NO: 8
  misc_difference 31..38: note = a,c,t,g, unknown, or other
  misc_feature 1..38: note = source = /note="Description of Artificial Sequence: Syntheticoligonucleotide"
  misc_feature 1..38: note = source = /note="Target seq and PAM region of plasmid library 1"
  source 1..38: mol_type = other DNA

SEQ ID NO: 34 - DNA, 38 bp, synthetic construct; identical to SEQ ID NO: 9
  misc_difference 31..38: note = a,c,t,g, unknown, or other
  misc_feature 1..38: note = source = /note="Description of Artificial Sequence: Syntheticoligonucleotide"
  misc_feature 1..38: note = source = /note="Target seq and PAM region of plasmid library 2"
  source 1..38: mol_type = other DNA

SEQ ID NO: 35 - RNA, 135 nt, synthetic construct
  misc_difference 1..25: note = a,c,t,g, unknown, or other
  misc_feature 1..135: note = source = /note="Description of Artificial Sequence: Syntheticpolynucleotide"
  misc_feature 1..135: note = source = /note="sgRNA with N's"
  source 1..135: mol_type = other RNA
nnnnnnnnnnnnnnnnnnnnnnnnngtcatagttccatgaaagccaaaagtggctttgatgtttctatgataagggtttcggcccgtggcgtcggggatcgcctgcccattccgatgggcttctccccatttatt

SEQ ID NO: 36 - protein, 1337 aa, Enterococcus sp.
  REGION 1..1337: note = source = /note="APG05459.1"
MKKDYVIGLDIGTNSVGWAVMTEDYQLVKKKMPIYGNTEKKKIKKNFWGVRLFEEGHTAEDRRLKRTARRRISRRRNRLRYLQAFFEEAMTALDENFFARLQESFLVPEDKKWHRHPIFAKLEDEVAYHETYPTIYHLRKKLADSSEQADLRLIYLALAHIVKYRGHFLIEGKLSTENISVKEQFQQFMIIYNQTFVNGESRLVSAPLPESVLIEEELTEKASRTKKSEKVLQQFPQEKANGLFGQFLKLMVGNKADFKKVFGLEEEAKITYASESYEEDLEGILAKVGDEYSDVFLAAKNVYDAVELSTILADSDKKSHAKLSSSMIVRFTEHQEDLKKFKRFIRENCPDEYDNLFKNEQKDGYAGYIAHAGKVSQLKFYQYVKKIIQDIAGAEYFLEKIAQENFLRKQRTFDNGVIPHQIHLAELQAIIHRQAAYYPFLKENQEKIEQLVTFRIPYYVGPLSKGDASTFAWLKRQSEEPIRPWNLQETVDLDQSATAFIERMTNFDTYLPSEKVLPKHSLLYEKFMVFNELTKISYTDDRGIKANFSGKEKEKIFDYLFKTRRKVKKKDIIQFYRNEYNTEIVTLSGLEEDQFNASFSTYQDLLKCGLTRAELDHPDNAEKLEDIIKILTIFEDRQRIRTQLSTFKGQFSAEVLKKLERKHYTGWGRLSKKLINGIYDKESGKTILDYLIKDDGVSKHYNRNFMQLINDSQLSFKNAIQKAQSSEHEETLSETVNELAGSPAIKKGIYQSLKIVDELVAIMGYAPKRIVVEMARENQTTSTGKRRSIQRLKIVEKAMAEIGSNLLKEQPTTNEQLRDTRLFLYYMQNGKDMYTGDELSLHRLSHYDIDHIIPQSFMKDDSLDNLVLVGSTENRGKSDDVPSKEVVKDMKAYWEKLYAAGLISQRKFQRLTKGEQGGLTLEDKAHFIQRQLVETRQITKNVAGILDQRYNANSKEKKVQIITLKASLTSQFRSIFGLYKVREVNDYHHGQDAYLNCVVATTLLKVYPNLAPEFVYGEYPKFQAFKENKATAKTIIYTNLMRFFTEDEPRFMKDGEILWSNSYLKNIKKELNYHQMNIVKKVEVQKGGFSKESIKPKGPSNKLIPVKNGLDPQKYGGFDSPVVAYTVLFTHEKGKKPLIKQEILGITIMEKTRFEQNPILFLEEKGFLRPRVLMKLPKYTLYEFPEGRRRLLASAKEAQKGNQMVLPEHLLTLLYHAKQCLLPNQSESLAYVEQHQPEFQEILERVVDFAEVHTLAKSKVQQIVKLFEANQTADVKEIAASFIQLMQFNAMGAPSTFKFFQKDIERARYTSIKEIFDATIIYQSTTGLYETRRKVVD

SEQ ID NO: 37 - RNA, 16 nt, Enterococcus sp.
  misc_feature 1..16: note = source = /note="crRNA"
  source 1..16: mol_type = other RNA
gttttagagtcatgtt

SEQ ID NO: 38 - RNA, 74 nt, Enterococcus sp.
  misc_feature 1..74: note = source = /note="tracrRNA"
  source 1..74: mol_type = other RNA
aacatagcaagttaaaataaggttttaaccgtaatcaactgtaaagtggcgctgtttcggcgctttttttgttt

SEQ ID NO: 39 - RNA, 124 nt, synthetic construct
  misc_feature 1..124: note = source = /note="Description of Artificial Sequence: Syntheticpolynucleotide"
  misc_feature 1..124: note = source = /note="sgRNA L1"
  source 1..124: mol_type = other RNA
gagcggacagcagcttcctatatctcgtacgttttagagtcatgttaaagaacatagcaagttaaaataaggttttaaccgtaatcaactgtaaagtggcgctgtttcggcgctttttttgttt

SEQ ID NO: 40 - RNA, 124 nt, synthetic construct
  misc_feature 1..124: note = source = /note="Description of Artificial Sequence: Syntheticpolynucleotide"
  misc_feature 1..124: note = source = /note="sgRNA L2"
  source 1..124: mol_type = other RNA
ccatgatatagacgttgtggctgttgtagtgttttagagtcatgttaaagaacatagcaagttaaaataaggttttaaccgtaatcaactgtaaagtggcgctgtttcggcgctttttttgttt

SEQ ID NO: 41 - skipped

SEQ ID NO: 42 - DNA, 38 bp, synthetic construct; identical to SEQ ID NO: 8
  misc_difference 31..38: note = a,c,t,g, unknown, or other
  misc_feature 1..38: note = source = /note="Description of Artificial Sequence: Syntheticoligonucleotide"
  misc_feature 1..38: note = source = /note="Target seq and PAM region of plasmid library 1"
  source 1..38: mol_type = other DNA

SEQ ID NO: 43 - DNA, 38 bp, synthetic construct; identical to SEQ ID NO: 9
  misc_difference 31..38: note = a,c,t,g, unknown, or other
  misc_feature 1..38: note = source = /note="Description of Artificial Sequence: Syntheticoligonucleotide"
  misc_feature 1..38: note = source = /note="Target seq and PAM region of plasmid library 2"
  source 1..38: mol_type = other DNA

SEQ ID NO: 44 - RNA, 119 nt, synthetic construct
  misc_difference 1..25: note = a,c,t,g, unknown, or other
  misc_feature 1..119: note = source = /note="Description of Artificial Sequence: Syntheticpolynucleotide"
  misc_feature 1..119: note = source = /note="sgRNA with N's"
  source 1..119: mol_type = other RNA
nnnnnnnnnnnnnnnnnnnnnnnnngttttagagtcatgttaaagaacatagcaagttaaaataaggttttaaccgtaatcaactgtaaagtggcgctgtttcggcgctttttttgttt

SEQ ID NO: 45 - protein, 1436 aa, Enterococcus sp.
  REGION 1..1436: note = source = /note="APG04583.1"
MAKNILGLDLGTNSIGWALVQQDFENKEGNILGMGSRIIPMSQDILGEFGKGNSISQTAERTGYRGVRRLRERHLLRRERLHRVLHLLGFLPKHYDEKIDFTQRFGKFINQAEPKLAFDSEFLFKDSFHEMLADFKQNQPEFLKDKNGEDCLVPYDWTIYYLRKKALTQKIEKYELAWLILNFNQKRGYYQLRGEEEKENPNKLVGFHSLKIVDVIPDAETNKKGETWYSLHLENGWVYRRSSKISLADWKDKVRDFIVTTDLNDDGSEKLDKDGIVKRSFRAPSADDWTLLKKKTEKDIDNSNKTVGTYIYDNLLLNPKQKIKGKMVRTIERKFYKQELEQILKTQKEFHSELQSENLLQDCVRELYRNNEQHQQMLEAKDFVHLFLNDIIFYQRPLRSQKSSISNCTLEFRKSKNENGEEVIHRLKVIAKSNPYYQEFRLLQWVQNLAIYTKDDDKNVTNEFLKSTQDWEDLLRWLHSKKEIKQDALIKFLIEKKGLKGKALTIEVAKYRWNYVQDKDYPGNETRYLIQSRLDKVEYAPKDFLTYENEMALWHIIYSINDKIEYEKALKSFANKKGLDEVTFVEAFKKFPPFKSDYGSFSEKAIKKLLPLMRFGTQWNWDNIDQNSKERIGKILTGEYDENIKGRVREKARHLNSETDFQALPLWLAQYVVYGRHSEADIAGKWNSVDDLKQFLDDFKQHSLRNPIVEQVITETLRAVKDIWNFYGKGAKDFFSEIHIELGREMKNTADERKRITTMVTDNENTNLRIKALLAEMALDQNVDNVRPYSPMQQEILKIYEEGVLNAEENIDDDILKISKTAQPSATDLKRYKLWLEQKYRSPYTGQMIPLNKLFTPEYEIEHIIPQSRYFDDSMSNKVICEAAVNKLKDNQIGLVFIKNHHGEVVDFGMGKQVKILEVSDYEDFVKQNYNKNRGKRNKLLLEDIPEKMIERQLNDTRYISKYITQVLSNIVRDDKEGSKDDGVNSKNIVPGNGKITTRLKQDWGLNDVWNDLVLPRFERMNTLTNSNDFTSKNTHGKTIPTVPIELSKGFSKKRIDHRHHAMDALVIACATRDHVNLLNNESSKSDTKRYDLNRKLRKYEKVAYNDPKTGERIEKEVPKDFIKPWETFTEDTRTLLENIVISFKQNLRVINKATNYYEKIENGKKVKVEQKGINWAVRKALHKETVSGQVHLDRIKVAKGKILTATRKTLDASFNEKTIESITDTGIQKILLNYLKSKDNNPEVAFSPEGIEELNKNIRLYNDGKAHQPILKVRVFEQGSKFTLGETGNKTTKFVEAAKGTNLFFGIYEDKSGKRSYETIPLNIVIERQKQGLQAVPETNEKGKQLLFTLSPNDLVYVPEEGVFDENNIKVDRIYKVVSFSTYQCFFVRNDVSTSVVNKVEYSALNKMEKSIDNIMIKENCVKLNVDRLGKISKA

SEQ ID NO: 46 - RNA, 16 nt, Enterococcus sp.
  misc_feature 1..16: note = source = /note="crRNA"
  source 1..16: mol_type = other RNA
gttgtgagttcctttc

SEQ ID NO: 47 - RNA, 78 nt, Enterococcus sp.
  misc_feature 1..78: note = source = /note="tracrRNA"
  source 1..78: mol_type = other RNA
gaaaggaactcacaataaggattattccgttgtgaaaacatttagcgcctcgactatcttcggggcttttttattttt

SEQ ID NO: 48 - RNA, 128 nt, synthetic construct
  misc_feature 1..128: note = source = /note="Description of Artificial Sequence: Syntheticpolynucleotide"
  misc_feature 1..128: note = source = /note="sgRNA L1"
  source 1..128: mol_type = other RNA
gagcggacagcagcttcctatatctcgtacgttgtgagttcctttcacttgaaaggaactcacaataaggattattccgttgtgaaaacatttagcgcctcgactatcttcggggcttttttattttt

SEQ ID NO: 49 - RNA, 128 nt, synthetic construct
  misc_feature 1..128: note = source = /note="Description of Artificial Sequence: Syntheticpolynucleotide"
  misc_feature 1..128: note = source = /note="sgRNA L2"
  source 1..128: mol_type = other RNA
ccatgatatagacgttgtggctgttgtagtgttgtgagttcctttcacttgaaaggaactcacaataaggattattccgttgtgaaaacatttagcgcctcgactatcttcggggcttttttattttt

SEQ ID NO: 50 - skipped

SEQ ID NO: 51 - DNA, 38 bp, synthetic construct; identical to SEQ ID NO: 8
  misc_difference 31..38: note = a,c,t,g, unknown, or other
  misc_feature 1..38: note = source = /note="Description of Artificial Sequence: Syntheticoligonucleotide"
  misc_feature 1..38: note = source = /note="Target seq and PAM region of plasmid library 1"
  source 1..38: mol_type = other DNA

SEQ ID NO: 52 - DNA, 38 bp, synthetic construct; identical to SEQ ID NO: 9
  misc_difference 31..38: note = a,c,t,g, unknown, or other
  misc_feature 1..38: note = source = /note="Description of Artificial Sequence: Syntheticoligonucleotide"
  misc_feature 1..38: note = source = /note="Target seq and PAM region of plasmid library 2"
  source 1..38: mol_type = other DNA

SEQ ID NO: 53 - RNA, 123 nt, synthetic construct
  misc_difference 1..25: note = a,c,t,g, unknown, or other
  misc_feature 1..123: note = source = /note="Description of Artificial Sequence: Syntheticpolynucleotide"
  misc_feature 1..123: note = source = /note="sgRNA with N's"
  source 1..123: mol_type = other RNA
nnnnnnnnnnnnnnnnnnnnnnnnngttgtgagttcctttcaaaggaaaggaactcacaataaggattattccgttgtgaaaacatttagcgcctcgactatcttcggggcttttttattttt

SEQ ID NO: 54 - protein, 1456 aa, Empedobacter sp.
  REGION 1..1456: note = source = /note="APG01688.1"
MMIKNILGLDLGTNSIGWALIKQDFENKHGEILGMGSRIIPMSQDILGDFGKGNSISQTADRTKYRSVRRLRERFLLRRERLHRVLHLLNFLPQHYASQIDFEKKFGKFKSETEPKLAWENWGGKFSFLFQNSFNEMLEDFKAAGQGLKIPYDWTIYYLRKKALSQKIEKEELAWILLNFNQKRGYYQLRGEEEEENPNKLVEFYSLKIVDVVADEPQKGKSDIWYSLILENGWVYRRASKIPLFDWKDKTRDFIVTTDLNDDRSVKTDKEGNEKRSFRAPSENDWTLVKKKTEQEIDQSHKTVGTYIYETLLLNPKQKIKGKLVRTIERKFYKDELKQILEKQKEFHQELKNDDLYNDCIRELYRNNEAHQLTLSKKDFVHLLMDDLIFYQRPLRSQKSSISNCTLEFRKYKDENGIEHTQYLKAIPKSNPYYQEFRLWQWMYNLNIYRKDDEANVTKEFLNTNKDFESLFEFLNNRKEIEQKPLIKFLLEQKDINKKLLNAEAEKYRWNYVEDKKYPCNETKTMISSRLDKVENISDDFLTRDIEQKIWHIIYSVNDKIEYEKALKSFATRNDLDENSFIEAFKKFSPFKSEYGSFSEKAIKKLLPLMRLGKYWYEDEIVKHSDIYFKNIENLLGDFSNRDKKISEEDKEKWNKSINLKLQEELKDFQTAEIDLFQGLRLHIAQYLVYGRHSEASMIGKWNSAEDLEEFLKDFKQHSLRNPIVEQVITETLRVVKDIWLKYGNGAKDFFNEIHIELGREMKLPADDRKKLTNQISENENTNFRIKALLAEMMNDSSVENVRPFSPMQQEILKIYEDDVLKSDIEIEDDILKISKTAQPSPSDLKRYKLWLEQKYKSPYTGQIIPLNKLFTPEYEIEHIIPQSRYFDDSFSNKVICESAVNKLKDNYIGLEFIKQFGGTIIELGFGKSIKVFETKEYEDFVKKHYANNQGKRNKLLMEDIPEKMIERQMNDTRYISKYISGVLSNIVRVEDGSDEGVNSKNIVPGNGKITTQLKQDWGLNDVWNDLILPRFERMNQLTNSKVFTAWNENYQKFLPTVPIEYSKGFSKKRIDHRHHALDALVIACATKDHVNLLNNQSAKSDTKRYDLKKKSMKFEKVVYNDAKTGEKIEREVPKQFLKPWENFTLDVKHNLETIIVSFKQNLRVINKATNYYEKYVEKDGTKNKERVEQTGTNWAIRKPMHKDTVSGKVDLPWVKVPKGKILTATRKSLDSSFDLKSIGSITDTGIQKILKNYLAFKDGNPELAFSPEGIDDLNKNIEKYNDGKPHQPINKVRVFELGSKFQVGQSGNKKDKYVEAAKGTNLFFAVYEDEKGKRNYETIPLNEVIERQKQGLSVVDLKGTNDFYLCPNDFVYIPSGDELENINNVDFKDIKKEINERIYKVVSFTGNRLSCIPYMVATTIVNKLEFTQLNKIEFTKEKEICIKLNVDRLGNISKA

SEQ ID NO: 55 - RNA, 18 nt, Empedobacter sp.
  misc_feature 1..18: note = source = /note="crRNA"
  source 1..18: mol_type = other RNA
gttgtgaattgctttcaa

SEQ ID NO: 56 - RNA, 75 nt, Empedobacter sp.
  misc_feature 1..75: note = source = /note="tracrRNA"
  source 1..75: mol_type = other RNA
ttgaaaagcaattcacaataaggattattccgttgtgaaaacattcaaggcggggcaactcgtcttttttctttt

SEQ ID NO: 57 - RNA, 127 nt, synthetic construct
  misc_feature 1..127: note = source = /note="Description of Artificial Sequence: Syntheticpolynucleotide"
  misc_feature 1..127: note = source = /note="sgRNA L1"
  source 1..127: mol_type = other RNA
gagcggacagcagcttcctatatctcgtacgttgtgaattgctttcaaaaagttgaaaagcaattcacaataaggattattccgttgtgaaaacattcaaggcggggcaactcgtcttttttctttt

SEQ ID NO: 58 - RNA, 127 nt, synthetic construct
  misc_feature 1..127: note = source = /note="Description of Artificial Sequence: Syntheticpolynucleotide"
  misc_feature 1..127: note = source = /note="sgRNA L2"
  source 1..127: mol_type = other RNA
ccatgatatagacgttgtggctgttgtagtgttgtgaattgctttcaaaaagttgaaaagcaattcacaataaggattattccgttgtgaaaacattcaaggcggggcaactcgtcttttttctttt

SEQ ID NO: 59 - skipped

SEQ ID NO: 60 - DNA, 38 bp, synthetic construct; identical to SEQ ID NO: 8
  misc_difference 31..38: note = a,c,t,g, unknown, or other
  misc_feature 1..38: note = source = /note="Description of Artificial Sequence: Syntheticoligonucleotide"
  misc_feature 1..38: note = source = /note="Target seq and PAM region of plasmid library 1"
  source 1..38: mol_type = other DNA

SEQ ID NO: 61 - DNA, 38 bp, synthetic construct; identical to SEQ ID NO: 9
  misc_difference 31..38: note = a,c,t,g, unknown,or other
  misc_feature 1..38: note = source = /note="Description of Artificial Sequence: Syntheticoligonucleotide"
  misc_feature 1..38: note = source = /note="Target seq and PAM region of plasmid library 2"
  source 1..38: mol_type = other DNA

SEQ ID NO: 62 - RNA, 122 nt, synthetic construct
  misc_difference 1..25: note = a,c,t,g, unknown, or other
  misc_feature 1..122: note = source = /note="Description of Artificial Sequence: Syntheticpolynucleotide"
  misc_feature 1..122: note = source = /note="sgRNA with N's"
  source 1..122: mol_type = other RNA
nnnnnnnnnnnnnnnnnnnnnnnnngttgtgaattgctttcaaaaagttgaaaagcaattcacaataaggattattccgttgtgaaaacattcaaggcggggcaactcgtcttttttctttt

SEQ ID NO: 63-66 - skipped (4 entries)

SEQ ID NO: 67 - protein, 7 aa, synthetic construct
  REGION 1..7: note = source = /note="Description of Artificial Sequence: Syntheticpeptide"
  REGION 1..7: note = source = /note="NLS"
PKKKRKV

SEQ ID NO: 68-72 - skipped (5 entries)

SEQ ID NO: 73 - DNA, 30 bp, synthetic construct
  misc_feature 1..30: note = source = /note="Description of Artificial Sequence: Syntheticoligonucleotide"
  misc_feature 1..30: note = source = /note="mismatch repair Table 4"
  source 1..30: mol_type = other DNA
gagcggacagcagcttcctatatctcgtac

SEQ ID NO: 74 - DNA, 30 bp, synthetic construct
  misc_feature 1..30: note = source = /note="Description of Artificial Sequence: Syntheticoligonucleotide"
  misc_feature 1..30: note = source = /note="mismatch repair Table 4"
  source 1..30: mol_type = other DNA
gagcggacagcagcttcctatatctcgtag

SEQ ID NO: 75 - DNA, 30 bp, synthetic construct
  misc_feature 1..30: note = source = /note="Description of Artificial Sequence: Syntheticoligonucleotide"
  misc_feature 1..30: note = source = /note="mismatch repair Table 4"
  source 1..30: mol_type = other DNA
gagcggacagcagcttcctatatctcgttc

SEQ ID NO: 76 - DNA, 30 bp, synthetic construct
  misc_feature 1..30: note = source = /note="Description of Artificial Sequence: Syntheticoligonucleotide"
  misc_feature 1..30: note = source = /note="mismatch repair Table 4"
  source 1..30: mol_type = other DNA
gagcggacagcagcttcctatatctcgaac

SEQ ID NO: 77 - DNA, 30 bp, synthetic construct
  misc_feature 1..30: note = source = /note="Description of Artificial Sequence: Syntheticoligonucleotide"
  misc_feature 1..30: note = source = /note="mismatch repair Table 4"
  source 1..30: mol_type = other DNA
gagcggacagcagcttcctatatctcctac

SEQ ID NO: 78 - DNA, 30 bp, synthetic construct
  misc_feature 1..30: note = source = /note="Description of Artificial Sequence: Syntheticoligonucleotide"
  misc_feature 1..30: note = source = /note="mismatch repair Table 4"
  source 1..30: mol_type = other DNA
gagcggacagcagcttcctatatctggtac

SEQ ID NO: 79 - DNA, 30 bp, synthetic construct
  misc_feature 1..30: note = source = /note="Description of Artificial Sequence: Syntheticoligonucleotide"
  misc_feature 1..30: note = source = /note="mismatch repair Table 4"
  source 1..30: mol_type = other DNA
gagcggacagcagcttcctatatcacgtac

SEQ ID NO: 80 - DNA, 30 bp, synthetic construct
  misc_feature 1..30: note = source = /note="Description of Artificial Sequence: Syntheticoligonucleotide"
  misc_feature 1..30: note = source = /note="mismatch repair Table 4"
  source 1..30: mol_type = other DNA
gagcggacagcagcttcctatatgtcgtac

SEQ ID NO: 81 - DNA, 30 bp, synthetic construct
  misc_feature 1..30: note = source = /note="Description of Artificial Sequence: Syntheticoligonucleotide"
  misc_feature 1..30: note = source = /note="mismatch repair Table 4"
  source 1..30: mol_type = other DNA
gagcggacagcagcttcctataactcgtac

SEQ ID NO: 82 - DNA, 30 bp, synthetic construct
  misc_feature 1..30: note = source = /note="Description of Artificial Sequence: Syntheticoligonucleotide"
  misc_feature 1..30: note = source = /note="mismatch repair Table 4"
  source 1..30: mol_type = other DNA
gagcggacagcagcttcctatttctcgtac

SEQ ID NO: 83 - DNA, 30 bp, synthetic construct
  misc_feature 1..30: note = source = /note="Description of Artificial Sequence: Syntheticoligonucleotide"
  misc_feature 1..30: note = source = /note="mismatch repair Table 4"
  source 1..30: mol_type = other DNA
gagcggacagcagcttcctaaatctcgtac

SEQ ID NO: 84 - DNA, 30 bp, synthetic construct
  misc_feature 1..30: note = source = /note="Description of Artificial Sequence: Syntheticoligonucleotide"
  misc_feature 1..30: note = source = /note="mismatch repair Table 4"
  source 1..30: mol_type = other DNA
gagcggacagcagcttcctttatctcgtac

SEQ ID NO: 85 - DNA, 30 bp, synthetic construct
  misc_feature 1..30: note = source = /note="Description of Artificial Sequence: Syntheticoligonucleotide"
  misc_feature 1..30: note = source = /note="mismatch repair Table 4"
  source 1..30: mol_type = other DNA
gagcggacagcagcttccaatatctcgtac

SEQ ID NO: 86 - DNA, 30 bp, synthetic construct
  misc_feature 1..30: note = source = /note="Description of Artificial Sequence: Syntheticoligonucleotide"
  misc_feature 1..30: note = source = /note="mismatch repair Table 4"
  source 1..30: mol_type = other DNA
gagcggacagcagcttcgtatatctcgtac

SEQ ID NO: 87 - DNA, 30 bp, synthetic construct
  misc_feature 1..30: note = source = /note="Description of Artificial Sequence: Syntheticoligonucleotide"
  misc_feature 1..30: note = source = /note="mismatch repair Table 4"
  source 1..30: mol_type = other DNA
gagcggacagcagcttgctatatctcgtac

SEQ ID NO: 88 - DNA, 30 bp, synthetic construct
  misc_feature 1..30: note = source = /note="Description of Artificial Sequence: Syntheticoligonucleotide"
  misc_feature 1..30: note = source = /note="mismatch repair Table 4"
  source 1..30: mol_type = other DNA
gagcggacagcagctacctatatctcgtac

SEQ ID NO: 89 - DNA, 30 bp, synthetic construct
  misc_feature 1..30: note = source = /note="Description of Artificial Sequence: Syntheticoligonucleotide"
  misc_feature 1..30: note = source = /note="mismatch repair Table 4"
  source 1..30: mol_type = other DNA
gagcggacagcagcatcctatatctcgtac

SEQ ID NO: 90 - DNA, 30 bp, synthetic construct
  misc_feature 1..30: note = source = /note="Description of Artificial Sequence: Syntheticoligonucleotide"
  misc_feature 1..30: note = source = /note="mismatch repair Table 4"
  source 1..30: mol_type = other DNA
gagcggacagcaggttcctatatctcgtac

SEQ ID NO: 91 - DNA, 30 bp, synthetic construct
  misc_feature 1..30: note = source = /note="Description of Artificial Sequence: Syntheticoligonucleotide"
  misc_feature 1..30: note = source = /note="mismatch repair Table 4"
  source 1..30: mol_type = other DNA
gagcggacagcaccttcctatatctcgtac

SEQ ID NO: 92 - DNA, 30 bp, synthetic construct
  misc_feature 1..30: note = source = /note="Description of Artificial Sequence: Syntheticoligonucleotide"
  misc_feature 1..30: note = source = /note="mismatch repair Table 4"
  source 1..30: mol_type = other DNA
gagcggacagctgcttcctatatctcgtac

SEQ ID NO: 93 - DNA, 30 bp, synthetic construct
  misc_feature 1..30: note = source = /note="Description of Artificial Sequence: Syntheticoligonucleotide"
  misc_feature 1..30: note = source = /note="mismatch repair Table 4"
  source 1..30: mol_type = other DNA
gagcggacaggagcttcctatatctcgtac

SEQ ID NO: 94 - DNA, 30 bp, synthetic construct
  misc_feature 1..30: note = source = /note="Description of Artificial Sequence: Syntheticoligonucleotide"
  misc_feature 1..30: note = source = /note="mismatch repair Table 4"
  source 1..30: mol_type = other DNA
gagcggacaccagcttcctatatctcgtac

SEQ ID NO: 95 - DNA, 30 bp, synthetic construct
  misc_feature 1..30: note = source = /note="Description of Artificial Sequence: Syntheticoligonucleotide"
  misc_feature 1..30: note = source = /note="mismatch repair Table 4"
  source 1..30: mol_type = other DNA
gagcggactgcagcttcctatatctcgtac

SEQ ID NO: 96 - DNA, 30 bp, synthetic construct
  misc_feature 1..30: note = source = /note="Description of Artificial Sequence: Syntheticoligonucleotide"
  misc_feature 1..30: note = source = /note="mismatch repair Table 4"
  source 1..30: mol_type = other DNA
gagcggagagcagcttcctatatctcgtac

SEQ ID NO: 97 - DNA, 30 bp, synthetic construct
  misc_feature 1..30: note = source = /note="Description of Artificial Sequence: Syntheticoligonucleotide"
  misc_feature 1..30: note = source = /note="mismatch repair Table 4"
  source 1..30: mol_type = other DNA
gagcggtcagcagcttcctatatctcgtac

SEQ ID NO: 98 - DNA, 30 bp, synthetic construct
  misc_feature 1..30: note = source = /note="Description of Artificial Sequence: Syntheticoligonucleotide"
  misc_feature 1..30: note = source = /note="mismatch repair Table 4"
  source 1..30: mol_type = other DNA
gagcgcacagcagcttcctatatctcgtac

SEQ ID NO: 99 - DNA, 30 bp, synthetic construct
  misc_feature 1..30: note = source = /note="Description of Artificial Sequence: Syntheticoligonucleotide"
  misc_feature 1..30: note = source = /note="mismatch repair Table 4"
  source 1..30: mol_type = other DNA
gagccgacagcagcttcctatatctcgtac

SEQ ID NO: 100 - DNA, 30 bp, synthetic construct
  misc_feature 1..30: note = source = /note="Description of Artificial Sequence: Syntheticoligonucleotide"
  misc_feature 1..30: note = source = /note="mismatch repair Table 4"
  source 1..30: mol_type = other DNA
gaggggacagcagcttcctatatctcgtac

SEQ ID NO: 101 - DNA, 30 bp, synthetic construct
  misc_feature 1..30: note = source = /note="Description of Artificial Sequence: Syntheticoligonucleotide"
  misc_feature 1..30: note = source = /note="mismatch repair Table 4"
  source 1..30: mol_type = other DNA
gaccggacagcagcttcctatatctcgtac

SEQ ID NO: 102 - DNA, 30 bp, synthetic construct
  misc_feature 1..30: note = source = /note="Description of Artificial Sequence: Syntheticoligonucleotide"
  misc_feature 1..30: note = source = /note="mismatch repair Table 4"
  source 1..30: mol_type = other DNA
gtgcggacagcagcttcctatatctcgtac

SEQ ID NO: 103 - DNA, 30 bp, synthetic construct
  misc_feature 1..30: note = source = /note="Description of Artificial Sequence: Syntheticoligonucleotide"
  misc_feature 1..30: note = source = /note="mismatch repair Table 4"
  source 1..30: mol_type = other DNA
cagcggacagcagcttcctatatctcgtac

SEQ ID NO: 104 - DNA, 30 bp, synthetic construct
  misc_feature 1..30: note = source = /note="Description of Artificial Sequence: Syntheticoligonucleotide"
  misc_feature 1..30: note = source = /note="mismatch repair Table 6"
  source 1..30: mol_type = other DNA
gagcggacagcagcttcctatatctcgtat

SEQ ID NO: 105 - DNA, 30 bp, synthetic construct
  misc_feature 1..30: note = source = /note="Description of Artificial Sequence: Syntheticoligonucleotide"
  misc_feature 1..30: note = source = /note="mismatch repair Table 6"
  source 1..30: mol_type = other DNA
gagcggacagcagcttcctatatctcgtgc

SEQ ID NO: 106 - DNA, 30 bp, synthetic construct
  misc_feature 1..30: note = source = /note="Description of Artificial Sequence: Syntheticoligonucleotide"
  misc_feature 1..30: note = source = /note="mismatch repair Table 6"
  source 1..30: mol_type = other DNA
gagcggacagcagcttcctatatctcgcac

SEQ ID NO: 107 - DNA, 30 bp, synthetic construct
  misc_feature 1..30: note = source = /note="Description of Artificial Sequence: Syntheticoligonucleotide"
  misc_feature 1..30: note = source = /note="mismatch repair Table 6"
  source 1..30: mol_type = other DNA
gagcggacagcagcttcctatatctcatac

SEQ ID NO: 108 - DNA, 30 bp, synthetic construct
  misc_feature 1..30: note = source = /note="Description of Artificial Sequence: Syntheticoligonucleotide"
  misc_feature 1..30: note = source = /note="mismatch repair Table 6"
  source 1..30: mol_type = other DNA
gagcggacagcagcttcctatatcttgtac

SEQ ID NO: 109 - DNA, 30 bp, synthetic construct
  misc_feature 1..30: note = source = /note="Description of Artificial Sequence: Syntheticoligonucleotide"
  misc_feature 1..30: note = source = /note="mismatch repair Table 6"
  source 1..30: mol_type = other DNA
gagcggacagcagcttcctatatcccgtac

SEQ ID NO: 110 - DNA, 30 bp, synthetic construct
  misc_feature 1..30: note = source = /note="Description of Artificial Sequence: Syntheticoligonucleotide"
  misc_feature 1..30: note = source = /note="mismatch repair Table 6"
  source 1..30: mol_type = other DNA
gagcggacagcagcttcctatatttcgtac

SEQ ID NO: 111 - DNA, 30 bp, synthetic construct
  misc_feature 1..30: note = source = /note="Description of Artificial Sequence: Syntheticoligonucleotide"
  misc_feature 1..30: note = source = /note="mismatch repair Table 6"
  source 1..30: mol_type = other DNA
gagcggacagcagcttcctatacctcgtac

SEQ ID NO: 112 - DNA, 30 bp, synthetic construct
  misc_feature 1..30: note = source = /note="Description of Artificial Sequence: Syntheticoligonucleotide"
  misc_feature 1..30: note = source = /note="mismatch repair Table 6"
  source 1..30: mol_type = other DNA
gagcggacagcagcttcctatgtctcgtac

SEQ ID NO: 113 - DNA, 30 bp, synthetic construct
  misc_feature 1..30: note = source = /note="Description of Artificial Sequence: Syntheticoligonucleotide"
  misc_feature 1..30: note = source = /note="mismatch repair Table 6"
  source 1..30: mol_type = other DNA
gagcggacagcagcttcctacatctcgtac

SEQ ID NO: 114 - DNA, 30 bp, synthetic construct
  misc_feature 1..30: note = source = /note="Description of Artificial Sequence: Syntheticoligonucleotide"
  misc_feature 1..30: note = source = /note="mismatch repair Table 6"
  source 1..30: mol_type = other DNA
gagcggacagcagcttcctgtatctcgtac

SEQ ID NO: 115 - DNA, 30 bp, synthetic construct
  misc_feature 1..30: note = source = /note="Description of Artificial Sequence: Syntheticoligonucleotide"
  misc_feature 1..30: note = source = /note="mismatch repair Table 6"
  source 1..30: mol_type = other DNA
gagcggacagcagcttcccatatctcgtac

SEQ ID NO: 116 - DNA, 30 bp, synthetic construct
  misc_feature 1..30: note = source = /note="Description of Artificial Sequence: Syntheticoligonucleotide"
  misc_feature 1..30: note = source = /note="mismatch repair Table 6"
  source 1..30: mol_type = other DNA
gagcggacagcagcttcttatatctcgtac

SEQ ID NO: 117 - DNA, 30 bp, synthetic construct
  misc_feature 1..30: note = source = /note="Description of Artificial Sequence: Syntheticoligonucleotide"
  misc_feature 1..30: note = source = /note="mismatch repair Table 6"
  source 1..30: mol_type = other DNA
gagcggacagcagctttctatatctcgtac

SEQ ID NO: 118 - DNA, 30 bp, synthetic construct
  misc_feature 1..30: note = source = /note="Description of Artificial Sequence: Syntheticoligonucleotide"
  misc_feature 1..30: note = source = /note="mismatch repair Table 6"
  source 1..30: mol_type = other DNA
gagcggacagcagctccctatatctcgtac

SEQ ID NO: 119 - DNA, 30 bp, synthetic construct
  misc_feature 1..30: note = source = /note="Description of Artificial Sequence: Syntheticoligonucleotide"
  misc_feature 1..30: note = source = /note="mismatch repair Table 6"
  source 1..30: mol_type = other DNA
gagcggacagcagcctcctatatctcgtac

SEQ ID NO: 120 - DNA, 30 bp, synthetic construct
  misc_feature 1..30: note = source = /note="Description of Artificial Sequence: Syntheticoligonucleotide"
  misc_feature 1..30: note = source = /note="mismatch repair Table 6"
  source 1..30: mol_type = other DNA
gagcggacagcagtttcctatatctcgtac

SEQ ID NO: 121 - DNA, 30 bp, synthetic construct
  misc_feature 1..30: note = source = /note="Description of Artificial Sequence: Syntheticoligonucleotide"
  misc_feature 1..30: note = source = /note="mismatch repair Table 6"
  source 1..30: mol_type = other DNA
gagcggacagcaacttcctatatctcgtac

SEQ ID NO: 122 - DNA, 30 bp, synthetic construct
  misc_feature 1..30: note = source = /note="Description of Artificial Sequence: Syntheticoligonucleotide"
  misc_feature 1..30: note = source = /note="mismatch repair Table 6"
  source 1..30: mol_type = other DNA
gagcggacagcggcttcctatatctcgtac

SEQ ID NO: 123 - DNA, 30 bp, synthetic construct
  misc_feature 1..30: note = source = /note="Description of Artificial Sequence: Syntheticoligonucleotide"
  misc_feature 1..30: note = source = /note="mismatch repair Table 6"
  source 1..30: mol_type = other DNA
gagcggacagtagcttcctatatctcgtac

SEQ ID NO: 124 - DNA, 30 bp, synthetic construct
  misc_feature 1..30: note = source = /note="Description of Artificial Sequence: Syntheticoligonucleotide"
  misc_feature 1..30: note = source = /note="mismatch repair Table 6"
  source 1..30: mol_type = other DNA
gagcggacaacagcttcctatatctcgtac

SEQ ID NO: 125 - DNA, 30 bp, synthetic construct
  misc_feature 1..30: note = source = /note="Description of Artificial Sequence: Syntheticoligonucleotide"
  misc_feature 1..30: note = source = /note="mismatch repair Table 6"
  source 1..30: mol_type = other DNA
gagcggacggcagcttcctatatctcgtac

SEQ ID NO: 126 - DNA, 30 bp, synthetic construct
  misc_feature 1..30: note = source = /note="Description of Artificial Sequence: Syntheticoligonucleotide"
  misc_feature 1..30: note = source = /note="mismatch repair Table 6"
  source 1..30: mol_type = other DNA
gagcggatagcagcttcctatatctcgtac

SEQ ID NO: 127 - DNA, 3210 bp, synthetic construct
  misc_feature 1..3210: note = source = /note="Description of Artificial Sequence: Syntheticpolynucleotide"
  misc_feature 1..3210: note = source = /note="APG05083.1 mammalian codon optimized sequence"
  source 1..3210: mol_type = other DNA
atgagagagctggattaccggatcggcctggatatcgggaccaactccattggatggggcatcatcgagctgtcttggaacaaagacagagaacagtacgagaaggcaagaatcgtggacaagggcgtgagaatgttcgacaaggccgaaatacccaagaccggagccagcctggccgagcctagaagaattgccagatcaagcagaagacggctcaacagaaagtctcagagaaaaaaagatattcggaacctgctggtccagcacgagatcatcagccaaaaggaactcgctagcctgtatcctctgaccaagagcagcatggacatttgggacatcagactggacggcctggacagactgctggatagattcgagtggaccagattgctgatccacctggctcagcggagaggcttcaaaagcaaccggaagagcgagctgaaggacgtggaaaccggcaaggtgctctccagcatccaggctaatgagaagcggctgtccctgtacagaactgtgggcgagatgtggatgaagaatgaagattttagcaagtacgacaaaagaagaaatagtagcaacgaatacgtgttctctgtgtcccgggccgacctggaaaaggaaatcgtgacactgtttgaagctcagcggaagttccagagcagctatgccagcgccgatcttcaaaaaacctacctccagatctgggcccatcaactgcctttcgcctctggcaacgccatcgttaacaaggtgggctactgcagcctactgaaaggcaaggagaagagagttcctaaggccacctacaccttccaatacttcagcaccctggatcagatcaacagaaccagactgggcccaaacttccagcccttcaccaaggaacagagagatgtgatcctggacgagatgtttaaccggaccgattattacaagaagaagaccatccctgaggtgacgtactacgatatcagaaaatggctggccctggacgagacaatccagttcaagggcctgacctacgaccctaatgaagaactgaagaaaattgagctaaagtcttttatcaatctgaagcctttctacgagataaagaaggtggtgacaaactacgccaagaagacaaatgaggcctttagcacactggactatgacacctttgcctacgccctgacagtgtacaagaccgacaaggacatccgctcctacctgaaaaagagtaacaacctgtccaaatgctgctacgacgaccaactgatcgaggaattgctgacactgagctacaccaaattcggccacctgagcttcaaggctatcaaccacgttctgcctatcatgcaggagggcagaacctaccaggaggccattcaccagctcggctacgatgccacaaacctcaaaaaagagaaccggtctatgttcctgcctctgttccctgacgagatcaccaaccccatcgtgaagagggccctgacccaggccaggaaggtggtcaacgccatcatcagacgatacgggtctccaaacagcgtgcacatcgagctggccagagagctgagcaagagccacgacgagagaacaaagatcatgaaagctcatgatgaaaactacaaaaagaacaagggcgctatcagcatcctgatcgagaacggtattctgaatcctacaggttatgacatcgtccggtacaagctgtggaaggaacagggcgagagatgcgcctattctctgaaacagatccccgccaacaccttcttcaacgaaatgaagaaggagcggtccggcagccctgtgctggaaatcgatcacatcctgccctacagccagagcttcatcgacagctaccacaacaaagtgctggtgtacggggatgagaaccagaaaaagggcaatagaatcccgtacacctacttcctggaaggcaacaaggactgggagtctttcgagagctatgtgcgcctgaactcctttttcagcaagaaaaagcgaggatatctgctgaagaaggcttacctgccaagagagagtaacatgatcaaggaacggcacctcaacgacacccggtacgccagctcctacctgaagaacttcatcgagaagaatctgaagttcaaggaggtggaaggctctacccggaagaagcacgtgcaaaccgtgaacggcataatcacagcccacctgagaaagagatggggcctggaaaaggaccgccaggagacatatcttcatcacgctatggacgccatcatcgtggcatgcaccgaccaccacatggtgacaaaggtgaccgagtactaccagatcaaagaaagcaataaatctattagaaagccttacttccccctgccttgggtgggctttagagaggaaattctgtcccacctggctcggcagcctatcgccagaaagatctctgaagagctgaagatcggataccagagcttcgattacatcctcgtgtctagaatgcctaaaagatcagtgaccggcgccgcccacgagcagaccattatgaaaaagggaggcatcgacaaaaaaggaaaaaccatcatcattaagcgggtctacctgaaggatatcaagttcgacgagaatggcgatttcaagatggttggaaaggaacaggacctggctacctacgaggccatcaagcagagatacatcgagtacggcaaggaatccaagaaggccttcgagacccctctgtataagcccagcaagaaaggcaaaggcaacctgatcaagaagatcaaagtggaagtgcaaaccaagagctttgtgagagaagtcaacggcggagtggcccagaacggcgatctggtgcgggttgacctgttcgagaaggataatagatactacatgatccccatctacgtgatggataccgtgcacagcgaacttcctaacaaggccgtgaccagcagcaaaggctatgagcaatggctgaccatcgacaacagcttcaccttcaagttcagcctatacccctacgacctggtgcggctggtcaagggtaacgaggacagattcctgtacttttccaccctggatattaacagtgatagactcaacttcaaagacgtcaacaagcccagcaagcaggccgagaacagatatagcctgaagacaatcgaaaacctggaaaaatacgaggtgggcgtcctgggcgacctcagatttgtgagacaggagatcagaaagaacttc

SEQ ID NO: 128 - DNA, 3213 bp, synthetic construct
  misc_feature 1..3213: note = source = /note="Description of Artificial Sequence: Syntheticpolynucleotide"
  misc_feature 1..3213: note = source = /note="APG07433.1 mammalian codon optimized sequence"
  source 1..3213: mol_type = other DNA
atgagagagctggactacagaattggcctggacatcggcaccaacagcatcggatggggcgtgatcgagctgtcctggaacaaagaccgggagagatacgagaaggtcagaatcgtggatcaaggcgtgagaatgttcgacagagccgagatgcccaagacaggcgccagcttagctgaacccagaagaatcgccagatccagcagacggagactgaatcgcaagtcccagagaaagaaaaacatccggaacctgctggtgcaacacggcgtgatcacacaggaggaactggatagcctgtaccccctgagcaaaaagagcatggacatctggggcattcggctcgacggcctggacagactcctcaatcatttcgagtgggccagactgctgatccacctggctcagagacggggctttaagtccaacagaaagagtgaactgaaagatacagagacaggcaaggtgctgagcagcatccaactgaacgagaaacggctgagcttgtatagaaccgtgggcgagatgtggatgaaggaccccgacttctctaaatacgataggaagagaaatagccccaacgaatacgtgttcagcgtgtctagagccgagctggaaaaggaaatcgtgaccctgttcgccgcccagcggagattccagagcccttacgccagcaaagatctgcaggagacatatctgcagatctggacccaccaactgcctttcgccagcggcaatgccatcctgaacaaggtcggatactgctccctgttgaaaggcaaagaaagaaggattcccaaggctacatacaccttccaatacttctctgctctggaccaggtgaatcggaccagactgggacctgatttccagcccttcaccaaggagcaacgggaaattatcttgaacaacatgttccagaggacagattactacaagaagaaaaccatccccgaggtgacctactatgacatacggaagtggctggaattggacgagacaattcagttcaagggcctgaactacgaccctaacgaggaactgaagaagatcgagaagaagccttttatcaatctgaaggccttctacgagatcaacaaggtggtggccaactacagcgaaagaaccaacgagaccttctccaccctggactacgacggcatcggctacgccctgaccgtgtacaaaaccgacaaggatatccgcagctacctgaagagcagtcacaacctacctaagagatgctacgacgaccaactgatcgaggaactgctgagcctgagctacacaaagttcggccacctgtccctgaaagccatcaaccacgtgctgtctatcatgcagaagggcaatacctacaaggaagccgtggaccaactgggctacgacaccagcggccttaagaaggagaagaggtccaagttcctgccacctatttctgatgaaatcacgaatccaatcgtgaaaagggccctgacccaggccagaaaagtggtgaacgccataattagaagacacggatctcctcactccgtgcacatcgagctggccagagagctgagcaagaaccacgacgagcggacaaagatcgtcagcgcccaggatgaaaactacaagaaaaacaagggcgctatcagcatcctgtctgagcacggcatcctgaaccctacaggctacgacatcgtgagatacaaactgtggaaggagcagggcgaacggtgcgcctacagcctgaaggaaatccctgccgatacatttttcaacgagctgaagaaggaacgcaacggcgcccctatccttgaagtggaccacatcctgccctacagccagtccttcatcgactcctaccacaacaaggtcctggtgtacagcgacgaaaaccggaaaaagggcaacagaatcccttatacctacttcctggaaaccaacaaggattgggaggcctttgagcggtacgtgcggagcaacaaattcttctccaagaaaaagcgagagtaccttctgaagcgggcttatctgcctagagaatctgagctgatcaaagaacgccacctgaacgacaccagatacgcctctaccttcctgaagaacttcatcgagcagaacctgcagttcaaggaagccgaggacaaccccagaaaaagacgggtgcaaaccgtgaacggcgttatcaccgcccacttcagaaagcggtggggcctggagaaggaccggcaggagacatacctccatcacgctatggacgccatcatcgtggcttgtacagaccaccacatggtcaccagagtgaccgagtactatcagatcaaggaaagcaacaagagcgtgaagaagccctattttcctatgccttgggaaggcttccgggacgagctgctgagccacttggcttctcagcctatcgccaagaaaatcagcgaggaactgaaggccggctaccagagcctggactacatcttcgtgtccagaatgcctaagagaagcattacaggcgctgctcataagcagaccatcatgcggaagggaggaattgacaagaagggcaaaacaatcatcatcgaacggctgcacctgaaggatatcaagttcgacgagaacggagatttcaagatggtgggcaaggaacaggacatggccacatacgaagctattaaacagagatacctggagcacggcaagaatagcaagaaggccttcgagacccctctgtacaagcccagcaaaaagggcacaggtaacctgatcaagcgggtgaaggtggaaggacaggccaagagctttgtgagggaagtgaacggcggagtggcccaaaatggcgatctggttagagttgatttgtttgagaaggatgataagtactacatggtccccatctacgtgccagacaccgtgtgtagcgagctgcccaaaaaggtggtcgccagctctaagggctatgagcagtggctgacactggataacagcttcacctttaagttcagcctgtacccttatgatctggtgcggctggtcaagggagatgaggatcggttcctgtactttggcaccctggacatcgacagcgacagacttaacttcaaggacgtgaacaagccaagcaagaagaacgagtaccggtacagcttgaaaaccatcgaggacttggagaagtacgaggtgggcgtgctgggcgatctaagactggtccggaaggaaactcgaagaaacttccac

SEQ ID NO: 129 - DNA, 3213 bp, synthetic construct
  misc_feature 1..3213: note = source = /note="Description of Artificial Sequence: Syntheticpolynucleotide"
  misc_feature 1..3213: note = source = /note="APG07513.1 mammalian codon optimized sequence"
  source 1..3213: mol_type = other DNA
atgcgggaactggattacagaattggactggacatcgggaccaactcaattggctggggagtgatcgagctgagctggaacaaggacagagagcagtacgagaagaccagaatcgtggacaagggcgttaggatgttcgacaaggccgagatccccaagaccggagccagcctggccgagcctagacgtatcgccagatcctccagacgtagactgaacagaaagtcccagaggaagaaggacattcggaacctgctggtgcaacacgagatcattagccaaaaagaactgaccagcctgtaccctctgtctaaatccagcatggacatctgggacatccggctggacggcctggacagactgcttgatagattcgagtgggcccggctcctgatccacctggctcagcggcggggctttaaaagcaaccggaagtctgagcttaaagacgtggaaacaggaaaagttctgtccagcatccaggtgaatgaaaagcggctgagcctgtacagaaccgtgggcgagatgtggatgaagaacgccgattgcagcaagtacggcaaacgtagaaatagccccaacgagtacgtgttcagcgtgtctagagccgacttggagaaagaaattgtgacacttttcgaggcccagcgaaaattccacagcagctacgccagtgtggacctgcagaagacatacatccaaatctgggctcatcaactgccatttgcctctggcaatgccattgtgaacaaggtgggatactgctctctgctgaagggcaaagaaaagagagtgcctaaggccacatacacctttcagtattttaacaccctggaccagatcaaccggacaagactgggccctaacttccaacctttcaccaaggagcagagagatatcatcctagacaaaatgttccagagaaccgactactacaagaaaaaaacaatccctgaggtgacatactacgatatcagaaagtggctggccctggacgaaaccatccagttcaagggcctgacctacgatcctaatgaagaactgaagaagatcgagatgaagccattcatcaacctgaaacctttctacgagatcaagaaggtggtgaccaactacgccaagaagacaaacgaggtgttctctgccctggactatgacaccgtggcttatgccctcaccgtgtacaaaacagacaaggatatcagaagctaccttaagcggtccaacaacctgagcaagagatgttacgacgaccaactgatcgaggaactgctgacactgagctacaccaagttcggccacctgtccttcaaggccatcaatcacgtgctgcccatcatgcaggagggcagaacctaccaagaggctattcaccaactgggctatgacacgaccaacctgaagaaggaaaatagaagcatgttcctgcccatcatccctgacgagatcaccaaccctatcgtgaagcgggccctgacgcaggcccggaaagtggtgaatgccatcatccgcagatacggctctcctaattctgtccacatcgagctggccagagagctgagcaaaagccacgacgagcggaagaagatcatgaccgcccacgacgagaactacaagaaaaacaagggcgccgtgtccatcctgatcgataacggcatcctgaatcctacaggatacgatatcgtgcggtacaagctgtggaaggaacagggcgaaagatgcgcctatagcctgaaaaaaatccccgccaacaccttcttcaacgagctaaaaaaggaacggagcggcccacctgtgctggaagtggaccacatcctgccctacagccagagcttcatcgacagctaccacaacaaggtgctggtgtacggcgacgagaaccagaagaagggcaatagaatcccttacacatttttcagcgaagaagataaggaatgggagagcttcgagagctacgttcggagcaacagcttcttcagcaagaaaaagcgcggctacctgctgaagaaggcctacctgcccagagaaagcaacctgatcaaggaacggcacctcaacgacacacggtacgccagcagttacctgaagaatttcatcgagaagaacctgaagttcaaggaagccgtggggatcacccggaagaagtacgtgcaaaccgtgaacggcgtgatcaccgcccacctgcggaagcggtggggccttgagaaggaccggcaggagacctacctgcaccacgctatggacgccatcatcgtggcctgcaccgatcaccacatggtgacgaaggtgaccgagtactaccagatcaaagaaggcaataagagcatcaagaagccttattttcctctgccctggatgggcttcagagaagaaatcctgtctcacctggagtctcaacctatcgccagaaaaatttctgaagagctgaaaattggataccagtcccccgattacatcctggtcagccggatgcctaagagaagcgtgaccggcagcgcccacgatcagaccgtgatgaagaagggcgatatcgataagaagggcaagacaatcatcatcaagcgggtgcacctgaaggatatcaagttcgacgaaaatggcgacttcaaaatggtgggcaaggagcaggacctggctacatacgaagctatcaaacagagatacctggagtaccggaaggaaagcaagaaggccttcgagacccctctgtacaagccatctaaaaaaggaaaaggtaacctgatcaaaaagatcaaggtggaagtgcaaaccaaatctttcgtgagagagattaacggcggagtggcccagaacggcgacctggttagagtggatctgttcgagaaggacaacagatattacatggtccccatctacgtggtggacaccgtgcggtctgaactccccaacaaagcagtgacaagctccaaaggctatgaacagtggctgagcatcgacaatagtttcaccttcaagtttagtctgtacccctacgacctcgtgcggctggtcaagggcgacgaggatcgcttcctgtacttctccaccctggatatcaacagcgacagactgaacttcaaggacgtgaacaagcctagcaagcaggctgaataccggtacagcctgaagacgatcgagaacctggaaaaatacgagatcggtgttctgggagatctgagactcgttagacaggagacaagaaaaattttcaag

SEQ ID NO: 130 - DNA, 3216 bp, synthetic construct
  misc_feature 1..3216: note = source = /note="Description of Artificial Sequence: Syntheticpolynucleotide"
  misc_feature 1..3216: note = source = /note="APG08290.1 mammalian codon optimized sequence"
  source 1..3216: mol_type = other DNA
atgagcgagctggattatagaatcggcctggatatcggcaccaattctatcggatggggagtgatcgagctgttctggaacaaggatcgggaacggtacgagaaggtccgcatcgtggacaaaggggtcagaatgtttgacaaggccgagatccccaacaagggcgccagcctggccgagcctcggagaatcgcccggagcagcagaagacgcctgaacaggaagtcccaaaggaagaaggagatccggaacctgctggtgcaacacggcatgatcacccaagaggaactggacctcctgtaccctctgagcaaaaagtccatcgatatctgggacatcagactagacggcctggacagactgctgaaccacttagagtgggctagactgctgattcacctggcccagcggcggggcttcaagagcaaccgcaaaagcgagctgaaggacgctgaaacaggcaaggtgttgtctagcatccaggtgaacgagaagcggctgttcctgtacagaaccgtgggggaaatgtggatcaaggacgcagagttcagcaagtacgacaggcgtagaaactccccaaacgaatacgtgttcagcgtgtcaagagccgacctggaaaaggaaatcgtgacactgtttgaggctcagagaaagttccagagcagctatgcctctaaaaatctgcaggagacctacctgcagatctgggcccaccaactgcctttcgccagcggcaatgccatcctgaacaaagtgggctactgcagcctgctgaaagggaaggaaaggcggattcccaaggccacatacaccttccagtacttctccgccctggatcaggttaaccggacccggctcggccctgacttccaacctttcacccaggaacaaaaggagatcatcctggataagatgttccagagaacagactactacaagaagaagaccatccccgaggtttcttattatgatatcagaaagtggctggaactcgacgagacaatccagtttaagggactgaattacgaccccaacgaagagctgaagaagatcgaaaaaaaacctttcatcaacctgaaggccttctacgagatcaagaaggtggttgctaactacgccgaaagaacaaatgaagccttttctaccctggactacgacgctatcgcctatgccctgacagtctacaagaccgacaaggacatccggtcctacctgaagaaatccaacaacctgtccaagcggtgctacgatgatcaactgatcgaggaactgtttaccctgagctacaccaaattcggccacctgtctttcaaggccattaaccacgtgctgcctatcatgcaggagggcagaacctaccaggaggccatacaccaactgggctacgacaccaccaacctgaagaaagagaatagaagcatgttcctgcctctgatccctgacgagatcacaaaccccattgtgaagcgggccatcacccaggccagaaaggtggtgaacgccatcatcagaagatacggctctcctaacagtgtgcacatcgaactggccagagagctgagcaagagccacgatgagcggaaaaagatcatgaccgcccacgacgagaactacaagaaaaataagggcgctatttctatcctgatcgagaacggcattctgaaccctaccggctacgacatcgtgagatacaagctgtggaaggaacaaggcgagagatgcgcctacagcctgaaagaaattccacctgatacttttttcaacgagctgaagaaagaaagaaacggcagccccattctggaagtggaccacatcctgccttacagccagtccttcatcgacagctaccacaacaaagtgctggtgtactctgacgagaacagaaacaagggcaacagaatcccttacacctacttcctggaaacaaacaaggactgggaggcctttgaaagatacgtgcggagtaacaaactgttttctaagaaaaagagagaatatctgctgaagaagacttacctgcctagagagtctgaactaatcaaggaacggcacctgaacgacactcggtatgcttctacattcctgaagaatttcatcgagcagaatctgcagttcaaagaggtcgaggtcaatctgagaaaaaagagagtgcaaaccgtgaatggcgtgatcaccgcccacctcagaaagcgttggggcctggagaagaaccggcaggagacgtacctgcaccacgctatggacgccatcatcgtggcttgtacagaccaccacatggtgacccggataacagagtactaccagatcaaggaatccaacaagagcgtgaagaaaccttacttccccatgccttgggagggctttagagatgagctgttgtctcacctcgctagccagcctatcgcaaagaagatcagcgaggaactgaaggccggctaccagagcagcgactacatcttcgtgtccagaatgcccaagagaagcgtgaccggcgccgcccatgatcagaccatcagaagaaagggcggcatcgacaagaagggcaagacaatcatcattaagcgggtgcggctgaaagatatcaagttcgacgaaaacggcgatttcaagatggtgggcaaagagcaggacctggcaacctacgaggccatcaagcagagatacctggagcacagaaagaacagtaagaaggccttcgagacccctctgtacaaacctagcaagaagggaacaggaaacctgattaagcgggtgaaaatcgagggacagactaaggccttcgtgcgggaagtgaacggaggcgtggcccaaaatagcgacctggtcagagtggacctgttcgagaaggacgacaagtactatatggtgcctatctacgtgccagacaccgtgtgtagcgagctgcctaagaaggtggttaagagcggaaaaggctatgagcagtggctgaccctggacaacagcttcaccttcaagtctagcctgtacccctacgatctggtgcggctcgtgaagggcaacgaggacagattcctgtacttcggcacactggacattgactccgatagactgaatttcaaggatgtgaacaagcccagcaagcagaacgagtaccggtacagcctgaaaacaatcgagaacctggaaaaatacgaggttggagtgctgggagatctgcggctggtgaaacaggagaccaggaggatctttaacaga

SEQ ID NO: 131 - DNA, 4011 bp, synthetic construct
  misc_feature 1..4011: note = source = /note="Description of Artificial Sequence: Syntheticpolynucleotide"
  misc_feature 1..4011: note = source = /note="APG05459.1 mammalian codon optimized sequence"
  source 1..4011: mol_type = other DNA
atgaaaaaagattacgtgatcggcctggacattggcaccaacagcgtcggctgggccgtgatgacagaggactaccaactggtgaagaagaagatgccaatctatggcaatactgagaagaaaaagataaaaaagaatttctggggcgtgcggctgtttgaggagggccacaccgccgaggatcggcggctgaaacggaccgctagaagacggatctctcgccgcagaaatagactgagatatctgcaggccttcttcgaggaagccatgaccgccctggacgagaacttcttcgccagactgcaggagagcttcctggtgcctgaggacaagaaatggcaccggcaccctatcttcgccaagctggaggatgaggtggcctatcacgaaacctaccctacaatctaccacctgagaaagaaactggctgattcctctgaacaggctgacctgagactgatctatctggccctggcccatatcgtgaagtacagaggccacttcctgatcgaaggaaagctgagtaccgagaacatcagcgtcaaggagcagttccagcagttcatgattatctataaccagacatttgtgaacggcgaaagccggctggtgtctgcccctctgcctgagagcgtgctgatcgaagaagagctgaccgaaaaggccagccggacaaagaaatctgagaaggtgctgcaacagtttcctcaggagaaagccaatggactgttcggccagttcctgaaacttatggtaggcaacaaagccgatttcaagaaagtctttggcctggaagaagaggccaaaataacatacgccagcgagtcctacgaggaggatctggaaggcattctggccaaggtgggcgacgagtacagcgatgttttcctggccgctaagaacgtctacgacgccgtggaactgtctaccatcctggccgactccgacaagaagagccacgccaagttgtctagtagcatgatcgttagattcaccgagcaccaggaggacctgaagaagttcaagcggtttatcagagagaattgccccgacgagtacgataacctgttcaagaacgagcaaaaagacggctacgccggctacatcgcccacgccggcaaggtgtcccaactgaagttctaccagtacgtgaagaagataatccaggacatcgccggcgccgaatacttcctggagaaaatcgcccaggagaacttcctgcgaaaacagaggaccttcgacaacggcgtgatcccccaccagatccacctggccgagctgcaggccatcatccacagacaggctgcttactaccctttcctgaaggaaaatcaggaaaagattgagcaactggtgacattcagaatcccctactacgtcggccctctgagcaaaggagatgccagcaccttcgcctggctgaaaagacaaagcgaggaacctatccggccttggaacctgcaagagacagtggacctggaccagtctgctaccgcattcatcgagagaatgaccaacttcgatacctacctgccttctgagaaggtgctgcccaagcacagcctgctctacgaaaaatttatggtgttcaacgagctgaccaagatttcttacactgatgacagaggcatcaaggccaacttcagcggcaaggagaaggagaagatattcgactacctgtttaagacccgccggaaggtgaagaaaaaggatatcatccagttctaccggaacgagtacaacaccgagatcgtcaccctgtctggcctggaagaggaccagttcaatgccagcttcagcacctaccaagatctgctgaagtgcggcctaactagagccgaactggaccaccctgataatgccgagaaactggaggacatcattaagatcctaaccatcttcgaggatagacagcggatcagaacacagctcagcaccttcaagggacagttcagcgccgaggtgctgaagaagctggaacggaagcactacaccggctggggcagactgtccaagaaactcatcaacggcatctacgacaaggaatccggaaagacaatcctggactacctgatcaaagatgacggcgtttctaagcactacaacagaaacttcatgcagctaatcaacgacagccaactgagcttcaagaacgccatccagaaggcccagagcagcgagcatgaggaaaccctgtctgagaccgtgaacgagctggccggcagccctgccatcaagaaaggcatctaccagagcttaaaaatcgttgatgagctggttgccatcatgggctacgcccctaagagaatcgtggtggagatggctagagagaaccagacaacaagcaccggaaagagaagaagcatccagaggctgaagatcgtggaaaaagctatggccgagattggaagcaacctgctcaaggaacagcctaccacaaacgagcaactgagagatacaagactcttcctgtattatatgcagaacggtaaggacatgtacaccggcgacgagctgagcctgcacagactgtctcactacgacatcgaccacatcattcctcagtccttcatgaaggacgattccctggataacctggtgctggtgggcagcaccgagaaccggggcaagtctgacgacgtgcccagcaaggaagtggtgaaggacatgaaagcctactgggagaagctctacgctgctggcttgatcagccagcggaaattccagagactgacgaagggcgagcagggcggcctgaccctggaggacaaagctcatttcatccagagacaactggtggagacaagacagatcaccaagaacgtggctggaattctggatcagagatacaacgccaacagcaaagaaaaaaaggtgcaaatcataacactgaaagcctctctgaccagccagttccggagcatcttcggcctgtataaggtcagagaagtgaacgactatcaccacggccaggatgcgtacctgaactgcgtggtggccactacactcctgaaagtgtaccccaacctggctcctgagttcgtgtacggcgagtaccccaagtttcaggcctttaaggaaaacaaggctacagccaagaccatcatctacaccaatctgatgcggtttttcaccgaggatgaacccagattcatgaaggacggcgagatcctgtggagcaacagctacctgaagaacattaagaaagaactcaactaccatcagatgaacatagtgaaaaaggtggaagtgcaaaagggtggcttctccaaggaaagcatcaagcctaagggccccagcaacaagctgatccctgtgaagaacgggttggacccccagaaatacggcggatttgactctccagtggtcgcttacacagtgctgtttacccacgagaagggcaaaaaaccactgatcaagcaggagatcctgggaatcaccatcatggaaaagaccagattcgagcagaatcctatcctgttcctggaagaaaaaggcttcctgaggcctagagtgctgatgaagctgcctaaatacaccctgtacgagttccctgagggaagacggcggctgctggccagcgccaaagaagcccagaaagggaatcagatggtgctccccgaacacctgctgaccctgctgtaccacgccaaacagtgtctgctgcctaaccagagcgaatctctcgcttacgtggaacaacaccaaccggagttccaagagatcctggagagagtggtggacttcgctgaggtgcacacactggccaagagcaaggtgcaacagatcgtgaaactgtttgaggcaaaccagaccgcagatgtgaaggaaatcgccgcctccttcatccaactgatgcagttcaacgcaatgggagccccatctacctttaaattcttccagaaggacatcgagcgggcccggtacactagcatcaaggaaatcttcgacgccaccatcatctaccagagcacaaccggcctctacgagacacggagaaaggtggtggac

SEQ ID NO: 132 - DNA, 4308 bp, synthetic construct
  misc_feature 1..4308: note = source = /note="Description of Artificial Sequence: Syntheticpolynucleotide"
  misc_feature 1..4308: note = source = /note="APG04583.1 mammalian codon optimized sequence"
  source 1..4308: mol_type = other DNA
atggccaagaatatcctgggcctggatctgggtacaaacagcatcggctgggctctggtccagcaggacttcgagaacaaggagggaaacatcctgggcatgggatctagaatcatccctatgagccaggacatcctgggcgaattcggtaagggcaacagcatcagccagaccgccgagagaacaggataccggggcgtgcgtagactgagagagagacacctcctgagaagagagagactgcatagagtgctgcacctgctcggctttctgcctaagcactacgatgaaaaaatcgactttacacaaagattcggcaagttcatcaaccaggctgagcctaagctggcttttgatagcgagttcctgttcaaggacagcttccacgagatgctggccgacttcaagcagaatcaacctgaattcctgaaagacaagaacggagaggactgcctggttccttacgactggaccatctactacctgagaaagaaggctctgacccagaagatcgagaaatacgaactagcttggctgatcctgaacttcaaccaaaagcggggctactaccagcttagaggcgaagaagagaaggaaaaccctaacaaactggtgggcttccactctctgaagattgttgatgtgatccctgatgccgagaccaacaaaaagggcgagacatggtacagcctgcacctggaaaacggctgggtgtacaggcggagcagcaagatcagcctggccgactggaaggacaaggttcgggacttcatcgtcactacagatctgaacgacgatggcagcgagaagctggacaaggacggcatcgtgaagaggtccttcagagccccttctgccgacgattggacactcctgaaaaaaaagactgagaaggacatcgacaactccaacaagactgtgggcacctacatctacgacaacttgctgctgaaccctaaacagaagatcaaggggaaaatggtcagaaccatcgaacgaaagttctacaagcaggagctggagcaaatcctgaaaacccagaaagaatttcactccgagctgcagtctgaaaacctgctgcaggactgcgtgagggagctgtaccggaacaacgagcagcaccagcagatgctggaagccaaggattttgtgcacctgttcctgaacgatatcatcttctaccagagacccctgcgcagccagaaaagctctattagcaactgcaccctggaattccggaagagcaagaacgagaatggagaagaagtgatccaccggctgaaggtgatcgccaagtccaacccctactatcaagagtttcggctgctgcagtgggtgcaaaacctggctatctacactaaggacgacgacaaaaacgtcacaaacgaattcctgaagagcacccaggactgggaggatctgctgagatggctgcacagcaagaaagaaatcaagcaggatgccctgatcaaattcctgatcgaaaagaaaggcctgaagggtaaggccctgaccattgaagtggctaagtacagatggaattacgtgcaagacaaggattatcctggcaacgagacaagatacctgattcagagccggctggacaaggtggaatacgcccctaaggacttcctcacgtacgaaaatgagatggccctgtggcacatcatctactctatcaacgataagatcgaatacgaaaaggccctaaagagcttcgccaacaagaaaggtctcgacgaggtgaccttcgtggaagcctttaagaaattcccacctttcaagagcgattacggcagcttcagcgagaaggccatcaagaagctgctgcctctcatgcggttcggcacacaatggaactgggacaacatcgaccagaactcgaaggaaaggattggaaaaatcctgaccggcgagtacgacgagaatatcaagggtagagtgcgggaaaaagctagacacctgaacagcgagacggactttcaggcgctccctctgtggctggcccagtacgtggtgtacggcagacatagcgaagctgacatcgccggcaagtggaatagtgtggacgacctgaagcagttcttggacgacttcaagcaacacagcctgagaaatcccattgtagaacaggtgattactgagacactgcgggccgtgaaggatatctggaacttctacggcaagggcgccaaggactttttctctgagatccacatcgagctgggaagagagatgaaaaacaccgccgacgagagaaaaaggattaccacaatggtgacagataatgagaataccaatctgagaatcaaagctctgctggctgagatggccctggatcagaacgtggacaatgtgcggccttacagccccatgcagcaagaaatcctgaaaatctatgaggaaggcgtgctgaacgccgaagagaacatcgacgatgacatcctgaagatctctaaaactgctcagcctagcgctaccgatctgaagagatacaagctgtggctggaacagaagtacagaagcccctataccggacagatgatccctctgaacaagctgttcacccctgagtatgaaatcgagcacattatcccccagagcagatacttcgacgattctatgagcaacaaggtgatctgcgaggccgccgtgaacaagctgaaggataaccagatcggcctggtgttcatcaagaaccaccacggcgaagtggtggactttggcatgggcaagcaggtgaaaatcctggaggtgtctgattacgaagatttcgtgaagcagaactacaacaaaaacagaggcaaacggaacaagctgctcctcgaagatatccccgagaaaatgattgaacggcaactgaacgataccagatatatcagcaagtacatcactcaggtgctgtctaatatcgtcagagacgacaaggaaggctctaaggatgacggagtgaacagcaagaacattgtgcccggcaacggcaagattacaaccagactcaagcaggattggggcctgaacgatgtgtggaacgacctggtgctgcctagattcgagagaatgaacaccctcacaaactccaatgattttacaagcaagaacacacacggcaagaccattcctaccgtgcctatcgagctgagcaaggggttcagcaaaaagcggatcgatcacagacaccacgctatggacgccctggtgatcgcctgcgccacccgggaccacgtgaacctgctgaataacgaatccagcaagtctgacacaaagcggtacgacctgaatagaaaactgagaaaatacgagaaggtggcctacaacgaccccaaaaccggcgagaggattgaaaaagaagtgccaaaagacttcatcaagccttgggaaacttttaccgaagataccagaacactgctggagaatatcgtgatctcattcaaacagaacctgagagtgatcaacaaggccaccaactactacgagaagatcgagaacggcaaaaaggtgaaggtggaacaaaagggaatcaactgggccgtgagaaaggctctccataaggagaccgtgtccggccaggtccaccttgacagaatcaaggtggccaagggcaagatcctgaccgccacaagaaagaccctggacgcttcttttaacgagaaaaccatagagagcatcaccgataccggcatccagaagatcctgctgaactacctgaagtcaaaggacaacaaccctgaggtggccttctccccagaaggaattgaggaactaaacaagaatatcagactgtacaatgacggcaaggcccaccagccaatcctaaaagtgcgggtgttcgagcagggcagcaagttcacactgggcgagacaggcaacaagacaaccaagttcgtggaagctgccaagggcaccaatcttttcttcggaatctacgaggacaagagcggaaaacgtagctacgagaccatccccctgaatatcgttattgaaagacagaaacagggcctccaggccgtgcccgagaccaacgagaagggcaagcaactgctgttcaccctgagccccaacgacctggtctacgtgccagaggaaggcgtattcgacgagaacaacatcaaggtggatagaatctacaaggtcgtgtctttcagcacataccaatgttttttcgtgcggaacgacgtatctaccagcgtggtcaacaaggtggagtacagcgccctgaacaagatggaaaaatccatcgacaatatcatgatcaaggaaaactgtgtgaagctgaatgtggaccggctgggtaagatcagcaaggcc

SEQ ID NO: 133 - DNA, 4368 bp, synthetic construct
  misc_feature 1..4368: note = source = /note="Description of Artificial Sequence: Syntheticpolynucleotide"
  misc_feature 1..4368: note = source = /note="APG01688.1 mammalian codon optimized sequence"
  source 1..4368: mol_type = other DNA
atgatgatcaagaacattctgggactggatttgggcacaaacagcattggatgggctctgatcaagcaggacttcgagaacaaacacggcgagatcctgggcatgggcagcagaatcatccctatgagccaggatatcctgggcgatttcggcaaagggaactcgataagccagactgctgacagaaccaagtacagaagcgtgcggagactgagagaaagattcttgctgcggcgggaacgcctgcaccgggtgctccacctgctgaacttcctccctcaacactacgcctctcagatcgacttcgagaagaagttcggcaagtttaagtctgagaccgaacctaagctggcctgggaaaactggggaggtaaattctctttcctcttccagaacagcttcaacgagatgctggaagacttcaaggccgccggccagggactcaagattccctatgactggaccatctactacctacggaagaaagctctgtcccagaagatcgagaaagaggagcttgcctggattctgctgaacttcaaccagaagcgaggctactaccagctcagaggcgaggaagaagaagagaacccgaacaagctggtggagttctactccctgaagatcgtggatgtggtcgccgacgagcctcagaaggggaagagcgacatctggtattctctgatcctggaaaacggctgggtctaccgcagagccagtaagatcccactgtttgattggaaggataagaccagagatttcatcgtcaccacagaccttaatgacgacagaagcgtgaagaccgacaaagagggcaacgagaagcggtcctttcgggcccctagcgaaaatgattggaccctggtcaagaagaagacagagcaggagattgaccagagccacaagaccgtgggcacctacatctacgagacactgctgctcaatccaaagcagaaaatcaagggcaagctggtgcgaacaatcgagagaaaattttataaggacgagctgaagcaaatcctggaaaagcagaaggaatttcaccaggagctgaaaaacgacgatctgtacaacgactgcatcagagagctgtaccggaacaacgaggcccaccaactgaccctgagcaagaaagatttcgtgcacctgctgatggacgatctgatcttctaccaaagacccctgcgaagccagaagtccagcatctctaactgcaccctggaattcagaaaatacaaggacgaaaacggcatcgaacacacccagtacctgaaggccatcccaaagagtaatccgtactaccaagagtttagactgtggcagtggatgtacaacctgaacatctacagaaaggacgacgaggctaatgtgaccaaggaattcctgaacaccaataaggacttcgagagcctgtttgagttcctgaataatagaaaggaaatcgaacagaagcctctgatcaagttcctcctggaacagaaagatattaacaagaagctgctgaacgccgaggccgaaaagtatcggtggaattacgtggaagataagaagtatccttgcaacgaaacgaagaccatgatctccagcagactggacaaagtggagaatatctctgacgacttcctgaccagagacattgagcagaagatctggcacatcatctacagcgtcaacgacaagatagaatacgagaaggccctgaagtccttcgccaccagaaacgatctcgacgagaacagctttatcgaagcctttaagaagttcagcccattcaagagcgagtacggatctttttctgagaaagccatcaagaaactgctgcccctgatgagactgggaaagtactggtacgaggacgagattgtgaagcactctgatatttactttaagaacatcgaaaatcttctgggcgacttctccaacagagataaaaaaatatctgaggaagacaaagagaaatggaacaagtctatcaacctgaaactgcaggaggaactgaaggactttcagaccgccgagatcgacctgttccagggccttagactccatatcgcccagtacctggtgtacggccggcacagcgaagccagcatgatcggaaagtggaacagcgccgaggatctggaagaattcctgaaggacttcaagcagcacagcctgagaaaccccatcgtcgagcaagtgatcaccgagaccctgagggtggttaaggatatatggctgaaatacggcaacggcgccaaggacttcttcaacgagattcacatcgagctgggcagagaaatgaagctgcctgccgacgaccggaaaaagctgaccaaccagatcagcgagaacgaaaacacaaatttcagaatcaaggccctgctggctgaaatgatgaacgacagcagtgtggaaaatgtgcggcctttcagccctatgcagcaggagatcctgaagatctatgaagatgacgtcctgaagtctgacattgaaatcgaggatgacatccttaagatctctaaaaccgcccagccttctcctagcgatctcaagcgatacaagctctggctggagcagaagtacaagtctccatacaccggccagatcatacctctgaacaagctgtttacccctgaatacgagatcgagcacattatccctcagtctagatatttcgacgacagcttcagcaacaaagtgatctgcgagagcgccgtgaacaagctgaaagacaactacattggcctggaattcatcaagcaatttggaggcaccatcatcgaactgggctttggcaagtccatcaaagtgttcgagaccaaagagtacgaggacttcgtgaagaaacactacgccaacaatcagggcaagagaaacaagctgctcatggaagacatccccgagaaaatgatcgagagacagatgaacgacaccagatacatctctaagtacatcagcggagtgctgagcaacatcgtcagagtggaagatggatctgatgagggcgtgaacagcaagaacatcgtgcccggcaacggcaagattacaacacaactgaagcaggactggggcctgaatgacgtgtggaacgaccttatcctgccgcggttcgagagaatgaatcaactgaccaacagcaaggtgttcacagcctggaacgaaaactaccagaagttcctgcctacagtgccaatcgaatacagcaaaggcttcagcaagaagcgtatcgatcacagacaccacgccctggatgctctggttatcgcctgcgccaccaaggaccacgtgaacctgctgaacaaccagtctgccaagagcgacaccaagagatacgacttaaagaaaaaaagtatgaaattcgagaaagtggtgtacaatgatgccaagaccggcgaaaagatcgagcgggaagtgcccaagcagttcctgaagccttgggagaacttcaccctggatgtgaagcacaacctggaaacgatcatcgtctcttttaaacaaaatctgcgggtgatcaataaagccacgaactactacgagaagtacgtcgagaaggacggcaccaaaaacaaagagcgcgtggagcagacagggacaaactgggccattagaaagcccatgcacaaggatacagtgtccggcaaagtggaccttccttgggtgaaggtgcctaagggaaagatcctgaccgccacacggaagagcttggatagcagcttcgacctcaagagcatcggctctataacagatacaggcattcagaagatcctaaagaattacctggcattcaaggacggcaaccctgagctggctttcagccctgagggcatcgacgatctgaacaagaacatagagaagtacaacgatggcaaacctcaccagcctatcaacaaggtgcgagtgtttgagctgggcagcaagttccaggtgggacaatctggtaacaagaaggacaagtatgtggaagctgctaagggcaccaatctcttcttcgccgtgtacgaggatgaaaaaggaaagcggaactacgagaccatccctctcaacgaggtgatcgagagacagaagcagggcctgagcgtggtggacctgaagggtacaaacgacttctacctgtgccctaacgactttgtgtacatcccaagcggcgacgagctggaaaacatcaacaacgtggacttcaaggacatcaagaaggagattaacgagcgcatctacaaagtggtgtcttttacaggcaatagactttcttgtatcccttacatggtggccacaacgatcgtcaacaaactcgaattcactcaactgaacaaaatcgagtttaccaaggaaaaagaaatttgtatcaagctcaacgtggacagactgggcaatatctccaaggcc

SEQ ID NO: 134 - DNA, 21 bp, synthetic construct
  misc_feature 1..21: note = source = /note="Description of Artificial Sequence: Syntheticoligonucleotide"
  misc_feature 1..21: note = source = /note="SV40 large T-antigen nuclear localization sequence"
  source 1..21: mol_type = other DNA
cctaagaagaaaagaaaggtg

SEQ ID NO: 135 - DNA, 66 bp, synthetic construct
  misc_feature 1..66: note = source = /note="Description of Artificial Sequence: Syntheticoligonucleotide"
  misc_feature 1..66: note = source = /note="Triple FLAG epitope tag"
  source 1..66: mol_type = other DNA
gactacaaggaccacgacggcgactacaaagatcacgatatcgactacaaggacgacgatgataag

SEQ ID NO: 136 - DNA, 48 bp, synthetic construct
  misc_feature 1..48: note = source = /note="Description of Artificial Sequence: Syntheticoligonucleotide"
  misc_feature 1..48: note = source = /note="Nucleoplasmin nuclear localization sequence"
  source 1..48: mol_type = other DNA
aaaagacctgccgctacaaagaaggccggccaggccaagaaaaagaag

SEQ ID NO: 137 - DNA, 203 bp, synthetic construct
  misc_feature 1..203: note = source = /note="Description of Artificial Sequence: Syntheticpolynucleotide"
  misc_feature 1..203: note = source = /note="Cytomegalovirus mammalian transcription promoter"
  source 1..203: mol_type = other DNA
tgatgcggttttggcagtacatcaatgggcgtggatagcggtttgactcacggggatttccaagtctccaccccattgacgtcaatgggagtttgttttggcaccaaaatcaacgggactttccaaaatgtcgtaacaactccgccccattgacgcaaatgggcggtaggcgtgtacggtgggaggtctatataagcagagct

SEQ ID NO: 138 - DNA, 304 bp, synthetic construct
  misc_feature 1..304: note = source = /note="Description of Artificial Sequence: Syntheticpolynucleotide"
  misc_feature 1..304: note = source = /note="Cytomegalovirus transcription enhancer"
  source 1..304: mol_type = other DNA
cgttacataacttacggtaaatggcccgcctggctgaccgcccaacgacccccgcccattgacgtcaataatgacgtatgttcccatagtaacgccaatagggactttccattgacgtcaatgggtggagtatttacggtaaactgcccacttggcagtacatcaagtgtatcatatgccaagtacgccccctattgacgtcaatgacggtaaatggcccgcctggcattatgcccagtacatgaccttatgggactttcctacttggcagtacatctacgtattagtcatcgctattaccatg

SEQ ID NO: 139 - DNA, 318 bp, synthetic construct
  misc_feature 1..318: note = source = /note="Description of Artificial Sequence: Syntheticpolynucleotide"
  misc_feature 1..318: note = source = /note="Human U6 RNA promoter"
  source 1..318: mol_type = other DNA
tgtacaaaaaagcaggctttaaaggaaccaattcagtcgactggatccggtaccaaggtcgggcaggaagagggcctatttcccatgattccttcatatttgcatatacgatacaaggctgttagagagataattagaattaatttgactgtaaacacaaagatattagtacaaaatacgtgacgtagaaagtaataatttcttgggtagtttgcagttttaaaattatgttttaaaatggactatcatatgcttaccgtaacttgaaagtatttcgatttcttggctttatatatcttgtggaaaggacgaaacacc

SEQ ID NO: 140 - DNA, 20 bp, synthetic construct
  misc_feature 1..20: note = source = /note="Description of Artificial Sequence: Syntheticoligonucleotide"
  misc_feature 1..20: note = source = /note="target for Guide 189"
  source 1..20: mol_type = other DNA
cctgaatgctgtgcggctct

SEQ ID NO: 141 - DNA, 20 bp, synthetic construct
  misc_feature 1..20: note = source = /note="Description of Artificial Sequence: Syntheticoligonucleotide"
  misc_feature 1..20: note = source = /note="target for Guide 185"
  source 1..20: mol_type = other DNA
ggacagtgcgcatctccctg

SEQ ID NO: 142 - DNA, 20 bp, synthetic construct
  misc_feature 1..20: note = source = /note="Description of Artificial Sequence: Syntheticoligonucleotide"
  misc_feature 1..20: note = source = /note="target for Guide 168"
  source 1..20: mol_type = other DNA
cacatctcgagcaagacgtt

SEQ ID NO: 143 - DNA, 20 bp, synthetic construct
  misc_feature 1..20: note = source = /note="Description of Artificial Sequence: Syntheticoligonucleotide"
  misc_feature 1..20: note = source = /note="target for Guide 135"
  source 1..20: mol_type = other DNA
gggccattaaaacctctcca

SEQ ID NO: 144 - DNA, 20 bp, synthetic construct
  misc_feature 1..20: note = source = /note="Description of Artificial Sequence: Syntheticoligonucleotide"
  misc_feature 1..20: note = source = /note="target for Guide 139"
  source 1..20: mol_type = other DNA
aggttttaatggcccagcct

SEQ ID NO: 145 - DNA, 20 bp, synthetic construct
  misc_feature 1..20: note = source = /note="Description of Artificial Sequence: Syntheticoligonucleotide"
  misc_feature 1..20: note = source = /note="target for Guide 143"
  source 1..20: mol_type = other DNA
catggcagtacattagagca

SEQ ID NO: 146 - DNA, 20 bp, synthetic construct
  misc_feature 1..20: note = source = /note="Description of Artificial Sequence: Syntheticoligonucleotide"
  misc_feature 1..20: note = source = /note="target for Guide 190"
  source 1..20: mol_type = other DNA
cctgaatgctgtgcggctct

SEQ ID NO: 147 - DNA, 20 bp, synthetic construct
  misc_feature 1..20: note = source = /note="Description of Artificial Sequence: Syntheticoligonucleotide"
  misc_feature 1..20: note = source = /note="target for Guide 194"
  source 1..20: mol_type = other DNA
gccgcacagcattcaggtcg

SEQ ID NO: 148 - DNA, 20 bp, synthetic construct
  misc_feature 1..20: note = source = /note="Description of Artificial Sequence: Syntheticoligonucleotide"
  misc_feature 1..20: note = source = /note="target for Guide 165"
  source 1..20: mol_type = other DNA
atggggaatgtagcaagacc

SEQ ID NO: 149 - DNA, 20 bp, synthetic construct
  misc_feature 1..20: note = source = /note="Description of Artificial Sequence: Syntheticoligonucleotide"
  misc_feature 1..20: note = source = /note="target for Guide 169"
  source 1..20: mol_type = other DNA
cacatctcgagcaagacgtt

SEQ ID NO: 150 - DNA, 20 bp, synthetic construct
  misc_feature 1..20: note = source = /note="Description of Artificial Sequence: Syntheticoligonucleotide"
  misc_feature 1..20: note = source = /note="target for Guide 173"
  source 1..20: mol_type = other DNA
cttctatagcctccttcccc

SEQ ID NO: 151 - DNA, 20 bp, synthetic construct
  misc_feature 1..20: note = source = /note="Description of Artificial Sequence: Syntheticoligonucleotide"
  misc_feature 1..20: note = source = /note="target for Guide 144"
  source 1..20: mol_type = other DNA
catggcagtacattagagca

SEQ ID NO: 152 - DNA, 20 bp, synthetic construct
  misc_feature 1..20: note = source = /note="Description of Artificial Sequence: Syntheticoligonucleotide"
  misc_feature 1..20: note = source = /note="target for Guide 136"
  source 1..20: mol_type = other DNA
gggccattaaaacctctcca

SEQ ID NO: 153 - DNA, 20 bp, synthetic construct
  misc_feature 1..20: note = source = /note="Description of Artificial Sequence: Syntheticoligonucleotide"
  misc_feature 1..20: note = source = /note="target for Guide 145"
  source 1..20: mol_type = other DNA
catggcagtacattagagca

SEQ ID NO: 154 - DNA, 20 bp, synthetic construct
  misc_feature 1..20: note = source = /note="Description of Artificial Sequence: Syntheticoligonucleotide"
  misc_feature 1..20: note = source = /note="target for Guide 188"
  source 1..20: mol_type = other DNA
ggacagtgcgcatctccctg

SEQ ID NO: 155 - DNA, 20 bp, synthetic construct
  misc_feature 1..20: note = source = /note="Description of Artificial Sequence: Syntheticoligonucleotide"
  misc_feature 1..20: note = source = /note="target for Guide 192"
  source 1..20: mol_type = other DNA
cctgaatgctgtgcggctct

SEQ ID NO: 156 - DNA, 20 bp, synthetic construct
  misc_feature 1..20: note = source = /note="Description of Artificial Sequence: Syntheticoligonucleotide"
  misc_feature 1..20: note = source = /note="target for Guide 196"
  source 1..20: mol_type = other DNA
gccgcacagcattcaggtcg

SEQ ID NO: 157 - DNA, 20 bp, synthetic construct
  misc_feature 1..20: note = source = /note="Description of Artificial Sequence: Syntheticoligonucleotide"
  misc_feature 1..20: note = source = /note="target for Guide 167"
  source 1..20: mol_type = other DNA
atggggaatgtagcaagacc

SEQ ID NO: 158 - DNA, 20 bp, synthetic construct
  misc_feature 1..20: note = source = /note="Description of Artificial Sequence: Syntheticoligonucleotide"
  misc_feature 1..20: note = source = /note="target for Guide 171"
  source 1..20: mol_type = other DNA
cacatctcgagcaagacgtt

SEQ ID NO: 159 - DNA, 20 bp, synthetic construct
  misc_feature 1..20: note = source = /note="Description of Artificial Sequence: Syntheticoligonucleotide"
  misc_feature 1..20: note = source = /note="target for Guide 175"
  source 1..20: mol_type = other DNA
cttctatagcctccttcccc

SEQ ID NO: 160 - DNA, 25 bp, synthetic construct
  misc_feature 1..25: note = source = /note="Description of Artificial Sequence: Syntheticoligonucleotide"
  misc_feature 1..25: note = source = /note="target for Guide 197"
  source 1..25: mol_type = other DNA
cctcacccccacgagcttgtaggaa

SEQ ID NO: 161 - DNA, 25 bp, synthetic construct
  misc_feature 1..25: note = source = /note="Description of Artificial Sequence: Syntheticoligonucleotide"
  misc_feature 1..25: note = source = /note="target for Guide 199"
  source 1..25: mol_type = other DNA
acagtgcgcatctccctggtcacca

SEQ ID NO: 162 - DNA, 25 bp, synthetic construct
  misc_feature 1..25: note = source = /note="Description of Artificial Sequence: Syntheticoligonucleotide"
  misc_feature 1..25: note = source = /note="target for Guide 146"
  source 1..25: mol_type = other DNA
ggctgggccattaaaacctctccag

SEQ ID NO: 163 - DNA, 25 bp, synthetic construct
  misc_feature 1..25: note = source = /note="Description of Artificial Sequence: Syntheticoligonucleotide"
  misc_feature 1..25: note = source = /note="target for Guide 148"
  source 1..25: mol_type = other DNA
gaggctgggccattaaaacctctcc

SEQ ID NO: 164 - DNA, 25 bp, synthetic construct
  misc_feature 1..25: note = source = /note="Description of Artificial Sequence: Syntheticoligonucleotide"
  misc_feature 1..25: note = source = /note="target for Guide 176"
  source 1..25: mol_type = other DNA
gaggctgagacaggagagttgcttg

SEQ ID NO: 165 - DNA, 25 bp, synthetic construct
  misc_feature 1..25: note = source = /note="Description of Artificial Sequence: Syntheticoligonucleotide"
  misc_feature 1..25: note = source = /note="target for Guide 177"
  source 1..25: mol_type = other DNA
cccacaaaccgatgtagctcaagag

SEQ ID NO: 166 - DNA, 25 bp, synthetic construct
  misc_feature 1..25: note = source = /note="Description of Artificial Sequence: Syntheticoligonucleotide"
  misc_feature 1..25: note = source = /note="target for Guide 209"
  source 1..25: mol_type = other DNA
tagggtcttactctgttgtccacgc

SEQ ID NO: 167 - DNA, 25 bp, synthetic construct
  misc_feature 1..25: note = source = /note="Description of Artificial Sequence: Syntheticoligonucleotide"
  misc_feature 1..25: note = source = /note="target for Guide 151"
  source 1..25: mol_type = other DNA
ttctcccgagccaagtacacgtttc

SEQ ID NO: 168 - DNA, 25 bp, synthetic construct
  misc_feature 1..25: note = source = /note="Description of Artificial Sequence: Syntheticoligonucleotide"
  misc_feature 1..25: note = source = /note="target for Guide 152"
  source 1..25: mol_type = other DNA
gaaaatctgctcttagggctcaagg

SEQ ID NO: 169 - DNA, 3210 bp, synthetic construct
  misc_feature 1..3210: note = source = /note="Description of Artificial Sequence: Syntheticpolynucleotide"
  misc_feature 1..3210: note = source = /note="APG05083.1 Soy optimized"
  source 1..3210: mol_type = other DNA
atgagagagctagattacaggatcggactcgatatcggaactaattcaatcgggtggggaataattgagctgtcctggaataaagatcgcgagcaatatgaaaaggctaggattgtggataagggagtgaggatgttcgataaggctgaaattcctaagactggagcttctcttgctgaaccaagaagaattgctagatctagcaggaggagattaaacaggaagtctcagcgcaagaaggatataaggaaccttctcgttcagcatgaaatcatttctcagaaggagcttgcttctctctaccctctaaccaaatcaagcatggacatctgggatataaggcttgatggactcgataggcttcttgatagatttgagtggaccaggcttctaatacaccttgctcaaagaaggggcttcaaatcaaaccgcaagtccgaattaaaggatgttgagactggaaaggtgctttcaagcatccaagctaatgaaaagaggctttctttgtacaggactgttggggagatgtggatgaaaaacgaggacttctcaaaatacgataaaaggaggaactcctccaacgagtacgtgttctctgtttctagggctgatcttgagaaggagattgtgactctttttgaggctcaacgcaagttccaatcaagctacgcttctgctgatcttcaaaagacctaccttcaaatttgggctcatcagcttccttttgcttctggaaacgccattgtgaataaagtgggatactgctccctattaaagggaaaggagaagagagtgcctaaggctacctatacattccagtacttctctaccctcgatcaaatcaatagaactaggcttggacctaacttccagccttttactaaggagcagagggatgtgatcctcgatgaaatgttcaacaggaccgactactataaaaagaagaccattcccgaggtgacctactacgatataagaaagtggcttgctctcgatgaaaccattcagttcaagggactaacttatgaccccaacgaggagctgaagaaaatagaactcaagtccttcataaacctcaagcccttctacgaaatcaagaaggtggtaaccaactacgccaagaagaccaacgaagcattctctaccctcgattacgatacattcgcttacgctcttaccgtgtataaaaccgacaaggatataaggtcctacctcaagaaatcaaacaacctctccaagtgctgctacgacgatcaattaattgaggagcttctcaccctctcctatactaagttcggacacctctctttcaaggcaatcaaccatgtgcttccaataatgcaagagggaagaacttaccaagaggcaatacaccaacttggatacgatgctaccaaccttaagaaggagaacaggtctatgttccttcctctcttccctgatgagattactaaccctattgtgaagagagctttgactcaagctaggaaggtggtgaatgctattattaggaggtacggatcacctaactctgtgcatattgagcttgctagggagctttctaagtctcatgatgagaggaccaagattatgaaggctcacgatgagaactacaagaagaacaagggggctatttccattctcattgagaacggaattcttaaccctaccggatacgatattgtgaggtacaagttgtggaaggagcaaggagagagatgcgcttactctcttaagcaaattcctgctaacaccttcttcaacgagatgaagaaggaaagatcaggatctcctgtgcttgagattgatcacattctcccttactcccagtccttcattgattcttaccacaacaaggtgcttgtttacggagatgagaaccaaaagaaggggaacaggattccttacacttacttccttgagggaaacaaggattgggagtctttcgagtcttacgtgaggcttaactccttcttctctaagaagaagaggggataccttcttaagaaggcttatcttcctagggagtccaatatgattaaggagaggcacctaaacgataccaggtacgcttcttcttacctcaagaacttcatcgagaagaaccttaagttcaaggaggttgagggatctactaggaagaagcatgttcagaccgtgaacggaattattactgctcatcttagaaagaggtggggacttgagaaggataggcaagagacttaccttcatcacgctatggatgctattattgtggcttgcactgatcaccatatggtgactaaggttaccgagtactaccagattaaggagtcaaacaagtccatcaggaagccttattttcctcttccttgggttggattcagggaggagattctttctcatcttgctagacaacctatcgctagaaagatttccgaggagcttaagattggataccagtccttcgattacattcttgtgtctaggatgcctaagaggtctgttactggagctgctcatgagcagactattatgaagaagggaggaattgataagaaggggaagaccatcatcattaagagggtgtacctaaaggacatcaagttcgatgagaacggggatttcaagatggttggaaaggagcaggatcttgctacttacgaggctattaagcagaggtacattgagtatggaaaggagtctaagaaggctttcgagactcctctttacaagccttctaagaagggaaaggggaacctcatcaagaagattaaggttgaggttcagactaagtctttcgttagggaggttaatggaggagttgctcagaatggagatcttgtgagggttgatctattcgagaaggacaacaggtactacatgatccctatctacgtgatggatactgttcattccgagcttcctaacaaggctgttacttcttctaagggatacgagcagtggcttaccattgataactctttcaccttcaagttctctctctacccttacgatcttgttaggcttgttaagggaaacgaggataggttcctctacttctccaccctcgatattaactctgataggctcaacttcaaggatgtgaacaagccttcaaagcaagctgagaacaggtactctcttaagaccattgagaaccttgagaagtacgaagtgggagttcttggagatcttaggttcgttaggcaagagattaggaagaacttc

SEQ ID NO: 170 - DNA, 3210 bp, synthetic construct
  misc_feature 1..3210: note = source = /note="Description of Artificial Sequence: Syntheticpolynucleotide"
  misc_feature 1..3210: note = source = /note="APG05083.1 Corn optimized"
  source 1..3210: mol_type = other DNA
atgcgcgagctagattacaggatcggcctggatatcggcactaactcaataggctggggcatcatcgagctgagctggaataaagaccgcgagcagtatgaaaaggccaggatcgtggacaagggcgtgaggatgttcgataaggccgagatcccaaagacaggcgcctctctggccgaaccaaggaggatcgccaggtcttctaggaggagattaaacaggaagtctcagcgcaagaaggatataaggaacctgctggtccagcatgaaatcatctctcagaaggagctggccagcctgtacccgctgaccaagtcaagcatggacatctgggatataaggctggatggcctggataggctgctggataggttcgagtggacaaggctgctgatacatctggcccagaggaggggcttcaaatcaaataggaagagcgaattaaaggacgtggagacaggcaaggtgctgtcaagcattcaggccaatgaaaagcgcctgagcctgtacaggacagtgggcgagatgtggatgaaaaacgaggacttctcaaaatacgacaagcgccgcaacagcagcaacgagtacgtgttcagcgtgagcagggccgacctggagaaggagatcgtgacactgttcgaggcccagaggaagttccaatcaagctacgcctctgccgatctgcagaagacatacctgcagatctgggcccaccagctgccattcgctagcggcaatgccatcgtgaataaagtgggctactgctctctattaaagggcaaggagaagagggtgccaaaggccacctatacattccagtacttcagcaccctggaccaaatcaataggacacgcctgggcccaaacttccagccattcacaaaggagcagcgcgacgtgatcctggatgaaatgttcaaccgcaccgactactataaaaagaagaccatcccggaggtgacatactacgatataaggaagtggctggccctggatgaaaccatccagttcaagggcctaacctacgacccgaacgaggagctgaagaaaatagaactgaagagcttcataaacctgaagccgttctacgaaatcaagaaggtggtaaccaactacgccaagaaaaccaacgaagcattcagcaccctggactacgatacattcgcctacgccctgaccgtgtataaaaccgacaaggatataaggagctacctgaagaaatcaaacaacctgagcaagtgctgctacgacgaccaattaatcgaggagctgctgaccctgagctatactaagttcggccacctgagcttcaaggcaatcaaccacgtgctgccaataatgcaggagggccgcacctaccaggaggcaatacaccagctgggctacgacgcaaccaacctgaagaaggagaaccgaagcatgttcctgccgctgttcccggacgagatcaccaacccgatcgtgaagcgcgccctgacccaggcccgcaaggtggtgaacgccatcatccgccgctacggctcaccgaacagcgtgcacattgagctggcccgcgagctgagcaagagccacgacgagcgcacaaagatcatgaaggcccacgacgagaactacaagaagaacaagggcgccatcagcatcctgatcgagaacggcatcctgaacccaacaggctacgacatcgtgaggtacaagctgtggaaggagcagggcgagaggtgcgcctactctctgaagcagatcccagccaatacattcttcaacgagatgaagaaggagaggtcaggctctccagtgctggagattgatcacatcctgccatacagccagagcttcatcgacagctaccacaacaaggtgctggtgtacggcgatgagaaccagaagaagggcaatcgcatcccatacacatacttcctggagggcaacaaggattgggagagcttcgagagctacgtgaggctgaacagcttcttcagcaagaagaagaggggctacctgctgaagaaggcctacctgccaagggagagcaacatgatcaaggagaggcacctaaacgatacaaggtacgccagcagctacctgaagaacttcatcgagaagaacctgaagttcaaggaggtggagggcagcacccgtaagaagcacgtccagaccgtgaacggcatcatcacagcccacctgaggaagaggtggggcctggagaaggataggcaggagacatacctgcatcacgccatggatgccatcatcgtggcttgcacagatcaccacatggtgacaaaggtgacagagtactaccagatcaaggagagcaacaagtcaatccgcaagccatacttcccactgccatgggtgggcttcagggaggagatcctgtctcacctggccaggcagccaatcgccaggaagatctctgaggagctgaagatcggctaccagtctttcgattacatcctggtgtctaggatgccaaagaggtctgtgacaggcgccgcccacgagcagacaatcatgaagaagggcggcatcgataagaagggcaagacaatcatcatcaagagggtgtacctgaaggatatcaagttcgatgagaacggcgatttcaagatggtgggcaaggagcaggatctagccacatacgaggccatcaagcagaggtacatcgagtacggcaaggagtctaagaaggccttcgagacaccactgtacaagccatctaagaagggcaagggcaacctgatcaagaagatcaaggtggaggttcagaccaagagcttcgtgagggaggtgaatggcggcgtggcccagaatggcgatctggtgagggtggatctgttcgagaaggataacaggtactacatgatcccgatctacgtgatggatacagtgcacagcgagctgccaaacaaggccgtgacatcttctaagggctacgagcagtggctaaccatcgacaacagcttcaccttcaagttcagcctgtacccatacgacctggtgaggctggtgaagggcaatgaggacaggttcctgtacttcagcaccctggacatcaacagcgacaggctgaacttcaaggacgtgaacaagccatctaagcaggccgagaacaggtacagcctgaagaccatcgagaacctggagaagtacgaggtgggcgtgctgggcgatctgaggttcgtgaggcaggagatcaggaagaatttc

SEQ ID NO: 171 - DNA, 3213 bp, synthetic construct
  misc_feature 1..3213: note = source = /note="Description of Artificial Sequence: Syntheticpolynucleotide"
  misc_feature 1..3213: note = source = /note="APG07433.1 Soy optimized"
  source 1..3213: mol_type = other DNA
atgagagagctagattacaggatcggactcgatatcggaactaattcaattggatggggcgtgattgagctttcctggaataaagatagggagcgttatgaaaaggttaggattgtggatcagggagttaggatgtttgatagagctgagatgcctaagactggagcttcattagctgaaccaagaaggattgctagatctagcaggaggagattaaacaggaagtctcagcgcaagaagaatataaggaaccttcttgttcagcacggagttattactcaggaggagcttgattctctctaccctctctccaagaaatcaatggatatctggggaattaggcttgatggactcgatcgcctattaaaccattttgagtgggctaggcttctaatacaccttgctcaaagaaggggcttcaaatcaaaccgcaagtccgaattaaaggatactgagactggaaaggtgctttcaagcatccagctcaatgaaaagaggctttctttgtataggactgttggggagatgtggatgaaagatcccgacttctcaaaatacgataggaagaggaactctcctaacgagtacgtgttttctgtttctagagctgagcttgagaaggagattgtgactttgtttgctgctcaaaggaggttccaatctccttacgcttctaaggatcttcaagagacctaccttcagatttggactcatcagcttccttttgcttccgggaacgctattctcaataaagtgggatactgctccttattaaagggaaaggagagaaggattcctaaggccacctatacattccagtacttctctgctcttgatcaagtgaatagaactaggcttggacctgatttccagccttttactaaggagcagcgcgagatcatcctcaataatatgttccagaggaccgactactataaaaagaagaccattcccgaggtgacctactacgatataagaaagtggcttgagcttgatgaaaccattcagttcaagggattaaactacgaccccaacgaggagctgaagaaaatagagaagaagcccttcataaacctcaaggccttctacgaaatcaacaaggtggtggctaactactctgagcgaaccaatgaaaccttctctaccctcgattacgatggaattggatacgctcttaccgtgtataaaaccgacaaggatataaggtcctacctcaaatcaagccataatctccctaagaggtgctacgacgatcaattaattgaggagcttctctccctctcctatactaagttcgggcacctctctcttaaggcaatcaaccatgttctaagcattatgcagaaggggaacacatataaggaggctgttgatcagcttggatacgatacttctggacttaagaaggagaagaggtctaagttcctccctcctatttctgatgagattaccaaccctattgtgaagagagctttgactcaagctaggaaggtggtgaatgctattattaggaggcatggatctcctcattctgtgcatattgagcttgctagggagctttcaaagaatcacgatgagaggactaagattgtttctgctcaggacgagaactacaagaagaacaagggggctatttctattctctctgagcacggaattcttaaccctaccggatacgatattgtgaggtataagttgtggaaggagcaaggagagagatgcgcttactctcttaaggaaattcctgctgataccttcttcaacgagcttaagaaggaaaggaacggtgctcctattctagaggtggatcacattcttccttactcccagtccttcattgattcttaccataacaaggtgcttgtgtattccgatgagaacaggaagaagggaaacaggattccttacacctacttccttgagactaataaggattgggaggcttttgagaggtacgtgaggtctaacaagttcttctctaagaagaagagggagtaccttcttaagagggcttatcttcctagggagtcagagcttattaaggagaggcatcttaacgataccaggtacgcttctaccttcctcaagaacttcattgagcagaaccttcaattcaaggaagctgaggataatcctagaaagaggagggttcagactgtgaacggagttattactgctcattttagaaagaggtggggacttgagaaggataggcaagagacttaccttcatcacgctatggatgctattattgtggcttgcactgatcatcatatggtgactagggttaccgagtactaccagatcaaggagtcaaacaagtctgtgaagaagccttattttcctatgccttgggaaggattcagggatgagcttctttctcatcttgcttctcagcctatcgctaagaagatttctgaagagcttaaggctggataccagtcccttgattacattttcgtgtctagaatgcctaagaggtctattactggagctgctcacaagcagactattatgaggaagggaggaattgataagaaggggaagaccatcattattgagaggctccacctcaaggatatcaagttcgatgagaacggagatttcaagatggttggaaaggagcaggatatggctacttacgaggctattaagcagagatatctagagcacggaaagaactctaagaaggctttcgagactcctctttacaagccttctaagaagggaaccggaaaccttattaagagagttaaggttgagggacaggctaagtctttcgttagagaggttaatggaggagttgctcagaatggagatcttgtgagggttgatcttttcgagaaggacgataagtactacatggtgcctatctacgttcctgatactgtttgttccgagcttcctaagaaggttgttgcttcttctaagggatacgagcaatggcttacccttgataactctttcaccttcaagttctctctctacccttacgatcttgttaggctagttaagggagatgaggataggttcctttacttcgggaccctcgatattgattctgataggctcaacttcaaggatgtgaacaagccttctaagaagaacgagtacaggtactctctcaagaccattgaggatcttgagaagtacgaagtgggagttcttggagatcttagacttgttagaaaggagactaggaggaacttccac

SEQ ID NO: 172 - DNA, 3213 bp, synthetic construct
  misc_feature 1..3213: note = source = /note="Description of Artificial Sequence: Syntheticpolynucleotide"
  misc_feature 1..3213: note = source = /note="APG07433.1 Corn optimized"
  source 1..3213: mol_type = other DNA
atgcgcgagctagattacaggatcggcctggatatcggcactaactcaatcggctggggcgtgatcgagctgagctggaataaagatcgcgagcgctatgaaaaggtgcgcatcgtggatcagggcgttaggatgttcgatagggccgagatgccaaagacaggcgcctcactggccgaaccaaggaggatagccaggtcttctaggaggagattaaacaggaagtctcagcgcaagaaaaatatcaggaacctgctggttcagcacggcgtgatcacacaggaggagctggattctctgtacccactgagcaagaaaagcatggacatctggggcattaggctagatggcctggaccgcctattaaaccacttcgagtgggcccgcctattaattcacctggcccagaggaggggcttcaaatcaaataggaagagcgaattaaaggacaccgagacaggcaaggtgctgtcaagcatccagctgaatgaaaagcgcctgagcctgtacaggacagtgggcgagatgtggatgaaagacccggacttctcaaaatacgaccgcaagcgcaacagcccgaacgagtacgtgttctctgtgtctagggccgagctggagaaggagatcgtgacactgttcgccgctcagaggaggttccagtctccatacgcctctaaggatctgcaagagacatacctgcagatctggacacaccagctgccattcgcctctggcaatgccatcctgaataaagtgggctactgctctctattaaagggcaaggagaggaggattccaaaggccacctatacattccagtacttcagcgccctggaccaggtgaataggacaaggctgggcccagatttccagccattcacaaaggagcagcgcgagatcatcctgaataatatgttccagcgcaccgactactataaaaagaagaccatcccggaggtgacatactacgatataaggaagtggctggagctggatgaaaccatccagttcaagggattaaactacgacccgaacgaggagctgaagaaaatagagaagaagccgttcataaacctgaaggccttctacgaaatcaacaaggtggtggccaactacagcgagcgaaccaacgagaccttcagcaccctggactacgacggcatcggctacgccctgaccgtgtataaaaccgacaaggatataaggagctacctgaaatcaagccacaacctgccgaagcgctgctacgacgaccaattaatcgaggagctgctgagcctgagctatactaagttcggccacctgagcctgaaggcaatcaaccacgtgctaagcatcatgcagaagggcaatacatacaaggaggccgtggaccagctgggctacgacaccagcggcctgaagaaggagaagcgcagcaagttcctgccgccgatcagcgacgagatcaccaacccgatcgtgaagcgcgccctgacccaggccaggaaggtggtgaacgccatcatcaggaggcacggctctccacatagcgtgcacatcgagctggccagggagctgtctaagaatcacgatgagaggacaaagatcgtgtcagcccaggacgagaactacaagaagaataagggcgccatctctatcctgtctgagcacggcatcctgaacccaacaggctacgacatcgtgaggtacaagctgtggaaggagcagggcgagaggtgcgcctactctctgaaggagatcccagccgatacattcttcaatgagctgaagaaggagaggaatggcgccccaatcctggaggtggatcacatcctgccatactctcagagcttcatcgattcataccacaacaaggtgctggtgtacagcgacgagaacaggaagaagggcaatcgcatcccatacacatacttcctggagaccaacaaggattgggaggccttcgagaggtacgtgcgcagcaacaagttcttcagcaagaagaagcgcgagtacctgctgaagagggcctacctgcctagggagtctgagctgatcaaggagaggcacctgaatgatacaaggtacgccagcaccttcctgaagaacttcatcgagcagaacctacagttcaaggaggccgaggataacccaaggaagaggagggttcagacagtgaatggcgtgatcacagcccacttcaggaagaggtggggcctggagaaggataggcaggagacatacctgcatcacgccatggatgccatcatcgtggcttgcacagatcaccacatggtgacaagggtgacagagtactaccagatcaaggagagcaacaagagcgtgaagaagccatacttcccaatgccatgggagggcttcagggatgagctactgtctcacctggcctctcagccaatcgccaagaagatctctgaggagctgaaggccggctaccagtctctggattacatcttcgtgtctaggatgccaaagaggtctatcacaggcgccgcccacaagcagacaatcatgaggaagggcggcatcgataagaagggcaagacaatcatcatcgagaggctgcatctgaaggacatcaagttcgatgagaacggcgatttcaagatggtgggcaaggagcaggatatggccacatacgaggccatcaagcagcgctacctagagcacggcaagaactctaagaaggccttcgagacaccactgtacaagccatctaagaagggcaccggcaatctgatcaagagggtgaaggtggagggccaggccaagtctttcgtgagggaggtgaatggcggcgtggcccagaatggcgatctggtgagggtggatctgttcgagaaggatgataagtactacatggtgccaatctacgtgccagatacagtgtgctctgagctgccaaagaaggtggtggcctcttctaagggctacgagcagtggctaacactggataacagcttcacattcaagttcagcctgtacccatacgatctggtgaggctggtgaagggcgatgaggataggttcctgtacttcggcacactggatatcgatagcgacaggctgaacttcaaggacgtgaacaagccgagcaagaagaacgagtaccgctacagcctgaagacaatcgaggacctggagaagtacgaggtgggcgtgctgggcgatctgaggctggtgaggaaggagacaaggaggaatttccac

SEQ ID NO: 173 - DNA, 3213 bp, synthetic construct
  misc_feature 1..3213: note = source = /note="Description of Artificial Sequence: Syntheticpolynucleotide"
  misc_feature 1..3213: note = source = /note="APG07513.1 Soy optimized"
  source 1..3213: mol_type = other DNA
atgagagagctagattacaggatcggactcgatatcggaactaattcaattggatggggcgtgattgagctttcctggaataaagatcgcgagcaatatgaaaagaccaggattgtggataagggagtgaggatgttcgataaggctgaaattcctaagactggagcttctcttgctgaaccaagaagaattgctagatctagcaggaggagattaaacaggaagtctcagcgcaagaaggatataaggaaccttctcgttcagcatgaaatcatttcccagaaggaattaacctctctctaccctctctccaaatcaagcatggacatctgggatataaggcttgatggactcgataggcttcttgatagatttgagtgggctaggcttctaatacaccttgctcaaagaaggggcttcaaatcaaaccgcaagtccgaattaaaggatgttgagactggaaaggtgctttcaagcatccaggtgaatgaaaagaggctttctttgtataggactgttggggagatgtggatgaaaaacgccgattgctcaaaatatggaaagaggaggaactctcctaacgagtacgtgttttctgtttctagggctgatcttgagaaggagattgtgactctttttgaggctcagaggaagttccactcttcttacgcttctgtggatctccaaaagacatacattcagatttgggctcatcagcttccttttgcttctggaaacgccattgtgaataaagtgggatactgctccctattaaagggaaaggagaagagagtgcctaaggctacctatacattccagtacttcaataccctcgatcaaatcaacagaactaggcttggacctaacttccagccttttactaaggagcagagggatataatcctcgataaaatgttccagcgcaccgactactataaaaagaagaccatccccgaggtgacctactacgatataagaaagtggcttgctctcgatgaaaccattcagttcaagggactaacttatgaccccaacgaggagctgaagaaaatagagatgaaacccttcataaacctcaagcccttctacgaaatcaagaaggtggtaaccaactacgccaagaaaaccaacgaggtgttctctgctcttgattacgatactgtggcttacgctcttaccgtgtataaaaccgacaaggatataaggtcttacctcaagcgctccaataatctctctaagaggtgctacgacgatcaattaattgaggagcttctcaccctctcctatactaagttcggacacctctctttcaaggcaatcaaccatgtgcttccaataatgcaagagggaagaacttaccaagaggcaatacaccagcttggatacgatacaaccaacctcaagaaggagaatagaagcatgttcctcccaatcatccctgatgaaataaccaaccctattgtgaagagagctttgactcaagctaggaaggtggtgaatgcaataattaggaggtacggatcacctaactctgtgcatattgagcttgccagggaattaagcaagtctcatgatgagaggaagaagattatgactgctcacgacgagaactacaagaagaacaagggagctgtgtccattctcattgataacggaattcttaaccctaccggatacgatattgtgaggtacaagttgtggaaggagcaaggagagagatgcgcttactctcttaagaagattcctgctaacaccttcttcaacgagcttaagaaggaaagatctggacctcctgttcttgaggtggatcacattctaccttactcccagtccttcattgattcttaccataacaaggtgcttgtttacggagatgagaaccaaaagaaggggaacaggattccttacactttcttctctgaagaagataaggagtgggagtctttcgagtcttacgtgaggtccaactccttcttctctaagaagaagaggggataccttcttaagaaggcttatcttcctagggagtctaaccttattaaggagaggcaccttaacgataccaggtacgcttcatcttacctcaagaacttcatcgagaagaaccttaagttcaaggaggctgtgggaattactaggaagaagtacgttcagactgtgaacggagtgattactgctcatcttagaaagagatggggacttgagaaggataggcaagagacttaccttcatcacgctatggatgctattattgtggcttgcactgatcaccatatggtgactaaggttaccgagtactaccaaattaaggaggggaacaagtccatcaagaagccttattttcctctaccttggatgggattcagggaggagattctttctcatcttgagtctcaacctatcgctagaaagatttccgaggagcttaagattggataccagtcccctgattacattcttgtgtctagaatgcctaagaggtctgttactggatctgctcatgatcagactgtgatgaagaagggggatattgataagaaggggaagaccatcattattaagagggtgcacctcaaggacatcaagttcgatgagaacggagatttcaagatggttggaaaggagcaggatctagctacttacgaggctattaagcagaggtatcttgagtataggaaggagtctaagaaggctttcgagactcctctttacaagccttctaagaagggaaaggggaacctcatcaagaagattaaggttgaggttcagactaagtctttcgtgagggagattaatggaggagttgctcagaatggagatcttgtgagggttgatcttttcgagaaggacaacaggtactacatggtgcctatctacgttgttgatactgttaggtctgagctacctaacaaggctgttacttcttctaagggatacgagcagtggctctctattgataactctttcaccttcaagttctctctctacccttacgatcttgttaggcttgttaagggagatgaggataggttcctctacttctccaccctcgatattaactctgataggctcaacttcaaggatgtgaacaagccttctaagcaagctgagtacaggtactctcttaagaccattgagaaccttgagaagtacgagattggagttcttggagatctaaggcttgttaggcaggagaccaggaagattttcaag

SEQ ID NO: 174 - DNA, 3213 bp, synthetic construct
  misc_feature 1..3213: note = source = /note="Description of Artificial Sequence: Syntheticpolynucleotide"
  misc_feature 1..3213: note = source = /note="APG07513.1 Corn optimized"
  source 1..3213: mol_type = other DNA
atgcgcgagctagattacaggatcggcctggatatcggcactaactcaatcggctggggcgtgatcgagctgagctggaataaagatcgcgagcagtatgaaaagaccaggatcgtggacaagggcgtgaggatgttcgataaggccgagatcccaaagacaggcgcctctctggccgaaccaaggaggatcgccaggtcttctaggaggagattaaacaggaagtctcagcgcaagaaggatataaggaacctgctggtccagcatgaaatcatcagccagaaggagctgacaagcctgtacccgctgagcaagtcaagcatggacatctgggatataaggctggatggcctggataggctgctggataggttcgagtgggccaggctgctgatacatctggcccagaggaggggcttcaaatcaaatcgcaagagcgaattaaaggacgtggagacaggcaaggtgctgtcaagcattcaggtgaatgaaaagaggctgagcctgtacaggacagtgggcgagatgtggatgaaaaacgccgactgctcaaaatacggcaagcgccgcaacagcccaaacgagtacgtgttctctgtgtctagggccgatctggagaaggagatcgtgacactgttcgaggcccagaggaagttccactcttcttacgcctctgtggacctgcagaagacatacatccagatctgggcccaccagctgccattcgcctctggcaatgccatcgtgaataaagtgggctactgctctctattaaagggcaaggagaagagggtgccaaaggccacctatacattccagtacttcaataccctggaccaaatcaacaggacccgcctgggcccaaacttccagccattcacaaaggagcagcgcgatataatcctggataaaatgttccagcgcaccgactactataaaaagaagaccatcccggaggtgacatactacgatataaggaagtggctggccctggatgaaaccatccagttcaagggcctaacctacgacccgaacgaggagctgaagaagatcgagatgaaaccgttcataaacctgaagccgttctacgaaatcaagaaggtggtaaccaactacgccaagaaaaccaacgaggtgttcagcgccctggactacgacaccgtggcctacgccctgaccgtgtataaaaccgacaaggatataaggagctacctgaagcgcagcaataatctgagcaagcgctgctacgacgaccaattaatcgaggagctgctgaccctgagctatactaagttcggccacctgagcttcaaggcaatcaaccacgtgctgccaataatgcaggagggccgcacctaccaggaggcaatacaccagctgggctacgacacaaccaacctgaagaaggagaaccgaagcatgttcctgccaataatcccggacgagataaccaacccgatcgtgaagcgcgccctgacccaggcccgcaaggtggtgaacgcaataatccgccgctacggctcaccgaacagcgtgcacattgagctggcccgcgaattaagcaagagccacgacgagcgcaagaagatcatgaccgcccacgatgaaaactacaagaaaaataagggcgccgtgagcatcctgatcgacaacggcatcctgaacccgaccggctacgacatcgtgcgctacaagctgtggaaggagcagggcgagaggtgcgcctactctctgaagaagatcccagccaacaccttcttcaacgagctgaagaaggagaggtctggcccaccagtgctggaggtggatcacatcctgccatactcacagagcttcatcgatagctaccacaacaaggtgctggtgtacggcgatgagaaccagaagaagggcaatcgcatcccatacacattcttcagcgaggaggataaggagtgggagagcttcgagagctacgtgaggagcaacagcttcttcagcaagaagaagaggggctacctgctgaagaaggcctacctgccaagggagtctaacctgatcaaggagaggcacctgaacgatacaaggtacgccagcagctacctaaagaacttcatcgagaagaacctgaagttcaaggaggccgtgggcatcacccgcaagaagtacgtccagacagtgaacggcgtgatcacagcccacctgaggaagaggtggggcctggagaaggataggcaggagacatacctgcatcacgccatggatgccatcatcgtggcttgcacagatcaccacatggtgacaaaggtgacagagtactaccagatcaaggagggcaacaagagcatcaagaagccatacttcccactaccatggatgggcttcagggaggagatcctgtctcacctggagtctcagccaatcgccaggaagatctctgaggagctgaagatcggctaccagtctccagattacatcctggtgtctaggatgccaaagaggtctgtgacaggctctgcccacgatcagacagtgatgaagaagggcgatatcgacaagaagggcaagaccatcatcatcaagagggtgcacctgaaggacatcaagttcgacgagaacggcgacttcaagatggtgggcaaggagcaggatctagccacatacgaggccatcaagcagcgctacctggagtacaggaaggagtctaagaaggccttcgagacaccactgtacaagccatctaagaagggcaagggcaacctgatcaagaagatcaaggtggaggtccagaccaagagcttcgtgagggagatcaatggcggcgtggcccagaatggcgatctggtgagggtggatctgttcgagaaggataacaggtactacatggtgccaatctacgtggtggatacagtgaggagcgagctaccaaacaaggccgtgacatcttctaagggctacgagcagtggctgagcatcgacaacagcttcaccttcaagttcagcctgtacccatacgatctggtgaggctggtgaagggcgatgaggacaggttcctgtacttcagcacactggacatcaacagcgacaggctgaacttcaaggacgtgaacaagccatctaagcaggccgagtacaggtacagcctgaagaccatcgagaacctggagaagtacgagatcggcgtgctgggcgatctaaggctggtgaggcaggagacaaggaagatcttcaag

SEQ ID NO: 175 - DNA, 3216 bp, synthetic construct
  misc_feature 1..3216: note = source = /note="Description of Artificial Sequence: Syntheticpolynucleotide"
  misc_feature 1..3216: note = source = /note="APG08290.1 Soy optimized"
  source 1..3216: mol_type = other DNA
atgtctgagctagattacaggatcggactcgatatcggaactaattcaattggatggggagtgattgagcttttctggaataaagatcgcgagcgctatgaaaaggttaggattgtggataagggagtgaggatgttcgataaggccgagattcctaataaaggagcttcacttgctgaaccaagaaggattgctagatctagcaggaggagattaaacaggaagtctcagaggaagaaggagattaggaaccttcttgttcagcacggaatgattactcaggaggagcttgatcttctctaccctctctccaagaaatcaatcgatatctgggatataaggcttgatggactcgataggctattaaaccatcttgagtgggctaggcttctaatacaccttgctcaaagaaggggcttcaaatcaaaccgcaagtccgaattaaaggatgctgagactggaaaggttctttcaagcatccaggtgaatgaaaagaggcttttcttgtataggactgtgggcgagatgtggataaaagatgccgagttctcaaaatatgataggaggaggaactctcctaacgagtacgtgttttctgtttctagggctgatcttgagaaggagattgtgactttgtttgaggctcaacgcaagttccaatcaagctacgcttctaagaaccttcaagagacctaccttcaaatttgggctcatcagcttccttttgcttccgggaacgctattctcaataaagtgggatactgctccttattaaagggaaaggagagaaggattcctaaggccacctatacattccagtacttctctgctcttgatcaagtgaatagaactaggcttggacctgatttccaacctttcactcaggagcagaaggaaataatcctcgataaaatgttccagcgcaccgactactataaaaagaagaccatccccgaggtgtcctactacgatataagaaagtggcttgagcttgatgaaaccattcagttcaagggattaaactacgaccccaacgaggagctgaagaaaatagagaagaagcccttcataaacctcaaggccttctacgaaatcaagaaggtggttgctaactacgctgaacgaaccaacgaagcattctctaccctcgattacgatgctattgcttacgctcttaccgtgtataaaaccgacaaggatataaggtcctacctcaagaaatcaaacaacctctccaagaggtgctacgacgatcaattaatcgaggagcttttcaccctctcctatactaagttcggacacctctctttcaaggcaatcaaccatgtgcttcctattatgcaagagggaagaacttaccaagaggctattcatcagcttggatacgataccaccaaccttaagaaggagaacaggtctatgttcctccctctcattcctgatgagattactaaccctattgtgaagagggctattactcaagctaggaaggtggtgaatgctattattaggaggtacggatcacctaactctgtgcatattgagcttgctagggagctttctaagtctcatgatgagaggaagaagattatgactgctcacgacgagaactacaagaagaacaagggggctatttccattctcattgagaacggaattcttaaccctaccggatacgatattgtgaggtacaagttgtggaaggagcaaggagagagatgcgcttactctcttaaggaaattcctcctgataccttcttcaacgagcttaagaaggagaggaacggatcacctattcttgaggtggatcacattcttccttactcccagtccttcattgattcttaccataacaaggtgcttgtgtattccgatgagaacaggaacaagggaaacaggattccttacacctacttccttgagactaataaggattgggaggcttttgagaggtatgtgaggtctaacaagctcttctctaagaagaagagggagtacctccttaagaagacttaccttcctagggagtctgagcttattaaggagaggcatctaaacgataccaggtacgcttctaccttcctcaagaacttcattgagcagaaccttcaattcaaggaggttgaggttaaccttaggaagaagagggttcagactgtgaacggagttattactgctcatcttagaaagagatggggacttgagaagaacaggcaagagacttaccttcatcacgctatggatgctattattgtggcttgcactgatcatcacatggtgactaggattaccgagtactaccagattaaggagtcaaacaagtctgtgaagaagccttattttcctatgccttgggagggattcagggatgagcttctttctcatcttgcttctcagcctatcgctaagaagatttctgaagagcttaaggctggataccagtcctctgattacattttcgtgtctagaatgcctaagaggtctgttactggagctgctcatgatcaaactattaggaggaagggaggaattgataagaaggggaagaccatcattattaagagggtgaggctaaaggacatcaagttcgatgagaacggggatttcaagatggttggaaaggagcaggatcttgctacttacgaggctattaagcagagatatcttgagcacaggaagaactctaagaaggctttcgagactcctctttacaagccttctaagaagggaaccggaaaccttatcaagagagttaagattgagggacagactaaggctttcgttagagaggttaatggaggagttgctcagaactctgatcttgtgagggttgatctattcgagaaggacgataagtactacatggtgcctatctacgttcctgatactgtttgttccgagcttcctaagaaggttgttaagtctggaaagggatacgagcaatggcttacccttgataactctttcaccttcaagtcttctctctacccttacgatcttgttaggcttgttaagggaaacgaggataggttcctttacttcgggaccctcgatattgattctgataggctcaacttcaaggatgtgaacaagccttcaaagcaaaacgagtacaggtactctctcaagaccattgagaaccttgagaagtacgaagtgggagttcttggagatcttaggcttgttaagcaagagaccaggaggattttcaatagg

SEQ ID NO: 176 - DNA, 3216 bp, synthetic construct
  misc_feature 1..3216: note = source = /note="Description of Artificial Sequence: Syntheticpolynucleotide"
  misc_feature 1..3216: note = source = /note="APG08290.1 Corn optimized"
  source 1..3216: mol_type = other DNA
atgtcagagctggactacaggatcggcctggacataggcactaattcaatcggctggggcgtgatcgagctgttctggaataaagaccgcgagcgctatgaaaaggtgcgcatcgtggacaagggcgttaggatgttcgataaggccgagatcccgaataaaggcgcctcactagccgaaccaaggaggatcgccaggtcttctaggaggagattaaacaggaagtctcagaggaagaaggagatcaggaacctgctggtccagcacggcatgatcacacaggaggagctggatctgctgtacccactgagcaagaaaagcattgacatctgggacatcaggctagatggcctggacaggctgctgaatcacctggagtgggccaggctgctgatacatctggcccagaggaggggcttcaaatcaaatcgcaagtctgaattaaaggatgccgagacaggcaaggtgctgtcaagcatccaggtgaatgaaaagaggctgttcctctaccgcacagtgggcgagatgtggataaaagacgccgagttcagcaagtacgacaggaggaggaacagcccaaacgagtacgtgttctctgtgtcaagggccgatctggagaaggagatcgtgacactgtttgaggctcagcgcaagttccaatcaagctacgccagcaagaacctgcaagagacctacctgcagatctgggcccaccagctgccattcgctagcggcaatgccatcctgaataaagtgggctactgctctctattaaagggcaaggagaggaggattccaaaggccacctatacattccagtacttcagcgccctggaccaggtgaataggacaaggctgggcccagatttccagccattcacacaggagcagaaggaaataatcctggataaaatgttccagcgcaccgactactataaaaagaagaccatcccggaggtgtcatactacgatataaggaagtggctggagctggatgaaaccatccagttcaagggattaaactacgacccgaacgaggagctgaagaaaatagagaagaagccgttcataaacctgaaggccttctacgaaatcaagaaggtggtggccaactacgccgagcgaaccaacgaagcattcagcaccctggactacgacgccatcgcctacgccctgaccgtgtataaaaccgacaaggatataaggtcatacctgaagaaatcaaacaacctgagcaagcgctgctacgacgaccaattaatcgaggagctgttcaccctgagctatactaagttcggccacctgagcttcaaggcaatcaaccacgtgctgccaataatgcaggagggccgcacctaccaggaggcaatacaccagctgggctacgacaccaccaacctgaagaaggagaaccgcagcatgttcctgccgctaatcccggacgagatcaccaacccgatcgtgaagcgcgccatcacccaggctaggaaggtggtgaacgccatcatccgccgctacggcagcccgaacagcgtgcacatcgagctggcccgcgagctgagcaagagccacgacgagcgcaagaagatcatgacagcccacgacgagaactacaagaagaacaagggcgccatctcaatcctgatcgagaacggcatcctgaacccaaccggctatgacatcgtgcgctacaagctgtggaaggagcagggcgagaggtgcgcctactctctgaaggagatcccaccagatacattcttcaacgagctgaagaaggagaggaatggctctccaatcctggaggtggatcacatcctgccatacagccagtcattcatcgacagctaccacaacaaggtgctggtgtacagcgatgagaacaggaacaagggcaaccgcatcccgtacacatacttcctggagaccaacaaggattgggaggccttcgagaggtacgtgaggagcaacaagctgttcagcaagaagaagcgcgagtacctgctgaagaagacctacctgccaagggagtcagagctgatcaaggagaggcacctgaacgatacaaggtacgctagcaccttcctgaagaacttcatcgagcagaacctgcagttcaaggaggtggaggtgaacctgaggaagaagcgcgttcagacagtgaacggcgtgatcacagcccacctgaggaagaggtggggcctggagaagaataggcaggagacatacctacaccacgccatggatgccatcatcgtggcttgcacagatcaccacatggtgacaaggatcacagagtactaccagatcaaggagagcaacaagagcgtgaagaagccatacttcccaatgccatgggagggcttcagggatgagctgctgtctcacctggcctctcagccaatcgccaagaagatctcagaggagctgaaggccggctaccagtcttctgattacatcttcgtgtctaggatgccaaagaggtctgtgacaggcgccgcccacgatcagacaatcaggaggaagggcggcatcgataagaagggcaagacaatcatcatcaagagggtgaggctgaaggatatcaagttcgatgagaacggcgatttcaagatggtgggcaaggagcaggatctagccacatacgaggccatcaagcagcgctacctggagcacaggaagaactctaagaaggccttcgagacaccactgtacaagccatctaagaagggcaccggcaatctgatcaagagggtgaagatcgagggccagacaaaggccttcgtgagggaggtgaatggcggcgtggcccagaattctgatctggtgagggtggatctattcgagaaggacgataagtactacatggtgccaatctacgtgccagatacagtgtgctccgagctgccaaagaaggtggtgaagtctggcaagggctacgagcagtggctcacactggataacagcttcacattcaagagcagcctgtacccatacgatctggtgaggctggtgaagggcaatgaggacaggttcctgtacttcggcacactagacatcgatagcgacaggctgaacttcaaggacgtgaacaagccaagcaagcagaacgagtaccgctacagcctgaagaccatcgagaacctggagaagtacgaggtgggcgtgctgggcgatctgaggctggtgaagcaggagacaaggaggatcttcaatagg

SEQ ID NO: 177 - DNA, 4011 bp, synthetic construct
  misc_feature 1..4011: note = source = /note="Description of Artificial Sequence: Syntheticpolynucleotide"
  misc_feature 1..4011: note = source = /note="APG05459.1 Soy optimized"
  source 1..4011: mol_type = other DNA
atgaagaaggactacgtgatcggactagatattggaactaactctgtgggatgggctgttatgactgaggattaccagctagttaagaagaagatgcccatctacgggaatacagagaagaagaagatcaagaagaacttctggggagtgagactatttgaagagggtcatactgctgaggataggagattaaagagaactgctaggagaaggatttctaggaggaggaacaggcttcgttaccttcaagcattctttgaagaggctatgaccgctctagatgaaaatttcttcgctaggcttcaggagtcttttcttgtgcctgaggataaaaagtggcacaggcatcctatttttgctaagttagaggatgaggtggcttaccatgaaacctaccctactatctaccaccttaggaagaagttggctgattcttcagagcaagccgacttgagattaatctaccttgctcttgcccacattgtaaaatataggggacacttccttatcgagggaaaactctccaccgaaaatatttcagtgaaggagcagtttcagcagttcatgatcatctataaccaaaccttcgtgaacggagaatcaaggcttgtgtctgctcctcttcctgagtccgtattaattgaggaggaacttactgagaaagcatccagaaccaagaagtctgagaaggttcttcaacagtttcctcaagagaaggctaacggacttttcggacagttcctcaaattaatggtggggaataaagccgacttcaagaaggtttttggacttgaggaggaggccaaaataacttacgcttctgagtcttatgaggaggatcttgagggaatactagctaaggtgggagatgaatacagcgatgttttccttgctgctaagaacgtttacgacgctgtggaattaagcaccatactagctgactccgataaaaagtctcacgccaaactctcttcaagcatgattgttaggttcactgagcatcaggaggatcttaagaagttcaagaggttcattagggagaactgccctgatgagtacgataaccttttcaagaacgagcaaaaggatgggtacgctggatacattgctcatgctggaaaggtgtcacaattaaagttctaccagtacgtgaagaaaataatccaggatatcgctggagccgagtacttccttgagaaaatagctcaggagaacttccttaggaagcagaggactttcgataacggagtgattcctcaccaaatacaccttgctgagctacaggcaataattcataggcaagctgcatactatcctttcctcaaggagaatcaagagaaaatagagcagctcgtgaccttcagaattccatactacgtgggacctctttctaagggagatgcttctacttttgcttggcttaagagacagtcagaggaaccaattaggccttggaatcttcaagagactgtggatcttgatcaatctgctactgctttcatagagaggatgaccaacttcgatacataccttccttctgagaaggtgctccctaagcattctctcctctatgaaaagttcatggtgttcaacgagctaaccaaaatatcctacaccgacgataggggaatcaaggctaatttctctggaaaggagaaggagaaaatattcgactacctcttcaagaccaggaggaaggtgaagaagaaggacataatacagttctaccgcaacgaatacaacaccgagattgtgaccttgtcaggacttgaggaggatcaattcaacgcttctttctctacctaccaggatctattaaagtgcggacttactagggctgagcttgatcatcctgataatgctgagaagctggaggacataatcaagatactaaccatcttcgaggataggcaaaggattaggacccagctttctactttcaagggacaattctctgctgaggttcttaagaagttggagaggaagcattatactggatggggaaggctctctaagaagctcattaacggaatctacgataaggagtcagggaagaccatcctagattacctcattaaggatgatggagtgtctaagcactacaacaggaacttcatgcagctcattaacgattcccagctctccttcaagaacgctattcaaaaggctcaatcttctgagcatgaagagactctttctgagactgttaacgaattagctgggtcccctgctattaagaagggaatctaccagtctctcaagattgtggatgagcttgtggctattatgggatatgctcctaagaggattgttgttgagatggctagggagaaccaaactacttctactggaaagaggaggtctattcagaggctaaagattgttgaaaaggctatggctgagattggatctaaccttcttaaggagcagcctactactaacgagcaacttagggataccaggctcttcctttactacatgcagaacggaaaggatatgtacactggagatgagctttctcttcataggctctcacactacgacatagatcacattatccctcagtccttcatgaaggatgattctctcgataaccttgtgcttgtgggatctactgagaataggggaaagtctgatgatgttccttctaaggaggtggttaaggatatgaaggcttactgggagaaactatacgctgctggacttatttctcaaaggaagttccagagacttactaagggagagcaaggaggacttactcttgaggataaggctcatttcattcaaaggcagcttgttgagaccaggcagattactaagaacgtggctggaattctagatcaaaggtacaacgctaactctaaggagaagaaggttcagatcattaccctcaaggcttctcttacctcccagttcaggtctattttcggactttacaaggttagggaggtgaacgattaccatcatggacaagatgcttaccttaactgcgtggttgctactactctacttaaggtttatcctaaccttgctcctgagttcgtttacggagagtatcctaagttccaggctttcaaggagaataaggctaccgctaagaccattatctacaccaaccttatgaggttctttactgaggatgagcctaggtttatgaaggatggagagattctctggtcaaactcctacctcaagaacatcaagaaggagcttaactaccaccagatgaacattgtgaagaaggtggaggttcaaaagggaggattctccaaggagtctattaagcctaagggaccttctaacaagctcattcctgtgaagaacggacttgatcctcaaaagtacggaggattcgattcacctgttgttgcttacactgttcttttcactcacgaaaaggggaagaagcctctcattaagcaggagattctcggaattaccattatggagaagactaggttcgagcagaaccctattctttttctagaggagaagggatttcttaggcctagggttcttatgaagctccctaagtacactctttatgagtttcctgagggaagaaggagacttcttgcttctgctaaggaggctcaaaagggaaaccaaatggttcttcctgagcaccttcttactcttctttaccatgctaagcaatgcctacttcctaaccaatctgagtctcttgcttacgtagaacaacatcaacctgagttccaagagattcttgagagggttgtggatttcgctgaggttcatacccttgctaagtctaaggttcagcagattgttaagttgttcgaggctaaccagactgctgatgttaaggagatcgctgcttcattcattcagcttatgcaattcaatgctatgggtgctccttctaccttcaagttcttccagaaggatatagagagggctaggtacacctccatcaaggagattttcgatgctaccattatctaccagtctactactggactttatgagactaggaggaaggtggttgat

SEQ ID NO: 178 - DNA, 4011 bp, synthetic construct
  misc_feature 1..4011: note = source = /note="Description of Artificial Sequence: Syntheticpolynucleotide"
  misc_feature 1..4011: note = source = /note="APG05459.1 Corn optimized"
  source 1..4011: mol_type = other DNA
atgaaaaaggactacgtgatcggcctggacatcggcactaattcagtgggctgggccgtgatgacagaggactaccagctggtgaagaagaagatgcctatctacggcaacactgagaagaagaagatcaagaagaacttctggggcgtgcgcctattcgaggagggccacacagccgaggaccgcagattaaagaggacagccaggaggaggatctctaggaggaggaataggctgcgctacctgcaagcattcttcgaggaggccatgacagccctggatgaaaatttcttcgccaggctgcaggagtctttcctagtgccggaggataaaaagtggcacaggcaccctatcttcgccaagctggaggatgaggtggcctaccatgaaacatacccaacaatctaccacctgaggaagaagctggccgattcttctgagcaggccgacctgagattaatctacctggccctggcccacatcgtcaaatacaggggccacttcctgatcgagggcaaactgagcacagaaaatatcagcgtgaaggagcagttccagcagttcatgatcatctataaccaaaccttcgtgaacggcgaatcaaggctggtgagcgccccactgccggagagcgtattaatcgaggaggaactgaccgagaaagcatcccgaaccaagaagagcgagaaggtgctgcagcagttcccgcaagagaaggctaatggcctgttcggtcagttcctgaaactgatggtgggcaataaagccgacttcaagaaggtgttcggcctagaggaggaggccaaaataacctacgccagcgagagctacgaggaggacctggagggcatactagccaaggtgggcgatgaatacagcgatgtgttcctggccgccaagaatgtgtacgatgccgtggagctgtctacaatactagccgacagcgataaaaagagccacgccaagctctcttcaagcatgatcgtgaggttcacagagcatcaggaggacctgaagaagttcaagcgcttcatcagggagaactgcccggacgagtacgacaacctgttcaagaacgagcagaaggatggctacgccggatacatcgcccacgccggtaaggtgtcccaattaaagttctaccagtacgtgaagaaaataatccaggacatcgccggcgccgagtacttcctggagaaaatagcccaggagaacttcctgcgcaagcagaggacattcgacaacggcgtcatcccgcaccagatacatctggccgagctgcaggccatcatacataggcaggccgcatactacccattcctaaaggagaaccaagagaaaatagagcagctggtgaccttccgcatcccatactacgtgggcccactgtctaagggcgatgcctctacattcgcctggctgaagaggcagtctgaggaaccaatcaggccatggaatctgcaagagacagtggatctggatcagtctgccacagccttcatcgagaggatgaccaacttcgatacatacctaccaagcgagaaggtgctgccaaagcatagcctgctgtatgaaaagttcatggtgttcaacgagctaaccaagatcagctacaccgacgaccgcggaatcaaggccaacttcagcggcaaggagaaggagaaaatattcgactacctgttcaagacccgccgcaaggtgaagaagaaggacataatacagttctaccgcaacgaatacaacaccgagatcgtgaccctgagcggccttgaggaggaccagttcaacgccagcttctcaacctaccaggacctattaaagtgcggcctgacccgcgccgagctggaccacccggataacgccgagaagctggaggacataatcaagatactaaccatcttcgaggaccgccagcgcatccgcacccaattaagcaccttcaagggccagttcagcgccgaggtattaaagaagctggagcgcaagcattacacaggctggggcaggctgagcaagaagctaatcaacggcatctacgacaaggagagcggcaagaccatccttgactacctgatcaaggacgatggcgtgagcaagcactacaaccgcaacttcatgcagctgatcaacgacagccagctgagcttcaagaacgccatccagaaggcccagtcttctgagcacgaggagacactgtctgagacagtgaatgagctggccggctcaccagccatcaagaagggcatctaccagtctctgaagatcgtggatgagctggtggccatcatgggctacgccccaaagaggatcgtggtggagatggccagggagaatcagacaacatcaacaggcaagaggaggtctatccagaggctgaagatcgtggagaaggccatggccgagatcggctctaatctgctgaaggagcagccaacaacaaatgagcagctgagggatacaaggctgttcctgtactacatgcagaatggcaaggatatgtacacaggcgatgagctgtctctgcataggctgagccactacgacatcgatcacatcatcccgcagtcattcatgaaggacgactctctggataatctggtgctggtgggctctacagagaacaggggcaagagcgatgatgtgccatctaaggaggtggtgaaggatatgaaggcctactgggagaagctgtacgccgccggcctgatctctcagaggaagttccagaggctgacaaagggcgagcagggcggcctgacactggaggataaggcccacttcatccagaggcagctagtggagacaaggcagatcacaaagaatgtggccggcatcctggatcagaggtacaatgccaattctaaggagaagaaggttcagatcatcacactgaaggcctctctgacatctcagttcaggtctatcttcggcctgtacaaggtgcgcgaggtgaatgattaccaccacggccaggatgcctacctgaattgcgtggtggccacaacactactgaaggtgtacccaaatctggccccagagttcgtgtacggcgagtacccaaagttccaggccttcaaggagaataaggccacagccaagacaatcatctacacaaacctgatgaggttcttcacagaggacgagccaaggttcatgaaggatggcgagatcctgtggagcaacagctacctgaagaacatcaagaaggagctgaactaccaccagatgaacatcgtgaagaaggtggaggtccagaagggcggcttctcaaaggagagcatcaagccgaagggcccgagcaacaagctgatcccagtgaagaatggcctggacccacagaagtacggcggctttgattctccagtggtggcctacacagtgctgttcacacacgagaagggcaagaagccactgatcaagcaggagatcctgggcatcacaatcatggagaagacaaggttcgagcagaacccaatcctgttcctggaggagaagggcttcctgaggccaagggtgctgatgaagctaccaaagtacacactgtacgagttcccagagggcaggaggaggctgctggcctctgccaaggaggcccagaagggcaatcagatggtgctgcctgagcacctgctgacactgctgtaccacgccaagcagtgcctgctgccaaatcagtctgagtctctggcctacgtggagcagcaccagccagagttccaggagatcctggagagggtggtggatttcgccgaggtgcacacactggctaagtctaaggttcagcagatcgtgaagctgttcgaggccaatcagacagccgatgtgaaggagatcgccgcctcattcatccagctgatgcagttcaatgccatgggcgccccatctacattcaagttcttccagaaggatatcgagagggccaggtacacatctatcaaggagatcttcgatgccacaatcatctaccagtctacaacaggcctgtacgagacaaggaggaaggtggtggat

SEQ ID NO: 179 - DNA, 4308 bp, synthetic construct
  misc_feature 1..4308: note = source = /note="Description of Artificial Sequence: Syntheticpolynucleotide"
  misc_feature 1..4308: note = source = /note="APG04583.1 Soy optimized"
  source 1..4308: mol_type = other DNA
atggccaaaaatattctaggactcgatctcggaaccaactctattggatgggctcttgttcagcaggactttgaaaataaggaggggaacatactaggaatggggtccagaataattcctatgtctcaggatatactaggagagttcgggaagggtaactctatttctcaaactgctgagagaactggatataggggagttagaaggttaagggagagacatcttcttagaagggagaggcttcatagggtgcttcatcttcttggattcctacctaagcattacgacgagaaaatagacttcactcagaggttcgggaagttcatcaatcaagctgaaccaaagttggctttcgattcagagttcctcttcaaggactccttccatgaaatgctagctgacttcaagcagaatcaacctgagttcctcaaggataaaaacggagaggattgccttgttccttacgactggactatatactacctaaggaagaaagcattgacccagaagatcgaaaaatatgagctggcctggctcatcctcaacttcaatcaaaagaggggatactatcaattaaggggagaggaggagaaggagaaccctaataaactcgtggggttccactctctcaaaatagtggatgttattcctgacgctgaaaccaataaaaagggagagacctggtactcacttcatcttgagaacggatgggtttataggaggtcctccaaaatatctctcgctgattggaaggacaaagtgagggatttcattgtgaccaccgatcttaatgatgatggatcagagaagctcgataaggatggaattgtgaagaggtcttttagggctccttctgctgatgactggaccctattaaagaagaagaccgagaaggatatcgacaactctaataaaaccgtggggacctacatctacgacaacctcctattaaaccccaagcagaaaatcaagggaaagatggttaggaccattgagaggaagttctacaagcaagagctggagcagatattaaagactcagaaggagttccattctgagcttcagtctgagaacttgcttcaagattgcgttagggagctgtacaggaataatgagcaacatcaacagatgcttgaggctaaggatttcgtgcacctcttcctcaacgatataattttctaccagaggcctcttaggtcccagaaatcaagcatttctaattgcacccttgagttccgcaagtccaagaatgaaaacggagaggaggtaatacacagattaaaggtgatcgccaaatcaaacccatactaccaggagttcaggcttcttcaatgggttcagaacctcgctatctatactaaggacgacgataagaacgtaaccaacgagttcctcaaatcaactcaggattgggaggatcttcttaggtggcttcactctaagaaggaaatcaagcaggatgctctaatcaagttcctcattgagaagaagggactcaaggggaaagcattgactattgaggtggcaaaatataggtggaactacgttcaggataaggattaccctggaaatgaaacccgctacctcattcaatcaaggcttgataaggttgagtacgctcctaaggatttcctcacctatgaaaatgaaatggccctctggcatatcatctactcaatcaacgacaagatcgagtatgaaaaggcattaaagtccttcgccaataaaaaggggctcgatgaggtgaccttcgtggaagcattcaagaagttccctcctttcaagtccgattacggatctttctctgagaaggcaatcaagaagctccttccattaatgaggttcggaactcaatggaactgggataacatcgaccaaaatagcaaggagaggattggaaaaatactaaccggggagtacgatgaaaatattaaagggagggttagggagaaggctaggcaccttaactctgagaccgattttcaagcattacctctttggcttgctcagtacgttgtttatggaaggcactctgaagctgatattgctggaaagtggaactctgtggatgatctcaagcagttccttgatgatttcaagcagcattccttgaggaaccctattgtggagcaggttattactgagactcttagggctgttaaggatatttggaacttctacggaaagggggctaaggatttcttctcagaaatacacattgagcttgggagggagatgaaaaataccgctgatgaaaggaagaggattaccaccatggtgaccgacaatgaaaataccaacctcagaatcaaagcattgcttgctgagatggctcttgatcagaacgttgataacgttaggccttactctcctatgcagcaggagattcttaagatctatgaggagggagttctaaacgctgaggagaacatcgatgatgatatcctcaagatttctaagactgctcagccttctgctaccgatcttaagaggtataagttgtggcttgagcaaaagtacaggtctccttacactggacagatgattcctcttaacaagttgttcacccctgagtacgagatcgagcacattattcctcagtctaggtacttcgacgattcaatgtccaacaaggttatttgcgaggctgctgtgaacaagttgaaggataaccagattggactcgtgttcattaagaaccatcatggagaggtggttgatttcggaatgggaaagcaggtgaagattcttgaggtttctgattacgaggatttcgtgaagcagaactataacaagaacaggggaaagaggaacaagctcctcttagaggatatccctgagaagatgattgagaggcagcttaacgataccaggtacatctctaagtacattacccaggtgctttccaacattgttagggatgataaggagggatctaaggatgatggagtgaactccaagaacattgttcctggaaacggaaagattaccaccaggcttaaacaggattggggacttaacgatgtgtggaacgatcttgttcttcctaggttcgagaggatgaacactcttaccaactctaacgatttcacctctaagaacactcacggaaagactattcctactgtgcctattgagctttcaaagggattctccaagaagaggattgatcacaggcatcatgctatggatgctcttgttattgcttgcgctactagggatcatgtgaaccttctcaacaacgagtcttctaagtctgataccaagaggtacgatcttaacaggaagttgaggaagtacgagaaggttgcttacaacgatcctaagactggagagagaattgagaaggaggtgcctaaggattttattaagccttgggagacctttactgaggatactaggacccttcttgagaacatcgtgatttctttcaagcagaacctcagggtgattaacaaggctaccaactactacgagaagattgagaacggaaagaaggtgaaggttgagcagaagggaattaattgggctgttaggaaggctctacataaggagactgtttctggacaggtgcaccttgataggattaaagtggctaagggaaagattcttaccgctactaggaagactcttgatgcttctttcaacgagaagaccattgagtctattaccgataccgggattcagaagattctcctcaactacctcaagtccaaggataacaatcctgaggttgctttctctcctgaaggaattgaggagcttaacaagaacatcaggctctataacgatggaaaggctcaccagcctattcttaaggttagggttttcgagcagggatctaagtttactcttggagagactggaaacaagactactaagtttgttgaggctgctaagggaaccaaccttttcttcggaatctacgaggataagtctggaaagaggtcttacgagaccatccctttgaacattgttattgagaggcaaaagcaaggactacaagctgttcctgagactaacgagaagggaaagcagcttcttttcaccctttctcctaacgatcttgtttatgttcctgaggagggagttttcgatgagaacaacatcaaggtggataggatctacaaggtggtgtctttctctacttaccaatgcttcttcgtgaggaacgatgtgtctacttctgtggttaacaaggttgagtactctgctctcaacaagatggagaagtccatcgacaacatcatgattaaggagaactgcgtgaagttgaacgttgataggctcggaaagatttccaaggct

SEQ ID NO: 180 - DNA, 4308 bp, synthetic construct
  misc_feature 1..4308: note = source = /note="Description of Artificial Sequence: Syntheticpolynucleotide"
  misc_feature 1..4308: note = source = /note="APG04583.1 Corn optimized"
  source 1..4308: mol_type = other DNA
atggccaagaacatactaggcctggacctcggaaccaattctatcggctgggccctggttcagcaggactttgagaacaaggagggcaacatactaggcatgggcagccgaataatccctatgtctcaggacatactgggcgagttcggtaagggcaacagcatctcacagacagccgagaggacaggctaccgcggcgtgaggaggctcagggagaggcacctgcttaggagggagaggctacacagggtgctgcatctgctgggcttcctgccaaagcattacgatgaaaagatagatttcacacagaggttcggcaagttcatcaatcaagccgaaccaaagctagccttcgattctgagttcctgttcaaggacagcttccatgaaatgctggccgacttcaagcagaatcaaccggagttcctgaaggataaaaacggcgaggactgcctagtgccgtacgactggaccatatactacctgcgcaagaaggccctcacccagaagatcgaaaaatacgagctggcctggctgatccttaacttcaaccaaaagcgcggatactaccagctacgcggcgaggaggagaaggagaacccgaataaactggtgggcttccacagcctgaaaatagtggacgtgatcccggacgccgagactaataaaaagggcgagacctggtactcacttcacctggagaacggctgggtgtaccgcaggagcagcaaaatatctctggccgactggaaggataaagtgagggacttcatcgtgaccacagacctgaacgacgatggctcagagaagctggacaaggatggcatcgtgaagaggtcattcagggccccatctgccgatgactggaccctattaaagaagaagaccgagaaggacatcgacaacagcaataaaaccgtgggcacctacatctacgacaacctgctattaaacccgaagcagaaaatcaagggcaagatggtgcgcaccatcgagcgcaagttctacaagcaggagctggagcagatactaaagacccagaaggagttccacagcgagctgcagagcgagaacctgctgcaggactgcgtgcgcgagctgtaccgcaataatgagcagcaccagcagatgctggaggccaaggacttcgtgcacctgttcctgaacgatataatcttctaccagaggccgctcaggagccagaagtcaagcatcagcaattgcaccctggagttccgcaagagcaagaatgaaaacggcgaggaggtgatacatcgattaaaggtgatcgccaagagcaacccatactaccaggagttccgcctgctgcagtgggtccagaacctggccatctatactaaggacgacgacaagaacgtaaccaacgagttcctgaaatcaacccaggactgggaggacctgctgcgctggctccacagcaagaaggaaatcaagcaggacgccctaatcaagttcctgatcgagaagaagggattaaagggcaaagcattgaccatcgaggtggcaaaatacaggtggaactacgtccaggacaaggactacccgggcaatgaaacccgctacctaatacagagccgcctggacaaggtggagtacgccccgaaggacttcctgacctacgagaatgaaatggccctgtggcatatcatctactcaatcaacgacaagatcgagtatgaaaaggcattaaagagcttcgccaataaaaagggcctggacgaggtgaccttcgtggaagcattcaagaagttcccgccgttcaagagcgactacggcagcttcagcgagaaggcaatcaagaagctgctgccattaatgcgcttcggcacccagtggaactgggacaacatcgaccaaaatagcaaggagcgcatcggcaaaatactaaccggcgagtacgacgagaacataaagggccgcgtgcgcgagaaggcccgccacctgaacagcgagaccgacttccaagcattgccgctgtggctggcccagtacgtggtctacggcaggcacagcgaggccgatatcgccggcaagtggaacagcgtggatgatctcaagcagttcctggacgatttcaagcagcacagcctgaggaatccaatcgtggagcaggtgatcacagagacactaagggccgtgaaggacatctggaatttctacggcaagggcgccaaggacttcttcagcgagatacatatcgagctgggccgcgagatgaaaaacaccgccgatgaaaggaagaggatcacaaccatggtgaccgacaatgaaaacaccaacctgcgaatcaaggccctgctggccgagatggccctggatcagaacgtggataacgtgaggccatactctccaatgcagcaggagatcctgaaaatatacgaggagggcgtattaaacgccgaggaaaatatcgacgacgacatcctgaaaataagcaagaccgcccaaccaagcgccaccgacctgaagcgatataagctgtggctggagcaaaaatacaggagcccgtacaccggccagatgatcccgctgaataaactgttcaccccggagtatgaaatcgagcatataatccctcagagccgctacttcgacgacagcatgagcaacaaggtgatctgcgaggccgccgtgaacaagctaaaggacaaccagatcggcctggtgttcatcaagaaccaccacggcgaggtggtggacttcggcatgggcaagcaggtgaagatcctggaggtgagcgactacgaggacttcgtgaagcagaactacaacaagaaccgcggcaagaggaacaagctgctgctggaggacatccctgagaagatgatcgagaggcagctgaacgacacccgctacatcagcaagtacatcacacaggtgctgagcaacatcgtgagggacgataaggagggctcaaaggatgatggcgtgaacagcaagaacatcgtgccaggcaacggcaagatcacaacaaggctgaagcaggattggggcctgaacgatgtgtggaatgatctggtgctgccaaggttcgagaggatgaacaccctgaccaacagcaacgacttcacctctaagaacacccacggcaagacaatcccaacagtgccgatcgagctgagcaagggcttcagcaagaagaggatcgatcacaggcaccacgccatggatgccctggtgatcgcctgcgccacaagggatcacgtgaatctactgaataacgagtctagcaagagcgatacaaagaggtacgatctgaacaggaagctgcgcaagtacgagaaggtggcctacaacgatccaaagacaggcgagaggatcgagaaggaggtgccgaaggatttcatcaagccatgggagacattcacagaggacacaaggaccctgctggagaacatcgtgatcagcttcaagcagaacctgcgcgtgatcaacaaggccaccaactactacgagaagatcgagaacggcaagaaggtgaaggtggagcagaagggcatcaattgggccgtgaggaaggccctacataaggagacagtgtctggccaggtgcacctggataggatcaaggtggccaagggcaagatcctgacagccacaaggaagacactggatgcctctttcaacgagaagacaatcgagagcatcacagacaccggcatccagaagatcctgctgaactacctgaagagcaaggacaacaacccagaggtggccttctctccagagggcatcgaggagctgaacaagaacatcaggctgtacaatgatggcaaggcccaccagccaatcctgaaggtgcgcgtgttcgagcagggctcaaagttcacactgggcgagacaggcaataagacaacaaagttcgtggaggccgccaagggcacaaatctgttcttcggcatctacgaggataagtctggcaagaggtcttacgagacaatcccgctgaatatcgtgatcgagaggcagaagcagggactgcaggccgtgccagagacaaatgagaagggcaagcagctgctgttcacactgtctccaaatgatctggtgtacgtgccagaggagggcgtgttcgatgagaacaatatcaaggtggacaggatctacaaggtggtgagcttctcaacctaccagtgcttcttcgtgaggaacgacgtgagcacaagcgtggtgaacaaggtggagtacagcgccctgaacaagatggagaagagcatcgacaacatcatgatcaaggagaactgcgtgaagctgaacgtggaccgcctgggcaagatctctaaggcc

SEQ ID NO: 181 - DNA, 4368 bp, synthetic construct
  misc_feature 1..4368: note = source = /note="Description of Artificial Sequence: Syntheticpolynucleotide"
  misc_feature 1..4368: note = source = /note="APG01688.1 Soy optimized"
  source 1..4368: mol_type = other DNA
atgatgatcaagaacatactaggactcgatctcggaaccaactctatcggatgggctctaatcaagcaggatttcgagaacaagcatggagaaatactagggatgggctccagaataattcctatgtcccaggatatactaggagatttcggaaagggtaactctatttctcagaccgctgatagaaccaagtataggtctgttagaaggcttagggagagatttcttcttaggagagagaggcttcatagggtgctccacctattaaacttccttcctcaacactacgcttctcagatcgatttcgagaagaagttcggaaagtttaagtctgagaccgaaccaaagttagcttgggaaaattggggaggaaagttctctttcctcttccaaaatagcttcaatgaaatgctggaggatttcaaggctgctggacaggggctcaaaataccttacgactggaccatatactatctcaggaagaaagcattgtcccagaaaatagagaaggaggagctagcttggatactcctcaacttcaatcaaaagaggggatactatcaattaagaggtgaggaggaggaggagaaccctaataaactcgtggagttctactccctcaaaatagtggatgttgttgctgatgagcctcagaagggaaagtccgatatctggtactcattaattcttgagaacggatgggtttatcgcagggcttccaaaatacctctcttcgactggaaggataaaaccagggatttcattgtgaccaccgatcttaacgatgataggtctgtgaagactgataaggagggaaatgaaaagaggtcttttagggctccttcagagaacgattggactcttgtgaagaagaagactgagcaggagattgatcagtctcataaaaccgtgggaacctacatctatgaaaccctcctattaaaccccaagcagaaaatcaagggaaagttggtgaggaccattgagaggaagttctacaaggacgagcttaagcagatactagagaagcaaaaggagttccaccaggaattaaagaacgacgacctatataacgactgcattagggagctgtacaggaataatgaggctcaccaattaaccctctccaagaaggatttcgtgcacctattaatggacgatctcattttctaccagaggcctcttaggtcccagaaatcaagcatttctaattgcaccctggagttcagaaaatacaaggatgaaaacgggattgagcacacccagtacctcaaggctatcccaaaatcaaacccatactaccaagagtttaggctttggcagtggatgtacaacttgaacatctacagaaaggatgatgaggctaacgtaaccaaggagttcctcaacaccaataaagacttcgagtctctcttcgagttcctcaataatcgcaaggagattgagcagaagcccctaatcaagttccttcttgagcagaaggacataaacaagaagctattaaacgccgaggctgagaaatacaggtggaactacgtggaggataaaaagtacccctgcaatgaaaccaagaccatgatttcctctaggcttgacaaggtggaaaatatctccgatgatttcctcaccagggacatcgagcagaaaatatggcatataatctactccgtgaacgacaagatcgagtatgaaaaggcattaaagtccttcgctaccaggaacgacctcgatgaaaatagcttcatcgaagcattcaagaagttctcccctttcaagtccgagtacggatctttctctgagaaggcaatcaagaagctccttccattaatgaggctcggaaaatactggtacgaggatgaaatcgtgaagcattccgacatctacttcaaaaatattgagaacctcctcggggatttctccaaccgcgacaagaaaatatctgaggaagacaaggagaagtggaacaagtcaatcaaccttaagctccaggaggaattaaaggatttccagaccgctgagattgatttgttccagggacttaggcttcacattgctcagtaccttgtttatggaaggcactccgaagcatctatgattggaaagtggaattctgctgaggatcttgaggagttccttaaggatttcaagcagcattcccttaggaaccctattgtggagcaggttattactgagactcttagggtggttaaggatatttggctaaagtacggaaacggggctaaggatttcttcaacgagattcatattgagcttggaagggaaatgaagttgcctgctgatgataggaagaagctcaccaaccaaatttctgagaacgagaacaccaacttcaggattaaggctctccttgctgagatgatgaacgattcttctgttgagaacgttaggcctttctctcctatgcagcaggagattctaaagatctacgaggatgatgtgctcaagtccgatatcgagatcgaggatgatatcctcaagatttctaagactgctcaaccttctccttctgatcttaagaggtacaagttgtggcttgagcagaagtacaagtctccttacaccggacagattattcctcttaacaagttgttcacccctgagtacgagatcgagcacattattcctcagtcaaggtacttcgatgattccttctccaataaggtgatttgcgagtctgctgtgaacaagctcaaggataactacatcgggcttgagttcattaagcagttcggaggaactattattgagcttggattcgggaagtctattaaggtgttcgagactaaggagtacgaggatttcgtgaagaagcattacgctaacaaccagggaaagaggaacaagctccttatggaagatatccctgagaagatgattgagaggcagatgaacgataccaggtacatctcaaagtacatttctggggtgctttctaacattgttagggtggaagatggatctgatgagggagtgaactctaagaacattgttcctggaaacggaaagattaccacccaacttaagcaggattggggacttaacgatgtgtggaacgatctcattcttcctaggttcgagaggatgaatcagcttactaactctaaggttttcactgcttggaacgagaactaccagaagttccttcctactgtgcctattgagtactccaagggattctcaaagaagaggattgatcacaggcatcatgctcttgatgctcttgttattgcttgcgctactaaggatcacgtgaaccttcttaacaaccagtctgctaagtctgataccaagaggtacgatctcaagaagaagtccatgaagttcgagaaggtggtttacaacgatgctaagactggagaaaagattgagagggaggttcctaagcaatttcttaagccttgggagaacttcactcttgatgtgaagcacaaccttgagaccatcattgtgtcattcaagcagaacctcagggtgattaacaaggctaccaactactacgagaagtacgttgagaaggatggaactaagaataaggagagggttgagcaaactggaactaactgggctattaggaagcctatgcacaaggatactgtgtctggaaaagttgatcttccttgggttaaggtgcctaagggaaagattcttactgctaccaggaagtctctcgattcttctttcgatctcaagtccattggatctattaccgataccgggattcagaagatcctaaagaactacctcgctttcaaggatggaaatcctgagcttgctttctctcctgagggaattgatgacctcaacaagaacatcgagaagtataacgatggaaagcctcaccagcctattaacaaggttagggttttcgagcttggatctaagttccaagttggacagtctggaaacaagaaggataagtatgttgaggctgctaagggaaccaaccttttcttcgctgtttatgaggatgagaagggaaagaggaactacgagactattcctctaaacgaggttattgagaggcaaaagcagggactttctgtggttgatcttaaggggaccaacgatttctatctttgccctaacgatttcgtgtacattccttctggagatgagctggagaacatcaacaacgtggacttcaaggatatcaagaaggagattaacgagaggatctacaaggtggtgtctttcactggaaacaggctttcttgcattccttacatggtggctaccactattgtgaacaagttggagttcacccagctaaacaagattgagttcaccaaggagaaggagatctgcattaagttgaacgtggataggctcggaaacatttctaaggct

SEQ ID NO: 182 - DNA, 4368 bp, synthetic construct
  misc_feature 1..4368: note = source = /note="Description of Artificial Sequence: Syntheticpolynucleotide"
  misc_feature 1..4368: note = source = /note="APG01688.1 Corn optimized"
  source 1..4368: mol_type = other DNA
atgatgatcaagaacatcctaggcctggacctcggaaccaattctatcggctgggccctgatcaagcaggacttcgagaacaagcatggcgagatactaggcatgggcagccgaataatcccgatgagccaggacatactaggcgatttcggcaagggcaatagcatctctcagaccgccgacagaaccaagtacaggtctgttaggaggctgagggagaggttccttcttaggagggagaggctgcatagggtgctccacctattaaacttcctgccacagcactacgccagccagatcgacttcgagaagaagttcggcaagttcaagagcgagacagaaccaaagctggcttgggaaaactggggcggcaagttcagcttcctgttccaaaatagcttcaatgaaatgctggaggacttcaaggccgccggccagggattaaagatcccctacgactggaccatatactacctgcgcaagaaagcattgagccagaaaatagagaaggaggagctggcctggatactgctgaacttcaaccaaaagcgcggatactaccagctgcgcggtgaggaggaggaggagaacccgaataaactggtggagttctactcactgaaaatagtggacgtggtggccgacgagccgcagaagggcaagagcgacatctggtacagcctgatactagagaacggctgggtgtaccgccgcgctagcaaaataccgctgttcgactggaaggataaaacccgcgacttcatcgtgaccaccgacctgaacgacgacaggagcgtgaagacagataaggagggcaatgaaaagaggagcttcagggccccaagcgagaacgattggaccctggtgaagaagaagacagagcaggagatcgatcagagccataaaaccgtgggcacatacatctatgaaaccctgctattaaacccgaagcagaaaatcaagggcaagctggtgcgcaccatcgagcgcaagttctacaaggacgagctgaagcagatactagagaagcagaaggagttccaccaggaattaaagaacgacgacctatataacgactgcatccgcgagctgtaccgcaataatgaggcccaccaattaaccctgagcaagaaggacttcgtgcacctattaatggacgacctgatcttctaccagcgcccgctgcgcagccagaagtcaagcatcagcaattgcaccctggagttccgcaaatacaaggatgaaaacggcatcgagcacacccagtacctgaaggccatcccgaagagcaacccatactaccaggagttccgcctgtggcagtggatgtacaacctgaacatctaccgcaaggacgacgaggccaacgtaaccaaggagttcctgaatacaaataaagacttcgagagcctgttcgagttcctgaataatcgcaaggagatcgagcagaagccgctaatcaagttcctgctggagcagaaggacataaacaagaagctattaaacgccgaggccgagaaatacaggtggaactacgtggaggataaaaagtacccgtgcaacgaaaccaagaccatgatcagcagccgcctggacaaggtggaaaatatcagcgacgacttcctgacccgcgacatcgagcagaaaatatggcatataatctacagcgtgaacgacaagatcgagtatgaaaaggcattaaagagcttcgccacccgcaacgacctggatgaaaacagcttcatcgaagcattcaagaagttcagcccgttcaagagcgagtacggcagcttcagcgagaaggcaatcaagaagctgctgccattaatgcgcctgggaaaatactggtacgaggacgagatcgtgaagcatagcgacatctacttcaaaaatatcgagaacctgctgggcgacttcagcaaccgcgacaagaaaataagcgaggaggacaaggagaagtggaacaaaagcatcaacctgaagctgcaggaggaattaaaggacttccagaccgccgagatcgacctgttccagggcctgcgcctccacatcgcccagtacctggtgtacggccgccacagcgaggcaagcatgatcggcaagtggaacagcgccgaggacctggaggagttcctgaaggacttcaagcagcatagcctgcgcaacccgatcgtggagcaggtgatcaccgagaccctgcgcgtggtgaaggacatctggctaaaatacggcaacggcgccaaggacttcttcaatgaaattcacatcgagctgggccgcgagatgaaactgccggccgacgaccgcaagaagctgaccaaccaaatcagcgagaatgaaaacaccaacttccgaatcaaggccctgctggccgagatgatgaacgacagcagcgtggagaacgtgcgcccgttcagcccgatgcagcaggagatcctgaaaatatacgaggacgacgtgctgaagagcgacatcgagatcgaggacgacatcctgaagatcagcaagaccgcccagccgagcccgagcgacctgaagcgctacaagctgtggctggagcagaagtacaagagcccgtacaccggccagatcatcccgctaaacaagctgttcaccccggagtacgagatcgagcacatcatcccgcagagccgctacttcgacgacagcttcagcaacaaggtgatctgcgagagcgccgtgaacaagctgaaggataactacatcggcctggagttcatcaagcagttcggcggcaccatcatcgagctgggcttcggcaagagcatcaaggtgttcgagaccaaggagtacgaggacttcgtgaagaagcactacgccaacaaccagggcaagcgcaacaagctgctgatggaggacatcccggagaagatgatcgagcgccagatgaacgacacccgctacatcagcaagtacatcagcggcgtgctgagcaacatcgtgcgcgtggaggatggctcagatgagggcgtgaacagcaagaacattgtgccgggcaacggcaagatcacaacacagcttaagcaggactggggcctgaacgatgtgtggaacgatctgattctgccaaggttcgagaggatgaaccagctgaccaacagcaaggtgttcaccgcctggaacgagaactaccagaagttcctgccaaccgtgccaatcgagtacagcaagggcttcagcaagaagaggatcgatcacaggcatcatgctctggatgctctggtgatcgcctgcgctacaaaggatcacgtgaacctgctgaacaaccagagcgccaagagcgacacaaagaggtacgacctgaagaagaagagcatgaagttcgagaaggtggtgtacaacgacgccaagaccggcgagaagattgagagggaggtgccgaagcagttcctaaagccatgggagaacttcacactggacgtgaagcacaacctggagaccatcatcgtgagcttcaagcagaacctgagggtgatcaacaaggccaccaactactacgagaagtacgtggagaaggacggcaccaagaacaaggagagggtggagcagacaggcacaaattgggccatccgcaagccaatgcacaaggatacagtgtctggcaaggtggatctgccatgggttaaggtgccaaagggcaagatcctgacagccacaaggaagagcctggatagcagcttcgatctgaagagcatcggctctatcacagacaccggcatccagaagatcctgaagaactacctggccttcaaggatggcaatccagagctggctttctctccagagggcatcgacgacctgaacaagaacatcgagaagtacaacgacggcaagccacaccagccaatcaataaggtgcgcgtgttcgagctaggctctaagttccaggttggccagagcggcaacaagaaggataagtacgttgaggccgccaagggcacaaatctgttcttcgctgtgtacgaggatgagaagggcaagcgcaactacgagacaatcccactgaacgaggtgatcgaaaggcagaagcagggcctgtctgttgtggatctgaagggcaccaacgatttctacctgtgcccgaacgacttcgtgtacattccatctggcgacgagctggagaacatcaacaacgtggacttcaaggacatcaagaaggagatcaacgagcgcatctacaaggtggtgagcttcaccggcaacaggctgagctgcatcccatacatggtggccaccaccatcgtgaacaagctggagttcacccagctgaacaagatcgagttcaccaaggagaaggagatctgcatcaagctgaacgtggacaggctgggcaacatcagcaaggcc

SEQ ID NO: 183 - DNA, 3210 bp, Bacillus sp.
  misc_feature 1..3210: note = source = /note="APG05083.1 Native Seq"
  source 1..3210: mol_type = genomic DNA
atgagagagttggattatcgcataggattagatattggaacgaattctattggctgggggatcattgaattatcttggaacaaagatagagaacaatatgagaaagcaagaattgtcgacaagggtgttcgtatgtttgataaggctgaaatacctaagactggtgcttctcttgctgaaccgaggcgtatagcacgctcatcacgtagaagattaaatcgcaaaagccagagaaaaaaagatatacgtaatttactcgttcaacatgaaattattagtcaaaaggaattggcttcgttatatcccctgacaaaaagttcaatggatatttgggatattcgcttggatggattagatcgcttgttagaccgttttgaatggactcgattattaattcatttagcgcaaagacgcggttttaaatcaaatcgaaagtctgaactgaaagatgtggagacaggaaaagtattatcaagtattcaagcaaatgaaaaacgattatcactgtaccgtacagtgggagagatgtggatgaagaatgaagattttagtaaatatgacaaaaggcgtaattcttctaatgagtatgtattttcggttagccgtgcagatttagaaaaagaaattgtgacactatttgaagcgcaaagaaaatttcagtcatcatatgcatcggctgatttacaaaaaacatacttacaaatttgggcacaccaacttccttttgcttctgggaatgcaattgtaaataaagtaggatattgttcattattaaaagggaaagaaaagagagttccgaaagcaacatatacttttcaatatttcagtacactagatcaaataaatcgaacacgattaggtcctaatttccaaccatttacgaaggaacagagagacgttattttagatgaaatgtttaatcgaacagattattataaaaaaaagacaatacccgaagtcacttactatgatattcggaaatggttagcattagatgaaacaattcaatttaaaggacttacctatgacccaaatgaagagctgaaaaaaatagaattgaaatcctttattaatttaaagccattctatgaaattaaaaaggtagttactaattacgccaaaaaaacaaatgaggcattctcaacattagactatgatacatttgcatatgctttaacagtttataaaacggacaaagatattagatcttatttaaagaaatctaataatttatcaaaatgttgctacgatgatcaattaatagaagagctattaactctctcctatacaaagtttggtcatttatcatttaaagcaattaatcatgtactgccaattatgcaagagggaaggacttatcaggaagcaatacaccaattaggatatgatgccactaatctaaaaaaagaaaacagaagtatgttcttgcccctttttcccgatgagataacaaatccaattgttaaaagagcactaactcaagcacgtaaagttgtaaatgctattattagaagatatggttcccccaattctgttcatattgaactagctcgtgagctttctaaaagtcatgatgagagaacgaaaataatgaaagctcatgatgaaaattataagaaaaataaaggagccatatcaattttgattgagaatggaattttaaatccgacaggatatgatattgtacgttataagttatggaaagagcaaggagaacgatgtgcttattcgctaaaacagattcctgctaatacgttttttaatgaaatgaaaaaagagcgaagtggctccccagttctagagatagatcacattttaccgtatagtcagagttttattgatagttatcataataaagtactagtttatggagatgagaatcaaaaaaagggaaatcgaattccatatacttattttttagaaggaaataaggactgggaaagctttgaaagctacgtacgattgaatagttttttttctaaaaagaagcgcggatatttattgaaaaaagcttacttgccaagagagagtaacatgattaaggagcgtcatttaaatgatactcgatatgctagtagctatttgaaaaacttcattgagaaaaatttgaaatttaaagaagttgaaggtagtacacgaaaaaaacatgtacagacggttaacggtataattacagcccatcttcgaaaaagatggggattagaaaaagataggcaggaaacatatttgcatcatgcaatggacgctattattgttgcttgtacagaccatcatatggtcactaaagtaacggagtactatcaaataaaagaaagtaataagtcaataaggaaaccatactttcctttgccatgggtgggctttagagaggaaattttatcacatttagcaaggcagccaattgctagaaaaattagtgaggaacttaaaattggatatcaatcatttgattatatacttgtatcgcgaatgccaaaaagatctgtcactggagcagctcatgaacagacaatcatgaaaaaaggtggtatcgacaaaaaaggaaaaactattatcataaagcgtgtgtacttaaaggatattaagtttgatgagaatggcgattttaaaatggttggaaaagaacaggatttagcaacttatgaagcgataaagcaaagatatatagagtatggaaaagaatcgaaaaaagcatttgaaacacctttatacaagcctagtaaaaaaggaaaaggaaacctcattaaaaagatcaaagtagaagtgcaaaccaaatcttttgttcgagaagttaatgggggcgtagctcaaaatggtgatttagtaagagtagatttgtttgaaaaggataatagatattatatgatacctatttatgtaatggatactgttcattccgaactaccaaataaagctgtaacaagcagtaaaggctatgagcaatggttaacaatagataacagctttacgttcaaattcagtttatatccttatgatttagtacgacttgtaaaaggtaatgaagatcgtttcctatattttagtacccttgatattaattcggatcgtcttaatttcaaagatgtaaacaagccatcaaagcaggctgaaaatcgttatagccttaaaacaattgagaatttagaaaaatatgaggttggtgttttaggtgatttaaggtttgtgagacaagaaatacgtaaaaatttt

SEQ ID NO: 184 - DNA, 3210 bp, synthetic construct
  misc_feature 1..3210: note = source = /note="Description of Artificial Sequence: Syntheticpolynucleotide"
  misc_feature 1..3210: note = source = /note="APG05083.1 E. coli optimized"
  source 1..3210: mol_type = other DNA
atgcgcgagctagattatcgcatcggcctggatattggcactaactcaataggctggggcatcatcgaactgagctggaataaagaccgcgagcagtatgaaaaggcgcgcatcgtggataaaggcgtgcgcatgttcgacaaagcggaaattccgaaaaccggtgcaagtctggcggaaccaagacgtattgcacgtagtagtcgccgccgattaaaccgcaaaagtcagcgcaagaaggatataaggaacctgctggtccagcatgaaatcatcagccagaaggaactggcgagcctgtacccgctgaccaaatcaagtatggacatctgggatataaggctggacggcctggatcgtctgctggatcgctttgaatggacccgcctattaatccatctggcacagcgccgtggcttcaaatcaaaccgcaagagcgaattaaaggacgtggagaccggtaaagtgctgtcaagcattcaggcgaatgaaaagcgcctgagcctgtatcgtaccgtgggcgagatgtggatgaaaaacgaggacttctcaaaatacgataaaaggcgcaacagcagcaacgagtacgtgttcagcgtgagccgcgcggacctggagaaagaaatcgtgaccctgtttgaggcgcagcgcaaattccaatcaagctatgcgagcgcggatctgcagaaaacctacctgcagatttgggcacatcagctgccgtttgcaagcggtaacgcgatcgtgaataaagtgggctattgcagcctattaaaaggcaaagaaaaacgcgtgccgaaagcgacctatacattccagtacttcagcaccctggaccaaatcaaccgcacccgcctgggcccgaacttccagccgttcaccaaagaacagcgcgacgtgatcctggatgaaatgttcaaccgcaccgactactataaaaagaaaaccatcccggaggtgacatactacgatataaggaaatggctggcgctggatgaaaccatccagttcaaaggcttaacctacgatccgaacgaggaattaaagaagatcgaattaaaatcgttcattaatctgaaaccgttctatgaaattaaaaaggtggtaaccaactacgcgaagaaaaccaacgaagcattcagcaccctggactacgatacattcgcgtacgcgctgaccgtgtataaaaccgacaaggatataaggagctacctgaagaaatcaaacaacctgagcaaatgctgctacgacgaccaattaatcgaagaactgctgaccctgagctacaccaaattcggccacctgagcttcaaagcgatcaaccacgtgctgccgatcatgcaggaaggccgcacctaccaggaagcgatccaccagctgggctacgatgcgaccaacctgaaaaaggaaaaccgcagcatgttcctgccgctgttccctgatgaaatcaccaacccgatcgtgaaacgcgcgctgacccaggcgcgcaaggtggtgaacgcgatcatccgccgctacggctcaccgaacagcgtgcacatcgaactggcgcgcgaactgagcaaaagccacgatgaacgcaccaaaatcatgaaagcgcacgatgaaaactacaaaaagaacaaaggcgcgatcagcatcctgatcgaaaacggcatcctgaacccgaccggctacgatatcgtgcgctacaaactgtggaaagaacagggcgaacgctgcgcgtacagcctgaaacagatcccggcgaacaccttcttcaacgaaatgaaaaaggaacgctcaggcagcccggtgctggaaatcgatcacatcctgccgtacagccagagcttcatcgatagctaccacaacaaagtgctggtgtacggcgatgaaaaccagaaaaagggcaaccgcatcccgtacacctacttcctggaaggcaacaaagattgggagagcttcgaaagctacgtgcgcctgaacagcttcttcagcaaaaagaaacgcggctacctgctgaaaaaggcgtacctgccgcgcgaaagcaacatgatcaaagaacgccacttaaacgatacccgctacgcgagcagctacctgaaaaacttcatcgagaaaaacctgaaattcaaagaagtggaaggcagcacccgtaaaaagcatgtccagaccgtgaacggcatcatcaccgcgcatctgcgcaaacgctggggcctggaaaaagatcgccaggaaacctatctgcatcatgcgatggatgcgatcatcgtggcgtgcaccgatcatcatatggtgaccaaagtgaccgaatattatcagatcaaagaaagcaacaaatcaatccgcaaaccgtattttccgctgccgtgggtgggctttcgcgaagaaatcctgagccatctggcgcgtcagccgatcgcgcgtaaaatcagcgaagaactgaaaatcggctatcagagctttgattatatcctggtgagccgcatgccgaaacgcagcgtgaccggcgcggcgcatgaacagaccatcatgaaaaagggcggcatcgataaaaagggcaaaaccatcatcatcaaacgcgtgtatctgaaagatatcaaatttgatgaaaacggcgattttaaaatggtgggcaaggaacaggacttagcgacctacgaagcgatcaaacagcgctacatcgagtacggcaaagagagcaaaaaggcgtttgaaaccccgctgtacaaaccgagcaaaaagggcaagggcaacctgatcaaaaagatcaaagtggaagtccagaccaaatcgtttgtgcgcgaagtgaacggcggcgtggcgcagaacggcgatctggtgcgcgtggatctgtttgaaaaagataaccgctactatatgatcccgatctacgtgatggataccgtgcatagcgagctgccgaacaaagcggtgaccagcagcaaaggctatgaacagtggttaaccatcgataacagctttaccttcaaattcagcctgtatccgtacgacctggtgcgcctggtgaaaggcaacgaagatcgcttcctgtatttcagcaccctggacatcaacagcgatcgcctgaacttcaaggacgtgaacaaaccgagcaaacaggcggaaaaccgctatagcctgaagaccatcgagaacctggagaaatatgaagtgggcgtgctgggcgatctgcgctttgtgcgccaggaaattcgcaaaaacttc

SEQ ID NO: 185 - DNA, 3213 bp, Bacillus sp.
  misc_feature 1..3213: note = source = /note="APG07433.1 Native Seq"
  source 1..3213: mol_type = genomic DNA
atgagggagttggactatcgcatagggttagatattgggacgaattctattggatggggtgttattgaattatcctggaacaaggacagagaacgatatgaaaaagtaaggattgtcgaccagggtgttcgtatgtttgatagggctgaaatgccaaaaacaggtgcttctcttgctgaaccgaggcgtatagcacgttcatcacgtagaaggttaaatcgtaaaagtcagaggaagaaaaatatacgtaatttacttgttcaacatggggtgattactcaagaagagctggattcgttatatcctctttcaaaaaaatcaatggatatttggggtattcgattggatggattagatcgtctgctaaatcattttgaatgggctcgattattaattcatttagctcaaagacgtggttttaaatcgaatcgtaagtctgaactgaaagatacggagacggggaaggtattatcgagtattcaattaaatgaaaaacgattatcactgtaccgtacagtgggagaaatgtggatgaaagatcctgattttagtaagtatgatagaaaacggaattctcctaatgagtatgtattttcggttagtcgtgcggaactagaaaaggaaatagttactttatttgcagcacaaagaaggtttcagtcaccatacgcatcgaaggatttacaagaaacatatttacaaatttggacacaccaacttccctttgcttctgggaatgcaattttaaataaagtgggatattgttcattattgaaagggaaagaaagaagaattccgaaagcaacatatacttttcagtattttagtgcactagatcaagtgaatcgaacacgattaggacctgattttcagccatttacgaaggaacaaagagaaattattttaaataacatgtttcaacgtacagattattataaaaaaaagactatacctgaagttacatactatgatatccggaaatggctagaactagatgaaactattcaatttaaaggacttaattatgatccaaacgaagaattgaaaaaaatagaaaagaaaccatttattaatttaaaggcattctatgaaattaataaggtagtcgcaaattattctgagagaacaaatgagacattttcaacgttagactatgatgggattggatatgctttaacagtttataaaacggacaaagatattaggtcttatttgaagagctctcataatttacctaaacgttgttacgatgatcaattaatagaggaactattaagtctttcttatacaaagtttggtcacttatcactgaaagcaatcaatcacgtactatcgattatgcaaaaaggcaatacttataaagaagcagtagaccagttagggtatgatacaagcggtttaaagaaagaaaaaagaagtaagttcttgcctcctatttcagatgagataacgaatccaattgttaaaagagcgttaacacaagcgcgtaaagttgtgaatgctataattagaagacatggttctccacattcagttcatattgaactggctcgtgaactttctaaaaatcatgacgagagaacaaaaatagtgtcagctcaagatgaaaattataagaagaataaaggggctatatcaattttaagtgagcatggaattttgaatccaacaggctatgatattgttcgttataagttatggaaagaacaaggagaacgatgtgcttattcgttaaaggagattcctgcggatacgttttttaatgaattaaaaaaagaacgaaatggtgctccaattctagaggtagatcacattttaccgtacagtcaaagttttattgatagttatcataataaagtattagtttacagtgatgaaaatcgaaaaaaggggaatcgaattccatatacctattttttagagacaaataaggattgggaagcttttgaaagatatgtaagatcaaataaatttttttctaaaaagaagcgtgagtatttattgaaaagagcatatttgccaagagaaagtgaactgataaaggagcgacatttaaatgatacgcgatatgctagtacctttttgaaaaacttcattgagcagaatttgcaatttaaagaagctgaagataatccgcgtaaaagacgtgtacaaacagttaacggtgtaattacagcacattttcgaaaaagatggggattagaaaaagatagacaagaaacatacttacatcatgcaatggacgctatcattgttgcttgtacagaccatcatatggttactagagtaacagagtattatcaaataaaagaaagtaataaatcagtaaagaaaccgtattttcctatgccatgggagggctttagagatgaactcttatcacatttagcgagtcagccaatagctaaaaaaattagtgaggagcttaaagctggatatcaatcattagattatatatttgtgtctcgaatgccaaaaagatctatcactggagcagcacataaacaaacgatcatgagaaaaggcggtattgataaaaaaggaaaaactattattatagagcgtttgcatttaaaggatattaagtttgatgagaatggtgattttaaaatggttggcaaagaacaagatatggcaacttacgaggcgataaagcaaagatatttggagcatggaaaaaactcgaaaaaagcatttgaaacacctctatacaaacctagtaaaaaaggaacaggaaatcttattaaaagagttaaagttgaaggacaagctaaatcttttgttcgagaagtaaatgggggcgtagcccaaaatggtgatttagtgagagttgatttatttgaaaaagatgataaatattacatggtgcctatttatgtaccagataccgtttgttcagaattacccaaaaaagttgtggcaagtagtaagggttatgagcaatggttaacactagataacagctttacgtttaaatttagtttatacccttatgatttagtacggcttgtaaaaggggacgaagatcgtttcttatactttggtactctcgatatcgattcagatcgtcttaattttaaagatgtaaataagccatcaaaaaagaatgaatatcgttatagccttaaaacaattgaggatttagaaaaatatgaggtgggtgttttaggagatttaaggttagtaagaaaagaaacacgtagaaattttcac

SEQ ID NO: 186 - DNA, 3213 bp, synthetic construct
  misc_feature 1..3213: note = source = /note="Description of Artificial Sequence: Syntheticpolynucleotide"
  misc_feature 1..3213: note = source = /note="APG07433.1 E. coli optimized"
  source 1..3213: mol_type = other DNA
atgcgcgagctagattatcgcatcggcctggatattggcactaactcaataggctggggcgtgatcgaactgagctggaataaagaccgcgagcgctatgaaaaggtgcgcattgtggatcagggcgtcagaatgtttgatcgtgcggaaatgccgaaaaccggtgcatcactggcagaaccaagacgtatagcacgtagtagtcgccgccgattaaaccgtaaaagccagcgcaagaaaaatatccgcaacctgctggttcagcatggcgtcatcacccaggaagaactggatagcctgtacccgctgagcaagaaatcaatggacatctggggcattcgtctggatggtctggaccgcctattaaaccactttgaatgggcccgcctattaattcatctggcgcagcgccgcggcttcaaatcaaaccgcaagagcgaattaaaggacaccgagaccggtaaagtgctgtcatcgatccagctgaatgaaaaacgcctgagcctgtatcgcaccgtgggcgagatgtggatgaaagacccggacttctcaaaatacgaccgcaaacgcaacagcccgaacgaatacgtgtttagcgttagccgtgcggaactggagaaagaaatcgtgaccctgtttgcagctcagcgccgttttcagagcccgtatgcgagcaaagatctgcaagaaacctacctgcagatctggacccatcagctgccgtttgcaagcggtaacgcgatattaaacaaagtgggctattgcagcctattaaaaggcaaagaacgccgcatcccgaaagcgacctatacattccagtacttcagcgcgctggaccaggtgaaccgtacccgtctgggtccggattttcagccgttcaccaaagaacagcgcgagatcatattaaacaacatgttccagcgcaccgactactataaaaagaaaaccatcccggaggtgacatattacgatataaggaaatggctggaactggatgaaaccatccagttcaaaggcctgaactacgatccgaacgaggagctgaaaaaaatcgagaaaaaaccgttcattaatctgaaagcgttctatgaaatcaacaaagtggtggcgaactacagcgaacgcaccaatgaaaccttctcaaccctggattacgatggcatcggctacgcgctgaccgtgtataaaaccgacaaggatataaggagctacctgaaatcaagccacaacctgccgaaacgctgctacgacgaccaattaatcgaagaactgctgagcctgagctatactaagttcggccacctgtcattaaaagcgattaatcacgtgttaagcatcatgcagaaaggcaacacatataaagaagcggtggatcagctgggctacgataccagcggattaaaaaaagaaaaacgcagcaaattcctgccgccgatcagcgatgaaatcaccaacccgatcgtgaaacgcgcgctgacccaggcgcgcaaagtggtgaacgcgatcatccgccgccacggcagcccgcacagcgtgcacatcgaactggcgcgcgaactgagcaaaaaccacgatgaacgcaccaaaatcgtgagcgcgcaggatgaaaactacaaaaagaacaaaggcgcgatcagcatcctgtcagaacacggcatcctgaacccgaccggctacgatatcgtgcgctacaaactgtggaaagagcagggcgaacgctgcgcgtacagcctgaaagaaatcccggcggataccttcttcaacgagctgaaaaaagaacgcaacggcgccccgatcctggaagtggatcacatcctgccgtacagccagagcttcatcgatagctaccacaacaaagtgctggtgtacagcgatgaaaaccgcaaaaaaggcaaccgcatcccgtacacctacttcttagagaccaacaaagattgggaagcgttcgaacgctacgtgcgcagcaacaagttcttcagcaaaaagaagcgcgagtacctgctgaaacgcgcgtacctgccgcgcgaaagcgaactgatcaaagaacgccatctgaacgatacccgctacgcgagcaccttcctgaaaaacttcatcgaacagaacctgcagttcaaagaagcggaagataacccgcgcaaacgccgcgtccagaccgtgaacggcgtgatcaccgcgcattttcgcaaacgctggggcttagaaaaagatcgccaggaaacctatctgcatcatgcgatggatgcgatcatcgtggcgtgcaccgatcatcatatggtgacccgcgtgaccgaatattatcagatcaaagaaagcaacaaaagcgtgaaaaaaccgtattttccgatgccgtgggaaggctttcgcgatgaactgctgagccatctggcgagccagccgatcgcgaaaaaaatcagcgaagaactgaaagcgggctatcagagcctggattatatctttgtgagccgcatgccgaaacgctcaatcaccggcgcggcgcataaacagaccatcatgcgcaaaggcggcatcgataaaaaaggcaaaaccatcatcatcgaacgcctgcatctgaaagatatcaaatttgatgaaaacggcgattttaaaatggtgggcaaagaacaggacatggcgacctacgaagcgatcaaacagcgctatctggagcatggcaagaacagcaaaaaagcgtttgagaccccgctgtacaaaccgagcaaaaaaggcaccggcaacctgatcaaacgcgtgaaagtggaaggccaggcgaaatcatttgtgcgcgaagtgaacggcggcgtggcgcagaacggcgatctggtgcgcgtggatctgtttgaaaaagatgacaaatattatatggtgccgatctatgtgccggataccgtgtgtagcgaactgccgaaaaaagtggtggcgagcagcaaaggctatgaacagtggctgaccctggataacagctttaccttcaaattcagcctgtatccgtatgatctggtgcgcctggtgaaaggcgatgaagatcgctttctgtattttggcaccctggacatcgattcagatcgcctgaacttcaaggacgtgaacaaaccgagcaaaaagaacgaatatcgctatagcctgaaaaccattgaagatctggaaaaatatgaagtgggcgtgctgggcgatctgcgcctggtgcgcaaagagacccgccgcaactttcat

SEQ ID NO: 187 - DNA, 3213 bp, Bacillus sp.
  misc_feature 1..3213: note = source = /note="APG07513.1 Native Seq"
  source 1..3213: mol_type = genomic DNA
atgagagagttggattatcgcataggattagatattggaacgaattctattggctggggtgttattgaattatcttggaacaaagatagagaacaatatgagaaaacgagaattgtcgacaagggtgttcgtatgtttgataaggctgaaatacctaagactggtgcttctcttgctgaaccgagacgtatagcgcgctcatcacgtagaaggttaaatcgtaaaagccagagaaaaaaagatatacgtaatttacttgttcaacatgaaattattagccaaaaggaattgacttcgttatatcccctgtcaaaaagttcaatggatatttgggatattcgcttagatggattagatcgcttgttagaccgttttgaatgggctcgattattaattcatttagcacaaagacgcggttttaaatcaaatcgaaagtctgaactgaaagatgtggagacaggaaaagtattatcaagtattcaagtaaatgaaaaacgattatctctgtaccgtacagtgggagagatgtggatgaagaatgcggattgtagtaaatatggcaaaaggcgtaattctcctaatgagtatgtattttcggttagccgtgcagatttagaaaaggaaattgtgactctatttgaggcgcaaagaaaattccattcatcatatgcatcggttgatttacaaaaaacatatatacaaatttgggcacaccaacttccttttgcttctgggaatgcaattgtaaataaagtaggatattgttcattattaaaaggtaaagaaaagagagttccaaaagcaacatatacttttcaatatttcaatacactagatcaaataaaccgaacacgattagggcccaatttccaaccatttacgaaggaacagagagacataattttagataaaatgtttcaacggacagattattataaaaaaaagacaatacccgaagttacttactatgatattcggaaatggttagcactagatgaaacaattcaatttaaaggacttacctatgacccaaacgaagagctgaaaaaaatagaaatgaaaccctttattaatttaaagccattctatgaaattaaaaaggtagttactaattacgcaaaaaaaacaaatgaggtattctcagcattagattatgatacagttgcatacgctttaacagtttataaaacggacaaagatattagatcttatttgaagagatctaataatttatcaaaacgttgctacgatgatcaattaatagaagagctattaactctctcctatacaaagtttggtcatttatcatttaaagcaattaatcatgtactgccaattatgcaagagggaaggacttatcaggaagcaatacaccaattagggtatgataccactaatcttaaaaaagaaaacagaagtatgttcttgcctattattccagatgagataacaaatccaattgttaaaagagcgttaactcaagcacgtaaagttgtaaatgctattattagaagatatggttctccaaattctgttcatattgaactagctcgtgagctttcgaaaagtcatgacgagagaaaaaaaataatgacagctcatgatgaaaattataagaaaaataaaggagctgtatcaattttgatcgataatggaattttaaatccgacaggatatgatattgtacgttataagttatggaaagagcaaggagaacgatgtgcttattcgttaaaaaagattcctgctaatacgttttttaatgaattgaaaaaagagcgaagtggccctccggttctagaggtagatcacattttaccgtatagtcagagttttattgatagttaccataataaagtattagtttatggggatgaaaatcaaaaaaagggaaatcgaattccatatacttttttttcagaagaagataaggagtgggaaagctttgaaagctacgtaagatcgaatagttttttttctaaaaagaagcgcggatatttattgaaaaaagcttacttgccaagagagagtaacttgattaaggagcgtcatttaaatgatacccgatatgctagtagctatttgaaaaacttcattgagaaaaatttaaaatttaaagaagctgtaggtattacacgaaaaaaatatgtacagacggttaacggtgtaattacagcccatctgcgaaaaaggtggggtttagaaaaagataggcaggaaacatatttgcatcatgcaatggacgctattattgttgcttgtacagatcatcatatggtcactaaagtaacggagtactatcaaataaaagaaggtaataagtcaataaagaaaccgtattttcctttgccatggatgggatttagagaggaaattttatcacatttagaaagtcagccaattgctagaaaaattagtgaggaacttaaaattggatatcaatcacctgattatatacttgtatcgcgaatgccaaaaagatctgtcactggatcagctcatgatcagacagtcatgaaaaaaggcgatatcgataaaaaaggaaagactattatcataaagcgtgtgcacttaaaggatattaagtttgatgagaatggcgattttaaaatggttggcaaagaacaagatttagcaacttacgaagcgataaagcaaagatatttagagtatagaaaagaatcgaaaaaagcatttgaaacacctttatacaagcctagtaaaaaaggaaaaggaaacctcattaaaaaaattaaagtagaagtgcaaaccaaatcttttgttcgagaaattaatgggggcgtagctcaaaatggtgatttagtaagagtagatttgtttgaaaaggataataggtattatatggtgcctatttacgtagtagatactgttcgttccgaactaccaaataaagctgtaacaagcagtaaaggctatgagcaatggttatcaatagataacagctttacgttcaaattcagtttatatccttatgatttagtacgacttgtaaaaggcgatgaagatcgttttctatactttagtactcttgatattaattcggaccgtcttaattttaaagatgtaaataagccatcaaagcaagctgaatatcgttatagtcttaaaacaattgagaatttagaaaaatatgagattggtgttttaggtgatttaaggttagtgagacaagaaacacgtaaaatttttaaa

SEQ ID NO: 188 - DNA, 3213 bp, synthetic construct
  misc_feature 1..3213: note = source = /note="Description of Artificial Sequence: Syntheticpolynucleotide"
  misc_feature 1..3213: note = source = /note="APG07513.1 E. coli optimized"
  source 1..3213: mol_type = other DNA
atgcgcgagctagattatcgcatcggcctggatattggcactaactcaataggctggggcgtgatcgaactgagctggaataaagaccgcgagcagtatgaaaagacccgcatcgtggataaaggcgtgcgcatgttcgacaaagcggaaattccgaaaaccggtgcaagtctggcggaaccaagacgtattgcacgtagtagtcgccgccgattaaaccgcaaaagtcagcgcaagaaggatatcaggaacctgctggtccagcatgaaatcatcagccagaaggaattaaccagcctgtacccgctgagcaaatcaagtatggacatctgggatataaggctggacggcctggaccgcctgctggatcgttttgaatgggcccgcctattaatccatctggcacagcgccgtggcttcaaatcaaaccgcaagagcgaattaaaggacgtggagaccggtaaagtgctgtcaagcattcaggtgaatgaaaagcgcctgagcctgtatcgcaccgtgggcgagatgtggatgaaaaacgcggactgctcaaaatatggcaaacgccgcaacagcccgaacgaatacgtgtttagcgttagccgtgcggacctggaaaaagaaatcgtgaccctgtttgaggcgcagcgcaaattccatagcagctatgcgagcgtggatctgcagaaaacatacatccagatctgggcacatcagctgccgtttgcgagcggtaacgcgatcgtgaataaagtgggctattgcagcctattaaaaggcaaagaaaaacgcgtgccgaaagcgacctatacattccagtacttcaatacactggaccaaatcaaccgcacccgcctgggcccgaacttccagccgttcaccaaagaacagcgcgatataatcctggataaaatgttccagcgcaccgactactataaaaagaaaaccatcccggaggtgacatactacgatataaggaaatggctggcgctggatgaaaccatccagttcaagggcttaacctacgatccgaacgaggagctgaaaaagatcgagatgaaaccgttcattaatctgaaaccgttctatgaaattaaaaaggtggtaaccaactacgcgaagaaaaccaacgaagtgttcagcgcgctggattacgataccgtggcgtacgcgctgaccgtgtataaaaccgacaaggatataaggagctacctgaaacgcagcaataatctgagcaaacgctgctacgacgaccaattaatcgaagaactgctgaccctgagctatactaagttcggccacctgagcttcaaagcgattaatcacgtgctgccaataatgcaggaaggccgcacctaccaggaagcaatacaccagctgggctacgatacaaccaacctgaaaaaggaaaataggagcatgttcctgccaataatcccggatgaaatcaccaacccgatcgtgaaacgcgcgctgacccaggcgcgcaaagtggtgaacgcaataatccgccgctacggctcaccgaacagcgtgcacatcgaactggcgcgcgaactgagcaaaagccacgatgaacgcaaaaagatcatgaccgcgcacgatgaaaactacaaaaagaacaaaggcgcggtgagcatcctgatcgataacggcatcctgaacccgaccggctacgatatcgtgcgctacaaactgtggaaagaacagggcgaacgctgcgcgtacagcctgaaaaagatcccggcgaacaccttcttcaacgaactgaaaaaggaacgctcaggcccgccggtgctggaagtggatcacatcctgccgtacagccagagcttcatcgatagctaccacaacaaagtgctggtgtacggcgacgaaaaccagaaaaagggcaaccgcatcccgtacaccttcttcagcgaagaagacaaagaatgggagagcttcgaaagctacgtgcgcagcaacagcttcttcagcaaaaagaaacgcggctacctgctgaaaaaggcgtacctgccgcgcgaaagcaacttaatcaaagaacgccatctgaacgatacccgctacgcgagcagctacctgaaaaacttcattgagaaaaacctgaaattcaaggaagcggtgggcatcacccgcaagaagtacgtccagaccgtgaacggcgtgatcaccgcgcatctgcgcaaacgctggggcctggaaaaagatcgccaggaaacctatctgcatcatgcgatggatgcgatcatcgtggcgtgcaccgatcatcatatggtgaccaaagtgaccgaatattatcagatcaaagaaggcaacaaatcaatcaaaaagccgtattttccgctgccgtggatgggcttccgcgaagaaatccttagccatctggaaagccagccgatcgcgcgcaaaatcagcgaagaactgaaaatcggctatcagagcccggattatatcctggtgagccgcatgccgaaacgcagcgtgaccggcagcgcgcatgatcagaccgtgatgaaaaagggcgatatcgataaaaagggcaaaaccatcatcatcaaacgcgtgcatctgaaagacatcaaattcgacgaaaacggcgacttcaaaatggtgggcaaggaacaggacttagcgacctacgaagcgatcaaacagcgctacctggaataccgcaaagagagcaaaaaggcgtttgaaaccccgctgtacaaaccgagcaaaaagggcaagggcaacctgatcaaaaagatcaaagtggaagtccagaccaaatcgtttgtgcgcgagatcaacggcggcgtggcgcagaacggcgatctggtgcgcgtggatctgtttgaaaaagataaccgctattatatggtgccgatctacgtggtggataccgtgcgcagcgaactgccgaacaaagcggtgaccagcagcaaaggctatgaacagtggttaagcatcgataacagcttcaccttcaaattcagcctgtacccgtatgatctggtgcgcctggtgaaaggcgatgaagatcgcttcctgtattttagcaccctggacatcaacagcgatcgcctgaacttcaaagacgtgaacaaaccgagcaaacaggcggaatatcgctacagcctgaagaccatcgagaacctggagaaatacgaaattggcgtgctgggcgatctgcgcctggtgcgccaggaaacccgcaaaatcttcaaa

SEQ ID NO: 189 - DNA, 3216 bp, Bacillus sp.
  misc_feature 1..3216: note = source = /note="APG08290.1 Native Seq"
  source 1..3216: mol_type = genomic DNA
atgagtgagttggattaccgcatagggttggatattggtacgaattccattggctggggtgttattgaattattttggaacaaggacagagaacgatatgaaaaagtaaggattgtcgacaagggcgttcgtatgtttgataaggctgaaatacctaataagggtgcttctcttgctgaaccgagacgtatagcgcgttcatcacgtagaaggttaaatcgcaaaagtcagaggaagaaagagatacgtaatttacttgttcaacacggaatgattacccaagaggaattggatttgttatatcctctttcaaaaaaatcaatagatatttgggatattcgtttggatggattagatcgtctgttgaatcatcttgaatgggctcgattattaattcatttagcacaaagacgtggttttaagtcgaatcgaaagtctgaattgaaagatgctgagacggggaaggtattatcgagtattcaagtaaatgaaaaacgactatttctgtaccgtacagtgggggaaatgtggataaaagatgctgagtttagtaagtatgatagaagacgtaattctcctaatgagtatgtattttcggttagtcgtgcggacttagaaaaggaaattgttactctatttgaagcacaaagaaagtttcagtcatcatacgcatcgaagaacttacaagaaacatatttacaaatttgggcacaccaacttccttttgcttctgggaatgcaattttaaacaaagtaggctattgttcattattgaaagggaaagaaaggagaattccgaaagcaacatatacttttcaatatttcagtgcactagatcaggtgaatcgaacacgattaggacctgattttcaaccatttacgcaggaacagaaagagattattttagataaaatgtttcaacgtacagattattataaaaaaaagactatacctgaagttagctactatgatatacggaaatggctagagttagatgaaactattcaatttaaaggacttaattatgatccaaacgaagaactgaaaaaaatagaaaaaaaaccatttattaatttaaaggcattctatgaaattaaaaaggtagttgcaaattatgctgagagaacaaatgaggcattttcaacgttagactatgatgcgattgcatatgctttaacagtttataaaacggacaaagatattagatcttatttgaagaaatctaataatttatcaaaacgttgctacgacgatcaattaatagaagagctatttactctctcctatacaaagtttggtcatttatcatttaaagcaattaatcatgtacttccaattatgcaagagggaaggacttatcaagaagcgatacaccaattaggatatgataccactaatcttaaaaaagaaaacagaagtatgttcttgcctcttattccagatgaaataacaaatccaattgttaaaagagcgataactcaagcacgtaaagttgtaaacgctattattagaagatatggttctccaaattctgttcatattgaactagctcgtgagctttctaaaagtcatgacgagagaaagaaaataatgacggctcatgatgaaaattataagaaaaataaaggagctatatccattttgatcgagaatggaattttaaatccgacaggatatgatattgtacgttataagttatggaaagagcaaggagaacgatgtgcttattcgttaaaggagattcctccggatacgttttttaatgaattaaaaaaagaacgaaatggttctccaattctagaggtagatcacattttaccgtatagccaaagttttattgatagttatcataataaagtattagtttacagtgatgaaaatcgaaacaagggaaatcgaattccatatacctattttttagagacaaataaggattgggaagcttttgaaaggtatgtaagatcaaataagcttttttctaaaaagaagcgtgagtatttattgaaaaaaacatatttgccaagagagagtgaactaataaaggagcgacatttaaatgatacgcgatatgctagtacctttttgaaaaacttcattgagcagaacttgcaatttaaagaagttgaagttaatctgcgtaaaaaacgtgtgcaaacagttaatggtgtaattacagcgcaccttcgaaaaagatggggattagaaaaaaatagacaggaaacatatctgcatcatgcaatggacgctatcattgttgcttgtacagaccatcatatggttactagaataacagagtattatcaaataaaagaaagtaataaatcagtaaagaaaccatattttccgatgccatgggagggttttagagatgaactcttatcacatttagcgagccagccaattgctaaaaaaattagtgaggagcttaaagctggatatcaatcatctgattatatatttgtgtctcgaatgccaaaaagatctgtcactggagcagctcatgatcaaacgattaggagaaaaggtggtattgataaaaaaggaaaaactattattataaagcgtgtgcgcttaaaggatattaagtttgatgagaatggcgattttaaaatggttggaaaagaacaagatttagcaacttatgaggcgataaagcaaagatatttggagcatagaaaaaactcgaaaaaagcatttgaaacacctctatacaagcctagtaaaaaagggacaggaaatctcatcaaaagagttaaaattgaaggacaaactaaagcttttgttcgagaagtaaatgggggagtagcccaaaatagtgatttagtaagagttgatttatttgaaaaagatgataaatattacatggtgcctatttatgtaccagataccgtttgttcagaattacccaaaaaagttgtgaaaagtggtaagggttatgagcaatggctaacactagataacagctttacgtttaaatctagtttatacccttatgatttagtacgtcttgtaaaaggtaatgaagatcgttttttatactttggtactctcgatatcgattctgaccgtcttaattttaaagatgtaaataagccatcaaaacagaatgaatatcgttatagtcttaaaacaattgagaatttagaaaaatatgaggttggtgttttaggtgatttaaggttagtgaaacaagaaacacgtagaatttttaataga

SEQ ID NO: 190 - DNA, 3216 bp, synthetic construct
  misc_feature 1..3216: note = source = /note="Description of Artificial Sequence: Syntheticpolynucleotide"
  misc_feature 1..3216: note = source = /note="APG08290.1 E. coli optimized"
  source 1..3216: mol_type = other DNA
atgagcgagctagattatcgcatcggcctggatatcggcactaactcaataggctggggcgtgatcgaactgttctggaataaagaccgcgagcgctatgaaaaggtgcgcatcgtggacaaaggcgtcaggatgttcgacaaagcggagatcccgaataaaggtgcatcactggcggaaccaagacgtatagcacgtagtagtcgccgccgattaaaccgcaaaagtcagcgcaagaaagagatccgtaacctgctggttcagcatggcatgatcacccaggaagaactggatctgctgtacccgctgagcaagaaatcaatcgacatctgggatataaggctggacggcctggaccgcctattaaaccatctggaatgggcccgcctattaatccatctggcgcagcgtagaggcttcaaatcaaaccgcaagagcgaattaaaggacgcggagaccggtaaagtgctgtcaagcattcaggtgaatgaaaagcgcctgttcctgtatcgcaccgtgggcgagatgtggattaaagacgcggagttctcaaaatacgaccgccgtcgcaacagcccgaacgaatacgtgtttagcgttagccgtgcggacctggagaaagaaatcgtgaccctgtttgaagcgcagcgcaaattccaatcaagctacgcgagcaagaacctgcaagagacctacctgcagatttgggcacatcagctgccgtttgcaagcggcaacgcgatattaaacaaagtgggctattgcagcctattaaaaggcaaagaacgccgcatcccgaaagcgacctatacattccagtacttcagcgcgctggaccaggtgaaccgtacccgtctgggccctgattttcagccgtttacccaggaacagaaagaaataatcctggataaaatgttccagcgcaccgactactataaaaagaaaaccatcccggaagtgtcatattacgatataaggaaatggctggagctggatgagaccatccagttcaagggcctgaactacgatccgaacgaggagctgaaaaaaatcgagaaaaaaccgttcattaatctgaaagcgttctatgaaattaaaaaagtggtggcgaactacgcggaacgaaccaacgaagcattcagcaccctggattacgatgcgatcgcgtacgcgttaaccgtgtataaaaccgacaaggatataaggagctacctgaaaaaatcaaacaacctgagcaaacgctgctacgacgaccaattaatcgaagaactgttcaccctgagctatactaagttcggccacctgagcttcaaagcgattaatcacgtgctgccaataatgcaggaaggccgcacctaccaggaagcgatccaccagctgggctacgataccaccaacctgaaaaaagaaaaccgcagcatgttcctgccgctgatcccggatgaaatcaccaacccgatcgtgaaacgcgcgatcacccaggcgcgcaaagtggtgaacgcgatcatccgccgctacggctcaccgaacagcgtgcacatcgagctggcgcgcgagctgagcaaaagccacgacgagcgcaaaaaaatcatgaccgcgcacgacgagaactacaagaaaaacaaaggcgcgatcagcatcctgatcgagaacggcatcctgaacccgaccggctacgatatcgtgcgctacaaactgtggaaagaacagggtgaacgctgcgcgtacagcctgaaagaaatcccgccggataccttcttcaacgaactgaaaaaagaacgcaacggctcaccgatcctggaagtggatcacatcctgccgtacagccagagcttcatcgatagctaccacaacaaagtgctggtgtacagcgatgaaaaccgcaacaaaggcaaccgcatcccgtacacctacttcctggaaaccaacaaagattgggaagcgttcgaacgctacgtgcgcagcaacaaactgttcagcaaaaagaaacgcgaatacctgctgaaaaaaacctacctgccgcgcgaaagcgaactgatcaaagaacgccacttaaacgatacccgctacgcgagcaccttcctgaaaaacttcatcgaacagaacctgcagttcaaagaagtggaggtgaacctgcgtaaaaagcgcgtccagaccgtgaacggcgtgatcaccgcgcatctgcgcaaacgctggggcctggaaaaaaaccgccaggaaacctatctgcatcatgcgatggatgcgatcatcgtggcgtgcaccgatcatcatatggtgacccgcatcaccgaatattatcagatcaaagaaagcaacaaatcagtgaaaaaaccgtattttccgatgccgtgggaaggctttcgcgatgaactgctgagccatctggcgagccagccgatcgcgaaaaaaatcagcgaagaactgaaagcgggctatcagagcagcgattatatctttgtgagccgcatgccgaaacgcagcgtgaccggcgcggcgcatgatcagaccatccgccgcaaaggcggcatcgataaaaaaggcaaaaccatcatcatcaaacgcgtgcgcctgaaagatatcaaatttgatgaaaacggcgattttaaaatggtgggcaaagaacaggacttagcgacctacgaagcgatcaaacagcgctatctggagcatcgcaagaacagcaaaaaagcgtttgagaccccgctgtacaaaccgagcaaaaaaggcaccggcaacctgatcaaacgcgtgaaaatcgagggccagaccaaagcgtttgtgcgcgaagtgaacggcggcgtggcgcagaacagcgatctggtgcgcgtggatctgtttgaaaaagatgacaaatattatatggtgccgatctatgtgccggataccgtgtgtagcgaactgccgaaaaaagtggtgaaaagcggcaaaggctatgaacagtggttaaccctggataacagcttcaccttcaagagcagcctgtacccgtatgatctggtgcgcctggtgaaaggcaacgaagatcgctttctgtattttggcaccctggacatcgatagcgatcgcctgaacttcaaagacgtgaacaaaccgagcaagcagaacgaataccgctacagcctgaagaccatcgagaacctggagaaatatgaagtgggcgtgctgggcgatctgcgcctggtgaaacaggaaacccgccgcatttttaaccgc

SEQ ID NO: 191 - DNA, 4011 bp, Enterococcus sp.
  misc_feature 1..4011: note = source = /note="APG05459.1 Native Seq"
  source 1..4011: mol_type = genomic DNA
atgaagaaagactacgttattggtctggatatagggactaattctgtcggctgggcagttatgacagaagactatcagttggtgaagaaaaaaatgcctatttatggaaacactgaaaaaaagaaaatcaagaaaaatttttggggtgtgcgtttatttgaagaagggcatacagccgaagatcgccgattaaaaagaacagcacgacgaagaattagtcgtcgacggaatcgtttacgctacttacaagctttttttgaagaagcgatgacagctttggatgaaaacttttttgctcgtttacaagagagttttttagtgcctgaagataagaagtggcacagacatccgatttttgctaagttggaagatgaagtagcttaccatgaaacgtatccgacaatctaccatttacgcaaaaaattagcagattcatctgagcaagcagatttacgactaatttatttggcgttggcacatattgtcaaatatcgtggacattttttaattgaaggaaaattaagtacagaaaatatttctgttaaagaacaatttcaacaatttatgatcatttataaccaaacctttgtgaatggagagagtcgcttagttagtgcgccattacctgaatctgtcttgattgaggaagagttgactgaaaaagcttctcgtactaaaaaatctgaaaaagtcttacaacaatttcctcaagaaaaagctaatggcttatttggtcagttcttaaagctaatggtagggaataaagctgactttaaaaaagtttttggtttggaagaagaagccaaaataacctacgctagtgaaagctatgaagaagatttagaaggcattttagcaaaggttggggatgaatatagtgacgtgtttttagctgctaaaaatgtgtacgatgcagttgaattatcaacgattttagcagattcggataaaaaaagtcacgcgaaattatcttctagcatgattgtccgttttacagaacatcaagaagatttaaaaaaattcaaacgatttattcgtgaaaattgtccagacgaatatgataatctctttaaaaatgaacagaaagacggctatgcaggctacattgcacacgcaggtaaggtttcacagcttaaattttaccagtatgttaagaaaatcattcaagatattgctggagcagaatattttttagaaaaaattgctcaagaaaactttttaagaaagcaacggacctttgataatggggtgattcctcatcaaattcatttggctgagttacaagcaatcattcatcgtcaagcggcctattatccatttttaaaagaaaatcaagaaaaaattgaacaactggttacatttcgaattccttattatgtcggaccattatcaaaaggagatgcaagtaccttcgcttggctaaaacgtcaaagtgaggaaccaattcgaccttggaaccttcaagaaaccgttgatttggaccaatcagcgacagcctttattgaacgaatgaccaattttgatacgtatttaccttctgaaaaagttttaccgaaacatagtttgttatatgaaaagtttatggtatttaatgaattgaccaagatttcttatacggatgatcgaggaatcaaagccaatttttcaggtaaagaaaaagaaaaaatctttgattatctgtttaagacgcgtcgaaaagttaagaaaaaggatatcattcaattctatcgaaacgaatataatacggagattgtcacgcttagtggacttgaagaagaccaatttaatgctagttttagcacgtatcaggatttactgaaatgtggtttaacaagagctgaattagaccaccctgataatgccgaaaaattggaagatatcataaaaattttaactatttttgaagatcggcaacgaattcggacgcaactttccacattcaaagggcagttctcagcagaagtactaaaaaaattagaacgcaagcactacactggctggggaagattgtcgaaaaaattaatcaatggtatctacgataaagaatcgggtaaaacaattttggactatttaattaaagatgatggggtctcaaaacactataatcgcaattttatgcaactgattaatgattcacaattatcttttaaaaatgctattcaaaaagcacagtccagtgaacatgaagaaacattaagtgaaactgtcaatgaattagctggtagtccagcaataaaaaaaggaatttatcaaagtttaaaaattgtcgatgaactagtcgcgattatgggttatgcgcccaagcggattgttgtcgaaatggcacgtgaaaatcaaacgactagcactggcaagagaagatccatccaacgcttgaaaatagttgaaaaagcaatggccgaaatcggcagcaatttattaaaagaacaaccaacgactaatgaacagttacgagatacccgtcttttcctttactatatgcaaaatggtaaagatatgtacacgggagatgaattatcgcttcatcgtttatctcactatgatattgatcatattatcccacaaagctttatgaaagacgattcattggataacctagttttagtgggctctactgaaaatcgagggaaatccgatgatgtacctagcaaggaagttgttaaggatatgaaagcttattgggagaaattatatgctgctggcttaattagtcaacggaaattccaacgtctgaccaagggggagcaaggtggcttgactctcgaagacaaagcgcattttatccaacgacaattagtagaaactcgtcaaattaccaaaaatgttgcagggatcttagatcaacgctacaatgctaattcaaaagagaaaaaagtccaaatcatcaccttgaaagctagtttaacgagccaatttcgttcgatttttggcttgtataaagttcgtgaagtgaatgattatcaccatggacaagatgcttatttaaactgtgtggtcgcaaccacgttattaaaagtttatcctaatttagcaccagaatttgtttacggagaatatcctaaattccaggcctttaaagaaaataaagccacggcgaagactataatttatacaaatttgatgcgctttttcacggaagatgaaccacggttcatgaaggatggcgaaattctttggagtaacagttatttaaaaaatatcaaaaaagaattaaattaccatcaaatgaatattgtcaaaaaagtagaagtgcaaaaaggcggtttttcaaaagagtcgattaaacccaaaggaccatcgaataaattgattcctgtcaaaaatggtttggatccccaaaaatatggcggttttgatagtcctgtagttgcttatacagtgttattcacgcatgaaaaaggtaaaaaacctcttattaaacaggagatactgggcattacgattatggaaaaaacaaggtttgaacaaaatcctattctttttttagaggagaaaggcttcctacggcctcgtgtattaatgaaattgcctaagtatacactgtatgaatttccagaggggcgcaggcgcttattagccagcgctaaagaagcgcaaaaagggaaccagatggttttacctgaacatttacttacgttactgtaccatgcgaaacaatgtttgttaccaaatcaatcagaaagtttggcttatgtagaacaacatcaaccagaatttcaagagattttagagagagtggttgactttgctgaagtgcatacattagccaagtcaaaagtccagcaaattgtgaaactttttgaagcaaatcaaacagcagatgtgaaagagattgcggcatcctttatccaacttatgcagtttaatgcgatgggcgcaccaagtacgtttaaatttttccaaaaagacattgagcgagcacgctacacgtcaatcaaagaaatttttgatgccactatcatttaccaatcgactacgggactgtatgaaacacgcagaaaggttgtcgac

SEQ ID NO: 192 - DNA, 4011 bp, synthetic construct
  misc_feature 1..4011: note = source = /note="Description of Artificial Sequence: Syntheticpolynucleotide"
  misc_feature 1..4011: note = source = /note="APG05459.1 E. coli optimized"
  source 1..4011: mol_type = other DNA
atgaaaaaggactacgtgatcggcctagacatcggcactaacagcgttggttgggcggtgatgaccgaagattaccagctagtgaagaagaagatgcctatctacggtaatacagagaagaagaagattaaaaagaacttctggggcgtgaggctattcgaggagggtcacaccgcggaggaccgccgcctgaagcgcaccgctagacgccgtatttcacgtcgtcgtaaccgtctgcgttacctgcaagcattcttcgaagaagcaatgaccgcgctggatgaaaacttcttcgctaggctgcaggagtcatttctggtgccggaggataaaaagtggcaccgtcatccgatcttcgcgaaactagaagacgaggtggcgtaccatgaaacctacccgactatctaccacctgcgcaaaaagctggcggatagcagcgaacaagcagacctgcgattaatctatctggcgctggcgcacatcgtaaaatacagaggccacttcctcatcgagggcaaattatcgaccgaaaatattagcgtgaaggagcagttccagcagttcatgatcatctacaaccaaaccttcgtgaacggcgaatcaaggctggtgagcgcgccgctgccggagagcgtattaattgaggaggaattaaccgagaaagcgagccgcactaagaaaagcgagaaagtgcttcagcagttcccgcaagaaaaagcgaacggcctgttcggccagttcctgaaattaatggtgggcaataaagcggacttcaaaaaggtgttcggcctggaagaggaggcgaaaataacctacgcgagcgaaagctacgaggaagacctggagggcatactagcgaaagtgggcgacgaatacagtgacgtgttcctggcggctaaaaacgtgtacgacgcggtggaattaagcaccatactagcggacagcgataaaaagagtcacgcgaaattaagctcaagcatgatcgtgcgcttcaccgaacaccaggaagacctgaaaaagttcaaacgcttcatccgcgaaaactgcccggacgaatacgataacctgttcaaaaacgaacagaaagatggctacgcgggatacatcgcgcacgcgggcaaagtgtcacaattaaagttctaccagtacgtgaagaaaataatccaggatatcgcgggcgcggaatacttcctggagaaaatagcgcaggagaacttccttaggaaacagcgcaccttcgacaacggcgtgatcccgcaccaaatacacctggcggaactacaggcaataattcaccgccaggcggcatactacccgttcctgaaagagaaccaggagaaaatagaacagctggtgaccttccgcatcccatactacgtgggcccgcttagcaaaggcgatgcgagcaccttcgcgtggctgaaacgccagagcgaagaaccaatccgcccgtggaacttacaagaaaccgtggatctggatcagagcgcgaccgcgttcatcgaacgcatgaccaacttcgatacatacctgccgagcgaaaaagtgctgccgaagcatagcctgctgtatgaaaaattcatggtgttcaacgaactgaccaaaataagctacaccgatgatcgcggcattaaagcgaacttcagcggcaaagaaaaagagaaaatattcgattacctattcaaaacccgccgcaaagtgaaaaagaaagacataatacagttctaccgcaacgaatacaacaccgaaatcgtgaccctgagcggcctggaagaagatcagttcaacgcgagcttcagcacctaccaggacttattaaaatgcggcctgacccgcgcggagcttgaccacccggacaacgcggaaaaactggaagatatcattaaaatactgaccatcttcgaagatcgccagcgcatccgcacccagctgagcaccttcaagggccagttcagcgcggaagtgctgaaaaagctggaacgcaaacattacaccggctggggccgcctgagcaaaaagctgatcaacggcatctacgataaagaatcaggcaaaaccatcctggactacctgatcaaagatgacggcgtgagcaaacactacaaccgcaacttcatgcagctgatcaacgatagccagctgagcttcaagaacgcgatccagaaagcgcagagcagcgaacatgaagaaaccctgagcgaaaccgtgaacgaactggcgggcagcccggcgatcaaaaagggcatctatcagagcctgaaaatcgtggatgaattagtggcgatcatgggctatgcgccgaaacgcatcgtggtggaaatggcgcgcgaaaaccagaccaccagcaccggcaaacgccgcagcatccagcgcctgaaaatcgtggaaaaagcgatggcggaaatcggcagcaacctgctgaaagaacagccgaccaccaacgaacagctgcgcgatacccgcctgtttctgtattatatgcagaacggcaaagatatgtataccggcgatgaactgtcactgcatcgcctcagccattatgatatcgatcatatcatcccgcagagctttatgaaagatgatagcctggataacctggtgctggtgggcagcaccgaaaaccgcggcaaaagcgatgatgtgccgagcaaagaagtggtgaaagatatgaaagcgtattgggaaaaactgtatgcggcgggcctgatcagccagcgcaaatttcagcgcctgaccaaaggcgaacagggcggcctgaccttagaagataaagcgcattttatccagcgccagctggtggaaacccgccagatcaccaaaaacgtggcgggcatcctggatcagcgctataacgcgaacagcaaagaaaagaaagtccagatcatcaccctgaaagcgagcctgaccagccagtttcgcagcatctttggcctgtataaagtgcgcgaagtgaacgattatcatcatggccaggatgcgtatctgaactgcgtggtggcgaccaccttactgaaagtgtatccgaacctggcgccggaatttgtgtatggcgaatatccgaaatttcaggcgtttaaagaaaacaaagcgaccgcgaaaaccatcatctataccaacctgatgcgcttctttaccgaagatgaaccgcgctttatgaaagatggcgaaattctgtggagcaacagctatctgaaaaacatcaaaaaggaactgaactaccaccagatgaacatcgtgaaaaaggtggaggtccagaaaggcggcttctcaaaggaaagcatcaaaccgaaaggcccgagcaacaaactgatcccggtgaaaaacggcctggacccgcagaaatatggcggctttgatagcccggtggtggcgtataccgtgctgtttacccatgaaaaaggcaaaaagccgctgatcaaacaggaaattctgggcatcaccatcatggagaaaacccgctttgaacagaacccgatcctgttcctggaagaaaaaggctttctgcgcccgcgcgtgctgatgaaactgccgaaatataccctctatgaatttccggaaggccgccgccgcctgctggcgagcgcgaaagaagcgcagaaaggcaaccagatggtgttaccggaacatctgctgaccctgctgtatcatgcgaaacagtgcctgctgccgaaccagagcgaaagcctggcgtatgtggaacagcatcagccggaatttcaggaaattctggaacgcgtggtggattttgcggaagtgcataccctggcgaaaagcaaagttcagcagattgttaaactgtttgaagcgaaccagaccgcggatgtgaaagaaattgcggcgagctttattcagctgatgcagtttaacgcgatgggcgccccgagcaccttcaaattctttcagaaagatattgaacgcgcgcgctataccagcattaaagaaatttttgatgcgaccattatctatcagtcaaccaccggcctgtatgaaacccgccgcaaagtggtggat

SEQ ID NO: 193 - DNA, 4308 bp, Enterococcus sp.
  misc_feature 1..4308: note = source = /note="APG04583.1 Native Seq"
  source 1..4308: mol_type = genomic DNA
atggctaaaaatatacttggattagatttgggaaccaatagtattggttgggcgttggtacagcaagactttgaaaacaaagaaggaaatattcttggaatgggaagtaggattattccgatgtcgcaagatattttaggagaattcggtaaggggaattctatttctcaaactgctgaacgtactggttatcgtggtgtccgtcggttaagagaacgacatttattacgtcgtgagcgtttgcaccgagttttgcatttgttgggtttcttgccaaaacattatgatgaaaaaatagattttacacaacgttttgggaaattcattaaccaagccgaacctaaattggcttttgatagtgaatttctttttaaagattctttccatgaaatgttagctgattttaaacaaaatcaaccagagtttttgaaagataaaaatggagaagattgtttagttccttatgattggacgatttattatttacgtaaaaaagcattaacgcaaaaaattgagaaatatgaattagcttggttgattcttaattttaatcaaaaacgtggttattatcaattaagaggtgaagaagagaaagaaaatccaaataaattggtgggatttcattctttgaaaatcgttgatgttattcccgatgctgaaacaaataaaaaaggagagacttggtattctttgcatttagaaaatggttgggtatatcgccgttcttctaaaatttcattagcggattggaaagataaagttcgagattttattgttacgactgatttaaacgatgatggttctgaaaaattggataaagatggaattgtgaaacgtagctttcgtgcaccaagtgcggatgattggactttgttgaaaaagaaaacagaaaaagatattgataactctaacaaaactgttggaacttatatttacgacaatcttttattgaacccaaaacaaaaaataaaaggaaaaatggttcgtaccatcgaacgtaagttttacaagcaagaattagaacaaattttaaaaactcaaaaagaatttcattcagaattacaaagtgaaaatttgctacaagattgtgttcgagaattgtatcgaaataatgaacaacatcaacaaatgttagaagctaaagattttgtgcatttgttcctaaatgatattattttctatcaacgtcctttgagaagtcaaaaatccagtatatcgaattgtactttggaatttagaaaatcgaaaaatgaaaatggtgaagaagttattcatcgtttaaaagtaattgcaaaatcgaatccatattatcaggaatttagattgttacaatgggtgcaaaatttagcaatttatacaaaagatgatgataaaaatgtaacaaacgaatttctaaagtctactcaagattgggaggatttattgagatggctacattctaaaaaagaaattaaacaggatgctttaattaagtttttgattgaaaagaaaggtttaaaaggcaaagctttaactattgaagtagcaaaatatcgttggaattatgttcaggacaaagattaccctggtaatgaaacccgatatttaattcaatctcgtttggataaagttgaatatgcacctaaggattttttaacttatgaaaatgaaatggctttgtggcacatcatttattcgataaacgataaaattgagtacgaaaaagccttaaaatcttttgccaacaaaaaaggtttggacgaagtaacttttgttgaagcgtttaagaaattcccgccttttaaaagtgattacggaagtttttctgaaaaagcaatcaagaaattattgcctttgatgcgttttggaactcaatggaattgggataatatcgatcaaaattctaaagaaagaattggaaaaatattgacaggcgaatatgatgaaaacatcaaaggtcgtgttcgcgaaaaagcaagacatctcaattctgaaaccgattttcaagctttacctttgtggttggcgcaatacgtagtttacggaagacattctgaagctgatattgcaggtaaatggaattcggtggatgatttaaagcaatttttagatgactttaaacaacattcgcttcgtaatcctattgtagagcaagtgattactgaaacgttgcgtgcggtaaaagatatttggaatttttatggaaaaggtgctaaagatttcttctctgaaattcatatcgagctggggcgtgaaatgaaaaatacggctgatgaacgcaagcgtattactacaatggttacggataacgaaaacaccaatttgcgtatcaaagctttgttggctgaaatggctttggatcaaaatgtagataatgttcgtccatattctccaatgcaacaagaaattttgaaaatctatgaagaaggtgttttgaatgctgaagaaaatatcgatgatgatattctgaaaattagtaaaacggctcaaccttctgctacagatttaaagcgttacaaattgtggttagaacaaaaatatcgttcgccttatacaggtcaaatgattcctttgaataagctgtttacacctgaatatgagattgaacacataattccgcaaagtcgctattttgatgatagtatgagcaataaagtgatttgcgaagcagcggtgaataaacttaaagacaatcaaattggtttggttttcattaagaatcatcacggagaagttgtggatttcggaatgggaaaacaagtgaagattttggaagtttccgattatgaggattttgtaaaacaaaattacaataaaaacagaggaaaacgtaataagttgttattggaagatattcctgagaaaatgattgaacgtcaactaaatgatacacgttacatcagcaaatatattacgcaagtgttatcgaatattgttcgtgatgataaagaaggtagtaaagatgatggtgtaaattctaaaaatattgttcctggaaacggaaaaattaccacaagacttaaacaagattggggattgaatgacgtttggaatgatttggttttacctcgttttgaacgaatgaatacattgactaattcaaatgattttacatcaaaaaatacacatggaaaaacaattccaacagttccaattgagttatccaaaggtttttctaaaaaacgtatcgatcatcgtcatcacgcaatggatgcgttggtaattgcctgtgcaacgagagatcacgtgaatttgttgaataacgaaagttcaaaatcggatacaaaacgttatgatttgaataggaaattaagaaaatacgagaaagtagcttacaatgatcccaaaacaggcgaacgaattgagaaagaagttccaaaagacttcattaaaccttgggagacctttaccgaagatacgcgaactttgttagaaaatattgtaattagtttcaagcaaaatctacgagttatcaataaagcaaccaattattatgaaaaaattgagaatgggaaaaaagtaaaagttgaacaaaagggaataaattgggctgtaagaaaagctttgcataaagaaaccgtttctggacaagtgcatttggatagaataaaagttgcaaaaggtaaaatattaacggctactcgtaaaactttggatgcctcttttaatgaaaaaacaattgagtcaattacggatacagggattcaaaagattttattgaattatttaaaatcaaaagataacaatccagaggttgcattttcaccagaaggaatagaagaattaaataaaaatattaggctatataatgatggaaaagcacatcaaccaattttgaaagttcgtgtttttgagcaaggaagcaaatttactttaggtgagacgggaaataaaaccactaagtttgtagaagcagcaaagggtactaatctatttttcggaatttatgaagacaaatcaggtaagagaagctacgaaaccattccattaaatattgtcatcgaaagacaaaaacaaggtctgcaagctgttcccgaaaccaatgagaaagggaaacaattgttgtttacgttatctccaaatgatttggtttacgttcctgaagaaggagtttttgatgagaataatatcaaggtagataggatttataaggtagtgagtttttctacctatcaatgtttttttgtaagaaatgatgtttctacttctgtagttaataaggttgaatattccgctttaaataaaatggaaaaatctattgacaacataatgataaaagaaaactgcgtcaaactgaatgtagaccgtttaggaaagatttcaaaagct

SEQ ID NO: 194 - DNA, 4308 bp, synthetic construct
  misc_feature 1..4308: note = source = /note="Description of Artificial Sequence: Syntheticpolynucleotide"
  misc_feature 1..4308: note = source = /note="APG04583.1 E. coli optimized"
  source 1..4308: mol_type = other DNA
atggcgaagaacatactaggcctggatctcggaaccaacagcattggttgggcactggtccagcaggacttcgagaataaagagggcaacatactaggcatgggcagccgaataatccctatgagtcaggacatactaggcgagttcggcaagggcaacagcattagccagaccgcagaacgtactggttatcgtggtgtgcgccgtttacgtgaacgtcatctgttacgtcgtgaacgtctgcatcgtgttctgcatctgttaggcttcctgccgaagcattacgatgaaaagatcgacttcacccagcgcttcggcaagttcattaatcaagcggaaccaaagctggcgttcgacagcgagttcctgttcaaggacagcttccatgaaatgctagcggacttcaagcagaatcaaccggagttcctgaaggataaaaacggcgaggactgcctggtgccgtacgactggaccatatactacctgcgcaagaaagcactgacccagaagatcgaaaaatacgagctagcgtggctcatcctgaacttcaatcaaaagcgcggatactaccagcttaggggcgaggaggagaaagagaacccgaataaactggtgggcttccacagcctgaaaatagtggacgtgatcccggacgcggaaaccaataaaaagggcgagacctggtactcactgcatctggaaaacggctgggtgtaccgccgcagcagcaaaataagcctggcggactggaaagacaaagtgcgcgacttcatcgtgaccaccgacctgaacgatgacggcagcgaaaaactggacaaagacggcatcgtgaaacgcagctttcgtgcaccgagcgcagatgattggaccctattaaagaaaaagaccgaaaaagacatcgacaacagcaataaaaccgtgggcacctacatctacgacaacctgttattaaacccgaagcagaaaatcaaaggcaaaatggtgcgcaccatcgaacgcaaattctacaaacaggagctggagcagatcctgaaaacccagaaggaattccacagcgaactgcagagcgaaaacctgctgcaggattgcgtgcgcgaactgtaccgcaataatgaacagcaccagcagatgctggaagcgaaagatttcgtgcacctgttcctgaacgatataatcttctaccagcgcccgctgcgcagccagaaatcaagcatcagcaattgcaccctggaattccgcaaaagcaagaatgaaaacggcgaagaagtgatccaccgcctgaaagtgatcgcgaaaagcaacccatactaccaggaattccgcctgctgcagtgggtccagaacctggcgatctatactaaagacgacgacaagaacgtaaccaacgagttcctgaaatcaacccaggactgggaagatctgctgcgctggctgcatagcaagaaggagattaaacaggacgcgctgatcaagttcctgatcgagaaaaagggcctgaagggcaaagcattgaccatcgaggtggcaaaataccgctggaactacgtccaggacaaagattacccgggcaatgaaacccgctacctgatccaatcaaggctggacaaagtggaatacgcgccgaaagatttcctgacctacgagaatgaaatggcgctgtggcacatcatctacagcattaatgataaaatcgaatatgaaaaagcattaaaatcgttcgcgaataaaaagggcctggatgaagtgaccttcgtggaagcattcaaaaagttcccgccgttcaaaagcgattacggcagcttcagcgaaaaagcgattaaaaagctgctgccattaatgcgcttcggcacccagtggaactgggataacatcgatcaaaatagcaaagaacgcatcggcaaaatactaaccggcgaatacgatgaaaatattaaaggccgcgtgcgcgaaaaagcgcgccatctgaacagcgaaaccgatttccaagcattgccgctgtggctggcgcagtacgtggtgtacggccgccatagcgaagcggatatcgcgggcaaatggaacagcgtggatgatctgaaacagttcctggatgatttcaaacagcatagcctgcgcaacccgatcgtggaacaggtgatcaccgaaaccctgcgcgcggtgaaagatatctggaacttctatggcaaaggcgcgaaagatttcttcagcgaaatacacatcgaactgggccgcgaaatgaaaaataccgcggatgaaagaaaacgcatcaccaccatggtgaccgataatgaaaataccaacttacgcattaaagcattgctggcggaaatggcgctggatcagaacgtggataacgtgcgcccgtatagcccgatgcagcaggaaatcctgaaaatatatgaagaaggcgtattaaacgcggaagaaaatatcgacgatgatatcctgaaaataagcaaaaccgcgcaaccaagcgcgaccgatctgaaacgctataaactgtggctggaacagaaatatcgcagcccgtataccggccagatgatcccgctgaacaaactgtttaccccggaatatgaaatcgaacatatcatcccgcagagccgctattttgatgatagcatgagcaacaaagtgatctgcgaagcggcggtgaacaaactgaaagataaccagatcggcctggtgtttatcaaaaaccatcatggcgaagtggtggattttggcatgggcaaacaggtgaaaatcctggaagtgagcgattatgaagattttgtgaaacagaactataacaaaaaccgcggcaaacgcaacaaattactgctggaagatatcccggagaaaatgatcgaacgccagctgaacgatacccgctatatcagcaaatatatcacccaggtgctgagcaacatcgtgcgcgatgataaagaaggcagcaaagatgatggcgtgaacagcaaaaacatcgtgccgggcaacggcaaaatcaccacccgcctgaaacaggattggggcctgaacgatgtgtggaacgatctggtgctgccgcgctttgaacgcatgaacaccctgaccaacagcaacgattttaccagcaaaaacacccatggcaaaaccattccgaccgtgccgattgaactgagcaaaggctttagcaaaaagcgcattgatcatcgccatcatgcgatggatgcgctggtgattgcgtgcgcgacccgcgatcatgtgaacttactgaacaacgaaagcagcaaaagcgataccaaacgctatgatctgaaccgcaaactgcgcaaatatgaaaaagtggcgtataacgatccgaaaaccggcgaacgcattgaaaaagaagtgccgaaagattttattaaaccgtgggaaacctttaccgaagatacccgcaccctgctggaaaacattgtgattagctttaaacagaacctgcgcgtgattaacaaagcgaccaactattatgagaaaattgaaaacggcaaaaaggtgaaagtggaacagaaaggcattaactgggcggtgcgcaaagcgctgcataaagaaaccgtgagcggccaggtgcatctggatcgcattaaagtggcgaaaggcaaaattctgaccgcgacccgcaaaaccctggatgcgtcattcaacgagaaaaccattgaaagcattaccgataccggcattcagaaaattctgctgaactatctgaaaagcaaagataacaacccggaagtggcgtttagcccggaaggcattgaagaactgaacaaaaacattcgcctgtataacgatggcaaagcgcatcagccgattctgaaagtgcgcgtgtttgaacagggcagcaaattcaccctgggcgaaaccggcaacaaaaccaccaaatttgtggaagcggcgaaaggcaccaacctgttctttggcatctatgaagataaaagcggcaaacgcagctatgaaaccattccgctgaacattgtgattgaacgccagaaacagggcctgcaagcggtgccggaaaccaacgaaaaaggcaaacagctgctgtttaccctgtcaccgaacgatctggtgtatgtgccggaagaaggcgtgtttgatgaaaacaacattaaagtggatcgcatctataaagtggtgagctttagcacctatcagtgcttctttgtgcgcaacgatgtgagcaccagcgtggtgaacaaagtggaatatagcgcgctgaacaaaatggaaaaatcgattgataacattatgattaaagaaaactgcgtgaaactgaacgtggatcgcctgggcaaaattagcaaagcg

SEQ ID NO: 195 - DNA, 4368 bp, Empedobacter sp.
  misc_feature 1..4368: note = source = /note="APG01688.1 Native Seq"
  source 1..4368: mol_type = genomic DNA
atgatgattaaaaatatacttggattagatttggggactaactctattgggtgggcattgataaaacaagattttgaaaataagcatggcgaaattcttggaatgggtagccggattattccgatgtcacaggatattctgggcgattttgggaaaggaaattctatttcgcaaaccgctgatcgtaccaaatacagaagcgtgagaagattacgtgaacgatttttattgaggagagaacgactacacagagttttacatcttttaaattttcttccacagcattatgcttcacaaattgattttgaaaaaaaattcgggaagtttaaatctgaaactgaacccaaattggcatgggaaaattggggtggaaagttttcattccttttccaaaactctttcaatgaaatgcttgaagattttaaagcagctggacagggtttaaaaattccttacgactggacaatttattatctccgtaaaaaagcactttcacaaaaaattgaaaaggaggaactggcctggattcttttaaactttaatcagaaacgaggatattatcaattgcgtggtgaggaagaagaagagaatcctaataagctggttgaattttattctttaaaaattgtagatgttgtagcagatgaacctcaaaaaggaaaatctgatatttggtattctttgattttagagaatggatgggtttacagacgagcaagcaaaatacccctatttgactggaaagataaaacaagagattttattgtaacaactgatttgaatgatgacagaagtgttaaaacagacaaagaaggaaatgaaaaaagaagtttcagagcaccaagcgaaaacgattggacattggtaaaaaagaaaaccgaacaggaaatcgaccaatctcacaaaaccgttggaacctatatctacgaaacacttcttctaaatccgaaacaaaaaattaaaggaaaattggttcggacgattgaaagaaaattctataaagatgagctaaaacaaattttagaaaaacaaaaggaatttcatcaggaacttaaaaatgatgatttgtataatgattgcattcgtgagttgtacagaaacaacgaagcacatcagctgactttgagcaagaaagattttgttcatcttttgatggatgatcttattttctaccaaagacctttgagaagccagaaatcatctatttccaactgtacgttagagtttagaaaatataaagatgaaaatggaatagagcatacacaatatttaaaagccattccaaaatccaatccgtattatcaggaatttcgtctttggcaatggatgtataatctgaatatttacagaaaggacgatgaagcgaatgttaccaaagaatttttaaatacgaacaaagattttgaaagtctgtttgaatttttaaataatagaaaagaaattgagcaaaagccattgattaaatttcttttggaacaaaaagatatcaataaaaaattgcttaacgctgaagcagaaaaatatcgctggaactatgtagaagacaagaaatatccttgcaatgaaaccaaaacgatgatttcttctcgtttggataaagtcgaaaacatttctgatgatttcctgacaagggacattgagcagaaaatttggcacatcatctattccgtcaatgataaaatagaatatgaaaaagctttgaaatcttttgcaactagaaacgatttggatgaaaactcttttatcgaagcgtttaagaaattctcgccttttaaaagtgaatatggttctttttcggaaaaagcaattaaaaagttactgcctttaatgcgattgggtaaatattggtatgaagatgaaattgtaaagcatagtgatatttatttcaaaaatattgagaatcttttgggtgatttttcaaatagagacaaaaaaatttctgaagaagacaaagagaaatggaataaatctataaatctaaagttacaggaagagttaaaagattttcaaacagctgaaatagatttatttcaaggattacgattgcatattgctcaataccttgtttatggaagacattcagaagcttcaatgattggaaaatggaattccgccgaagatttagaagaatttttaaaggattttaaacagcattcgcttcgcaacccgattgtagaacaagtgattacagaaactttgcgtgttgtaaaagatatttggttgaaatacggaaatggagcaaaggatttcttcaatgaaattcatattgagttaggaagagaaatgaaacttcccgcagatgatcgaaaaaaactaacgaaccagatttctgaaaacgaaaataccaatttccgcatcaaagctctattggctgaaatgatgaatgacagttcggtagaaaatgtccgtccgttttcgccgatgcagcaagaaattttaaaaatttatgaagacgatgttttaaaatcagatatagaaattgaagatgatattctgaaaatcagcaaaaccgctcaaccttctccttccgatttgaaacgatataaactttggttggaacagaaatacaaatcgccttacacggggcaaattattcctttgaataaattgtttacaccagaatacgaaattgagcacattattccgcagagccgatattttgatgacagttttagcaataaagtaatttgtgagtctgcggttaataaattgaaagataactacatcggacttgaatttattaagcagttcggaggaacgattattgaacttggttttggtaaaagcataaaagtttttgaaacaaaagaatacgaagatttcgtcaaaaaacattacgccaacaatcaaggtaaaagaaacaaacttttgatggaagatattccagagaaaatgattgaacgtcaaatgaacgatacacgatatatcagcaaatatatttcgggcgttttgtctaatattgttcgggtagaagatggttcagatgaaggggtaaattctaaaaatattgttcccggaaacggaaaaatcaccacacagctgaaacaagattggggattgaatgatgtttggaatgatttgattttaccacgctttgaaagaatgaaccaactcaccaattcaaaagtttttactgcctggaatgagaattatcaaaagtttttaccaactgttcctattgaatattccaaagggttttcaaagaaaagaatagaccaccgccatcacgctttagatgctttggtgattgcctgtgctacaaaagatcacgtgaatttattaaataatcaatcggcaaaatcggataccaaacgatacgatttgaaaaagaaatcgatgaagtttgaaaaagtagtttacaatgatgccaaaacaggagagaaaatcgaaagggaagtgccaaaacaatttttaaaaccttgggaaaattttacgctagatgttaaacataatttggaaactattattgtaagttttaagcaaaatcttcgtgttattaataaagcgactaattattacgaaaagtatgttgagaaagacggtacaaaaaataaggaaagagtagagcagaccggaacaaactgggcgattaggaaaccaatgcataaagacacggtttccggtaaagtagatttaccttgggtaaaagtcccaaaagggaaaattttaacagcaacaaggaaaagccttgatagttcgtttgacttaaagtcaataggctctattacggatacaggaattcagaaaatactcaaaaattatttagcatttaaagacggaaatcctgaactggctttttcaccagaaggaattgacgatttgaataaaaatattgaaaaatacaatgatggaaaaccgcatcaacccatcaataaagtaagggtttttgaattgggaagtaaatttcaggtaggacaaagtggaaataaaaaagataaatatgtagaagctgcaaaaggaactaatctattctttgctgtttatgaagatgaaaaaggaaagagaaattatgaaaccattcctttgaatgaagtgattgaaaggcaaaagcaaggtttatctgtggttgatttaaaaggtacaaatgatttctacttatgtccgaatgattttgtatatattccatcaggcgacgaacttgaaaatataaataatgttgattttaaagacattaaaaaagagataaacgaaagaatttacaaagtagtaagttttacaggtaatagactttcctgtattccatatatggttgcaacaacgattgttaataaattagagtttacgcaacttaataaaattgaattcacaaaagaaaaagaaatttgtataaaactaaatgtcgatcgtttaggtaacatttcaaaagcg

SEQ ID NO: 196 - DNA, 4368 bp, synthetic construct
  misc_feature 1..4368: note = source = /note="Description of Artificial Sequence: Syntheticpolynucleotide"
  misc_feature 1..4368: note = source = /note="APG01688.1 E. coli optimized"
  source 1..4368: mol_type = other DNA
atgatgattaaaaatatcctaggcctggacctgggaaccaacagcatcggctgggcgctgattaaacaggacttcgaaaataagcatggcgagatactaggcatgggcagccgaataatcccgatgagtcaggacatactaggcgacttcggcaagggcaacagcatcagccagaccgcggaccgcacaaaatatcgcagcgtgcgtagactgcgcgaacgctttctgttacgtcgtgaacgtctgcatcgtgttcttcacctattaaacttcctgccgcagcattacgctagccagatcgacttcgagaagaagttcggcaagttcaagagcgagaccgaaccaaaactggcgtgggaaaactggggcggcaaattcagcttcctattccaaaatagcttcaacgagatgctagaggacttcaaggcggcgggtcagggattaaaaataccgtacgactggaccatatactacctgcgcaagaaagcgctgagccagaagatcgagaaggaggagctggcgtggatactactgaactttaatcaaaagcgcggatactaccagctgcgcggcgaggaggaggaggagaacccgaataaactggtggagttctacagcctgaaaatagtggacgtggtggcggacgagccgcagaaaggcaaaagcgacatctggtactcactcatactagaaaacggctgggtgtatcgccgcgcgagcaaaataccgctgttcgactggaaagataaaacccgcgacttcatcgtgaccaccgacctgaacgacgaccgcagcgtgaaaaccgacaaagaaggcaatgaaaaacgcagctttcgcgcgccgagcgaaaacgattggaccctggtgaaaaagaaaaccgaacaggaaatcgatcagagccataaaaccgtgggcacatatatctatgaaaccctgttattaaacccgaagcagaagattaaaggcaaactggtgcgcaccatcgaacgcaaattctacaaagacgaattaaaacagatactagaaaaacagaaagaattccaccaggaattaaagaacgacgacttatataacgattgcatccgcgaactgtaccgcaataatgaagcgcaccaattaaccctgagcaaaaaggatttcgtgcacttattaatggatgatctgatcttctaccagcgcccgctgcgcagccagaaatcaagcatcagcaattgcaccctggaattccgcaaatacaaagatgaaaacggcatcgaacacacccagtacctgaaagcgatcccgaaatcaaacccatactaccaggaattccgcctgtggcagtggatgtacaacctgaacatctaccgcaaagatgatgaagcgaacgtaaccaaagaattcctgaacaccaataaagatttcgaaagcctgttcgaattcctgaataatcgcaaagaaatcgaacagaaaccattaatcaaattcctgctggaacagaaagatattaataaaaagttattaaacgcggaagcggaaaaatacagatggaactacgtggaagataaaaagtacccgtgcaatgaaaccaaaaccatgatcagcagccgcctggataaagtggaaaatatcagcgatgatttcctgacccgcgatatcgaacagaaaatatggcatataatctacagcgtgaacgataaaatcgaatatgaaaaagcattaaaatcgttcgcgacccgcaacgatctggatgaaaatagcttcatcgaagcattcaaaaagttcagcccgttcaaaagcgaatacggcagcttcagcgaaaaagcgattaaaaagctgctgccattaatgcgcctgggaaaatactggtacgaagatgaaatcgtgaaacacagcgatatctacttcaaaaacatcgaaaacctgctgggcgatttcagcaaccgcgataaaaagatcagcgaagaagataaagaaaaatggaacaaaagcatcaacctgaaactgcaggaagaactgaaagatttccagaccgcggaaatcgatctgttccagggcctgcgcctgcatatcgcgcagtacctggtgtacggccgccatagcgaagcgagcatgatcggcaaatggaactcagcggaagatctggaagaattcctgaaagatttcaaacagcatagcctgcgcaacccgatcgtggaacaggtgatcaccgaaaccctgcgcgtggtgaaagatatctggctgaaatatggcaacggcgcgaaagatttctttaacgaaattcatatcgaactgggccgcgaaatgaaactgccggcggatgatcgcaaaaagctgaccaaccagatcagcgaaaacgaaaacaccaactttcgcatcaaagcgctgctggcggaaatgatgaacgatagcagcgtggaaaacgtgcgcccgtttagcccgatgcagcaggaaatcctgaaaatctatgaagatgatgtgctgaaaagcgatatcgaaatcgaagatgatatcttaaaaatcagcaaaaccgcgcagccgagcccgagcgatctgaaacgctataaactgtggctggaacagaaatataaaagcccgtataccggccagatcatcccgctgaacaaactgtttaccccggaatatgaaatcgaacatatcatcccgcagagccgctattttgatgatagctttagcaacaaagtgatctgcgaaagcgcggtgaacaaactgaaagataactatatcggcctggaattcatcaaacagtttggcggcaccatcatcgaactgggctttggcaaaagcatcaaagtgtttgaaaccaaagaatatgaagattttgtgaaaaagcattatgcgaacaaccagggcaaacgcaacaaactgttaatggaagatatcccggagaaaatgatcgaacgccagatgaacgatacccgctatatcagcaaatatatcagcggcgtgctgagcaacatcgtgcgcgtggaagatggcagcgatgaaggcgtgaacagcaaaaacatcgtgccgggcaacggcaaaatcaccacccagctgaaacaggattggggcctgaacgatgtgtggaacgatctgatcctgccgcgctttgaacgcatgaaccagctgaccaacagcaaagtgtttaccgcgtggaacgaaaactatcagaaatttctgccgaccgtgccgattgaatatagcaaaggctttagcaaaaagcgcattgatcatcgccatcatgcgctggatgcgttagtgattgcgtgcgcgaccaaagatcatgtgaacctgctgaacaaccagagcgcgaaaagcgataccaaacgctatgatctgaaaaagaaaagcatgaaatttgaaaaagtggtgtataacgatgcgaaaaccggcgagaaaattgaacgcgaagtgccgaaacagtttctgaaaccgtgggaaaactttaccctggatgtgaaacataacctggaaaccattattgtgagctttaaacagaacctgcgcgtgattaacaaagcgaccaactattatgaaaaatatgtggaaaaagatggcaccaaaaacaaagaacgcgtggaacagaccggcaccaactgggcgattcgcaaaccgatgcataaagataccgtgtcaggcaaagtggatctgccgtgggtgaaagtgccgaaaggcaaaattctgaccgcgacccgcaaaagcctggatagcagctttgatctgaaaagcattggcagcattaccgataccggcattcagaaaattctgaaaaactatctggcgtttaaagatggcaacccggaactggcgtttagcccggaaggcattgatgatctgaacaaaaacattgaaaaatataacgatggcaaaccgcatcagccgattaacaaagtgcgcgtgtttgaactgggcagcaaatttcaggtgggccagagcggcaacaaaaaggacaaatatgtggaagcggcgaaaggcaccaacctgttctttgcggtgtatgaagatgaaaaaggcaaacgcaactatgaaaccatcccgttaaacgaagtgattgaacgccagaaacagggcctgagcgtggtggatctgaaaggcaccaacgatttttatctgtgcccgaacgattttgtgtatattccgagcggcgatgaactggaaaacattaacaacgtggattttaaagatattaaaaaggaaattaacgaacgcatctataaagtggtgagctttaccggcaaccgcctgagctgcattccgtatatggtggcgaccaccattgtgaacaaactggaattcacccagctgaacaaaattgaattcaccaaagaaaaagaaatttgcattaaactgaacgtggatcgcctgggcaacattagcaaagcg

SEQ ID NO: 197 - DNA, 25 bp, Homo sapiens
  misc_feature 1..25: note = source = /note="target seq for Ataxia-telangiectasia syndrome"
  source 1..25: mol_type = genomic DNA
gaattattccagaaagccaaagtag

SEQ ID NO: 198 - DNA, 20 bp, Homo sapiens
  misc_feature 1..20: note = source = /note="target seq for Very long chain acyl-CoAdehydrogenase deficiency"
  source 1..20: mol_type = genomic DNA
ggcttcatgaaggtacagga

SEQ ID NO: 199 - DNA, 25 bp, Homo sapiens
  misc_feature 1..25: note = source = /note="target seq for Abnormality of T cell physiology"
  source 1..25: mol_type = genomic DNA
ggtgtgctcaccagaatggagtaca

SEQ ID NO: 200 - DNA, 25 bp, Homo sapiens
  misc_feature 1..25: note = source = /note="target seq for Cardiovascular phenotype"
  source 1..25: mol_type = genomic DNA
gcagatcattggggtggatcccgaa

SEQ ID NO: 201 - DNA, 25 bp, Homo sapiens
  misc_feature 1..25: note = source = /note="target seq for 3-Oxo-5 alpha-steroid delta4-dehydrogenase deficiency"
  source 1..25: mol_type = genomic DNA
ggctgcaagcttttcaccaccayag

SEQ ID NO: 202 - DNA, 25 bp, Homo sapiens
  misc_feature 1..25: note = source = /note="target seq for Acute myeloid leukemia"
  source 1..25: mol_type = genomic DNA
gggcggcatgaaccggaggcccatc

SEQ ID NO: 203 - DNA, 20 bp, Homo sapiens
  misc_feature 1..20: note = source = /note="target seq for Acute myeloid leukemia"
  source 1..20: mol_type = genomic DNA
gcatgggcggcatgaaccgg

SEQ ID NO: 204 - DNA, 20 bp, Homo sapiens
  misc_feature 1..20: note = source = /note="target seq for Cutaneous malignant melanoma 3"
  source 1..20: mol_type = genomic DNA
gtggccactgtggggatcac

SEQ ID NO: 205 - DNA, 20 bp, Homo sapiens
  misc_feature 1..20: note = source = /note="target seq for Alpha-1-antitrypsin deficiency"
  source 1..20: mol_type = genomic DNA
gtgctgaccatcgacgagaa

SEQ ID NO: 206 - DNA, 20 bp, Homo sapiens
  misc_feature 1..20: note = source = /note="target seq for Charcot-Marie-Tooth disease, type 2"
  source 1..20: mol_type = genomic DNA
ggcgagctgcatgatctgcg

SEQ ID NO: 207 - DNA, 25 bp, Homo sapiens
  misc_feature 1..25: note = source = /note="target seq for Hereditary cancer-predisposing syndrome"
  source 1..25: mol_type = genomic DNA
gcacatgacggaggttgtgaggcgc

SEQ ID NO: 208 - DNA, 25 bp, Homo sapiens
  misc_feature 1..25: note = source = /note="target seq for Hereditary cancer-predisposing syndrome"
  source 1..25: mol_type = genomic DNA
gaggttgtgaggcactgcccccacc

SEQ ID NO: 209 - DNA, 20 bp, Homo sapiens
  misc_feature 1..20: note = source = /note="target seq for Hereditary cancer-predisposing syndrome"
  source 1..20: mol_type = genomic DNA
gcagcatccggctgcaggta

SEQ ID NO: 210 - DNA, 25 bp, Homo sapiens
  misc_feature 1..25: note = source = /note="target seq for Brugada syndrome"
  source 1..25: mol_type = genomic DNA
ggccaaggggatccgcacgctgctc

SEQ ID NO: 211 - DNA, 20 bp, Homo sapiens
  misc_feature 1..20: note = source = /note="target seq for Brugada syndrome"
  source 1..20: mol_type = genomic DNA
gcctgatgacgcaggactgc

SEQ ID NO: 212 - DNA, 20 bp, Homo sapiens
  misc_feature 1..20: note = source = /note="target seq for GRACILE syndrome"
  source 1..20: mol_type = genomic DNA
ggtacgaagtctcgacactg

SEQ ID NO: 213 - DNA, 20 bp, Homo sapiens
  misc_feature 1..20: note = source = /note="target seq for Enhanced s-cone syndrome"
  source 1..20: mol_type = genomic DNA
ggcattggcggtggacccca

SEQ ID NO: 214 - DNA, 25 bp, Homo sapiens
  misc_feature 1..25: note = source = /note="target seq for Charcot-Marie-Tooth disease, type 2"
  source 1..25: mol_type = genomic DNA
gaagaacaggttctggacgtcaaag

SEQ ID NO: 215 - DNA, 20 bp, Homo sapiens
  misc_feature 1..20: note = source = /note="target seq for Charcot-Marie-Tooth disease, type 2"
  source 1..20: mol_type = genomic DNA
gaacaggttctggacgtcaa

SEQ ID NO: 216 - DNA, 20 bp, Homo sapiens
  misc_feature 1..20: note = source = /note="target seq for Arylsulfatase a, allele a"
  source 1..20: mol_type = genomic DNA
gacaggtcatagagcagcgg

SEQ ID NO: 217 - DNA, 20 bp, Homo sapiens
  misc_feature 1..20: note = source = /note="target seq for Familial hypercholesterolemia"
  source 1..20: mol_type = genomic DNA
gaacgtggtcgctctggaca

SEQ ID NO: 218 - DNA, 20 bp, Homo sapiens
  misc_feature 1..20: note = source = /note="target seq for Familial hypercholesterolemia"
  source 1..20: mol_type = genomic DNA
gaacgtggtcgctctggaca

SEQ ID NO: 219 - DNA, 25 bp, Homo sapiens
  misc_feature 1..25: note = source = /note="target seq for HEMOGLOBIN ARLINGTON PARK"
  source 1..25: mol_type = genomic DNA
ggtgcatctgactcctgaggagaag

SEQ ID NO: 220 - DNA, 20 bp, Homo sapiens
  misc_feature 1..20: note = source = /note="target seq for Familial hypertrophic cardiomyopathy 1"
  source 1..20: mol_type = genomic DNA
gaagtccgaggctcgccgca

SEQ ID NO: 221 - DNA, 20 bp, Homo sapiens
  misc_feature 1..20: note = source = /note="target seq for Cardiovascular phenotype"
  source 1..20: mol_type = genomic DNA
gtcaaggtcatcggtgaggc

SEQ ID NO: 222 - DNA, 25 bp, Homo sapiens
  misc_feature 1..25: note = source = /note="target seq for Cardiovascular phenotype"
  source 1..25: mol_type = genomic DNA
ggtcatcagtgaggccggccggggt

SEQ ID NO: 223 - DNA, 25 bp, Homo sapiens
  misc_feature 1..25: note = source = /note="target seq for Brugada syndrome"
  source 1..25: mol_type = genomic DNA
gtctcagccttacgcaccttccgag

SEQ ID NO: 224 - DNA, 25 bp, Homo sapiens
  misc_feature 1..25: note = source = /note="target seq for Brugada syndrome"
  source 1..25: mol_type = genomic DNA
gcaccttccaagtcctccgggccct

SEQ ID NO: 225 - DNA, 26 bp, Homo sapiens
  misc_feature 1..26: note = source = /note="target seq for Hereditary cancer-predisposing syndrome"
  source 1..26: mol_type = genomic DNA
gaagccagcccctcagggcaactgac

SEQ ID NO: 226 - DNA, 20 bp, Homo sapiens
  misc_feature 1..20: note = source = /note="target seq for Deficiency of butyryl-CoA dehydrogenase"
  source 1..20: mol_type = genomic DNA
ggcgactcatgggttctgaa

SEQ ID NO: 227 - DNA, 25 bp, Homo sapiens
  misc_feature 1..25: note = source = /note="target seq for Deficiency of butyryl-CoA dehydrogenase"
  source 1..25: mol_type = genomic DNA
gcgactcacgggttctgaatggaac

SEQ ID NO: 228 - DNA, 20 bp, Homo sapiens
  misc_feature 1..20: note = source = /note="target seq for Benign scapuloperoneal musculardystrophy with cardiomyopathy"
  source 1..20: mol_type = genomic DNA
ggaactgcgggcccagcatg

SEQ ID NO: 229 - DNA, 20 bp, Homo sapiens
  misc_feature 1..20: note = source = /note="target seq for Benign scapuloperoneal musculardystrophy with cardiomyopathy"
  source 1..20: mol_type = genomic DNA
ggacgagtaccaggagcttc

SEQ ID NO: 230 - DNA, 20 bp, Homo sapiens
  misc_feature 1..20: note = source = /note="target seq for Cone-rod dystrophy 6"
  source 1..20: mol_type = genomic DNA
ggatctgatccgggagcgca

SEQ ID NO: 231 - DNA, 25 bp, Homo sapiens
  misc_feature 1..25: note = source = /note="target seq for Cone-rod dystrophy 6"
  source 1..25: mol_type = genomic DNA
gaatgcactatgttctattccatcc

SEQ ID NO: 232 - DNA, 25 bp, Homo sapiens
  misc_feature 1..25: note = source = /note="target seq for Stargardt disease 1"
  source 1..25: mol_type = genomic DNA
gagctgctcacaggacgagaacatc

SEQ ID NO: 233 - DNA, 20 bp, Homo sapiens
  misc_feature 1..20: note = source = /note="target seq for Leber congenital amaurosis 2"
  source 1..20: mol_type = genomic DNA
gtctatccagtaagtatctc

SEQ ID NO: 234 - DNA, 20 bp, Homo sapiens
  misc_feature 1..20: note = source = /note="target seq for Cone-rod dystrophy 3"
  source 1..20: mol_type = genomic DNA
ggtacgtccatgccacaccc

SEQ ID NO: 235 - DNA, 20 bp, Homo sapiens
  misc_feature 1..20: note = source = /note="target seq for Nonsyndromic Oculocutaneous Albinism"
  source 1..20: mol_type = genomic DNA
ggacctttacggcgtaatcc

SEQ ID NO: 236 - DNA, 20 bp, Homo sapiens
  misc_feature 1..20: note = source = /note="target seq for Phenylketonuria"
  source 1..20: mol_type = genomic DNA
gtcatcctttggtgaattac

SEQ ID NO: 237 - DNA, 25 bp, Homo sapiens
  misc_feature 1..25: note = source = /note="target seq for Phenylketonuria"
  source 1..25: mol_type = genomic DNA
gtattacgtggcagagagttttaat

SEQ ID NO: 238 - DNA, 20 bp, Homo sapiens
  misc_feature 1..20: note = source = /note="target seq for Breast-ovarian cancer, familial 1"
  source 1..20: mol_type = genomic DNA
ggacgctcttgtattatctg

SEQ ID NO: 239 - DNA, 25 bp, Homo sapiens
  misc_feature 1..25: note = source = /note="target seq for Hyperphenylalaninemia, non-pku"
  source 1..25: mol_type = genomic DNA
gcccttctcagttcgctacgaccca

SEQ ID NO: 240 - DNA, 20 bp, Homo sapiens
  misc_feature 1..20: note = source = /note="target seq for Hyperphenylalaninemia, non-pku"
  source 1..20: mol_type = genomic DNA
gctacgacccatacacccaa

SEQ ID NO: 241 - DNA, 20 bp, Homo sapiens
  misc_feature 1..20: note = source = /note="target seq for Hereditary cancer-predisposing syndrome"
  source 1..20: mol_type = genomic DNA
gcgctatgttctattccatc

SEQ ID NO: 242 - DNA, 25 bp, Homo sapiens
  misc_feature 1..25: note = source = /note="target seq for Hereditary cancer-predisposing syndrome"
  source 1..25: mol_type = genomic DNA
ggggctggtattcatgaaaggcaac

SEQ ID NO: 243 - DNA, 20 bp, Homo sapiens
  misc_feature 1..20: note = source = /note="target seq for Hereditary cancer-predisposing syndrome"
  source 1..20: mol_type = genomic DNA
gcgctatgttctattccatc

SEQ ID NO: 244 - DNA, 25 bp, Homo sapiens
  misc_feature 1..25: note = source = /note="target seq for Hereditary cancer-predisposing syndrome"
  source 1..25: mol_type = genomic DNA
gtgttctcaggttatcggtaagttt

SEQ ID NO: 245 - DNA, 25 bp, Homo sapiens
  misc_feature 1..25: note = source = /note="target seq for Hereditary cancer-predisposing syndrome"
  source 1..25: mol_type = genomic DNA
ggaaatgctgttagtcggtatgtcg

SEQ ID NO: 246 - DNA, 25 bp, Homo sapiens
  misc_feature 1..25: note = source = /note="target seq for Hereditary cancer-predisposing syndrome"
  source 1..25: mol_type = genomic DNA
ggaaatgctgttagtcagtatgtcg

SEQ ID NO: 247 - DNA, 20 bp, Homo sapiens
  misc_feature 1..20: note = source = /note="target seq for Anterior segment dysgenesis 6"
  source 1..20: mol_type = genomic DNA
gtggccactgatcggaaacg

SEQ ID NO: 248 - DNA, 25 bp, Homo sapiens
  misc_feature 1..25: note = source = /note="target seq for Brugada syndrome"
  source 1..25: mol_type = genomic DNA
gaacctgatcctggccgtggtcgca

SEQ ID NO: 249 - DNA, 20 bp, Homo sapiens
  misc_feature 1..20: note = source = /note="target seq for Brugada syndrome"
  source 1..20: mol_type = genomic DNA
gatcctggccgtggtcgcaa

SEQ ID NO: 250 - DNA, 25 bp, Homo sapiens
  misc_feature 1..25: note = source = /note="target seq for Ornithine carbamoyltransferasedeficiency"
  source 1..25: mol_type = genomic DNA
gaagggccatgaccttctcactcta

SEQ ID NO: 251 - DNA, 25 bp, Homo sapiens
  misc_feature 1..25: note = source = /note="target seq for Osteogenesis imperfecta type I"
  source 1..25: mol_type = genomic DNA
ggtgctcgaggattgcccggaacag

SEQ ID NO: 252 - DNA, 25 bp, Homo sapiens
  misc_feature 1..25: note = source = /note="target seq for Osteogenesis imperfecta type I"
  source 1..25: mol_type = genomic DNA
gctcgaggattgcccggaacagctg

SEQ ID NO: 253 - DNA, 25 bp, Homo sapiens
  misc_feature 1..25: note = source = /note="target seq for Constipation"
  source 1..25: mol_type = genomic DNA
gattccagttaaatggatggcaatt

SEQ ID NO: 254 - DNA, 25 bp, Homo sapiens
  misc_feature 1..25: note = source = /note="target seq for Dopamine beta hydroxylase deficiency"
  source 1..25: mol_type = genomic DNA
ggacactgcctattttgcggtgagt

SEQ ID NO: 255 - DNA, 25 bp, Homo sapiens
  misc_feature 1..25: note = source = /note="target seq for Cystic fibrosis"
  source 1..25: mol_type = genomic DNA
gacttcatccaggtatgtaaaaata

SEQ ID NO: 256 - DNA, 25 bp, Homo sapiens
  misc_feature 1..25: note = source = /note="target seq for Phenylketonuria"
  source 1..25: mol_type = genomic DNA
gatgtaaacctgacccacactgaat

SEQ ID NO: 257 - DNA, 20 bp, Homo sapiens
  misc_feature 1..20: note = source = /note="target seq for Deficiency ofUDPglucose-hexose-1-phosphate uridylyltransferase"
  source 1..20: mol_type = genomic DNA
gagcccctgacacccttacc

SEQ ID NO: 258 - DNA, 20 bp, Homo sapiens
  misc_feature 1..20: note = source = /note="target seq for Amyloid Cardiomyopathy,Transthyretin-related"
  source 1..20: mol_type = genomic DNA
gtcaccaatcccaaggaatg

SEQ ID NO: 259 - DNA, 25 bp, Homo sapiens
  misc_feature 1..25: note = source = /note="target seq for Carbohydrate-deficientglycoprotein syndrome type I"
  source 1..25: mol_type = genomic DNA
ggctactccatgacagcgcctgagg

SEQ ID NO: 260 - DNA, 25 bp, Homo sapiens
  misc_feature 1..25: note = source = /note="target seq for Metachromatic leukodystrophy"
  source 1..25: mol_type = genomic DNA
gcatcccgtactcccacgaccagat

SEQ ID NO: 261 - DNA, 25 bp, Homo sapiens
  misc_feature 1..25: note = source = /note="target seq for Smith-Lemli-Opitz syndrome"
  source 1..25: mol_type = genomic DNA
gttcttcaatgggcgccccgggatc

SEQ ID NO: 262 - DNA, 20 bp, Homo sapiens
  misc_feature 1..20: note = source = /note="target seq for Deafness, autosomal recessive 1A"
  source 1..20: mol_type = genomic DNA
gcaggtgagcccgccggccc

SEQ ID NO: 263 - DNA, 25 bp, Homo sapiens
  misc_feature 1..25: note = source = /note="target seq for Congenital omphalocele"
  source 1..25: mol_type = genomic DNA
gccagcgctcctagtggccatgcac

SEQ ID NO: 264 - DNA, 25 bp, Homo sapiens
  misc_feature 1..25: note = source = /note="target seq for Congenital omphalocele"
  source 1..25: mol_type = genomic DNA
gcgctcctagtggccatgcacgtgg

SEQ ID NO: 265 - DNA, 20 bp, Homo sapiens
  misc_feature 1..20: note = source = /note="target seq for Congenital omphalocele"
  source 1..20: mol_type = genomic DNA
gtccacgccagcgctcctag

SEQ ID NO: 266 - DNA, 20 bp, Homo sapiens
  misc_feature 1..20: note = source = /note="target seq for Congenital omphalocele"
  source 1..20: mol_type = genomic DNA
gctcctagtggccatgcacg

SEQ ID NO: 267 - DNA, 25 bp, Homo sapiens
  misc_feature 1..25: note = source = /note="target seq for Congenital myotonia, autosomaldominant form"
  source 1..25: mol_type = genomic DNA
gagaggattctttgcagccacgttc

SEQ ID NO: 268 - DNA, 20 bp, Homo sapiens
  misc_feature 1..20: note = source = /note="target seq for Breast-ovarian cancer, familial 1"
  source 1..20: mol_type = genomic DNA
ggtgacccgagagtgggtgt

SEQ ID NO: 269 - DNA, 20 bp, Homo sapiens
  misc_feature 1..20: note = source = /note="target seq for Breast and/or ovarian cancer"
  source 1..20: mol_type = genomic DNA
gatgcctggacagaggacaa

SEQ ID NO: 270 - DNA, 20 bp, Homo sapiens
  misc_feature 1..20: note = source = /note="target seq for Breast-ovarian cancer, familial 1"
  source 1..20: mol_type = genomic DNA
ggacaatggcttccatggta

SEQ ID NO: 271 - DNA, 20 bp, Homo sapiens
  misc_feature 1..20: note = source = /note="target seq for Breast-ovarian cancer, familial 1"
  source 1..20: mol_type = genomic DNA
gggctagaaatctgttgcta

SEQ ID NO: 272 - DNA, 20 bp, Homo sapiens
  misc_feature 1..20: note = source = /note="target seq for Breast-ovarian cancer, familial 1"
  source 1..20: mol_type = genomic DNA
ggtgacccgagagtgggtgt

SEQ ID NO: 273 - DNA, 20 bp, Homo sapiens
  misc_feature 1..20: note = source = /note="target seq for Breast-ovarian cancer, familial 1"
  source 1..20: mol_type = genomic DNA
gattctgcaactttcaattg

SEQ ID NO: 274 - DNA, 20 bp, Homo sapiens
  misc_feature 1..20: note = source = /note="target seq for Breast-ovarian cancer, familial 1"
  source 1..20: mol_type = genomic DNA
ggacaatggcttccatggta

SEQ ID NO: 275 - DNA, 25 bp, Homo sapiens
  misc_feature 1..25: note = source = /note="target seq for Inborn genetic diseases"
  source 1..25: mol_type = genomic DNA
gaaagcccgacttatagccagtaat

SEQ ID NO: 276 - DNA, 20 bp, Homo sapiens
  misc_feature 1..20: note = source = /note="target seq for Breast-ovarian cancer, familial 2"
  source 1..20: mol_type = genomic DNA
gattacatgaacaaatgggc

SEQ ID NO: 277 - DNA, 20 bp, Homo sapiens
  misc_feature 1..20: note = source = /note="target seq for Breast-ovarian cancer, familial 2"
  source 1..20: mol_type = genomic DNA
gattacatgaacaaatgggc

SEQ ID NO: 278 - DNA, 20 bp, Homo sapiens
  misc_feature 1..20: note = source = /note="target seq for Breast-ovarian cancer, familial 2"
  source 1..20: mol_type = genomic DNA
gactggaaaaggaatacagt

SEQ ID NO: 279 - DNA, 25 bp, Homo sapiens
  misc_feature 1..25: note = source = /note="target seq for Breast and/or ovarian cancer"
  source 1..25: mol_type = genomic DNA
gttggctgatggtggatggctcata

SEQ ID NO: 280 - DNA, 25 bp, Homo sapiens
  misc_feature 1..25: note = source = /note="target seq for Breast-ovarian cancer, familial 2"
  source 1..25: mol_type = genomic DNA
gttggctgatggtggatggctcata

SEQ ID NO: 281 - DNA, 20 bp, Homo sapiens
  misc_feature 1..20: note = source = /note="target seq for Breast-ovarian cancer, familial 2"
  source 1..20: mol_type = genomic DNA
ggtcagaagattattcttca

SEQ ID NO: 282 - DNA, 20 bp, Homo sapiens
  misc_feature 1..20: note = source = /note="target seq for Breast-ovarian cancer, familial 2"
  source 1..20: mol_type = genomic DNA
ggcttctagtctcttttgtt

SEQ ID NO: 283 - DNA, 20 bp, Homo sapiens
  misc_feature 1..20: note = source = /note="target seq for Breast-ovarian cancer, familial 2"
  source 1..20: mol_type = genomic DNA
ggcttctagtctcttttgtt

SEQ ID NO: 284 - DNA, 20 bp, Homo sapiens
  misc_feature 1..20: note = source = /note="target seq for Smith-Lemli-Opitz syndrome"
  source 1..20: mol_type = genomic DNA
gttgcgattttgcagccatt

SEQ ID NO: 285 - DNA, 25 bp, Homo sapiens
  misc_feature 1..25: note = source = /note="target seq for Alport syndrome 1, X-linked recessive"
  source 1..25: mol_type = genomic DNA
ggcctatgggtccccctggtttcgg

SEQ ID NO: 286 - DNA, 20 bp, Homo sapiens
  misc_feature 1..20: note = source = /note="target seq for Acute neuronopathic Gaucher's disease"
  source 1..20: mol_type = genomic DNA
ggcatcaggtgagtgagtca

SEQ ID NO: 287 - DNA, 20 bp, Homo sapiens
  misc_feature 1..20: note = source = /note="target seq for Gonadotropin deficiency"
  source 1..20: mol_type = genomic DNA
gtaactctccagcataccat

SEQ ID NO: 288 - DNA, 20 bp, Homo sapiens
  misc_feature 1..20: note = source = /note="target seq for Distal arthrogryposis type 1A"
  source 1..20: mol_type = genomic DNA
gaagctggaggaggccgaga

SEQ ID NO: 289 - DNA, 20 bp, Homo sapiens
  misc_feature 1..20: note = source = /note="target seq for Distal arthrogryposis type 1A"
  source 1..20: mol_type = genomic DNA
gctggaggaggccgagaagg

SEQ ID NO: 290 - DNA, 20 bp, Homo sapiens
  misc_feature 1..20: note = source = /note="target seq for Hereditary cancer-predisposing syndrome"
  source 1..20: mol_type = genomic DNA
gctgccaccttcagggcctc

SEQ ID NO: 291 - DNA, 20 bp, Homo sapiens
  misc_feature 1..20: note = source = /note="target seq for Inborn genetic diseases"
  source 1..20: mol_type = genomic DNA
gataaacttcttgaagagga

SEQ ID NO: 292 - DNA, 25 bp, Homo sapiens
  misc_feature 1..25: note = source = /note="target seq for Death in early adulthood"
  source 1..25: mol_type = genomic DNA
gtgttctccatgttcgaacagaccc

SEQ ID NO: 293 - DNA, 20 bp, Homo sapiens
  misc_feature 1..20: note = source = /note="target seq for Death in early adulthood"
  source 1..20: mol_type = genomic DNA
gttcgaacagacccaaatcc

SEQ ID NO: 294 - DNA, 20 bp, Homo sapiens
  misc_feature 1..20: note = source = /note="target seq for Severe autosomal recessive musculardystrophy of childhood - North African type"
  source 1..20: mol_type = genomic DNA
gaaatctgtgtgtgtccaga

SEQ ID NO: 295 - DNA, 20 bp, Homo sapiens
  misc_feature 1..20: note = source = /note="target seq for Cardiovascular phenotype"
  source 1..20: mol_type = genomic DNA
ggtcatcattgagagcgacc

SEQ ID NO: 296 - DNA, 20 bp, Homo sapiens
  misc_feature 1..20: note = source = /note="target seq for Carbohydrate-deficient glycoproteinsyndrome type I"
  source 1..20: mol_type = genomic DNA
gaatgctgaagatgatcgac

SEQ ID NO: 297 - DNA, 20 bp, Homo sapiens
  misc_feature 1..20: note = source = /note="target seq for Charcot-Marie-Tooth disease, type I"
  source 1..20: mol_type = genomic DNA
gaatgctgaagatgatcgac

SEQ ID NO: 298 - DNA, 25 bp, Homo sapiens
  misc_feature 1..25: note = source = /note="target seq for Inborn genetic diseases"
  source 1..25: mol_type = genomic DNA
gctcagtacaccaccgtcggccgca

SEQ ID NO: 299 - DNA, 20 bp, Homo sapiens
  misc_feature 1..20: note = source = /note="target seq for Inborn genetic diseases"
  source 1..20: mol_type = genomic DNA
gtacaccaccgtcggccgca

SEQ ID NO: 300 - DNA, 25 bp, Homo sapiens
  misc_feature 1..25: note = source = /note="target seq for Familial Mediterranean fever"
  source 1..25: mol_type = genomic DNA
ggacacgtgatggagggaagaacac

SEQ ID NO: 301 - DNA, 25 bp, Homo sapiens
  misc_feature 1..25: note = source = /note="target seq for Deafness, autosomal recessive 2"
  source 1..25: mol_type = genomic DNA
ggacctttgtcaatgggacacggac

SEQ ID NO: 302 - DNA, 25 bp, Homo sapiens
  misc_feature 1..25: note = source = /note="target seq for Deafness, autosomal recessive 2"
  source 1..25: mol_type = genomic DNA
ggacctttgtcaatgggacacagac

SEQ ID NO: 303 - DNA, 25 bp, Homo sapiens
  misc_feature 1..25: note = source = /note="target seq for Deafness, X-linked 2"
  source 1..25: mol_type = genomic DNA
gcgctcctagtggccatgcacgtgg

SEQ ID NO: 304 - DNA, 25 bp, Homo sapiens
  misc_feature 1..25: note = source = /note="target seq for Enlarged vestibular aqueduct"
  source 1..25: mol_type = genomic DNA
gccaccactgctctttcccgcacgg

SEQ ID NO: 305 - DNA, 20 bp, Homo sapiens
  misc_feature 1..20: note = source = /note="target seq for Congenital sensorineuralhearing impairment"
  source 1..20: mol_type = genomic DNA
gtggtcattaacacaaactc

SEQ ID NO: 306 - DNA, 20 bp, Homo sapiens
  misc_feature 1..20: note = source = /note="target seq for Deficiency ofUDPglucose-hexose-1-phosphate uridylyltransferase"
  source 1..20: mol_type = genomic DNA
gccagatattgcccagcgtg

SEQ ID NO: 307 - DNA, 20 bp, Homo sapiens
  misc_feature 1..20: note = source = /note="target seq for Very long chain acyl-CoAdehydrogenase deficiency"
  source 1..20: mol_type = genomic DNA
gccactaatcgtacccagtt

SEQ ID NO: 308 - DNA, 20 bp, Homo sapiens
  misc_feature 1..20: note = source = /note="target seq for Cardiovascular phenotype"
  source 1..20: mol_type = genomic DNA
gatattccactggtggtcga

SEQ ID NO: 309 - DNA, 20 bp, Homo sapiens
  misc_feature 1..20: note = source = /note="target seq for Pyruvate kinase deficiency of red cells"
  source 1..20: mol_type = genomic DNA
ggaagactcctgggcataag

SEQ ID NO: 310 - DNA, 25 bp, Homo sapiens
  misc_feature 1..25: note = source = /note="target seq for Autosomal dominant progressiveexternal ophthalmoplegia with mitochondrial DNAdeletions 1"
  source 1..25: mol_type = genomic DNA
gaagtcgttgatggatctggccaat

SEQ ID NO: 311 - DNA, 20 bp, Homo sapiens
  misc_feature 1..20: note = source = /note="target seq for Very long chain acyl-CoAdehydrogenase deficiency"
  source 1..20: mol_type = genomic DNA
gaagatcacagcttttgtgg

SEQ ID NO: 312 - DNA, 20 bp, Homo sapiens
  misc_feature 1..20: note = source = /note="target seq for Cystinosis, ocular nonnephropathic"
  source 1..20: mol_type = genomic DNA
gtccatctccttctaccctc

SEQ ID NO: 313 - DNA, 20 bp, Homo sapiens
  misc_feature 1..20: note = source = /note="target seq for Pyruvate kinase deficiency of redcells"
  source 1..20: mol_type = genomic DNA
gctcagcccagcttctgtct

SEQ ID NO: 314 - DNA, 25 bp, Homo sapiens
  misc_feature 1..25: note = source = /note="target seq for Distal myopathy, Tateyama type"
  source 1..25: mol_type = genomic DNA
gattgacctggtgaaccaagacccc

SEQ ID NO: 315 - DNA, 25 bp, Homo sapiens
  misc_feature 1..25: note = source = /note="target seq for Malignant hyperthermia,susceptibility to, 1"
  source 1..25: mol_type = genomic DNA
ggccctgcggatccgcgccatcctc

SEQ ID NO: 316 - DNA, 25 bp, Homo sapiens
  misc_feature 1..25: note = source = /note="target seq for Malignant hyperthermia,susceptibility to, 1"
  source 1..25: mol_type = genomic DNA
ggatccgcgccatcctccgctccct

SEQ ID NO: 317 - DNA, 25 bp, Homo sapiens
  misc_feature 1..25: note = source = /note="target seq for Myopathy, Central Core"
  source 1..25: mol_type = genomic DNA
ggtctgatcatcgacgcttttggtg

SEQ ID NO: 318 - DNA, 20 bp, Homo sapiens
  misc_feature 1..20: note = source = /note="target seq for Myopathy, Central Core"
  source 1..20: mol_type = genomic DNA
ggtctgatcatcgacgcttt

SEQ ID NO: 319 - DNA, 25 bp, Homo sapiens
  misc_feature 1..25: note = source = /note="target seq for Myopathy, Central Core"
  source 1..25: mol_type = genomic DNA
gatcatcgacacttttggtgagctc

SEQ ID NO: 320 - DNA, 25 bp, Homo sapiens
  misc_feature 1..25: note = source = /note="target seq for Malignant hyperthermia,susceptibility to, 1"
  source 1..25: mol_type = genomic DNA
ggcggaggcattggggacgagatcg

SEQ ID NO: 321 - DNA, 20 bp, Homo sapiens
  misc_feature 1..20: note = source = /note="target seq for Ceroid lipofuscinosis neuronal 2"
  source 1..20: mol_type = genomic DNA
gtgacagtggggccgggtgt

SEQ ID NO: 322 - DNA, 25 bp, Homo sapiens
  misc_feature 1..25: note = source = /note="target seq for Ceroid lipofuscinosis neuronal 2"
  source 1..25: mol_type = genomic DNA
ggggccgggtattggtctgtctctg

SEQ ID NO: 323 - DNA, 25 bp, Homo sapiens
  misc_feature 1..25: note = source = /note="target seq for Niemann-Pick disease type C1"
  source 1..25: mol_type = genomic DNA
ggatcgacgattatttcgactgggt

SEQ ID NO: 324 - DNA, 25 bp, Homo sapiens
  misc_feature 1..25: note = source = /note="target seq for Glutaric aciduria, type 1"
  source 1..25: mol_type = genomic DNA
gagtatcacgtgatccggcacgcca

SEQ ID NO: 325 - DNA, 25 bp, Homo sapiens
  misc_feature 1..25: note = source = /note="target seq for CAPN3-Related Disorders"
  source 1..25: mol_type = genomic DNA
gccctgatgcagaagaaccggcgga

SEQ ID NO: 326 - DNA, 20 bp, Homo sapiens
  misc_feature 1..20: note = source = /note="target seq for CAPN3-Related Disorders"
  source 1..20: mol_type = genomic DNA
gatgcagaagaaccggcgga

SEQ ID NO: 327 - DNA, 20 bp, Homo sapiens
  misc_feature 1..20: note = source = /note="target seq for Glycogen storage disease, type II"
  source 1..20: mol_type = genomic DNA
gtcccagaacagctcccctc

SEQ ID NO: 328 - DNA, 25 bp, Homo sapiens
  misc_feature 1..25: note = source = /note="target seq for Nonsyndromic Oculocutaneous Albinism"
  source 1..25: mol_type = genomic DNA
gtacagggatctgccaacgatccta

SEQ ID NO: 329 - DNA, 20 bp, Homo sapiens
  misc_feature 1..20: note = source = /note="target seq for Familial hypercholesterolemia"
  source 1..20: mol_type = genomic DNA
gcgaagatggctcggatgag

SEQ ID NO: 330 - DNA, 20 bp, Homo sapiens
  misc_feature 1..20: note = source = /note="target seq for Familial hypercholesterolemia"
  source 1..20: mol_type = genomic DNA
gagtggccgcagcgctgtag

SEQ ID NO: 331 - DNA, 20 bp, Homo sapiens
  misc_feature 1..20: note = source = /note="target seq for Deafness, autosomal recessive 7"
  source 1..20: mol_type = genomic DNA
ggtctcaagctctctcttcg

SEQ ID NO: 332 - DNA, 20 bp, Homo sapiens
  misc_feature 1..20: note = source = /note="target seq for Chronic infantile neurological,cutaneous and articular syndrome"
  source 1..20: mol_type = genomic DNA
gacggcttcgatgagctgca

SEQ ID NO: 333 - DNA, 20 bp, Homo sapiens
  misc_feature 1..20: note = source = /note="target seq for Eichsfeld type congenitalmuscular dystrophy"
  source 1..20: mol_type = genomic DNA
gactctccgggagactgtcc

SEQ ID NO: 334 - DNA, 20 bp, Homo sapiens
  misc_feature 1..20: note = source = /note="target seq for Inborn genetic diseases"
  source 1..20: mol_type = genomic DNA
gctcaaaagtggatgagcgc

SEQ ID NO: 335 - DNA, 20 bp, Homo sapiens
  misc_feature 1..20: note = source = /note="target seq for Hyperkalemic Periodic ParalysisType 1"
  source 1..20: mol_type = genomic DNA
gcagctgcgggtcttcaagc

SEQ ID NO: 336 - DNA, 20 bp, Homo sapiens
  misc_feature 1..20: note = source = /note="target seq for Inclusion body myopathy 2"
  source 1..20: mol_type = genomic DNA
ggacgtggatgtggtggttt

SEQ ID NO: 337 - DNA, 25 bp, Homo sapiens
  misc_feature 1..25: note = source = /note="target seq for Severe APG05083.1, APG07433.1,APG07513.1, APG08290.1 immunodeficiency due to ADADeficiency"
  source 1..25: mol_type = genomic DNA
gaagagcggcattcaccgtactgtc

SEQ ID NO: 338 - DNA, 25 bp, Homo sapiens
  misc_feature 1..25: note = source = /note="target seq for Severe APG05083.1, APG07433.1,APG07513.1, APG08290.1 immunodeficiency due to ADADeficiency"
  source 1..25: mol_type = genomic DNA
gcggtacagtccgcacctgctggcc

SEQ ID NO: 339 - DNA, 20 bp, Homo sapiens
  misc_feature 1..20: note = source = /note="target seq for Cardiovascular phenotype"
  source 1..20: mol_type = genomic DNA
gtgtccgagcagcgccactg

SEQ ID NO: 340 - DNA, 20 bp, Homo sapiens
  misc_feature 1..20: note = source = /note="target seq for Cystic fibrosis"
  source 1..20: mol_type = genomic DNA
ggacacttcgtgccttcgga

SEQ ID NO: 341 - DNA, 20 bp, Homo sapiens
  misc_feature 1..20: note = source = /note="target seq for Cystic fibrosis"
  source 1..20: mol_type = genomic DNA
ggacacttcgtgccttcgga

SEQ ID NO: 342 - DNA, 25 bp, Homo sapiens
  misc_feature 1..25: note = source = /note="target seq for Adrenocortical carcinoma, pediatric"
  source 1..25: mol_type = genomic DNA
gggcgtgagcacttcgagatgttcc

SEQ ID NO: 343 - DNA, 20 bp, Homo sapiens
  misc_feature 1..20: note = source = /note="target seq for Fumarase deficiency"
  source 1..20: mol_type = genomic DNA
gattggacgtactcatactc

SEQ ID NO: 344 - DNA, 20 bp, Homo sapiens
  misc_feature 1..20: note = source = /note="target seq for Adenocarcinoma of prostate"
  source 1..20: mol_type = genomic DNA
gaacactgtccattggcatg

SEQ ID NO: 345 - DNA, 20 bp, Homo sapiens
  misc_feature 1..20: note = source = /note="target seq for Familial hypertrophic cardiomyopathy 1"
  source 1..20: mol_type = genomic DNA
gcatcctctacggggacttc

SEQ ID NO: 346 - DNA, 25 bp, Homo sapiens
  misc_feature 1..25: note = source = /note="target seq for Adult hypophosphatasia"
  source 1..25: mol_type = genomic DNA
gacaacgagatgccccctgaggcct

SEQ ID NO: 347 - DNA, 25 bp, Homo sapiens
  misc_feature 1..25: note = source = /note="target seq for Adult hypophosphatasia"
  source 1..25: mol_type = genomic DNA
ggtactcagacaacaagatgccccc

SEQ ID NO: 348 - DNA, 25 bp, Homo sapiens
  misc_feature 1..25: note = source = /note="target seq for Adult hypophosphatasia"
  source 1..25: mol_type = genomic DNA
gacaacaagatgccccctgaggcct

SEQ ID NO: 349 - DNA, 25 bp, Homo sapiens
  misc_feature 1..25: note = source = /note="target seq for Inborn genetic diseases"
  source 1..25: mol_type = genomic DNA
gccttcttggacaacgtcaccacca

SEQ ID NO: 350 - DNA, 25 bp, Homo sapiens
  misc_feature 1..25: note = source = /note="target seq for Inborn genetic diseases"
  source 1..25: mol_type = genomic DNA
ggtttgccatccgaggggtagtgct

SEQ ID NO: 351 - DNA, 20 bp, Homo sapiens
  misc_feature 1..20: note = source = /note="target seq for Crouzon syndrome"
  source 1..20: mol_type = genomic DNA
gcaaatgcctccacagtggt

SEQ ID NO: 352 - DNA, 20 bp, Homo sapiens
  misc_feature 1..20: note = source = /note="target seq for Propionyl-CoA carboxylase deficiency"
  source 1..20: mol_type = genomic DNA
gacatcataggcacctccat

SEQ ID NO: 353 - DNA, 25 bp, Homo sapiens
  misc_feature 1..25: note = source = /note="target seq for Cardiovascular phenotype"
  source 1..25: mol_type = genomic DNA
ggtggaagggatcggctacgacttc

SEQ ID NO: 354 - DNA, 25 bp, Homo sapiens
  misc_feature 1..25: note = source = /note="target seq for Dysostosis multiplex"
  source 1..25: mol_type = genomic DNA
ggagcagctctgggccgaagtgtcg

SEQ ID NO: 355 - DNA, 20 bp, Homo sapiens
  misc_feature 1..20: note = source = /note="target seq for Multiple sulfatase deficiency"
  source 1..20: mol_type = genomic DNA
ggcgactcctttgtctttga

SEQ ID NO: 356 - DNA, 20 bp, Homo sapiens
  misc_feature 1..20: note = source = /note="target seq for Bifunctional peroxisomal enzymedeficiency"
  source 1..20: mol_type = genomic DNA
ggtggtactggtcaccggcg

SEQ ID NO: 357 - DNA, 25 bp, Homo sapiens
  misc_feature 1..25: note = source = /note="target seq for Bifunctional peroxisomal enzymedeficiency"
  source 1..25: mol_type = genomic DNA
gtactggtcaccagcgcgggggcag

SEQ ID NO: 358 - DNA, 20 bp, Homo sapiens
  misc_feature 1..20: note = source = /note="target seq for Hereditary cancer-predisposingsyndrome"
  source 1..20: mol_type = genomic DNA
ggaaacttgtaagggcttcg

SEQ ID NO: 359 - DNA, 25 bp, Homo sapiens
  misc_feature 1..25: note = source = /note="target seq for Cardiovascular phenotype"
  source 1..25: mol_type = genomic DNA
gtgcagacattgacgaatgccgcat

SEQ ID NO: 360 - DNA, 25 bp, Homo sapiens
  misc_feature 1..25: note = source = /note="target seq for Cardiovascular phenotype"
  source 1..25: mol_type = genomic DNA
gacattgacgaatgccgcatatctc

SEQ ID NO: 361 - DNA, 20 bp, Homo sapiens
  misc_feature 1..20: note = source = /note="target seq for Limb-girdle muscular dystrophy,type 2L"
  source 1..20: mol_type = genomic DNA
gcatagtagtaaactagacg

SEQ ID NO: 362 - DNA, 25 bp, Homo sapiens
  misc_feature 1..25: note = source = /note="target seq for Familial hypercholesterolemia"
  source 1..25: mol_type = genomic DNA
gcatcgatgtcaacgagggcaaccg

SEQ ID NO: 363 - DNA, 20 bp, Homo sapiens
  misc_feature 1..20: note = source = /note="target seq for Spastic Paraplegia, Recessive"
  source 1..20: mol_type = genomic DNA
gcactgctgctcggcccccc

SEQ ID NO: 364 - DNA, 20 bp, Homo sapiens
  misc_feature 1..20: note = source = /note="target seq for Isovaleryl-CoA dehydrogenasedeficiency"
  source 1..20: mol_type = genomic DNA
ggagcagtggggctcagtta

SEQ ID NO: 365 - DNA, 20 bp, Homo sapiens
  misc_feature 1..20: note = source = /note="target seq for Familial hypercholesterolemia"
  source 1..20: mol_type = genomic DNA
gaggagctgcctcacaggtg

SEQ ID NO: 366 - DNA, 20 bp, Homo sapiens
  misc_feature 1..20: note = source = /note="target seq for Biotinidase deficiency"
  source 1..20: mol_type = genomic DNA
gctccagcgcctgagttgta

SEQ ID NO: 367 - DNA, 20 bp, Homo sapiens
  misc_feature 1..20: note = source = /note="target seq for Biotinidase deficiency"
  source 1..20: mol_type = genomic DNA
gcctgagttgtatggccatc

SEQ ID NO: 368 - DNA, 25 bp, Homo sapiens
  misc_feature 1..25: note = source = /note="target seq for Leber congenital amaurosis"
  source 1..25: mol_type = genomic DNA
gcataatttgtacagctctaagagt

SEQ ID NO: 369 - DNA, 25 bp, Homo sapiens
  misc_feature 1..25: note = source = /note="target seq for Familial hyperinsulinism"
  source 1..25: mol_type = genomic DNA
ggtggctgagcccagcccggccccc

SEQ ID NO: 370 - DNA, 25 bp, Homo sapiens
  misc_feature 1..25: note = source = /note="target seq for Familial cancer of breast"
  source 1..25: mol_type = genomic DNA
ggatgcttggcagtgggaaaaactt

SEQ ID NO: 371 - DNA, 20 bp, Homo sapiens
  misc_feature 1..20: note = source = /note="target seq for Cohen syndrome"
  source 1..20: mol_type = genomic DNA
ggaggtctactacaggtctg

SEQ ID NO: 372 - DNA, 25 bp, Homo sapiens
  misc_feature 1..25: note = source = /note="target seq for Cardiovascular phenotype"
  source 1..25: mol_type = genomic DNA
gctccctctgtactgtgcaggagtc

SEQ ID NO: 373 - DNA, 20 bp, Homo sapiens
  misc_feature 1..20: note = source = /note="target seq for Wilson disease"
  source 1..20: mol_type = genomic DNA
ggcaatgaacacaaagagca

SEQ ID NO: 374 - DNA, 25 bp, Homo sapiens
  misc_feature 1..25: note = source = /note="target seq for Wilson disease"
  source 1..25: mol_type = genomic DNA
gccctggatgggctcagcggccatg

SEQ ID NO: 375 - DNA, 20 bp, Homo sapiens
  misc_feature 1..20: note = source = /note="target seq for Wilson disease"
  source 1..20: mol_type = genomic DNA
gcagccctggatgggctcag

SEQ ID NO: 376 - DNA, 20 bp, Homo sapiens
  misc_feature 1..20: note = source = /note="target seq for Familial hypercholesterolemia"
  source 1..20: mol_type = genomic DNA
gtggcccagcgaagatgcga

SEQ ID NO: 377 - DNA, 20 bp, Homo sapiens
  misc_feature 1..20: note = source = /note="target seq for Familial hypercholesterolemia"
  source 1..20: mol_type = genomic DNA
gaagatgcgaaggtgatttc

SEQ ID NO: 378 - DNA, 20 bp, Homo sapiens
  misc_feature 1..20: note = source = /note="target seq for Floating-Harbor syndrome"
  source 1..20: mol_type = genomic DNA
gctgaagctggagtgggtcg

SEQ ID NO: 379 - DNA, 25 bp, Homo sapiens
  misc_feature 1..25: note = source = /note="target seq for Congenital long QT syndrome"
  source 1..25: mol_type = genomic DNA
gatgctacacgtcgaccgccaggga

SEQ ID NO: 380 - DNA, 20 bp, Homo sapiens
  misc_feature 1..20: note = source = /note="target seq for Congenital long QT syndrome"
  source 1..20: mol_type = genomic DNA
gatgctacacgtcgaccgcc

SEQ ID NO: 381 - DNA, 25 bp, Homo sapiens
  misc_feature 1..25: note = source = /note="target seq for Andersen Tawil syndrome"
  source 1..25: mol_type = genomic DNA
gaggaagagatcaaggtcctttcca

SEQ ID NO: 382 - DNA, 25 bp, Homo sapiens
  misc_feature 1..25: note = source = /note="target seq for Cardiovascular phenotype"
  source 1..25: mol_type = genomic DNA
gagctgataaccaccctgtacatcg

SEQ ID NO: 383 - DNA, 20 bp, Homo sapiens
  misc_feature 1..20: note = source = /note="target seq for Familial hypercholesterolemia"
  source 1..20: mol_type = genomic DNA
ggaaaactgcggtatgggcg

SEQ ID NO: 384 - DNA, 25 bp, Homo sapiens
  misc_feature 1..25: note = source = /note="target seq for Cardiovascular phenotype"
  source 1..25: mol_type = genomic DNA
gtatttgaaggtctcctccggggtc

SEQ ID NO: 385 - DNA, 20 bp, Homo sapiens
  misc_feature 1..20: note = source = /note="target seq for Gastrointestinal stroma tumor"
  source 1..20: mol_type = genomic DNA
gagggctaaagtgggctcgg

SEQ ID NO: 386 - DNA, 20 bp, Homo sapiens
  misc_feature 1..20: note = source = /note="target seq for Dyskeratosis congenita"
  source 1..20: mol_type = genomic DNA
gctgccaagcctgctggcaa

SEQ ID NO: 387 - DNA, 25 bp, Homo sapiens
  misc_feature 1..25: note = source = /note="target seq for Dyskeratosis congenita"
  source 1..25: mol_type = genomic DNA
gccctgcctgtgacttccagcactg

SEQ ID NO: 388 - DNA, 25 bp, Homo sapiens
  misc_feature 1..25: note = source = /note="target seq for Glycogen storage disease IIIa"
  source 1..25: mol_type = genomic DNA
gatgagtagaacagaaaaatacaag

SEQ ID NO: 389 - DNA, 25 bp, Homo sapiens
  misc_feature 1..25: note = source = /note="target seq for Dilated cardiomyopathy 1DD"
  source 1..25: mol_type = genomic DNA
gtctcgtagtccggtgagccggtca

SEQ ID NO: 390 - DNA, 20 bp, Homo sapiens
  misc_feature 1..20: note = source = /note="target seq for Renal carnitine transport defect"
  source 1..20: mol_type = genomic DNA
gtggccatggaatagcgccg

SEQ ID NO: 391 - DNA, 25 bp, Homo sapiens
  misc_feature 1..25: note = source = /note="target seq for Baraitser-Winter syndrome 1"
  source 1..25: mol_type = genomic DNA
gatcctcaccgagcgcggctacagc

SEQ ID NO: 392 - DNA, 25 bp, Homo sapiens
  misc_feature 1..25: note = source = /note="target seq for Very long chain acyl-CoAdehydrogenase deficiency"
  source 1..25: mol_type = genomic DNA
gggcatgcatgaccttggcgtgggc

SEQ ID NO: 393 - DNA, 20 bp, Homo sapiens
  misc_feature 1..20: note = source = /note="target seq for Familial hypercholesterolemia"
  source 1..20: mol_type = genomic DNA
gtcagatttgtccttgcagt

SEQ ID NO: 394 - DNA, 20 bp, Homo sapiens
  misc_feature 1..20: note = source = /note="target seq for Limb-girdle muscular dystrophy,type 2A"
  source 1..20: mol_type = genomic DNA
gtacggggttgctctgccgg

SEQ ID NO: 395 - DNA, 25 bp, Homo sapiens
  misc_feature 1..25: note = source = /note="target seq for Familial hypercholesterolemia"
  source 1..25: mol_type = genomic DNA
gacagtagcccctgctcggccttcg

SEQ ID NO: 396 - DNA, 20 bp, Homo sapiens
  misc_feature 1..20: note = source = /note="target seq for Aortic aneurysm, familial thoracic 6"
  source 1..20: mol_type = genomic DNA
gccccatgccatcatgcgtc

SEQ ID NO: 397 - DNA, 25 bp, Homo sapiens
  misc_feature 1..25: note = source = /note="target seq for Acromicric dysplasia"
  source 1..25: mol_type = genomic DNA
gctttgtcatcgacatttataccgg

SEQ ID NO: 398 - DNA, 25 bp, Homo sapiens
  misc_feature 1..25: note = source = /note="target seq for Charcot-Marie-Tooth disease type 2C"
  source 1..25: mol_type = genomic DNA
ggcggacatgcggcaccaggactcg

SEQ ID NO: 399 - DNA, 25 bp, Homo sapiens
  misc_feature 1..25: note = source = /note="target seq for Breast-ovarian cancer, familial 2"
  source 1..25: mol_type = genomic DNA
gtgtaactgtatacgtatggcgttt

SEQ ID NO: 400 - DNA, 20 bp, Homo sapiens
  misc_feature 1..20: note = source = /note="target seq for Breast-ovarian cancer, familial 1"
  source 1..20: mol_type = genomic DNA
gatgcctggacagaggacaa

SEQ ID NO: 401 - DNA, 25 bp, Homo sapiens
  misc_feature 1..25: note = source = /note="target seq for Charcot-Marie-Tooth disease type 2C"
  source 1..25: mol_type = genomic DNA
gcctaactgatgaggagtttcgagg

SEQ ID NO: 402 - DNA, 25 bp, Homo sapiens
  misc_feature 1..25: note = source = /note="target seq for Charcot-Marie-Tooth disease type 2C"
  source 1..25: mol_type = genomic DNA
gcctaactgatgaggagtttcaagg

SEQ ID NO: 403 - DNA, 20 bp, Homo sapiens
  misc_feature 1..20: note = source = /note="target seq for Hereditary cancer-predisposingsyndrome"
  source 1..20: mol_type = genomic DNA
gagcgctgctcagatagcga

SEQ ID NO: 404 - DNA, 25 bp, Homo sapiens
  misc_feature 1..25: note = source = /note="target seq for Early infantile epilepticencephalopathy"
  source 1..25: mol_type = genomic DNA
gatgatccgcatggaccggcgggga

SEQ ID NO: 405 - DNA, 20 bp, Homo sapiens
  misc_feature 1..20: note = source = /note="target seq for Early infantile epilepticencephalopathy"
  source 1..20: mol_type = genomic DNA
ggatgatccgcatggaccgg

SEQ ID NO: 406 - DNA, 25 bp, Homo sapiens
  misc_feature 1..25: note = source = /note="target seq for Early infantile epilepticencephalopathy"
  source 1..25: mol_type = genomic DNA
gcggatgatccgcatggaccagcgg

SEQ ID NO: 407 - DNA, 20 bp, Homo sapiens
  misc_feature 1..20: note = source = /note="target seq for Acromicric dysplasia"
  source 1..20: mol_type = genomic DNA
gtacgtgatccatcctaggt

SEQ ID NO: 408 - DNA, 25 bp, Homo sapiens
  misc_feature 1..25: note = source = /note="target seq for Hypertrophic cardiomyopathy"
  source 1..25: mol_type = genomic DNA
gacaccacggtctccctcaagtggc

SEQ ID NO: 409 - DNA, 25 bp, Homo sapiens
  misc_feature 1..25: note = source = /note="target seq for Cardiovascular phenotype"
  source 1..25: mol_type = genomic DNA
gctgtccggggtagccccaagatag

SEQ ID NO: 410 - DNA, 25 bp, Homo sapiens
  misc_feature 1..25: note = source = /note="target seq for Cardiovascular phenotype"
  source 1..25: mol_type = genomic DNA
gtccacggtgagggggccctggtgt

SEQ ID NO: 411 - DNA, 25 bp, Homo sapiens
  misc_feature 1..25: note = source = /note="target seq for Cardiovascular phenotype"
  source 1..25: mol_type = genomic DNA
gcctagactgcaggacacagggact

SEQ ID NO: 412 - DNA, 25 bp, Homo sapiens
  misc_feature 1..25: note = source = /note="target seq for Familial hypertrophiccardiomyopathy 1"
  source 1..25: mol_type = genomic DNA
gcatctgcagacatagagacctgtg

SEQ ID NO: 413 - DNA, 20 bp, Homo sapiens
  misc_feature 1..20: note = source = /note="target seq for Benign scapuloperoneal musculardystrophy with cardiomyopathy"
  source 1..20: mol_type = genomic DNA
gccctccaagagcttgcggt

SEQ ID NO: 414 - DNA, 25 bp, Homo sapiens
  misc_feature 1..25: note = source = /note="target seq for Glycogen storage disease, type II"
  source 1..25: mol_type = genomic DNA
ggccctcaccctgcgctacgcactc

SEQ ID NO: 415 - DNA, 25 bp, Homo sapiens
  misc_feature 1..25: note = source = /note="target seq for Diffuse mesangial sclerosis"
  source 1..25: mol_type = genomic DNA
gtttaggcacttgttttacctgtat

SEQ ID NO: 416 - DNA, 20 bp, Homo sapiens
  misc_feature 1..20: note = source = /note="target seq for Colobomatous microphthalmia"
  source 1..20: mol_type = genomic DNA
gggtcgaggcggacgccata

SEQ ID NO: 417 - DNA, 20 bp, Homo sapiens
  misc_feature 1..20: note = source = /note="target seq for Ataxia-telangiectasia syndrome"
  source 1..20: mol_type = genomic DNA
gtaaatacatatttactact

SEQ ID NO: 418 - DNA, 20 bp, Homo sapiens
  misc_feature 1..20: note = source = /note="target seq for Familial cancer of breast"
  source 1..20: mol_type = genomic DNA
ggctacagcacacagctcgt

SEQ ID NO: 419 - DNA, 25 bp, Homo sapiens
  misc_feature 1..25: note = source = /note="target seq for Limb-girdle muscular dystrophy,type 2A"
  source 1..25: mol_type = genomic DNA
gctacgagatgcaaaatgcagtcaa

SEQ ID NO: 420 - DNA, 20 bp, Homo sapiens
  misc_feature 1..20: note = source = /note="target seq for Hereditary cancer-predisposingsyndrome"
  source 1..20: mol_type = genomic DNA
gccgcttaccaaaaggagta

SEQ ID NO: 421 - DNA, 25 bp, Homo sapiens
  misc_feature 1..25: note = source = /note="target seq for Asymmetric septal hypertrophy"
  source 1..25: mol_type = genomic DNA
gtgctgcaggttgttggtgcatggc

SEQ ID NO: 422 - DNA, 20 bp, Homo sapiens
  misc_feature 1..20: note = source = /note="target seq for Hereditary cancer-predisposingsyndrome"
  source 1..20: mol_type = genomic DNA
gtaattctataactccttag

SEQ ID NO: 423 - DNA, 25 bp, Homo sapiens
  misc_feature 1..25: note = source = /note="target seq for Familial hypertrophiccardiomyopathy 2"
  source 1..25: mol_type = genomic DNA
gctaaagtcaccgggcgctggaaat

SEQ ID NO: 424 - DNA, 25 bp, Homo sapiens
  misc_feature 1..25: note = source = /note="target seq for Familial hypertrophiccardiomyopathy 2"
  source 1..25: mol_type = genomic DNA
ggctaaagtcaccgggcgctagaaa

SEQ ID NO: 425 - DNA, 25 bp, Homo sapiens
  misc_feature 1..25: note = source = /note="target seq for Familial hypertrophiccardiomyopathy 2"
  source 1..25: mol_type = genomic DNA
gctaaagtcaccgggcgctagaaat

SEQ ID NO: 426 - DNA, 25 bp, Homo sapiens
  misc_feature 1..25: note = source = /note="target seq for Erythrocytosis, familial, 2"
  source 1..25: mol_type = genomic DNA
gaaagagcaatgcctccaggttgtc

SEQ ID NO: 427 - DNA, 25 bp, Homo sapiens
  misc_feature 1..25: note = source = /note="target seq for Death in infancy"
  source 1..25: mol_type = genomic DNA
gtattggaatccggagcatccacgt

SEQ ID NO: 428 - DNA, 20 bp, Homo sapiens
  misc_feature 1..20: note = source = /note="target seq for Muscular Diseases"
  source 1..20: mol_type = genomic DNA
gcatcttccggatctttgag

SEQ ID NO: 429 - DNA, 25 bp, Homo sapiens
  misc_feature 1..25: note = source = /note="target seq for Familial hypercholesterolemia"
  source 1..25: mol_type = genomic DNA
gctgcgagcatggggccctgaggct

SEQ ID NO: 430 - DNA, 20 bp, Homo sapiens
  misc_feature 1..20: note = source = /note="target seq for Familial cancer of breast"
  source 1..20: mol_type = genomic DNA
ggcagcgttacccagtccga

SEQ ID NO: 431 - DNA, 25 bp, Homo sapiens
  misc_feature 1..25: note = source = /note="target seq for Hereditary cancer-predisposingsyndrome"
  source 1..25: mol_type = genomic DNA
gtgtaggcaacttctatagccacag

SEQ ID NO: 432 - DNA, 25 bp, Homo sapiens
  misc_feature 1..25: note = source = /note="target seq for Familial hypercholesterolemia"
  source 1..25: mol_type = genomic DNA
ggaactcccgccaagatcaagaaag

SEQ ID NO: 433 - DNA, 25 bp, Homo sapiens
  misc_feature 1..25: note = source = /note="target seq for Familial hypercholesterolemia"
  source 1..25: mol_type = genomic DNA
gcggctgccagtatctgtgcctccc

SEQ ID NO: 434 - DNA, 25 bp, Homo sapiens
  misc_feature 1..25: note = source = /note="target seq for Familial hypercholesterolemia"
  source 1..25: mol_type = genomic DNA
gaatgatctgcaggtgagcgtcgcc

SEQ ID NO: 435 - DNA, 25 bp, Homo sapiens
  misc_feature 1..25: note = source = /note="target seq for Inclusion body myopathy 2"
  source 1..25: mol_type = genomic DNA
gtgctgtagtgcaccaatgtaatct

SEQ ID NO: 436 - DNA, 20 bp, Homo sapiens
  misc_feature 1..20: note = source = /note="target seq for Ataxia-telangiectasia syndrome"
  source 1..20: mol_type = genomic DNA
gctttgatgttaacaatcgc

SEQ ID NO: 437 - DNA, 25 bp, Homo sapiens
  misc_feature 1..25: note = source = /note="target seq for Benign familialneonatal-infantile seizures"
  source 1..25: mol_type = genomic DNA
gtcagttctccgatcattccagctg

SEQ ID NO: 438 - DNA, 20 bp, Homo sapiens
  misc_feature 1..20: note = source = /note="target seq for Marfan Syndrome/Loeys-DietzSyndrome/Familial Thoracic Aortic Aneurysms andDissections"
  source 1..20: mol_type = genomic DNA
gtatctccattgtctcctcg

SEQ ID NO: 439 - DNA, 25 bp, Homo sapiens
  misc_feature 1..25: note = source = /note="target seq for Dilated cardiomyopathy 1G"
  source 1..25: mol_type = genomic DNA
gtttcagattcccctggcccacgtg

SEQ ID NO: 440 - DNA, 20 bp, Homo sapiens
  misc_feature 1..20: note = source = /note="target seq for Familial hypercholesterolemia"
  source 1..20: mol_type = genomic DNA
gcggtgagtctcggtgcagg

SEQ ID NO: 441 - DNA, 20 bp, Homo sapiens
  misc_feature 1..20: note = source = /note="target seq for Breast-ovarian cancer, familial 2"
  source 1..20: mol_type = genomic DNA
gatacagtattaattgactg

SEQ ID NO: 442 - DNA, 20 bp, Homo sapiens
  misc_feature 1..20: note = source = /note="target seq for Familial hypercholesterolemia"
  source 1..20: mol_type = genomic DNA
gcgagtgcatccactccagc

SEQ ID NO: 443 - DNA, 25 bp, Homo sapiens
  misc_feature 1..25: note = source = /note="target seq for Familial hypercholesterolemia"
  source 1..25: mol_type = genomic DNA
ggctacaagtgccagtgtgaggaag

SEQ ID NO: 444 - DNA, 25 bp, Homo sapiens
  misc_feature 1..25: note = source = /note="target seq for Familial hypercholesterolemia"
  source 1..25: mol_type = genomic DNA
gggtggctacaagtgccagcgtgag

SEQ ID NO: 445 - DNA, 25 bp, Homo sapiens
  misc_feature 1..25: note = source = /note="target seq for Familial hypercholesterolemia"
  source 1..25: mol_type = genomic DNA
gtacaccagcctcacccccaacctg

SEQ ID NO: 446 - DNA, 25 bp, Homo sapiens
  misc_feature 1..25: note = source = /note="target seq for Familial cancer of breast"
  source 1..25: mol_type = genomic DNA
gcctgcccgatagacgagcctcccg

SEQ ID NO: 447 - DNA, 20 bp, Homo sapiens
  misc_feature 1..20: note = source = /note="target seq for Hereditary hemorrhagictelangiectasia type 2"
  source 1..20: mol_type = genomic DNA
gatccgcagcgcggtgagtc

SEQ ID NO: 448-449 - skipped (2 entries)

SEQ ID NO: 450 - protein, 415 aa, synthetic construct
  REGION 1..415: note = source = /note="Description of Artificial Sequence: Syntheticpolypeptide"
  REGION 1..415: note = source = /note="ADAT"
MAKRPAATKKAGQAKKKKSEVEFSHEYWMRHALTLAKRAWDEREVPVGAVLVHNNRVIGEGWNRPIGRHDPTAHAEIMALRQGGLVMQNYRLIDATLYVTLEPCVMCAGAMIHSRIGRVVFGARDAKTGAAGSLMDVLHHPGMNHRVEITEGILADECAALLSDFFRMRRQEIKAQKKAQSSTDSGGSSGGSSGSETPGTSESATPESSGGSSGGSSEVEFSHEYWMRHALTLAKRARDEREVPVGAVLVLNNRVIGEGWNRAIGLHDPTAHAEIMALRQGGLVMQNYRLIDATLYVTFEPCVMCAGAMIHSRIGRVVFGVRNAKTGAAGSLMDVLHYPGMNHRVEITEGILADECAALLCYFFRMPRQVFNAQKKAQSSTDSGGSSGGSSGSETPGTSESATPESSGGSSGGSS

SEQ ID NO: 451 - protein, 1494 aa, synthetic construct
  REGION 1..1494: note = source = /note="Description of Artificial Sequence: Syntheticpolypeptide"
  REGION 1..1494: note = source = /note="Nuc-ADAT-Linker-dAPG08290.1-Linker-SV40"
MAKRPAATKKAGQAKKKKSEVEFSHEYWMRHALTLAKRAWDEREVPVGAVLVHNNRVIGEGWNRPIGRHDPTAHAEIMALRQGGLVMQNYRLIDATLYVTLEPCVMCAGAMIHSRIGRVVFGARDAKTGAAGSLMDVLHHPGMNHRVEITEGILADECAALLSDFFRMRRQEIKAQKKAQSSTDSGGSSGGSSGSETPGTSESATPESSGGSSGGSSEVEFSHEYWMRHALTLAKRARDEREVPVGAVLVLNNRVIGEGWNRAIGLHDPTAHAEIMALRQGGLVMQNYRLIDATLYVTFEPCVMCAGAMIHSRIGRVVFGVRNAKTGAAGSLMDVLHYPGMNHRVEITEGILADECAALLCYFFRMPRQVFNAQKKAQSSTDSGGSSGGSSGSETPGTSESATPESSGGSSGGSSMSELDYRIGLAIGTNSIGWGVIELFWNKDRERYEKVRIVDKGVRMFDKAEIPNKGASLAEPRRIARSSRRRLNRKSQRKKEIRNLLVQHGMITQEELDLLYPLSKKSIDIWDIRLDGLDRLLNHLEWARLLIHLAQRRGFKSNRKSELKDAETGKVLSSIQVNEKRLFLYRTVGEMWIKDAEFSKYDRRRNSPNEYVFSVSRADLEKEIVTLFEAQRKFQSSYASKNLQETYLQIWAHQLPFASGNAILNKVGYCSLLKGKERRIPKATYTFQYFSALDQVNRTRLGPDFQPFTQEQKEIILDKMFQRTDYYKKKTIPEVSYYDIRKWLELDETIQFKGLNYDPNEELKKIEKKPFINLKAFYEIKKVVANYAERTNEAFSTLDYDAIAYALTVYKTDKDIRSYLKKSNNLSKRCYDDQLIEELFTLSYTKFGHLSFKAINHVLPIMQEGRTYQEAIHQLGYDTTNLKKENRSMFLPLIPDEITNPIVKRAITQARKVVNAIIRRYGSPNSVHIALARELSKSHDERKKIMTAHDENYKKNKGAISILIENGILNPTGYDIVRYKLWKEQGERCAYSLKEIPPDTFFNELKKERNGSPILEVDHILPYSQSFIDSYHNKVLVYSDENRNKGNRIPYTYFLETNKDWEAFERYVRSNKLFSKKKREYLLKKTYLPRESELIKERHLNDTRYASTFLKNFIEQNLQFKEVEVNLRKKRVQTVNGVITAHLRKRWGLEKNRQETYLHHAMDAIIVACTDHHMVTRITEYYQIKESNKSVKKPYFPMPWEGFRDELLSHLASQPIAKKISEELKAGYQSSDYIFVSRMPKRSVTGAAHDQTIRRKGGIDKKGKTIIIKRVRLKDIKFDENGDFKMVGKEQDLATYEAIKQRYLEHRKNSKKAFETPLYKPSKKGTGNLIKRVKIEGQTKAFVREVNGGVAQNSDLVRVDLFEKDDKYYMVPIYVPDTVCSELPKKVVKSGKGYEQWLTLDNSFTFKSSLYPYDLVRLVKGNEDRFLYFGTLDIDSDRLNFKDVNKPSKQNEYRYSLKTIENLEKYEVGVLGDLRLVKQETRRIFNRPKKKRKV

SEQ ID NO: 452 - protein, 1494 aa, synthetic construct
  REGION 1..1494: note = source = /note="Description of Artificial Sequence: Syntheticpolypeptide"
  REGION 1..1494: note = source = /note="Nuc-ADAT-Linker-nAPG08290.1-Linker-SV40"
MAKRPAATKKAGQAKKKKSEVEFSHEYWMRHALTLAKRAWDEREVPVGAVLVHNNRVIGEGWNRPIGRHDPTAHAEIMALRQGGLVMQNYRLIDATLYVTLEPCVMCAGAMIHSRIGRVVFGARDAKTGAAGSLMDVLHHPGMNHRVEITEGILADECAALLSDFFRMRRQEIKAQKKAQSSTDSGGSSGGSSGSETPGTSESATPESSGGSSGGSSEVEFSHEYWMRHALTLAKRARDEREVPVGAVLVLNNRVIGEGWNRAIGLHDPTAHAEIMALRQGGLVMQNYRLIDATLYVTFEPCVMCAGAMIHSRIGRVVFGVRNAKTGAAGSLMDVLHYPGMNHRVEITEGILADECAALLCYFFRMPRQVFNAQKKAQSSTDSGGSSGGSSGSETPGTSESATPESSGGSSGGSSMSELDYRIGLAIGTNSIGWGVIELFWNKDRERYEKVRIVDKGVRMFDKAEIPNKGASLAEPRRIARSSRRRLNRKSQRKKEIRNLLVQHGMITQEELDLLYPLSKKSIDIWDIRLDGLDRLLNHLEWARLLIHLAQRRGFKSNRKSELKDAETGKVLSSIQVNEKRLFLYRTVGEMWIKDAEFSKYDRRRNSPNEYVFSVSRADLEKEIVTLFEAQRKFQSSYASKNLQETYLQIWAHQLPFASGNAILNKVGYCSLLKGKERRIPKATYTFQYFSALDQVNRTRLGPDFQPFTQEQKEIILDKMFQRTDYYKKKTIPEVSYYDIRKWLELDETIQFKGLNYDPNEELKKIEKKPFINLKAFYEIKKVVANYAERTNEAFSTLDYDAIAYALTVYKTDKDIRSYLKKSNNLSKRCYDDQLIEELFTLSYTKFGHLSFKAINHVLPIMQEGRTYQEAIHQLGYDTTNLKKENRSMFLPLIPDEITNPIVKRAITQARKVVNAIIRRYGSPNSVHIELARELSKSHDERKKIMTAHDENYKKNKGAISILIENGILNPTGYDIVRYKLWKEQGERCAYSLKEIPPDTFFNELKKERNGSPILEVDHILPYSQSFIDSYHNKVLVYSDENRNKGNRIPYTYFLETNKDWEAFERYVRSNKLFSKKKREYLLKKTYLPRESELIKERHLNDTRYASTFLKNFIEQNLQFKEVEVNLRKKRVQTVNGVITAHLRKRWGLEKNRQETYLHHAMDAIIVACTDHHMVTRITEYYQIKESNKSVKKPYFPMPWEGFRDELLSHLASQPIAKKISEELKAGYQSSDYIFVSRMPKRSVTGAAHDQTIRRKGGIDKKGKTIIIKRVRLKDIKFDENGDFKMVGKEQDLATYEAIKQRYLEHRKNSKKAFETPLYKPSKKGTGNLIKRVKIEGQTKAFVREVNGGVAQNSDLVRVDLFEKDDKYYMVPIYVPDTVCSELPKKVVKSGKGYEQWLTLDNSFTFKSSLYPYDLVRLVKGNEDRFLYFGTLDIDSDRLNFKDVNKPSKQNEYRYSLKTIENLEKYEVGVLGDLRLVKQETRRIFNRPKKKRKV

SEQ ID NO: 453 - DNA, 25 bp, Homo sapiens
  misc_feature 1..25: note = source = /note="Hurler target 1"
  source 1..25: mol_type = genomic DNA
ggagcagctctaggccgaagtgtcg

SEQ ID NO: 454 - DNA, 25 bp, Homo sapiens
  misc_feature 1..25: note = source = /note="Hurler target 2"
  source 1..25: mol_type = genomic DNA
taggccgaagtgtcgcaggccggga

SEQ ID NO: 455 - DNA, 25 bp, Homo sapiens
  misc_feature 1..25: note = source = /note="Hurler target 3"
  source 1..25: mol_type = genomic DNA
gctctaggccgaagtgtcgcaggcc

SEQ ID NO: 456 - DNA, 135 bp, synthetic construct
  misc_feature 1..135: note = source = /note="Description of Artificial Sequence: Syntheticpolynucleotide"
  misc_feature 1..135: note = source = /note="sgRNA Hurler target 1"
  source 1..135: mol_type = other DNA
ggagcagctctaggccgaagtgtcggtcatagttccatgaaagccaaaagtggctttgatgtttctatgataagggtttcggcccgtggcgtcggggatcgcctgcccattccgatgggcttctccccatttatt

SEQ ID NO: 457 - DNA, 135 bp, synthetic construct
  misc_feature 1..135: note = source = /note="Description of Artificial Sequence: Syntheticpolynucleotide"
  misc_feature 1..135: note = source = /note="sgRNA Hurler target 2"
  source 1..135: mol_type = other DNA
taggccgaagtgtcgcaggccgggagtcatagttccatgaaagccaaaagtggctttgatgtttctatgataagggtttcggcccgtggcgtcggggatcgcctgcccattccgatgggcttctccccatttatt

SEQ ID NO: 458 - DNA, 135 bp, synthetic construct
  misc_feature 1..135: note = source = /note="Description of Artificial Sequence: Syntheticpolynucleotide"
  misc_feature 1..135: note = source = /note="sgRNA Hurler target 3"
  source 1..135: mol_type = other DNA
ggcctgcgacacttcggcctagagcgtcatagttccatgaaagccaaaagtggctttgatgtttctatgataagggtttcggcccgtggcgtcggggatcgcctgcccattccgatgggcttctccccatttatt

SEQ ID NO: 459 - DNA, 15 bp, synthetic construct
  misc_feature 1..15: note = source = /note="Description of Artificial Sequence: Syntheticoligonucleotide"
  misc_feature 1..15: note = source = /note="Hurler Forward Amplification Primer"
  source 1..15: mol_type = other DNA
gactccttcaccaag

SEQ ID NO: 460 - DNA, 14 bp, synthetic construct
  misc_feature 1..14: note = source = /note="Description of Artificial Sequence: Syntheticoligonucleotide"
  misc_feature 1..14: note = source = /note="Hurler Reverse Amplification Primer"
  source 1..14: mol_type = other DNA
gtagatcagcaccg

SEQ ID NO: 461 - DNA, 14 bp, synthetic construct
  misc_feature 1..14: note = source = /note="Description of Artificial Sequence: Syntheticoligonucleotide"
  misc_feature 1..14: note = source = /note="Hurler Wild Type Probe"
  source 1..14: mol_type = other DNA
ctctgggccgaagt

SEQ ID NO: 462 - DNA, 14 bp, synthetic construct
  misc_feature 1..14: note = source = /note="Description of Artificial Sequence: Syntheticoligonucleotide"
  misc_feature 1..14: note = source = /note="Hurler W402X Probe-beta"
  source 1..14: mol_type = other DNA
ctctaggccgaagt

SEQ ID NO: 463 - DNA, 13 bp, synthetic construct
  misc_feature 1..13: note = source = /note="Description of Artificial Sequence: Syntheticoligonucleotide"
  misc_feature 1..13: note = source = /note="Hurler NGS forward"
  source 1..13: mol_type = other DNA
acttcctccagcc

SEQ ID NO: 464 - DNA, 13 bp, synthetic construct
  misc_feature 1..13: note = source = /note="Description of Artificial Sequence: Syntheticoligonucleotide"
  misc_feature 1..13: note = source = /note="Hurler NGS Reverse"
  source 1..13: mol_type = other DNA
gaaccccggctta

SEQ ID NO: 465 - DNA, 31 bp, Homo sapiens
  misc_feature 1..31: note = source = /note="Human W402X"
  source 1..31: mol_type = genomic DNA
ggagcagctctaggccgaagtgtcgcaggcc

SEQ ID NO: 466 - DNA, 31 bp, Mus musculus
  misc_feature 1..31: note = source = /note="Mouse W392X"
  source 1..31: mol_type = genomic DNA
agaacaactctaggcagaggtctcaaaggct

SEQ ID NO: 467 - DNA, 31 bp, synthetic construct; identical to SEQ ID NO: 465
  misc_feature 1..31: note = source = /note="Description of Artificial Sequence: Syntheticoligonucleotide"
  misc_feature 1..31: note = source = /note="humanized mouse"
  source 1..31: mol_type = other DNA

SEQ ID NO: 468 - DNA, 25 bp, Homo sapiens
  misc_feature 1..25: note = source = /note="FRDA target 1"
  source 1..25: mol_type = genomic DNA
atcacctgaggtccggagttcaaga

SEQ ID NO: 469 - DNA, 25 bp, Homo sapiens
  misc_feature 1..25: note = source = /note="FRDA target 2"
  source 1..25: mol_type = genomic DNA
gtcttgaactccggacctcaggtga

SEQ ID NO: 470 - DNA, 25 bp, Homo sapiens
  misc_feature 1..25: note = source = /note="FRDA target 3"
  source 1..25: mol_type = genomic DNA
tgaactccggacctcaggtgatcca

SEQ ID NO: 471 - DNA, 25 bp, Homo sapiens
  misc_feature 1..25: note = source = /note="FRDA target 4"
  source 1..25: mol_type = genomic DNA
gaaaagttagccgggcgtggtgtcg

SEQ ID NO: 472 - DNA, 500 bp, synthetic construct
  misc_feature 1..500: note = source = /note="Description of Artificial Sequence: Syntheticpolynucleotide"
  misc_feature 1..500: note = source = /note="BCL11A enhancer region"
  source 1..500: mol_type = other DNA
aaaaatggacaattatgaggaggggagagtgcagacaggggaagcttcacctcctttacaattttgggagtccacacggcatggcatacaaattatttcattcccattgagaaataaaatccaattctccatcaccaagagagccttccgaaagaggcccccctgggcaaacggccaccgatggagaggtctgccagtcctcttctaccccacccacgcccccaccctaatcagaggccaaacccttcctggagcctgtgataaaagcaactgttagcttgcactagactagcttcaaagttgtattgaccctggtgtgttatgtctaagagtagatgccatatctcttttctggcctatgttattacctgtatggactttgcactggaatcagctatctgctcttacttatgcacacctggggcatagagccagccctgtatcgcttttcagccatctcactacagataactcccaagtcctgtctagctgccttcctt

SEQ ID NO: 473 - DNA, 26 bp, Homo sapiens
  misc_feature 1..26: note = source = /note="SCD target seq 1"
  source 1..26: mol_type = genomic DNA
gcactagactagcttcaaagttgtag

SEQ ID NO: 474 - DNA, 26 bp, Homo sapiens
  misc_feature 1..26: note = source = /note="SCD target seq 2"
  source 1..26: mol_type = genomic DNA
cctaatcagaggccaaacccttcctg

SEQ ID NO: 475 - DNA, 26 bp, Homo sapiens
  misc_feature 1..26: note = source = /note="SCD target seq 3"
  source 1..26: mol_type = genomic DNA
caagctaacagttgcttttatcacag

SEQ ID NO: 476 - DNA, 26 bp, Homo sapiens
  misc_feature 1..26: note = source = /note="SCD target seq 4"
  source 1..26: mol_type = genomic DNA
gcactagactagcttcaaagttgtag

SEQ ID NO: 477 - DNA, 26 bp, Homo sapiens
  misc_feature 1..26: note = source = /note="SCD target seq 5"
  source 1..26: mol_type = genomic DNA
cctaatcagaggccaaacccttcctg

SEQ ID NO: 478 - DNA, 26 bp, Homo sapiens
  misc_feature 1..26: note = source = /note="SCD target seq 6"
  source 1..26: mol_type = genomic DNA
caagctaacagttgcttttatcacag

SEQ ID NO: 479 - DNA, 22 bp, synthetic construct
  misc_feature 1..22: note = source = /note="Description of Artificial Sequence: Syntheticoligonucleotide"
  misc_feature 1..22: note = source = /note="RelA FWD"
  source 1..22: mol_type = other DNA
cttagtttcaccgcaggttcta

SEQ ID NO: 480 - DNA, 22 bp, synthetic construct
  misc_feature 1..22: note = source = /note="Description of Artificial Sequence: Syntheticoligonucleotide"
  misc_feature 1..22: note = source = /note="RelA REV"
  source 1..22: mol_type = other DNA
ctgtgcactcaacactgatcta

SEQ ID NO: 481 - DNA, 21 bp, synthetic construct
  misc_feature 1..21: note = source = /note="Description of Artificial Sequence: Syntheticoligonucleotide"
  misc_feature 1..21: note = source = /note="AurkB FWD"
  source 1..21: mol_type = other DNA
cccagccctaggttgtttatt

SEQ ID NO: 482 - DNA, 23 bp, synthetic construct
  misc_feature 1..23: note = source = /note="Description of Artificial Sequence: Syntheticoligonucleotide"
  misc_feature 1..23: note = source = /note="AurkB REV"
  source 1..23: mol_type = other DNA
ctggctacatcttccttgactac

SEQ ID NO: 483 - DNA, 20 bp, synthetic construct
  misc_feature 1..20: note = source = /note="Description of Artificial Sequence: Syntheticoligonucleotide"
  misc_feature 1..20: note = source = /note="HPRT1 FWD"
  source 1..20: mol_type = other DNA
gtggcagaagcagtgagtaa

SEQ ID NO: 484 - DNA, 22 bp, synthetic construct
  misc_feature 1..22: note = source = /note="Description of Artificial Sequence: Syntheticoligonucleotide"
  misc_feature 1..22: note = source = /note="HPRT1 REV"
  source 1..22: mol_type = other DNA
tcccatctaggcactaggtaaa

SEQ ID NO: 485 - DNA, 54 bp, synthetic construct
  misc_feature 1..54: note = source = /note="Description of Artificial Sequence: Syntheticoligonucleotide"
  misc_feature 1..54: note = source = /note="FWD_Guide 134, Guide 135, Guide 136, Guide 137"
  source 1..54: mol_type = other DNA
gtctcgtgggctcggagatgtgtataagagacagacaattctcctgcctcagcc

SEQ ID NO: 486 - DNA, 53 bp, synthetic construct
  misc_feature 1..53: note = source = /note="Description of Artificial Sequence: Syntheticoligonucleotide"
  misc_feature 1..53: note = source = /note="REV_Guide 134, Guide 135, Guide 136, Guide 137"
  source 1..53: mol_type = other DNA
tcgtcggcagcgtcagatgtgtataagagacagactgccatgggaagaaggtg

SEQ ID NO: 487 - DNA, 54 bp, synthetic construct; identical to SEQ ID NO: 485
  misc_feature 1..54: note = source = /note="Description of Artificial Sequence: Syntheticoligonucleotide"
  misc_feature 1..54: note = source = /note="FWD_Guide 138, Guide 139, Guide 140, Guide 141"
  source 1..54: mol_type = other DNA

SEQ ID NO: 488 - DNA, 53 bp, synthetic construct; identical to SEQ ID NO: 486
  misc_feature 1..53: note = source = /note="Description of Artificial Sequence: Syntheticoligonucleotide"
  misc_feature 1..53: note = source = /note="REV_Guide 138, Guide 139, Guide 140, Guide 141"
  source 1..53: mol_type = other DNA

SEQ ID NO: 489 - DNA, 53 bp, synthetic construct
  misc_feature 1..53: note = source = /note="Description of Artificial Sequence: Syntheticoligonucleotide"
  misc_feature 1..53: note = source = /note="REV_Guide 142, Guide 143, Guide 144, Guide 145"
  source 1..53: mol_type = other DNA
tcgtcggcagcgtcagatgtgtataagagacaggagctgcacatttgacgagc

SEQ ID NO: 490 - DNA, 54 bp, synthetic construct
  misc_feature 1..54: note = source = /note="Description of Artificial Sequence: Syntheticoligonucleotide"
  misc_feature 1..54: note = source = /note="FWD_Guide 142, Guide 143, Guide 144, Guide 145"
  source 1..54: mol_type = other DNA
gtctcgtgggctcggagatgtgtataagagacagattacaggtgtgagccacgg

SEQ ID NO: 491 - DNA, 53 bp, synthetic construct
  misc_feature 1..53: note = source = /note="Description of Artificial Sequence: Syntheticoligonucleotide"
  misc_feature 1..53: note = source = /note="REV_Guide 164, Guide 165, Guide 166, Guide 167"
  source 1..53: mol_type = other DNA
tcgtcggcagcgtcagatgtgtataagagacagctgacctcaggtgatacgcc

SEQ ID NO: 492 - DNA, 54 bp, synthetic construct
  misc_feature 1..54: note = source = /note="Description of Artificial Sequence: Syntheticoligonucleotide"
  misc_feature 1..54: note = source = /note="FWD_Guide 164, Guide 165, Guide 166, Guide 167"
  source 1..54: mol_type = other DNA
gtctcgtgggctcggagatgtgtataagagacagctttgggaggctgagacagg

SEQ ID NO: 493 - DNA, 53 bp, synthetic construct
  misc_feature 1..53: note = source = /note="Description of Artificial Sequence: Syntheticoligonucleotide"
  misc_feature 1..53: note = source = /note="REV_Guide 168, Guide 169, Guide 170, Guide 171"
  source 1..53: mol_type = other DNA
tcgtcggcagcgtcagatgtgtataagagacagtgctctattgtccaggctgg

SEQ ID NO: 494 - DNA, 54 bp, synthetic construct
  misc_feature 1..54: note = source = /note="Description of Artificial Sequence: Syntheticoligonucleotide"
  misc_feature 1..54: note = source = /note="FWD_Guide 168, Guide 169, Guide 170, Guide 171"
  source 1..54: mol_type = other DNA
gtctcgtgggctcggagatgtgtataagagacagtccagcaggtcagcaaagaa

SEQ ID NO: 495 - DNA, 53 bp, synthetic construct
  misc_feature 1..53: note = source = /note="Description of Artificial Sequence: Syntheticoligonucleotide"
  misc_feature 1..53: note = source = /note="REV_Guide 172, Guide 173, Guide 174, Guide 175"
  source 1..53: mol_type = other DNA
tcgtcggcagcgtcagatgtgtataagagacaggcagtataactggccagcct

SEQ ID NO: 496 - DNA, 56 bp, synthetic construct
  misc_feature 1..56: note = source = /note="Description of Artificial Sequence: Syntheticoligonucleotide"
  misc_feature 1..56: note = source = /note="FWD_Guide 172, Guide 173, Guide 174, Guide 175"
  source 1..56: mol_type = other DNA
gtctcgtgggctcggagatgtgtataagagacagtcagttgaggagttcagcttaa

SEQ ID NO: 497 - DNA, 53 bp, synthetic construct
  misc_feature 1..53: note = source = /note="Description of Artificial Sequence: Syntheticoligonucleotide"
  misc_feature 1..53: note = source = /note="REV_Guide 185, Guide 186, Guide 187, Guide 188"
  source 1..53: mol_type = other DNA
tcgtcggcagcgtcagatgtgtataagagacagtggcccctatgtggagatca

SEQ ID NO: 498 - DNA, 54 bp, synthetic construct
  misc_feature 1..54: note = source = /note="Description of Artificial Sequence: Syntheticoligonucleotide"
  misc_feature 1..54: note = source = /note="FWD_Guide 185, Guide 186, Guide 187, Guide 188"
  source 1..54: mol_type = other DNA
gtctcgtgggctcggagatgtgtataagagacagggcagagctcagcctcatag

SEQ ID NO: 499 - DNA, 53 bp, synthetic construct
  misc_feature 1..53: note = source = /note="Description of Artificial Sequence: Syntheticoligonucleotide"
  misc_feature 1..53: note = source = /note="REV_Guide 189, Guide 190, Guide 191, Guide 192"
  source 1..53: mol_type = other DNA
tcgtcggcagcgtcagatgtgtataagagacagatatccccacttcccctgct

SEQ ID NO: 500 - DNA, 54 bp, synthetic construct
  misc_feature 1..54: note = source = /note="Description of Artificial Sequence: Syntheticoligonucleotide"
  misc_feature 1..54: note = source = /note="FWD_Guide 189, Guide 190, Guide 191, Guide 192"
  source 1..54: mol_type = other DNA
gtctcgtgggctcggagatgtgtataagagacagcacctcaaggacagctctgg

SEQ ID NO: 501 - DNA, 53 bp, synthetic construct; identical to SEQ ID NO: 499
  misc_feature 1..53: note = source = /note="Description of Artificial Sequence: Syntheticoligonucleotide"
  misc_feature 1..53: note = source = /note="REV_Guide 193, Guide 194, Guide 195, Guide 196"
  source 1..53: mol_type = other DNA

SEQ ID NO: 502 - DNA, 54 bp, synthetic construct; identical to SEQ ID NO: 500
  misc_feature 1..54: note = source = /note="Description of Artificial Sequence: Syntheticoligonucleotide"
  misc_feature 1..54: note = source = /note="FWD_Guide 193, Guide 194, Guide 195, Guide 196"
  source 1..54: mol_type = other DNA

SEQ ID NO: 503 - DNA, 54 bp, synthetic construct; identical to SEQ ID NO: 485
  misc_feature 1..54: note = source = /note="Description of Artificial Sequence: Syntheticoligonucleotide"
  misc_feature 1..54: note = source = /note="FWD_Guide 146"
  source 1..54: mol_type = other DNA

SEQ ID NO: 504 - DNA, 53 bp, synthetic construct; identical to SEQ ID NO: 486
  misc_feature 1..53: note = source = /note="Description of Artificial Sequence: Syntheticoligonucleotide"
  misc_feature 1..53: note = source = /note="REV_Guide 146"
  source 1..53: mol_type = other DNA

SEQ ID NO: 505 - DNA, 54 bp, synthetic construct; identical to SEQ ID NO: 485
  misc_feature 1..54: note = source = /note="Description of Artificial Sequence: Syntheticoligonucleotide"
  misc_feature 1..54: note = source = /note="FWD_Guide 147"
  source 1..54: mol_type = other DNA

SEQ ID NO: 506 - DNA, 53 bp, synthetic construct; identical to SEQ ID NO: 486
  misc_feature 1..53: note = source = /note="Description of Artificial Sequence: Syntheticoligonucleotide"
  misc_feature 1..53: note = source = /note="REV_Guide 147"
  source 1..53: mol_type = other DNA

SEQ ID NO: 507 - DNA, 53 bp, synthetic construct; identical to SEQ ID NO: 486
  misc_feature 1..53: note = source = /note="Description of Artificial Sequence: Syntheticoligonucleotide"
  misc_feature 1..53: note = source = /note="REV_Guide 148"
  source 1..53: mol_type = other DNA

SEQ ID NO: 508 - DNA, 54 bp, synthetic construct; identical to SEQ ID NO: 485
  misc_feature 1..54: note = source = /note="Description of Artificial Sequence: Syntheticoligonucleotide"
  misc_feature 1..54: note = source = /note="FWD_Guide 148"
  source 1..54: mol_type = other DNA

SEQ ID NO: 509 - DNA, 53 bp, synthetic construct
  misc_feature 1..53: note = source = /note="Description of Artificial Sequence: Syntheticoligonucleotide"
  misc_feature 1..53: note = source = /note="REV_Guide 176"
  source 1..53: mol_type = other DNA
tcgtcggcagcgtcagatgtgtataagagacaggtagctcactgcagcctcaa

SEQ ID NO: 510 - DNA, 54 bp, synthetic construct
  misc_feature 1..54: note = source = /note="Description of Artificial Sequence: Syntheticoligonucleotide"
  misc_feature 1..54: note = source = /note="FWD_Guide 176"
  source 1..54: mol_type = other DNA
gtctcgtgggctcggagatgtgtataagagacagtgggtgatgaacatacgggt

SEQ ID NO: 511 - DNA, 57 bp, synthetic construct
  misc_feature 1..57: note = source = /note="Description of Artificial Sequence: Syntheticoligonucleotide"
  misc_feature 1..57: note = source = /note="REV_Guide 177"
  source 1..57: mol_type = other DNA
tcgtcggcagcgtcagatgtgtataagagacagtcagactgaagagctattgtgtga

SEQ ID NO: 512 - DNA, 54 bp, synthetic construct
  misc_feature 1..54: note = source = /note="Description of Artificial Sequence: Syntheticoligonucleotide"
  misc_feature 1..54: note = source = /note="FWD_Guide 177"
  source 1..54: mol_type = other DNA
gtctcgtgggctcggagatgtgtataagagacagccccacaaaccgatgtagct

SEQ ID NO: 513 - DNA, 53 bp, synthetic construct
  misc_feature 1..53: note = source = /note="Description of Artificial Sequence: Syntheticoligonucleotide"
  misc_feature 1..53: note = source = /note="REV_Guide 209"
  source 1..53: mol_type = other DNA
tcgtcggcagcgtcagatgtgtataagagacagtggagtgcagtggtgtgatc

SEQ ID NO: 514 - DNA, 54 bp, synthetic construct
  misc_feature 1..54: note = source = /note="Description of Artificial Sequence: Syntheticoligonucleotide"
  misc_feature 1..54: note = source = /note="FWD_Guide 209"
  source 1..54: mol_type = other DNA
gtctcgtgggctcggagatgtgtataagagacagttgaggctgcagtgagctac

SEQ ID NO: 515 - DNA, 53 bp, synthetic construct; identical to SEQ ID NO: 497
  misc_feature 1..53: note = source = /note="Description of Artificial Sequence: Syntheticoligonucleotide"
  misc_feature 1..53: note = source = /note="REV_Guide 197"
  source 1..53: mol_type = other DNA

SEQ ID NO: 516 - DNA, 54 bp, synthetic construct; identical to SEQ ID NO: 498
  misc_feature 1..54: note = source = /note="Description of Artificial Sequence: Syntheticoligonucleotide"
  misc_feature 1..54: note = source = /note="FWD_Guide 197"
  source 1..54: mol_type = other DNA

SEQ ID NO: 517 - DNA, 53 bp, synthetic construct
  misc_feature 1..53: note = source = /note="Description of Artificial Sequence: Syntheticoligonucleotide"
  misc_feature 1..53: note = source = /note="REV_Guide 198"
  source 1..53: mol_type = other DNA
tcgtcggcagcgtcagatgtgtataagagacagccaagccgaccaaacaagtg

SEQ ID NO: 518 - DNA, 54 bp, synthetic construct
  misc_feature 1..54: note = source = /note="Description of Artificial Sequence: Syntheticoligonucleotide"
  misc_feature 1..54: note = source = /note="FWD_Guide 198"
  source 1..54: mol_type = other DNA
gtctcgtgggctcggagatgtgtataagagacaggatgcgctgactgatagcct

SEQ ID NO: 519 - DNA, 53 bp, synthetic construct; identical to SEQ ID NO: 497
  misc_feature 1..53: note = source = /note="Description of Artificial Sequence: Syntheticoligonucleotide"
  misc_feature 1..53: note = source = /note="REV_Guide 199"
  source 1..53: mol_type = other DNA

SEQ ID NO: 520 - DNA, 54 bp, synthetic construct; identical to SEQ ID NO: 498
  misc_feature 1..54: note = source = /note="Description of Artificial Sequence: Syntheticoligonucleotide"
  misc_feature 1..54: note = source = /note="FWD_Guide 199"
  source 1..54: mol_type = other DNA

SEQ ID NO: 521 - DNA, 54 bp, synthetic construct
  misc_feature 1..54: note = source = /note="Description of Artificial Sequence: Syntheticoligonucleotide"
  misc_feature 1..54: note = source = /note="FWD_Guide 149"
  source 1..54: mol_type = other DNA
gtctcgtgggctcggagatgtgtataagagacagggtaaggggaaactggaggc

SEQ ID NO: 522 - DNA, 53 bp, synthetic construct
  misc_feature 1..53: note = source = /note="Description of Artificial Sequence: Syntheticoligonucleotide"
  misc_feature 1..53: note = source = /note="REV_Guide 149"
  source 1..53: mol_type = other DNA
tcgtcggcagcgtcagatgtgtataagagacagtccactttctaagcaggcgg

SEQ ID NO: 523 - DNA, 54 bp, synthetic construct
  misc_feature 1..54: note = source = /note="Description of Artificial Sequence: Syntheticoligonucleotide"
  misc_feature 1..54: note = source = /note="FWD_Guide 150"
  source 1..54: mol_type = other DNA
gtctcgtgggctcggagatgtgtataagagacaggtgggcctggatttcgatct

SEQ ID NO: 524 - DNA, 53 bp, synthetic construct
  misc_feature 1..53: note = source = /note="Description of Artificial Sequence: Syntheticoligonucleotide"
  misc_feature 1..53: note = source = /note="REV_Guide 150"
  source 1..53: mol_type = other DNA
tcgtcggcagcgtcagatgtgtataagagacagatgaacaggcaggaagtcgg

SEQ ID NO: 525 - DNA, 53 bp, synthetic construct
  misc_feature 1..53: note = source = /note="Description of Artificial Sequence: Syntheticoligonucleotide"
  misc_feature 1..53: note = source = /note="REV_Guide 151"
  source 1..53: mol_type = other DNA
tcgtcggcagcgtcagatgtgtataagagacagcggttctgagttgccttcct

SEQ ID NO: 526 - DNA, 54 bp, synthetic construct; identical to SEQ ID NO: 521
  misc_feature 1..54: note = source = /note="Description of Artificial Sequence: Syntheticoligonucleotide"
  misc_feature 1..54: note = source = /note="FWD_Guide 151"
  source 1..54: mol_type = other DNA

SEQ ID NO: 527 - DNA, 53 bp, synthetic construct
  misc_feature 1..53: note = source = /note="Description of Artificial Sequence: Syntheticoligonucleotide"
  misc_feature 1..53: note = source = /note="REV_Guide 179"
  source 1..53: mol_type = other DNA
tcgtcggcagcgtcagatgtgtataagagacagtcagtggtccacatgcaagt

SEQ ID NO: 528 - DNA, 54 bp, synthetic construct
  misc_feature 1..54: note = source = /note="Description of Artificial Sequence: Syntheticoligonucleotide"
  misc_feature 1..54: note = source = /note="FWD_Guide 179"
  source 1..54: mol_type = other DNA
gtctcgtgggctcggagatgtgtataagagacagaaggcaagttgatcgctcga

SEQ ID NO: 529 - DNA, 53 bp, synthetic construct
  misc_feature 1..53: note = source = /note="Description of Artificial Sequence: Syntheticoligonucleotide"
  misc_feature 1..53: note = source = /note="REV_Guide 180"
  source 1..53: mol_type = other DNA
tcgtcggcagcgtcagatgtgtataagagacagagtggttctgttgcacacgt

SEQ ID NO: 530 - DNA, 54 bp, synthetic construct
  misc_feature 1..54: note = source = /note="Description of Artificial Sequence: Syntheticoligonucleotide"
  misc_feature 1..54: note = source = /note="FWD_Guide 180"
  source 1..54: mol_type = other DNA
gtctcgtgggctcggagatgtgtataagagacagtcgcttaagcccaggagttc

SEQ ID NO: 531 - DNA, 55 bp, synthetic construct
  misc_feature 1..55: note = source = /note="Description of Artificial Sequence: Syntheticoligonucleotide"
  misc_feature 1..55: note = source = /note="REV_Guide 181"
  source 1..55: mol_type = other DNA
tcgtcggcagcgtcagatgtgtataagagacagtctggctgatccgtactaatcc

SEQ ID NO: 532 - DNA, 54 bp, synthetic construct
  misc_feature 1..54: note = source = /note="Description of Artificial Sequence: Syntheticoligonucleotide"
  misc_feature 1..54: note = source = /note="FWD_Guide 181"
  source 1..54: mol_type = other DNA
gtctcgtgggctcggagatgtgtataagagacagtaggctcaagggatgctcct

SEQ ID NO: 533 - DNA, 53 bp, synthetic construct
  misc_feature 1..53: note = source = /note="Description of Artificial Sequence: Syntheticoligonucleotide"
  misc_feature 1..53: note = source = /note="REV_Guide 200"
  source 1..53: mol_type = other DNA
tcgtcggcagcgtcagatgtgtataagagacagccagagctgtccttgaggtg

SEQ ID NO: 534 - DNA, 54 bp, synthetic construct
  misc_feature 1..54: note = source = /note="Description of Artificial Sequence: Syntheticoligonucleotide"
  misc_feature 1..54: note = source = /note="FWD_Guide 200"
  source 1..54: mol_type = other DNA
gtctcgtgggctcggagatgtgtataagagacaggtccatacccaccttggcaa

SEQ ID NO: 535 - DNA, 53 bp, synthetic construct; identical to SEQ ID NO: 517
  misc_feature 1..53: note = source = /note="Description of Artificial Sequence: Syntheticoligonucleotide"
  misc_feature 1..53: note = source = /note="REV_Guide 201"
  source 1..53: mol_type = other DNA

SEQ ID NO: 536 - DNA, 54 bp, synthetic construct; identical to SEQ ID NO: 518
  misc_feature 1..54: note = source = /note="Description of Artificial Sequence: Syntheticoligonucleotide"
  misc_feature 1..54: note = source = /note="FWD_Guide 201"
  source 1..54: mol_type = other DNA

SEQ ID NO: 537 - DNA, 53 bp, synthetic construct
  misc_feature 1..53: note = source = /note="Description of Artificial Sequence: Syntheticoligonucleotide"
  misc_feature 1..53: note = source = /note="REV_Guide 202"
  source 1..53: mol_type = other DNA
tcgtcggcagcgtcagatgtgtataagagacagaggctatcagtcagcgcatc

SEQ ID NO: 538 - DNA, 54 bp, synthetic construct
  misc_feature 1..54: note = source = /note="Description of Artificial Sequence: Syntheticoligonucleotide"
  misc_feature 1..54: note = source = /note="FWD_Guide 202"
  source 1..54: mol_type = other DNA
gtctcgtgggctcggagatgtgtataagagacagagcaggggaagtggggatat

SEQ ID NO: 539 - DNA, 54 bp, synthetic construct; identical to SEQ ID NO: 490
  misc_feature 1..54: note = source = /note="Description of Artificial Sequence: Syntheticoligonucleotide"
  misc_feature 1..54: note = source = /note="FWD_Guide 152"
  source 1..54: mol_type = other DNA

SEQ ID NO: 540 - DNA, 53 bp, synthetic construct; identical to SEQ ID NO: 489
  misc_feature 1..53: note = source = /note="Description of Artificial Sequence: Syntheticoligonucleotide"
  misc_feature 1..53: note = source = /note="REV_Guide 152"
  source 1..53: mol_type = other DNA

SEQ ID NO: 541 - DNA, 54 bp, synthetic construct; identical to SEQ ID NO: 485
  misc_feature 1..54: note = source = /note="Description of Artificial Sequence: Syntheticoligonucleotide"
  misc_feature 1..54: note = source = /note="FWD_Guide 153"
  source 1..54: mol_type = other DNA

SEQ ID NO: 542 - DNA, 53 bp, synthetic construct; identical to SEQ ID NO: 486
  misc_feature 1..53: note = source = /note="Description of Artificial Sequence: Syntheticoligonucleotide"
  misc_feature 1..53: note = source = /note="REV_Guide 153"
  source 1..53: mol_type = other DNA

SEQ ID NO: 543 - DNA, 54 bp, synthetic construct; identical to SEQ ID NO: 490
  misc_feature 1..54: note = source = /note="Description of Artificial Sequence: Syntheticoligonucleotide"
  misc_feature 1..54: note = source = /note="FWD_Guide 154"
  source 1..54: mol_type = other DNA

SEQ ID NO: 544 - DNA, 53 bp, synthetic construct; identical to SEQ ID NO: 489
  misc_feature 1..53: note = source = /note="Description of Artificial Sequence: Syntheticoligonucleotide"
  misc_feature 1..53: note = source = /note="REV_Guide 154"
  source 1..53: mol_type = other DNA

SEQ ID NO: 545 - DNA, 54 bp, synthetic construct; identical to SEQ ID NO: 510
  misc_feature 1..54: note = source = /note="Description of Artificial Sequence: Syntheticoligonucleotide"
  misc_feature 1..54: note = source = /note="FWD_Guide 182"
  source 1..54: mol_type = other DNA

SEQ ID NO: 546 - DNA, 53 bp, synthetic construct; identical to SEQ ID NO: 509
  misc_feature 1..53: note = source = /note="Description of Artificial Sequence: Syntheticoligonucleotide"
  misc_feature 1..53: note = source = /note="REV_Guide 182"
  source 1..53: mol_type = other DNA

SEQ ID NO: 547 - DNA, 54 bp, synthetic construct
  misc_feature 1..54: note = source = /note="Description of Artificial Sequence: Syntheticoligonucleotide"
  misc_feature 1..54: note = source = /note="FWD_Guide 183"
  source 1..54: mol_type = other DNA
gtctcgtgggctcggagatgtgtataagagacagtgcctgtagtcccagctact

SEQ ID NO: 548 - DNA, 53 bp, synthetic construct
  misc_feature 1..53: note = source = /note="Description of Artificial Sequence: Syntheticoligonucleotide"
  misc_feature 1..53: note = source = /note="REV_Guide 183"
  source 1..53: mol_type = other DNA
tcgtcggcagcgtcagatgtgtataagagacagtcagctcagtgcaacctctg

SEQ ID NO: 549 - DNA, 54 bp, synthetic construct; identical to SEQ ID NO: 492
  misc_feature 1..54: note = source = /note="Description of Artificial Sequence: Syntheticoligonucleotide"
  misc_feature 1..54: note = source = /note="FWD_Guide 184"
  source 1..54: mol_type = other DNA

SEQ ID NO: 550 - DNA, 53 bp, synthetic construct; identical to SEQ ID NO: 491
  misc_feature 1..53: note = source = /note="Description of Artificial Sequence: Syntheticoligonucleotide"
  misc_feature 1..53: note = source = /note="REV_Guide 184"
  source 1..53: mol_type = other DNA

SEQ ID NO: 551 - DNA, 54 bp, synthetic construct; identical to SEQ ID NO: 518
  misc_feature 1..54: note = source = /note="Description of Artificial Sequence: Syntheticoligonucleotide"
  misc_feature 1..54: note = source = /note="FWD_Guide 203"
  source 1..54: mol_type = other DNA

SEQ ID NO: 552 - DNA, 53 bp, synthetic construct; identical to SEQ ID NO: 517
  misc_feature 1..53: note = source = /note="Description of Artificial Sequence: Syntheticoligonucleotide"
  misc_feature 1..53: note = source = /note="REV_Guide 203"
  source 1..53: mol_type = other DNA

SEQ ID NO: 553 - DNA, 54 bp, synthetic construct; identical to SEQ ID NO: 500
  misc_feature 1..54: note = source = /note="Description of Artificial Sequence: Syntheticoligonucleotide"
  misc_feature 1..54: note = source = /note="FWD_Guide 204"
  source 1..54: mol_type = other DNA

SEQ ID NO: 554 - DNA, 53 bp, synthetic construct; identical to SEQ ID NO: 499
  misc_feature 1..53: note = source = /note="Description of Artificial Sequence: Syntheticoligonucleotide"
  misc_feature 1..53: note = source = /note="REV_Guide 204"
  source 1..53: mol_type = other DNA

SEQ ID NO: 555 - DNA, 54 bp, synthetic construct; identical to SEQ ID NO: 498
  misc_feature 1..54: note = source = /note="Description of Artificial Sequence: Syntheticoligonucleotide"
  misc_feature 1..54: note = source = /note="FWD_Guide 205"
  source 1..54: mol_type = other DNA

SEQ ID NO: 556 - DNA, 53 bp, synthetic construct; identical to SEQ ID NO: 497
  misc_feature 1..53: note = source = /note="Description of Artificial Sequence: Syntheticoligonucleotide"
  misc_feature 1..53: note = source = /note="REV_Guide 205"
  source 1..53: mol_type = other DNA

SEQ ID NO: 557-558 - skipped (2 entries)

SEQ ID NO: 559 - DNA, 30 bp, synthetic construct
  misc_feature 1..30: note = source = /note="Description of Artificial Sequence: Syntheticoligonucleotide"
  misc_feature 1..30: note = source = /note="sequence 2 for cleavage site assay"
  source 1..30: mol_type = other DNA
ccatgatatagacgttgtggctgttgtagt

SEQ ID NO: 560 - protein, 6 aa, synthetic construct
  REGION 1..6: note = source = /note="Description of Artificial Sequence: Synthetic6xHis tag"
HHHHHH

SEQ ID NO: 561 - protein, 10 aa, synthetic construct
  REGION 1..10: note = source = /note="Description of Artificial Sequence: Synthetic10xHis tag"
HHHHHHHHHH

SEQ ID NO: 562 - DNA, 34 bp, synthetic construct
  misc_feature 1..34: note = source = /note="Description of Artificial Sequence: Syntheticoligonucleotide"
  source 1..34: mol_type = other DNA
cctgggtgtgaggctgggccattaaaacctctcc

SEQ ID NO: 563 - DNA, 15 bp, synthetic construct
  misc_feature 1..15: note = source = /note="Description of Artificial Sequence: Syntheticoligonucleotide"
  source 1..15: mol_type = other DNA
cctgaaaacctctcc

SEQ ID NO: 564 - DNA, 33 bp, synthetic construct
  misc_feature 1..33: note = source = /note="Description of Artificial Sequence: Syntheticoligonucleotide"
  source 1..33: mol_type = other DNA
cctgggtgtgagctgggccattaaaacctctcc

SEQ ID NO: 565 - DNA, 22 bp, synthetic construct
  misc_feature 1..22: note = source = /note="Description of Artificial Sequence: Syntheticoligonucleotide"
  source 1..22: mol_type = other DNA
cctgggccattaaaacctctcc

SEQ ID NO: 566 - DNA, 11 bp, synthetic construct
  misc_feature 1..11: note = source = /note="Description of Artificial Sequence: Syntheticoligonucleotide"
  source 1..11: mol_type = other DNA
cctggctctcc

SEQ ID NO: 567 - DNA, 20 bp, synthetic construct
  misc_feature 1..20: note = source = /note="Description of Artificial Sequence: Syntheticoligonucleotide"
  source 1..20: mol_type = other DNA
cgggccattaaaacctctcc

SEQ ID NO: 568 - DNA, 40 bp, synthetic construct
  misc_feature 1..40: note = source = /note="Description of Artificial Sequence: Syntheticoligonucleotide"
  source 1..40: mol_type = other DNA
cctgggtgtgaggccagacctgggccattaaaacctctcc

SEQ ID NO: 569 - DNA, 79 bp, synthetic construct
  misc_feature 1..79: note = source = /note="Description of Artificial Sequence: Syntheticoligonucleotide"
  source 1..79: mol_type = other DNA
cctgggtgtgaggggaagctgacgtcctttccatggctgctcgcctgtgttgccaccgctgggccattaaaacctctcc

SEQ ID NO: 570 - DNA, 33 bp, synthetic construct
  misc_feature 1..33: note = source = /note="Description of Artificial Sequence: Syntheticoligonucleotide"
  source 1..33: mol_type = other DNA
cctgggtgtgacctgggccattaaaacctctcc

SEQ ID NO: 571 - DNA, 35 bp, synthetic construct
  misc_feature 1..35: note = source = /note="Description of Artificial Sequence: Syntheticoligonucleotide"
  source 1..35: mol_type = other DNA
cctgggtgtgaggactgggccattaaaacctctcc

SEQ ID NO: 572 - DNA, 34 bp, synthetic construct
  misc_feature 1..34: note = source = /note="Description of Artificial Sequence: Syntheticoligonucleotide"
  source 1..34: mol_type = other DNA
agttggcagatgctctaatgtactgccatgggaa

SEQ ID NO: 573 - DNA, 31 bp, synthetic construct
  misc_feature 1..31: note = source = /note="Description of Artificial Sequence: Syntheticoligonucleotide"
  source 1..31: mol_type = other DNA
agttggcagatgcaatgtactgccatgggaa

SEQ ID NO: 574 - DNA, 30 bp, synthetic construct
  misc_feature 1..30: note = source = /note="Description of Artificial Sequence: Syntheticoligonucleotide"
  source 1..30: mol_type = other DNA
agttggcagatgcatgtactgccatgggaa

SEQ ID NO: 575 - DNA, 31 bp, synthetic construct
  misc_feature 1..31: note = source = /note="Description of Artificial Sequence: Syntheticoligonucleotide"
  source 1..31: mol_type = other DNA
agttggcagatgctatgtactgccatgggaa

SEQ ID NO: 576 - DNA, 32 bp, synthetic construct
  misc_feature 1..32: note = source = /note="Description of Artificial Sequence: Syntheticoligonucleotide"
  source 1..32: mol_type = other DNA
agttggcagatgctaatgtactgccatgggaa

SEQ ID NO: 577 - DNA, 31 bp, synthetic construct
  misc_feature 1..31: note = source = /note="Description of Artificial Sequence: Syntheticoligonucleotide"
  source 1..31: mol_type = other DNA
agttggcagatgctatgtaatgccatgggaa

SEQ ID NO: 578 - DNA, 33 bp, synthetic construct
  misc_feature 1..33: note = source = /note="Description of Artificial Sequence: Syntheticoligonucleotide"
  source 1..33: mol_type = other DNA
agttggcagatgctctatgtactgccatgggaa

SEQ ID NO: 579 - DNA, 39 bp, synthetic construct
  misc_feature 1..39: note = source = /note="Description of Artificial Sequence: Syntheticoligonucleotide"
  source 1..39: mol_type = other DNA
cgacctgaatgctgtgcggcgctctggcttcattcaatc

SEQ ID NO: 580 - DNA, 35 bp, synthetic construct
  misc_feature 1..35: note = source = /note="Description of Artificial Sequence: Syntheticoligonucleotide"
  source 1..35: mol_type = other DNA
cgacctgaatgctgtgcggctctgcttccaggtga

SEQ ID NO: 581 - DNA, 36 bp, synthetic construct
  misc_feature 1..36: note = source = /note="Description of Artificial Sequence: Syntheticoligonucleotide"
  source 1..36: mol_type = other DNA
cgacctgaatgctgtgcggcatctgcttccaggtga

SEQ ID NO: 582 - DNA, 25 bp, synthetic construct
  misc_feature 1..25: note = source = /note="Description of Artificial Sequence: Syntheticoligonucleotide"
  source 1..25: mol_type = other DNA
cgacctgaatgctgcttccaggtga

SEQ ID NO: 583 - DNA, 28 bp, synthetic construct
  misc_feature 1..28: note = source = /note="Description of Artificial Sequence: Syntheticoligonucleotide"
  source 1..28: mol_type = other DNA
cgacctgaatgcttctgcttccaggtga

SEQ ID NO: 584 - DNA, 22 bp, synthetic construct
  misc_feature 1..22: note = source = /note="Description of Artificial Sequence: Syntheticoligonucleotide"
  source 1..22: mol_type = other DNA
cgacctgaatgcttccaggtga

SEQ ID NO: 585 - DNA, 35 bp, synthetic construct
  misc_feature 1..35: note = source = /note="Description of Artificial Sequence: Syntheticoligonucleotide"
  source 1..35: mol_type = other DNA
gcgtggggactacgacctgaatgctgtgcggctct

SEQ ID NO: 586 - DNA, 24 bp, synthetic construct
  misc_feature 1..24: note = source = /note="Description of Artificial Sequence: Syntheticoligonucleotide"
  source 1..24: mol_type = other DNA
gcgacctgaatgctgtgcggctct

SEQ ID NO: 587 - DNA, 28 bp, synthetic construct
  misc_feature 1..28: note = source = /note="Description of Artificial Sequence: Syntheticoligonucleotide"
  source 1..28: mol_type = other DNA
gcgtggggactacgagctgtgcggctct

SEQ ID NO: 588 - DNA, 28 bp, synthetic construct
  misc_feature 1..28: note = source = /note="Description of Artificial Sequence: Syntheticoligonucleotide"
  source 1..28: mol_type = other DNA
gcgtggggactgaatgctgtgcggctct

SEQ ID NO: 589 - DNA, 31 bp, synthetic construct
  misc_feature 1..31: note = source = /note="Description of Artificial Sequence: Syntheticoligonucleotide"
  source 1..31: mol_type = other DNA
gcgtggggactcctgaatgctgtgcggctct

SEQ ID NO: 590 - DNA, 36 bp, synthetic construct
  misc_feature 1..36: note = source = /note="Description of Artificial Sequence: Syntheticoligonucleotide"
  source 1..36: mol_type = other DNA
gcgtggggactacgaacctgaatgctgtgcggctct

SEQ ID NO: 591 - DNA, 30 bp, synthetic construct
  misc_feature 1..30: note = source = /note="Description of Artificial Sequence: Syntheticoligonucleotide"
  source 1..30: mol_type = other DNA
gcgtggggactacgaatgctgtgcggctct

SEQ ID NO: 592 - DNA, 32 bp, synthetic construct
  misc_feature 1..32: note = source = /note="Description of Artificial Sequence: Syntheticoligonucleotide"
  source 1..32: mol_type = other DNA
gcgtggggactacctgaatgctgtgcggctct

SEQ ID NO: 593 - DNA, 21 bp, synthetic construct
  misc_feature 1..21: note = source = /note="Description of Artificial Sequence: Syntheticoligonucleotide"
  source 1..21: mol_type = other DNA
gcgtgaatgctgtgcggctct

SEQ ID NO: 594 - DNA, 24 bp, synthetic construct
  misc_feature 1..24: note = source = /note="Description of Artificial Sequence: Syntheticoligonucleotide"
  source 1..24: mol_type = other DNA
gcgacctgactgctgtgcggctct

SEQ ID NO: 595 - DNA, 34 bp, synthetic construct
  misc_feature 1..34: note = source = /note="Description of Artificial Sequence: Syntheticoligonucleotide"
  source 1..34: mol_type = other DNA
gcgtggggactacgcctgaatgctgtgcggctct

SEQ ID NO: 596 - DNA, 42 bp, synthetic construct
  misc_feature 1..42: note = source = /note="Description of Artificial Sequence: Syntheticoligonucleotide"
  source 1..42: mol_type = other DNA
atggaggagttggcagatgctctaatgtactgccatgggaag

SEQ ID NO: 597 - DNA, 40 bp, synthetic construct
  misc_feature 1..40: note = source = /note="Description of Artificial Sequence: Syntheticoligonucleotide"
  source 1..40: mol_type = other DNA
atggaggagttggcagatgctaatgtactgccatgggaag

SEQ ID NO: 598 - DNA, 34 bp, synthetic construct
  misc_feature 1..34: note = source = /note="Description of Artificial Sequence: Syntheticoligonucleotide"
  source 1..34: mol_type = other DNA
atggaggagttggcagatgtactgccatgggaag

SEQ ID NO: 599 - DNA, 18 bp, synthetic construct
  misc_feature 1..18: note = source = /note="Description of Artificial Sequence: Syntheticoligonucleotide"
  source 1..18: mol_type = other DNA
atgtactgccatgggaag

SEQ ID NO: 600 - DNA, 30 bp, synthetic construct
  misc_feature 1..30: note = source = /note="Description of Artificial Sequence: Syntheticoligonucleotide"
  source 1..30: mol_type = other DNA
atggaggagttggtgtactgccatgggaag

SEQ ID NO: 601 - DNA, 43 bp, synthetic construct
  misc_feature 1..43: note = source = /note="Description of Artificial Sequence: Syntheticoligonucleotide"
  source 1..43: mol_type = other DNA
atggaggagttggcagatgctctaaatgtactgccatgggaag

SEQ ID NO: 602 - DNA, 45 bp, synthetic construct
  misc_feature 1..45: note = source = /note="Description of Artificial Sequence: Syntheticoligonucleotide"
  source 1..45: mol_type = other DNA
atggaggagttggcagatgctcttctaatgtactgccatgggaag

SEQ ID NO: 603 - DNA, 44 bp, synthetic construct
  misc_feature 1..44: note = source = /note="Description of Artificial Sequence: Syntheticoligonucleotide"
  source 1..44: mol_type = other DNA
atggaggagttggcagatgccctctaatgtactgccatgggaag

SEQ ID NO: 604 - DNA, 40 bp, synthetic construct
  misc_feature 1..40: note = source = /note="Description of Artificial Sequence: Syntheticoligonucleotide"
  source 1..40: mol_type = other DNA
atggaggagttggcagataatgtactgccatgggaagaag

SEQ ID NO: 605 - DNA, 24 bp, synthetic construct
  misc_feature 1..24: note = source = /note="Description of Artificial Sequence: Syntheticoligonucleotide"
  source 1..24: mol_type = other DNA
atggcgtactgccatgggaagaag

SEQ ID NO: 606 - DNA, 46 bp, synthetic construct
  misc_feature 1..46: note = source = /note="Description of Artificial Sequence: Syntheticoligonucleotide"
  source 1..46: mol_type = other DNA
atggaggagttggcagatgcttctaatgtactgccatgggaagaag

SEQ ID NO: 607 - DNA, 32 bp, synthetic construct
  misc_feature 1..32: note = source = /note="Description of Artificial Sequence: Syntheticoligonucleotide"
  source 1..32: mol_type = other DNA
atggaggagttggcatctgccatgggaagaag

SEQ ID NO: 608 - DNA, 42 bp, synthetic construct
  misc_feature 1..42: note = source = /note="Description of Artificial Sequence: Syntheticoligonucleotide"
  source 1..42: mol_type = other DNA
atggaggagttggcagatgcaatgtactgccatgggaagaag

SEQ ID NO: 609 - DNA, 124 bp, synthetic construct
  misc_feature 1..124: note = source = /note="Description of Artificial Sequence: Syntheticpolynucleotide"
  source 1..124: mol_type = other DNA
atggaggagttggcagatgccaaactgaaaaacaaatcaaagcactcttattgagtgctggcgatccccgacgccacgggccgaaacccttatcatagaaactctaatgtactgccatgggaag

SEQ ID NO: 610 - DNA, 84 bp, synthetic construct
  misc_feature 1..84: note = source = /note="Description of Artificial Sequence: Syntheticoligonucleotide"
  source 1..84: mol_type = other DNA
atggaggagttggcagatgctgcttatatagacctcccaccgtacacgcctaccgcccattttctaatgtactgccatgggaag

SEQ ID NO: 611 - DNA, 34 bp, synthetic construct
  misc_feature 1..34: note = source = /note="Description of Artificial Sequence: Syntheticoligonucleotide"
  source 1..34: mol_type = other DNA
atggaggagttgtctaatgtactgccatgggaag

SEQ ID NO: 612 - DNA, 16 bp, synthetic construct
  misc_feature 1..16: note = source = /note="Description of Artificial Sequence: Syntheticoligonucleotide"
  source 1..16: mol_type = other DNA
ctgccatgggaagaag

SEQ ID NO: 613 - DNA, 90 bp, synthetic construct
  misc_feature 1..90: note = source = /note="Description of Artificial Sequence: Syntheticoligonucleotide"
  source 1..90: mol_type = other DNA
atggaggagttggcagatgcgcggctgttcctgtacagaaccgtgggcgagatgtggatcaaggatgctctaatgtactgccatgggaag

SEQ ID NO: 614 - DNA, 41 bp, synthetic construct
  misc_feature 1..41: note = source = /note="Description of Artificial Sequence: Syntheticoligonucleotide"
  source 1..41: mol_type = other DNA
atggaggagttggcagatgcctaatgtactgccatgggaag

SEQ ID NO: 615 - DNA, 97 bp, synthetic construct
  misc_feature 1..97: note = source = /note="Description of Artificial Sequence: Syntheticoligonucleotide"
  source 1..97: mol_type = other DNA
atggaggagttggcagatgctgtcatgatctttttccgctcgtcgtgggacttgctcagttctctggccagctcgtctaatgtactgccatgggaag

SEQ ID NO: 616 - DNA, 41 bp, synthetic construct
  misc_feature 1..41: note = source = /note="Description of Artificial Sequence: Syntheticoligonucleotide"
  source 1..41: mol_type = other DNA
atggaggagttggcagatgctctatgtactgccatgggaag

SEQ ID NO: 617 - DNA, 32 bp, synthetic construct
  misc_feature 1..32: note = source = /note="Description of Artificial Sequence: Syntheticoligonucleotide"
  source 1..32: mol_type = other DNA
cagggacagtgcgcatctccctggtcaccaag

SEQ ID NO: 618 - DNA, 17 bp, synthetic construct
  misc_feature 1..17: note = source = /note="Description of Artificial Sequence: Syntheticoligonucleotide"
  source 1..17: mol_type = other DNA
cagggacagtcaccaag

SEQ ID NO: 619 - DNA, 31 bp, synthetic construct
  misc_feature 1..31: note = source = /note="Description of Artificial Sequence: Syntheticoligonucleotide"
  source 1..31: mol_type = other DNA
cagggacagtgcgcatctcctggtcaccaag

SEQ ID NO: 620 - DNA, 30 bp, synthetic construct
  misc_feature 1..30: note = source = /note="Description of Artificial Sequence: Syntheticoligonucleotide"
  source 1..30: mol_type = other DNA
cagggacagtgcgcatctctggtcaccaag

SEQ ID NO: 621 - DNA, 33 bp, synthetic construct
  misc_feature 1..33: note = source = /note="Description of Artificial Sequence: Syntheticoligonucleotide"
  source 1..33: mol_type = other DNA
cagggacagtgcgcatctcctctggtcaccaag

SEQ ID NO: 622 - DNA, 29 bp, synthetic construct
  misc_feature 1..29: note = source = /note="Description of Artificial Sequence: Syntheticoligonucleotide"
  source 1..29: mol_type = other DNA
cagggacagtgcgcatcctggtcaccaag

SEQ ID NO: 623 - DNA, 17 bp, synthetic construct
  misc_feature 1..17: note = source = /note="Description of Artificial Sequence: Syntheticoligonucleotide"
  source 1..17: mol_type = other DNA
cagggacggtcaccaag

SEQ ID NO: 624 - DNA, 31 bp, synthetic construct
  misc_feature 1..31: note = source = /note="Description of Artificial Sequence: Syntheticoligonucleotide"
  source 1..31: mol_type = other DNA
cggggacagggcgcatctcctggtcaccaag

SEQ ID NO: 625 - DNA, 32 bp, synthetic construct
  misc_feature 1..32: note = source = /note="Description of Artificial Sequence: Syntheticoligonucleotide"
  source 1..32: mol_type = other DNA
cgacctgaatgctgtgcggctctgcttccagg

SEQ ID NO: 626 - DNA, 33 bp, synthetic construct
  misc_feature 1..33: note = source = /note="Description of Artificial Sequence: Syntheticoligonucleotide"
  source 1..33: mol_type = other DNA
cgacctgaatgctgtgcggcatctgcttccagg

SEQ ID NO: 627 - DNA, 33 bp, synthetic construct
  misc_feature 1..33: note = source = /note="Description of Artificial Sequence: Syntheticoligonucleotide"
  source 1..33: mol_type = other DNA
cgacctgaatgctgtgcggcttctgcttccagg

SEQ ID NO: 628 - DNA, 28 bp, synthetic construct
  misc_feature 1..28: note = source = /note="Description of Artificial Sequence: Syntheticoligonucleotide"
  source 1..28: mol_type = other DNA
cgacctgaatgctgtgtctgcttccagg

SEQ ID NO: 629 - DNA, 33 bp, synthetic construct
  misc_feature 1..33: note = source = /note="Description of Artificial Sequence: Syntheticoligonucleotide"
  source 1..33: mol_type = other DNA
cgacctgcatgctgtgcggcatctgcttccagg

SEQ ID NO: 630 - DNA, 33 bp, synthetic construct
  misc_feature 1..33: note = source = /note="Description of Artificial Sequence: Syntheticoligonucleotide"
  source 1..33: mol_type = other DNA
cgacctgcatgctgtgcggcttctgcttccagg

SEQ ID NO: 631 - DNA, 28 bp, synthetic construct
  misc_feature 1..28: note = source = /note="Description of Artificial Sequence: Syntheticoligonucleotide"
  source 1..28: mol_type = other DNA
cgacctgcatgctgtgtctgcttccagg

SEQ ID NO: 632 - DNA, 33 bp, synthetic construct
  misc_feature 1..33: note = source = /note="Description of Artificial Sequence: Syntheticoligonucleotide"
  source 1..33: mol_type = other DNA
cgacctgaatgctgtgcgacatctgcttccagg

SEQ ID NO: 633 - DNA, 32 bp, synthetic construct
  misc_feature 1..32: note = source = /note="Description of Artificial Sequence: Syntheticoligonucleotide"
  source 1..32: mol_type = other DNA
tggggactacgacctgaatgctgtgcggctct

SEQ ID NO: 634 - DNA, 27 bp, synthetic construct
  misc_feature 1..27: note = source = /note="Description of Artificial Sequence: Syntheticoligonucleotide"
  source 1..27: mol_type = other DNA
tggggactacgaatgctgtgcggctct

SEQ ID NO: 635 - DNA, 66 bp, synthetic construct
  misc_feature 1..66: note = source = /note="Description of Artificial Sequence: Syntheticoligonucleotide"
  source 1..66: mol_type = other DNA
tggggactacgagcaggcagaagtatgcaaagcatgcatctcaattcctgaatgctgtgcggctct

SEQ ID NO: 636 - DNA, 72 bp, synthetic construct
  misc_feature 1..72: note = source = /note="Description of Artificial Sequence: Syntheticoligonucleotide"
  source 1..72: mol_type = other DNA
tggggactacgaagaaggcgatagaaggccatgcgctgcgaatcgggagcggcctgaatgctgtgcggctct

SEQ ID NO: 637 - DNA, 99 bp, synthetic construct
  misc_feature 1..99: note = source = /note="Description of Artificial Sequence: Syntheticoligonucleotide"
  source 1..99: mol_type = other DNA
tggggactacgatgactcgctgcgctcggtcgttcggctgcggcgagcggtatcagctcactcaaaggcggtaatacggcctgaatgctgtgcggctct

SEQ ID NO: 638 - DNA, 14 bp, synthetic construct
  misc_feature 1..14: note = source = /note="Description of Artificial Sequence: Syntheticoligonucleotide"
  source 1..14: mol_type = other DNA
tggggtgcggctct

SEQ ID NO: 639 - DNA, 27 bp, synthetic construct
  misc_feature 1..27: note = source = /note="Description of Artificial Sequence: Syntheticoligonucleotide"
  source 1..27: mol_type = other DNA
tggggactacgactgctgtgcggctct

SEQ ID NO: 640 - DNA, 39 bp, synthetic construct; identical to SEQ ID NO: 579
  misc_feature 1..39: note = source = /note="Description of Artificial Sequence: Syntheticoligonucleotide"
  source 1..39: mol_type = other DNA

SEQ ID NO: 641 - DNA, 35 bp, synthetic construct; identical to SEQ ID NO: 580
  misc_feature 1..35: note = source = /note="Description of Artificial Sequence: Syntheticoligonucleotide"
  source 1..35: mol_type = other DNA

SEQ ID NO: 642 - DNA, 36 bp, synthetic construct; identical to SEQ ID NO: 581
  misc_feature 1..36: note = source = /note="Description of Artificial Sequence: Syntheticoligonucleotide"
  source 1..36: mol_type = other DNA

SEQ ID NO: 643 - DNA, 25 bp, synthetic construct
  misc_feature 1..25: note = source = /note="Description of Artificial Sequence: Syntheticoligonucleotide"
  source 1..25: mol_type = other DNA
cgacctgaatgctgcttccaggtga

SEQ ID NO: 644 - DNA, 28 bp, synthetic construct
  misc_feature 1..28: note = source = /note="Description of Artificial Sequence: Syntheticoligonucleotide"
  source 1..28: mol_type = other DNA
cgacctgaatgcttctgcttccaggtga

SEQ ID NO: 645 - DNA, 22 bp, synthetic construct
  misc_feature 1..22: note = source = /note="Description of Artificial Sequence: Syntheticoligonucleotide"
  source 1..22: mol_type = other DNA
cgacctgaatgcttccaggtga

SEQ ID NO: 646 - protein, 4 aa, Homo sapiens
EEQL

SEQ ID NO: 647 - protein, 6 aa, Homo sapiens
AEVSQA

SEQ ID NO: 648 - protein, 4 aa, Mus musculus
GEQL

SEQ ID NO: 649 - protein, 6 aa, Mus musculus
AEVSKA

SEQ ID NO: 650 - protein, 4 aa, synthetic construct
  REGION 1..4: note = source = /note="Description of Artificial Sequence: Syntheticpeptide"
GEQL

SEQ ID NO: 651 - protein, 6 aa, synthetic construct
  REGION 1..6: note = source = /note="Description of Artificial Sequence: Syntheticpeptide"
AEVSQA